European Patent Specification EP 3 681 307 B1, published June 4, 2025. Title: Low Fiber Pennycress Meal and Methods of Making. Applicant: Ulmasov, Tim Handel, Cristine Hartnell, Gary Sedbrook, John C. Chopra, Ratan Esfahanian, Maliheh Marks, Michael David. Application US 62/559,122. The sequence listing filed with the application follows.

SEQUENCE LISTING (183 sequences)

SEQ ID NO: 1 - DNA, 795 bp, Thlaspi arvense
atggggaagagaacaagtaacagtttgaagaaagatgagttaaacagaggagcttggactgatcaagaagacaagatccttaaagattatatcatgatccatggcgaaggcaaatggagcactctcccaaaccaagccggtctcaagaggtgtggcaaaagctgcagactcaggtggaagaactacttgagaccggggataaagcgcggaaacatctcatctgatgaagaagaactcataatccgcctccataatctccttggaaacagatggtctctgatagctgggaggcttccggggcgaacagacaatgaaataaagaaccattggaactcaaacctccgcaaaagacttcccaaaacaaaaaccaaccaaccaaaacttcgaaaacattcaaccaacatcaagaacaatgtctgtgttatacgcacaaaggcgattaggtgctcaaaggctctgacttttcagaaccagagtagtagtggtagtaccaatcttcttcctatgaaagaacaagtgagctctatgatggatcatgaagctggttcttcgttgttggaagatcttgaaattgattttgataaaatccaatcagagtttctcttccctgatctgatggatttggaaggtttgggttgtggaaacgtaacatcacttgtttcatctgaggagattttaggagattatgttcgtgctgatgaatcttctcagggtaatcttgatctcaatagacctttcactccttgtcttcatcgtggcaacgatgaagattggctccgagttttcaattgttag

SEQ ID NO: 2 - protein, 264 aa, Thlaspi arvense
MGKRTSNSLKKDELNRGAWTDQEDKILKDYIMIHGEGKWSTLPNQAGLKRCGKSCRLRWKNYLRPGIKRGNISSDEEELIIRLHNLLGNRWSLIAGRLPGRTDNEIKNHWNSNLRKRLPKTKTNQPKLRKHSTNIKNNVCVIRTKAIRCSKALTFQNQSSSGSTNLLPMKEQVSSMMDHEAGSSLLEDLEIDFDKIQSEFLFPDLMDLEGLGCGNVTSLVSSEEILGDYVRADESSQGNLDLNRPFTPCLHRGNDEDWLRVFNC

SEQ ID NO: 3 - DNA, 3512 bp, Thlaspi arvense
tctcagccaaattgacaaataaaaatcacatttagaaaacatttcacggttttgtatgtaaactagtaaaaaaaaaaaaagagaacatgttatttcaatatataacattggaaagtatagtatattgattctctcactaatctaaaaatttatgcatcaataatttttaatagattaaaaatctaaagttaatcttattggaaattaaatataattattaagtttcaatatatatagacatgttatctctttcatttttaaccaactagtgatatgggacaaagtacaaaatgttagttacatcagttttaatctgatataaaatttgtatcaatttttttaatgttaacaaaattattgattacattgattatttaaatagtgtaaatttataattttatatcagttttgtttaactgatgtaaactaatataagtttgtatcaattttattgaacggaagtcaaataatcaataaaaatatcaattttcagaactgatgttaaatcacatattttatatcatttattaataagtaattcaccttttttgtagtgtgatatgagttattggcgtttaataataattttaaaaaattatagtttcatgttaaatcttacaaaattatataaatcttttaaaatcaaaaattatttatttgagcatttgcaataatgaacagttgcgaatgaataattaataaaatatttaaaaattaaaaatgtaaataacaaaatgtatttaaactctgaatatatgtatataataacataaattgacttaaaaaataataaatcatatgtacaaagttgacgccttcttaaatactgtttttataatttctaatataataattattcaaatggaaaaattaaacttgaatatgaaccttttaactctttgattgtcaaaaataaaaagttttcatgaaatagagttccgaacttaaaaaagagacatttgaaacttgggaccccaaatttatgtaacactgaaagatcttaaggagttttattttttgtttgttcatgacgcaggactatgtgtactgtgtaggcatgaagaccatgtgttaccgtcttaactgtatcaaatgatgattgcttacatactagaatgtggctagcaatgactattttcactctgtatacatacttataccccatatgcaatacaataatgatcaaggtcgttttaggacctatatgattggagtctaaggcacgagagactagactagcgatcatcgtgtgaagtgagttcaaaggatttcagatccttagtaataagtacaaaagtatattcttgatgacaaaattcggtagagttaaatctcaccaaaactgatacactattattaccaggtgagaaaaggattgatatttcaaagtgtgtgtgtgtgacagaagttttggaaagcgacatgtgtacggacattgcaacaactccatataaagttactttgttaacacaaaaagaatctattctctactcaacactaaagacaattgtaccaaccaaacaaccacaagagagagaaagagagtatggggaagagaacaagtaacagtttgaagaaagatgagttaaacagaggagcttggactgatcaagaagacaagatccttaaagattatatcatgatccatggcgaaggcaaatggagcactctcccaaaccaagccggtacatatccatctatctattgatctatccgtctttaaatgcaaatcttcatctacttacaataattgcacataaaggtctcaagaggtgtggcaaaagctgcagactcaggtggaagaactacttgagaccggggataaagcgcggaaacatctcatctgatgaagaagaactcataatccgcctccataatctccttggaaacaggttaattaacttcctctttcaccgaaacacagattgttttcttttcaagttaagtttttccataatttttgcggcgtaatgcagatggtctctgatagctgggaggcttccggggcgaacagacaatgaaataaagaaccattggaactcaaacctccgcaaaagacttcccaaaacaaaaaccaaccaaccaaaacttcgaaaacattcaaccaacatcaagaacaatgtctgtgttatacgcacaaaggcgattaggtgctcaaaggctctgacttttcagaaccagagtagtagtggtagtaccaatcttcttcctatgaaagaacaagtgagctctatgatggatcatgaagctggttcttcgttgttggaagatcttgaaattgattttgataaaatccaatcagagtttctcttccctgatctgatggatttggaaggtttgggttgtggaaacgtaacatcacttgtttcatctgaggagattttaggagattatgttcgtgctgatgaatcttctcagggtaatcttgatctcaatagacctttcactccttgtcttcatcgtggcaacgatgaagattggctccgagttttcaattgttagagcgtatcactagtctacataattacatacatatatatctgtacgaacaaaattatatttgtattttgtttgaaagcttctaatttctaattactaattttgttgtgttttctaatccatagattatcaattttgcactctttttcaattaaagacttatggaaatggcttttgtctttagaataaaatacaaattgcaaaatatcgcaaatacgcaatgaagattatttattttcgatagattttattcaattattatgtgcatgcataaatgatagagcttttattatagcctaactaccgcttaactaccctaccaataaattatacgagggtcattgttcttggtaatacgaaaaaaatctttgcaatattgtcttaacgaaattgaattttaatatacacacatatccatttataggcagacacggtcatacatctaaggatttattgttttttgtttcttatcattcttcggaatcattgtataaatggttattgttgtaacaagagaaaggacatcgggttataattttatagaggaaacctaaatttgtgattgtcgactgtggccgctgacggcggttcagtgtcactagtttatggtcttttatctatgctattgtgggtgcgaatatgtccttttgttaaccttcttaaatattgaaataaggttgttttcggattgtcaatgttattaaacaaatccattctcaatagtttgacaaaaaaaaaaaaaaaatccattctcaataaatagctgatgcaggaaagactattggtttttctgtattttaagttatcggatcttttatatgatataatccattacaaatagacactaattagacaagtgttaaaaatagttcttattatcaatttggcagtgatacataaataaacctattacacctacctattaggtgattatctgcgtatacatacatacacacggatttacattttattatagattttaaaatgtataaataatataccatattttattt

SEQ ID NO: 4 - DNA, 795 bp, Thlaspi arvense
atggggaagagaacaagtaacagtttgaagaaagatgagttaaacagaggagcttggactgatcaagaagacaagatccttaaagattatatcatgatccatggcgaaggcaaatggagcactctcccaaaccaagccggtctcaagaggtgtggcaaaagctgcagactcaggtggaagaactacttgagaccggggataaagcgcggaaacatctcatctgatgaagaagaactcataatccgcctccataatctccttggaaacagatggtctctgatagctgggaggcttccggggcgaacagacaatgaaataaagaaccattgaaactcaaacctccgcaaaagacttcccaaaacaaaaaccaaccaaccaaaacttcgaaaacattcaaccaacatcaagaacaatgtctgtgttatacgcacaaaggcgattaggtgctcaaaggctctgacttttcagaaccagagtagtagtggtagtaccaatcttcttcctatgaaagaacaagtgagctctatgatggatcatgaagctggttcttcgttgttggaagatcttgaaattgattttgataaaatccaatcagagtttctcttccctgatctgatggatttggaaggtttgggttgtggaaacgtaacatcacttgtttcatctgaggagattttaggagattatgttcgtgctgatgaatcttctcagggtaatcttgatctcaatagacctttcactccttgtcttcatcgtggcaacgatgaagattggctccgagttttcaattgttag

SEQ ID NO: 5 - protein, 109 aa, Thlaspi arvense
MGKRTSNSLKKDELNRGAWTDQEDKILKDYIMIHGEGKWSTLPNQAGLKRCGKSCRLRWKNYLRPGIKRGNISSDEEELIIRLHNLLGNRWSLIAGRLPGRTDNEIKNH

SEQ ID NO: 6 - DNA, 813 bp, Thlaspi arvense
atgagagattcaaactcaatccttgatctgtctcttcagatcagccttcctaactctcacgccggagaacttcttcacggcggtgaccgaagctccaccacaagtagtgattctggaagcagtctcagtgagttgggccatgagaacaacttcttcaacaaacctctcctaagcttaggttttgatcatcattatcgttatcaaaggcactcaaacatgatccaaccacaaatctacggtcgagatttcaagagaagctcatcatcaatggtttgtcttaaacgaagcattcgagctccaagaatgagatggacttctactctccatgcgcactttgtccatgctgttcagcttcttggcggccatgaaagagctacgcctaaatcagtgttggagttgatgaatgtgaaggatctaaccctagctcatgtcaagagtcacttgcagatgtatagaacagtgaaatgcactgataaaggatcatcaggagaaggaaaggtagagaaagatacagagctgatgacagaggacaataataataatgaagaagctgacgaaggaactgacacaaattcgccaaactcatcatctgtgcaaaagacccaaagggcttcttgttcatccaaaaagagagtgtgtatgaacatatctacacaagcagaacctcacttgggatcaactcgtcacactaatgatgatgggaagaaagaggcgatcaacgctcatctcaatttggaattcacattaggccggcaaagttgggggatggactattcggaacccttaagagatctaactcttctcaagtgctaa

SEQ ID NO: 7 - protein, 270 aa, Thlaspi arvense
MRDSNSILDLSLQISLPNSHAGELLHGGDRSSTTSSDSGSSLSELGHENNFFNKPLLSLGFDHHYRYQRHSNMIQPQIYGRDFKRSSSSMVCLKRSIRAPRMRWTSTLHAHFVHAVQLLGGHERATPKSVLELMNVKDLTLAHVKSHLQMYRTVKCTDKGSSGEGKVEKDTELMTEDNNNNEEADEGTDTNSPNSSSVQKTQRASCSSKKRVCMNISTQAEPHLGSTRHTNDDGKKEAINAHLNLEFTLGRQSWGMDYSEPLRDLTLLKC

SEQ ID NO: 8 - DNA, 4752 bp, Thlaspi arvense
gaggtcggtcgattcaaacttcttttccctttttgtcttttgtgtatatttccatatctatcctttattctccgagtaataaggaaattcttctttatcttttgaattagtccgatgtttccggtcttcaaaggttatccttaagagatttccttaaatccgaactaggtcggcacggtcttcctagtcttgatgggcttaagttattgcgagggaaaaccttttaggaaatgtattcattttccctctaacaatgttttaagtatgtattaacaaaataaaaattaatatatgaaaacaattaataaaaataagtaagatgcttatgtgaagcagaatattcccgaccgtgtgtctacttaccgtggccaaagacatcgcatgaaaaaacaaaccaaagagtaaggtaaattaaatagaatgtatttaactagattgaacttggagtaattagttgtctttctctttttgcacttttgaaaagataaacaaaatttccttttggagctactttgtggttcaaacaagaatccccatggcaaaacggcagttactttgtcagtcaacttttgaaatctgaggctttcaaggattgtaagaaatattaaatacaaaactctgttgtattttccatcgaccctaagagacaggccttttcaagcctatctttttagcattggaaattttaaagtgttttattttatttatttaaaatagtaaaaacatgcaaatcatagggtactcattatctaattatcacactcactctctttcctcggcttggtttaacctttttaaccactgatcaaataatacgtagccaatttgtccaaaatcttccaacttcttttcctcctttcttacttctttaaattattttagtattcgtcataaatcaaaagatacgttgtcttgaacatgtacacaggttgtagtatttgtgtgaaacacaaaagtgtatactagtattttagttaggaaatctacaccatatatttacttttcttataaattaagtatatgactttgacattattttaatgatacataatcttttgattactttcatcagttattttttttgctaaaaattaatttaaatgttgtttttaacctactaaagatttcatgcgtacgtcagagactattttttgtttctcatatcatgatatgtaatcagaaaagtgaaaacaggttgccatgtacattcatttatgatacacaattgattttttttttctttttaccaaataacaggttattcatcagttgccacattggcgaaagatgaaaatactattttcattgatccgcataaataaaaaatcctttgattttaccactttgttatggtagtcatttacgtagttttaattcggttatctacccgaattacgttttttttgcttaaaagttgaaaatgttattctacgtagggactaacatctggtaatacagtactacgataagagtgaataattaagagttttataaataggttatatatttaaatcatttgtacacgtagaaaataaaacatattattcttaaaaaaagacgatagactatgtttattgagataaagacaatagttacgtcgttgcttttcttgctctctctctctccatttctttctctctccgctatttaaatagacaaaggattaatgaaaaagtagagagatgatgatgttagactccagaagcagtatgagagattcaaactcaatccttgatctgtctcttcagatcagccttcctaactctcacgccggagaacttcttcacggcggtgaccgaagctccaccacaagtagtgattctggaagcagtctcagtgagttgggccatgagaacaacttcttcaacaaacctctcctaagcttaggttttgatcatcattatcgttatcaaaggcactcaaacatgatccaaccacaaatctacggtcgagatttcaagagaagctcatcatcaatggtttgtcttaaacgaagcattcgagctccaagaatgagatggacttctactctccatgcgcactttgtccatgctgttcagcttcttggcggccatgaaagtattttgctttcacattttcctttttaaaagaaataatcaagatttatgtcaagtaaaatgttttgaaaccaaagtactaagatttgttgcttatttgctggtctcaggagctacgcctaaatcagtgttggagttgatgaatgtgaaggatctaaccctagctcatgtcaagagtcacttgcaggtccatctctattttaatttatttttcttatatattttattataaaaatagtaatggaatctcataagaatgcaataggtttaagtaaacatttatgaaagtgtatctatttggtccactagctaacacatgattgcgtagttgaaataaacttgtattagctatactttttttattttttatttggttttgatttttaaaggatgtgtgtttgttgatgcagatgtatagaacagtgaaatgcactgataaaggatcatcaggtatgcattcaaaccggattggctgatttttgaattcctactggatgtaaatgtaactatctcatttttttttttttgttttaatttgtatttgtttcttcttgggaataacaggagaaggaaaggtagagaaagatacagagctgatgacagaggacaataataataatgaagaagctgacgaaggaactgacacaaattcgccaaactcatcatctgtgcaaaagacccaaaggttactcttttatctattctattttgtaaaaactttgcatttaatctctttgcctttgttatgcgcgaattttgatgaatccctcttctagtcgtatgtgaccctgcttgtccatttttataaatagaaaaaatttctatgatctcagttaaattgtgtgtattcactgttgatagtaaataagtaggttcaaataaaacaatatatgaatatgaatgtccaacaatatgaattattattagtagatttctcaaatgtgttttttatcatttaaatttgaacagggcttcttgttcatccaaaaagagagtgtgtatgaacatatctacacaagcagaacctcacttgggatcaactcgtcacactaatgtacattctttaacaaattgttacaatgttattatagatgtgcactctcacatatacgtacatatacccttctgtatactgtttctaaaatgtgaaatctttggaaataggatgatgggaagaaagaggcgatcaacgctcatctcaatttggaattcacattaggccggcaaagttgggggatggactattcggaacccttaagagatctaactcttctcaagtgctaatcgtttagcttggagaactacaacaaataagtcagcttaggttatcaatttaacataattaacttgtttgatcgtaatagacattggaagaatcattatcatcatatatgaatttcttacaaaaaatgttctcatttttttttttgggatgtaaacaagagattcggattaagtagtagctatgttatggttgtagtggatgagaagggagtgcaagttcaagtagagatgaacttatgattggttgccaccaaatatgcatggtggatttgttggtagtttttttttatgttttcattgactgctattcatattgtcgcagtgaatatatatttaaatgattttgttttgattctttgtcttgatttggattagaaagtagaattcggcaaaactagaggtttttttactgatattctgcatgacaataaaactctcagttctatttaaatttttcgctttgttattgatacatataccgtttaaaaggatacattaaacaatactgaatagtactctcaaattctgtttttcgaaggatatgagttggtagatatttcacaacatcaaaaaacgaaggtgaaaataccttcttcagattgcaaagaattacagaaattttgtgccaggtttcgcagaccgcctgttgtaagagatcgcaacatatatcttgaaccaatccctcgaaagcataaataaacaaagtagacactaagaaatgattatataaataatataatatgtttaatttattaattatatgtagctgcaattgcttcatgaatattatgtggtagagactgacaaaaataaatggaaagagacacttcatcacaacatggtaatcataactcttcatccagaaaacttccatacctcttcatttatatgagaatttaatgttataggcaatctaataaatactctccctttgaaggtgcatccaactgaaaagcagggaccgatgccttccctttctaggaaacttgtcgcgccttaccagaacagtactctgccaagtccaatctagacttcatattgtcctttgtcttcctttgacattgagaacggtgttgattatgttgtctataaaattcttcgtattgtgcataacatctagattatgccttatcaaatggtccttccaaaaagacaattcccaaaatatactcatcttatacaaactatgttggtcaccacaagcgttcacatgataatgataaccttccatgcattggccatcagaataacatgccatatgctggaaaaaggctaatagtccacattaatactgaccccatgacaatattctgctgacaagaaacatgaaatgcctgaacactatgctcctataatatttgcagctcataaaacaatgattggagaaatt

SEQ ID NO: 9 - DNA, 1041 bp, Thlaspi arvense
atgacaatcttggatcagaccgttgtaacaaccggatcgaagaaggcttgtgtcatcggtggcacaggaaacttagcttctactctcatcaagcatttgcttcaaagtggctacaaagttaacactacagttagagatccagagaatgagaagaaaatggctcacttaagggtacttcaagaacttggggacctcaagatcttcaaggcggaatttactgatgaagagagtttcgattcaccagtttcgggctgtgattacgttttccatgtcgcaacgcctatcaactttacatctgaagatcccgagaaagacatgatcaagccagggatacaaggagtgaccaatgtgttgaaatcttgcttaaaatcgaaatcagtcaagcgtgtgatctacacttcttcagctgctgcggtttccatcaacaatctttctggacctggacttgtgatgaacgaagaaaactggactgaccttgattatctcacaaaggagaagccgtttaactggggctacccagtgtcaaagatactagcagaaaaggcagcttgtaaatttgcggaagagaacaagatcgatctagttaccgtgattccggcactcatatccggaaaatctctcctctcggatcctcctccgagcagctcatttctctctatgtctttaatcaccgggaatgaaatgtatctgaaaggtctcaaggaaatgcagaagcaatctggctccatctcgttcagccacgtgaaggatttggctcgtgcccatttgtttcttgcggagaaagaaactgcgtctggtcgttacatttgctgtacttacaacacaagtgttccggagattgcagattttctcaggcagagatatcctaagtacaatgtgctgtctgaattcgaagagtgcttatcaagtgcgaagctgacgctatcttcggaaaaactcatcaatgaaggctttcgattcgaatatgggattaatgagatctatgatgagatgatagagcacttcgagtccaaaggattaatcaaagctaaagaatcttga

SEQ ID NO: 10 - protein, 346 aa, Thlaspi arvense
MTILDQTVVTTGSKKACVIGGTGNLASTLIKHLLQSGYKVNTTVRDPENEKKMAHLRVLQELGDLKIFKAEFTDEESFDSPVSGCDYVFHVATPINFTSEDPEKDMIKPGIQGVTNVLKSCLKSKSVKRVIYTSSAAAVSINNLSGPGLVMNEENWTDLDYLTKEKPFNWGYPVSKILAEKAACKFAEENKIDLVTVIPALISGKSLLSDPPPSSSFLSMSLITGNEMYLKGLKEMQKQSGSISFSHVKDLARAHLFLAEKETASGRYICCTYNTSVPEIADFLRQRYPKYNVLSEFEECLSSAKLTLSSEKLINEGFRFEYGINEIYDEMIEHFESKGLIKAKES

SEQ ID NO: 11 - DNA, 4124 bp, Thlaspi arvense
gccgccgccgccgcgaaggccaagaagaaggatgtggaggctccgctgacaattgctttaggcttacaggcgccgaaatcgggaacgaagcggccgagtgaagggacttcaagggaggctaattcaaagcgagctaagaaggttacttcaggggacgacgagaagaagatcggcgaagactcaaagaaacctgcttttcagagactgtggtctgaggaagacgaaatcactgtgcttcaaggtatgatcgatttcaatgctgatacaggcaagtctccttacgaagacacgaatgtgtattacgatttcatcaagaaaaagattagctttgaggttagcaagaaccagttcatggataagattaggagcttgaagaagaagtatataggcaaaggaaagactgccttcacgaaacctcacgatcagagatctttcaagctgtgccaacacatatggggacctgaaggaatggctctcgagtcagcggttaagtccaatggcgtatcgagaaagagccagaagaagaagaagcttgactctgtgaagcaagagctgtcttttgcttcttcccctaatggcaaaacggttgatgatgataaaaaagtgttgatccatggaggagatgtggagtcttcggttgctgcgaagaagcatgattggttcgagagctcgtttcttgttcgcgccattgccggtttgggagttgatgagtatactgtgaaacagaggtggagcttggtgcctgttgagacgaagaagaaggttgaagagaagatgaagatgttgcaggccaaggagattgattttgtgttggagaagacacagtttttgcatgaggttacatcgatgatcgctgaagcatctaagaagaagacattagatatatagatttgatccgaaaatgccaatgccaatgcctctctcttttgttttttgaatcttaggaattatctcttttacttcccttttatgatctatcaatctatgtaatttttctggtttttctggtggtttttaatatggaactctctctcttttggatttgttgcttatacataaaagcaccatggaagtaaattctacatggtgaaatatgaagaagatccaaacaaactgttttttttttttttatgaaatgggtttattcaggatgaattttgttgaattgaggctaaaaaattttggtgttctctaaaacaaaaagttaaatgaaactttcagctcaaagatcaaattggttgaagaaagcaaaactcttttcacaagtagatgatatcaaatcagcaagtcaattaaaagtttgactctttttttgattcttaggtgagagagttagttattaaagaagaggaaggtaacacaaaattagttgcttcaaaactcacgtgcttaccttctaaaaagactttttgatcaatggttgtaccaaatgtgcaagaccataagctttgccactataaaaacgagtgctaaggccataaactcataacagtcagatctaaatatctgtgtttaagaactagtatcagatgacaatcttggatcagaccgttgtaacaaccggatcgaagaaggcttgtgtcatcggtggcacaggaaacttagcttctactctcatcaagcatttgcttcaaagtggctacaaagttaacactacagttagagatccaggttcttcatttcttctttctttcttctcttgaggttctttgagtgtttagtgactcttttattctgaatttgcagagaatgagaagaaaatggctcacttaagggtacttcaagaacttggggacctcaagatcttcaaggcggaatttactgatgaagagagtttcgattcaccagtttcgggctgtgattacgttttccatgtcgcaacgcctatcaactttacatctgaagatcccgaggtctgattttcaacagattgtgtatgtttttttttctctgactcttaagagaaacgttttcagctatcctttgtttgtgtttccatgtacagaaagacatgatcaagccagggatacaaggagtgaccaatgtgttgaaatcttgcttaaaatcgaaatcagtcaagcgtgtgatctacacttcttcagctgctgcggtttccatcaacaatctttctggacctggacttgtgatgaacgaagaaaactggactgaccttgattatctcacaaaggagaagccgtttaactgggtaatttacaatttcttgcgagccaagatagggtttacttggaccagtttacttactacatctctgttcttttctagggctacccagtgtcaaagatactagcagaaaaggcagcttgtaaatttgcggaagagaacaagatcgatctagttaccgtgattccggcactcatatccggaaaatctctcctctcggatcctcctccgagcagctcatttctctctatgtctttaatcaccggtaaacaccaattttactgtttgactccttctgttaaagtttcacaataagaaagtcaaagatgaatggtttttttttgttagggaatgaaatgtatctgaaaggtctcaaggaaatgcagaagcaatctggctccatctcgttcagccacgtgaaggatttggctcgtgcccatttgtttcttgcggagaaagaaactgcgtctggtcgttacatttgctgtacttacaacacaagtgttccggagattgcagattttctcaggcagagatatcctaagtacaatgtgctgtctgagtaagcatttatatccacagaaactgaaaatcttaatggaaaattctgaattttctcgttaattttcgctgtgaaatttggcagattcgaagagtgcttatcaagtgcgaagctgacgctatcttcggaaaaactcatcaatgaaggctttcgattcgaatatgggattaatgagatctatgatgagatgatagagcacttcgagtccaaaggattaatcaaagctaaagaatcttgaaatttataatgtgaagatatggatttatgagtatatgagtctttgttctcattctcattctataaatggcattaaataataagttggttgatttgatatgtattttgatatacacacctagaaaatgaaaaacaagatttttcaagctttatattactctacgaagctgattagtaattttacttctaagtttctcacatttcacaactaccttttttctttcccatgttataaatatataacttttttttcagcataaaaagaagttgtggaaagaatgcgacgaactattttaccaaaaaaaaaggtgacaatctacatggaaaaaagtaaataaaatgtgttaataaactttcgatttaaacaagttgtgtatttacatacaattgatatatatatatataatactttataatactgtattcttttatcaaaaggatatatactgtaatatttagcaaattatacataaaactatcaaattaaagagtatgatgtattccactgaaaacataaaaaatgatatatgtagaaaccaacctgagtgtatgcgcgtggatattcgtttagtaataatgataatgatatgagtagactatattacctaaagccaatcaacatatgaccaatctacaagctcgagctttattagatcaaaacataaaaattggtatatgtagaaatgttgtctaaattaaaccaagatgaaaaacatgagaaaacattaaaacatcactttttattcttggtgatttgttattagaactccgagcaaagaacgaatctgtgaggacatcatgcatgtatgtcttactcagcgtaatagggacattgtgcaagtcactgcaagagatctccaatgatgatctaacggatccaagaaagtaaaggaaaagaagaaggaagagcagattggtgagactcggatccaagaattagaggaagatctgaaggatctgaagcggatgtgcactgttctagaaacctttctagggaaagaaaaggcaaatgtgtttgaagccagagcccctgctatgacgttagatgagttgtataatgacttaggttctgcatgatgcgttgtggtattgtatgttcagggccggctctaagattatgggagtttgaaacaaaataaaaaat

SEQ ID NO: 12 - DNA, 1461 bp, Thlaspi arvense
atggatccgacgacgccgtttctcggtggcgaggtcgaagaggattatgctccggcgaggacatggagcgacgtcaagcgagtttttgctacggagtcggccaaaatgtggatgatcgccgctcccattggtttcaacatcatctgtcagtacggagttacctccatcaccaatattttcgtcggccatatcggcgaggtcgagctctccgccgtcgccatctccctctccgtcatcggcaccttttccttcggcttcctgcttggcatgggaagtgcacttgaaacactctgtggacaagcatttggagctggtcaagtccatatgttaggcgtttacatgcagagatcttggattatcttattcgtctcctgcatctttctccttcctatttacatattcgccacgccgattctgagactcctcggccaagcagaggagatcgccgttccagctggagaattcactcttttaaccatccctcagctattctcactcgccatcaacttcccaacctccaagttccttcaagcgcagagcaaagtcatcgcgattgcttggatcgggttcatcgctttcgtcctacacgtcggtatgctctggctgtttataatcgtgtttggttggggaacaaacggtgctgccttggcgtttaatctcaccaactggggaacagcgatctctcaagtcgtttatgtgattggttggtgtaatgaaggctggtctggtttgtcttggttggcatttaaagagatttgggctttcgttagactctccatagcatctgctgttatgctttgtcttgagatctggtacatgatgagtatcatcgtccttactggtcgccttgacaacgctgttatcgctgttgattccctttccatatgcatgaatctcaatggtctggaggccatgttgttcatcggaataaacgctgctataagtgtccgtgtctccaatgagcttggcttaggccgtccacgagcagcgaaatactctgtctatgtcacggtgttcgagtctctcctcatcggtcttgtctttatggtggctatcatcataggcagagaccattttgcgatcatcttcacgagcagcaaagtacttcaacgcgcagtgtctaagctagcttatcttcttggtataaccatggttctcaacagcgtgcagccagtcatttccggtgtggctgttggaggaggttggcaaagtttggtggcttatataaacttgggttgttactacattttcggccttccctttggatatcttcttggttacaaagcaaacttaggagtgatgggactttggtcgggaatgatagccgggacagcgcttcaaacgttgctactgatgtttgtcttgtacaagacaaactggaataaagaggttgaagagacgatggaacgtatgaagaaatggggagggagcgagacgacatcgaatgatgtaactgcgtga

SEQ ID NO: 13 - protein, 486 aa, Thlaspi arvense
MDPTTPFLGGEVEEDYAPARTWSDVKRVFATESAKMWMIAAPIGFNIICQYGVTSITNIFVGHIGEVELSAVAISLSVIGTFSFGFLLGMGSALETLCGQAFGAGQVHMLGVYMQRSWIILFVSCIFLLPIYIFATPILRLLGQAEEIAVPAGEFTLLTIPQLFSLAINFPTSKFLQAQSKVIAIAWIGFIAFVLHVGMLWLFIIVFGWGTNGAALAFNLTNWGTAISQVVYVIGWCNEGWSGLSWLAFKEIWAFVRLSIASAVMLCLEIWYMMSIIVLTGRLDNAVIAVDSLSICMNLNGLEAMLFIGINAAISVRVSNELGLGRPRAAKYSVYVTVFESLLIGLVFMVAIIIGRDHFAIIFTSSKVLQRAVSKLAYLLGITMVLNSVQPVISGVAVGGGWQSLVAYINLGCYYIFGLPFGYLLGYKANLGVMGLWSGMIAGTALQTLLLMFVLYKTNWNKEVEETMERMKKWGGSETTSNDVTA

SEQ ID NO: 14 - DNA, 4540 bp, Thlaspi arvense
gcagttcacatttaaatagtccaatatgttattattggcaagcaacccgaattgaaatgagacagtggaaacattagcaatccaaaacatcatacgaacctacttctacttataccttagagaagaataatcagattacgagtaacaagaatgaagaacctgagtcgcttagccttaatgttctaaatcaaataactaatctgagctcatttgcaaaacattggcccattttaaaattcttggcactgatacgcagcacaaaaggaggttactgtaaaagcccaatgtgcgtacattcattattcacaaaaaaaaatcttgtttgacttaaaattgtggccccctttttgggtttgtcttttaatttcatgtattttttaattaattgttttctattttggcattaatatggctctattaattataatttatgatacaaaatcagaatggaccgggctgggcctttggtgaagttggtgggctcggtttaagaattttatttttttcattattttgacttgcattaaataaaacaagtcaatgggaaatgtcatcatttatctgactggtttaatgacaaaggtttaatgatgaaacagggaaataaatacaaacgatgacgtaaactgaaaggggaccacaggaccctgtcgtttccgatgaaaaagaagaagaaaattccctctccgattcttcttcctgttcatattcattttacaaacggtacgtaactcactttttaatacttcacttaaggacatcaacctattttcggaaacgacaacttttccactcttggttcgagcttagattgattcaacatttttttcctaattaacttacatatactgtattcattttactgtctaacagtaaactcgagctatcctggcaagtttaatcttctcgacaacttactatatagttgatactatatcactaggatcaattttataaaaaaaaaaacaaattaatcacgtgaaaataattctcacacatgataaataaactaggagtaacaagtttgatgtgacattacactaacaaactttcacaacactaccctatcaatattaaatgtcaaatgatggaaaagagaaaagcagttttatgcttttgaataatcttgtatgcatatttctgatatgtcaaagtacgtggtgtctcatgcaccacccgttagcctcacctacctaatctacttctcaattccatgccgaattcggtaataaatttctcgtacgttttgtttttcctttccgctaattacccaaaaactaaaataggctaataactccttcaatttttattattgttattatttgattagtatggcaaaacaaggggagagagaagtgcgtgattcaacggttttgttatataaaccaaaaccccataattccgcaacaaacattgactcagagtgagagagagagagagagagagagagaagtctgtctgtgtgagctttgggtttaacattttgagactcgcacggagatggatccgacgacgccgtttctcggtggcgaggtcgaagaggattatgctccggcgaggacatggagcgacgtcaagcgagtttttgctacggagtcggccaaaatgtggatgatcgccgctcccattggtttcaacatcatctgtcagtacggagttacctccatcaccaatattttcgtcggccatatcggcgaggtcgagctctccgccgtcgccatctccctctccgtcatcggcaccttttccttcggcttcctggtatgcttttctcttcttctaactgatatctttcatgtaactctgctatgtatcaatcaagagcatcttcttgtgacaaatcgacaagaaacagagtctaatttaggtttgaaaactgcagcttggcatgggaagtgcacttgaaacactctgtggacaagcatttggagctggtcaagtccatatgttaggcgtttacatgcagagatcttggattatcttattcgtctcctgcatctttctccttcctatttacatattcgccacgccgattctgagactcctcggccaagcagaggagatcgccgttccagctggagaattcactcttttaaccatccctcagctattctcactcgccatcaacttcccaacctccaagttccttcaagcgcagagcaaagtcatcgcgattgcttggatcgggttcatcgctttcgtcctacacgtcggtatgctctggctgtttataatcgtgtttggttggggaacaaacggtgctgccttggcgtttaatctcaccaactggggaacagcgatctctcaagtcgtttatgtgattggttggtgtaatgaaggctggtctggtttgtcttggttggcatttaaagagatttgggctttcgttagactctccatagcatctgctgttatgctttgtcttgagatctggtacatgatgagtatcatcgtccttactggtcgccttgacaacgctgttatcgctgttgattccctttccatatggtgagttttgatcaacattttacaatgcttcttgtatcatcaacatctttcccactctttttttttgcatttcatttcagcatgaatctcaatggtctggaggccatgttgttcatcggaataaacgctgctataaggtagtactatcattatctgacacaacttttgtttaacccattgttcagcttgtaaactgatcatgtgtctacctacttgtgtactatatattagtgtccgtgtctccaatgagcttggcttaggccgtccacgagcagcgaaatactctgtctatgtcacggtgttcgagtctctcctcatcggtcttgtctttatggtggctatcatcataggcagagaccattttgcgatcatcttcacgagcagcaaagtacttcaacgcgcagtgtctaagctagcttatcttcttggtataaccatggttctcaacagcgtgcagccagtcatttccggtaacaaaaatctaaaattctcatgttccatcaaaacaaaaaccagaggtctcataagaccataaccgtcccggtttgttcatcttgttttaggtgtggctgttggaggaggttggcaaagtttggtggcttatataaacttgggttgttactacattttcggccttccctttggatatcttcttggttacaaagcaaacttaggagtgatggtaagcgaatacaaagaatgacatgaataatgtagatctttcggacatgcatgtttcataaactgatacgtgagagattataacgttttcagggactttggtcgggaatgatagccgggacagcgcttcaaacgttgctactgatgtttgtcttgtacaagacaaactggaataaagaggtaaagaacacctgagacacaaaaccgtagtatatacactggttcattgagatcgattgacttatggaaatataaaattgtaaaaactgtgatgaacaggttgaagagacgatggaacgtatgaagaaatggggagggagcgagacgacatcgaatgatgtaactgcgtgactatttcttttgttaatattaattaattaattattgtttagctttatatatatgaacatgtaggtctcagcttttttgtttgttttccattggtttggcagcaccagtaactctctatttactatttacgctgtaggaaacttttcattcagtgatgtaacgatgcatgcttttgtcactttgtttctcttggagtaaactaaatgttaggtacattttctcgtgtaacacaaattttattagacggcttttagtcttcaatgcaaattcaagtgacttgtacatagattcctgtcttctacttccatttccttcagaagtcaattgtatgtttccattttattcttctaccggtggaaaataatatagtatcagtacgtaatttttagcgtgcttgtaacacaggatggccgagcggtctaagccacgagactcaagttcttgtcctcctataggaggatatggattcaaatccctcttgtgacataataatttctttaaaaaaaaaatcattttgctatactttgcatatttttctttttctttttaagaatgcatgcatgtcttactttctcgtttctgcttgataggtcgtagtgtcctaataagctcttctgagaaatctcttatttttcttcttgaacgttggattcagcatttcttcattgtgatttttgacttgcgaagatacgcacacttatacattgattagggtcatcctcgtctcaagtgttattgcaatgtctaggtttggacatagcacactagtctttgctatttcatcacccaaaatccattaaatcatggtgatgatttgatttaaagctaatggttttgctaatttgattttttttatgtgtattttttgttctgtaataggtggcgtgagtggaacaacagaagggtggaacacaaacacttattaggtctccctgttttcaacatgatgcatttgattttgttggttatatctcctcaaatgcttgttgcattgcctaaa

SEQ ID NO: 15 - DNA, 2322 bp, Thlaspi arvense
atgtcaatggccgtcgaaatgtcatcgaaacaacccaccaaagatttcttctcctctccagccctctccctctctctcgctggtatattccggaatgcatcctccggcagcaggaaccctgaggaggactttttggggagaagggtagttgacgatgaggatcggacggtggagatgagcagcgagaactcgggacccacgagatccagatcagaggaagacttggaggatcaagaggaggaggaggaggatgaggaggaagacggagcaggaaacaagggcaacaagaggaagaggaagaagtatcaccgccacaccaccgatcagattagacacatggaagcgctgttcaaagagacgccccatccagacgagaagcaaagacagcagctgagcaagcaattagggctggctcctcgccaggtcaaattctggttccaaaaccgccgcacccagatcaaggctattcaagaacggcacgagaactcgctgctgaaagcggaactagagaagctgagggaggaaaacaaaggcatgagagagtcttttgccaaggctaattcttgctgcccaaactgcggaggaggcaccgatgatgtccacatcgagaactccaaactgaaggcggagctggataagcttcgtgcggctctcggacgcactccctacccactccaggcctcatgctccgatgatcaaccacaccgtctcgacttctacacgggcgtctttgccctcgacaagtcccgcatcgtggagattgccagccgagccacccttgagctccagaagatggcctcctccggccaacctctttggctccgcagccttgagactggccgtgacattctcaactacgacgagtatctcaaggacttccctcaagctcaggcctctcccctccatgcaaggagatccatcgaagcatccagggatgtggggatcgtgtttatggacgcacacaaacttgctcagagttttatggacgtggggcaatggaaagagatgtttgcgtgcttgatctcaaaggcggcgacggttgatgtaatccggcagggtgaagggccttcaaggatcgacggtgcgattcagttgatgtttggggagatgcaactgctcactccggttgtccccacaagagaagtgtacttcgtgagaagctgccggcagcttagccctgagaaatgggccatcgtggacgtatcagtctctctggaggaagacgacaacaacaacaacacggaggacaaggaggcttcgctgcttaaatgccggaaacgcccctcaggttgcatcatcgaggacacctccaacggccactccaaggtcacctgggtggagcacctcgacttgtctgcctccaccgttcagcctctcttccgctcctttgtcaacaccggtttggcctttggggctcgacactgggtcgccaccctccagctccactgcgaacgcctcgtcttcttcatggctaccaacgtccctaccaaggactctctcggtccgtccattatttacactctctctctccctctctctctttctccctctcaccttttcttaaccccaatcctcctctcaggagttacaacgcttgccgggagaaagagcgtgctcaagatggcccagaggatgacacaaagcttctaccgcgccattgctgcttccagctaccaccaatggaccaaaatcaccaccaaaactggacaagacatgagggtttcttccaggaagaacctccatgatcctggtgagcccaccggagtcatcgtctgcgcttcttcctccctctggttacctgtttctcccactctcctcttcgatttctttagagatgaagctcgtcgccatgagtgggatgctttgtcaaacggagctcatgttcagtctatcgcaagcttatccaagggacaagacagaggcaactcagtgtctatccagacagtgaaatcgagagaaaagagcatatgggtgctgcaggacagcagcacaaactcatatgagtcggtggtcgtatacgctcccgtagatataaacacgacacagctggtgattgcaggacatgatccaagcaacatccaaatcctgccttgtggattctcaatcatacccgatggagtagaatcaagaccactggtaatcacgtctgcacaagaggacagaaacagccaaggagggtctctgctcacactggccctccaaacgctcatcaacacttctcctgcagcaaagctgaatatggagtccgtggaatccgtcacaaacctcgtctctctcaccctccacaacattaagagaagcctccaaatcgaagattgttga

SEQ ID NO: 16 - protein, 773 aa, Thlaspi arvense
MSMAVEMSSKQPTKDFFSSPALSLSLAGIFRNASSGSRNPEEDFLGRRVVDDEDRTVEMSSENSGPTRSRSEEDLEDQEEEEEDEEEDGAGNKGNKRKRKKYHRHTTDQIRHMEALFKETPHPDEKQRQQLSKQLGLAPRQVKFWFQNRRTQIKAIQERHENSLLKAELEKLREENKGMRESFAKANSCCPNCGGGTDDVHIENSKLKAELDKLRAALGRTPYPLQASCSDDQPHRLDFYTGVFALDKSRIVEIASRATLELQKMASSGQPLWLRSLETGRDILNYDEYLKDFPQAQASPLHARRSIEASRDVGIVFMDAHKLAQSFMDVGQWKEMFACLISKAATVDVIRQGEGPSRIDGAIQLMFGEMQLLTPVVPTREVYFVRSCRQLSPEKWAIVDVSVSLEEDDNNNNTEDKEASLLKCRKRPSGCIIEDTSNGHSKVTWVEHLDLSASTVQPLFRSFVNTGLAFGARHWVATLQLHCERLVFFMATNVPTKDSLGPSIIYTLSLPLSLSPSHLFLTPILLSGVTTLAGRKSVLKMAQRMTQSFYRAIAASSYHQWTKITTKTGQDMRVSSRKNLHDPGEPTGVIVCASSSLWLPVSPTLLFDFFRDEARRHEWDALSNGAHVQSIASLSKGQDRGNSVSIQTVKSREKSIWVLQDSSTNSYESVVVYAPVDINTTQLVIAGHDPSNIQILPCGFSIIPDGVESRPLVITSAQEDRNSQGGSLLTLALQTLINTSPAAKLNMESVESVTNLVSLTLHNIKRSLQIEDC

SEQ ID NO: 17 - DNA, 5982 bp, Thlaspi arvense
aacccataaagagcattcatttccttttaaggtcgctgaaattaatgagtaacgatcagtcaatgcgtctcgttgaccttccaaaacatccgacgtctctttccgttgcatatccctcggctctgtccctgcagctcccacgtcatccatatttcccctctatccaatttttaactttctaacttattcaacaactcttcctccatgcatttacctcattatctaatcgtattgtttactagtagtaatatagcatactagagtagtagattcggattcccggaataatatatattagcataagttattggagcacaaggcatttcaggtttccatgtagctccaataatatcctcttcactctctcttaccaatgcttttccactttcctatgtcacgcaattactagcttgcttgctttacaaccaagttttattaaccaacataaaatatagagatttaatgttgcattttgtaatcataagttactaattgcttgaagaaagagatcacaataacagacaatacgtacacattacatcataaccaggtaagtatatagtatataataaataaataaatagaagtcataataagagaaatgatgatgataatcaaggaggaaagaagaaagcagaaaatgcggttggagaattaggtgcttaaagttagttgagtccatcccagtatctaacggtcaactctctcctctttcgtccttatttgtattttattttgtttttgaaacaataaactgacatacaatatgtctttctctcactactctctctctctctctctctatacacaaattcaattaaagaagagacagagaagttcgccttttgtctgtatacccttaaatcatgcaacccccttattctcattccttctctctgcctacagtaaactctaggaacgacattatgtggtttaaaccgattcaattcatgattagtggcaaaattctatatgattttcaaccacatgatatatgattttcaacagtaatattgtgcggaaaaataatgcacagcattttattctatatacaaaaggtaaattggaaaggagaattttccagatgcaatagcgaatttgctcgaatatttttataaaaaaaaacgaagtcgatatcgacgcctgcaaataatgtagctggccatgtttgcaaagtaatcaagtgtgaataaaattgtaaaactaatggagtatatatagatattaaaaagaagaaggggttggttaaatataattaaatgaagcacctaaaagtcaagcaatagagaaatatctgaaaaacgaccgtttgtatgtataattagaattgaagggctagcttagctatatagccatatacagtatatgtgaaagagtacattttggtacacacacacacaaaaaaaaagaaataaggaaaatatatagagatatataaatagcacaaggaagaaggaggagagggaagataaagcaaataaaaaaattgggagcgttcgtatgtcaatggccgtcgaaatgtcatcgaaacaacccaccaaagatttcttctcctctccagccctctccctctctctcgtacgcgtactctctgttctactactctcgtaaactcatctaaataaaaatttactgtattgtatatatgtatctatttgtgaatggtactgatataaatacaggctggtatattccggaatgcatcctccggcagcaggaaccctgaggaggactttttggggagaagggtagttgacgatgaggatcggacggtggagatgagcagcgagaactcgggacccacgagatccagatcagaggaagacttggaggatcaagaggaggaggaggaggatgaggaggaagacggagcaggaaacaagggcaacaagaggaagaggaagaagtatcaccgccacaccaccgatcagattagacacatggaagcgtacgttcttccttccttaattattattctttatatttcatctgtagctctaatggattaccatttaatcaaattagggtttcaaaacatggaacatttcgattaattggtcttgatgatatatgaatttgatgacctcaactcctccatatatacttcaattatgactagtcatcatcatcatgccctacacatagggattagagtatatagtagtcagtctgtgctgaacagtaggcctcttcatttctactgccatataaaaaggaagaatgcatatttcatgtatttattagtagtgatgaacaaattaatatatattgcagatcgatgatccagcaatagttaattatttgaatgcgtttaattacatatcttgctctttaattttctctcgtactccctagtatatacatgtgtttatactataacataggacgggacaagtgtttccattcaatcaccctatgattaaactaaaaccaagttctttcaaaacaaaaaactaaaaccaagagcactaatgtgtatagctagttagggctcatataattaagagtttaattcatactatgttttcgaataggaggataaaaaaaagatatgaaagaattaattaaatatgaagaatgatcatggagctatgaatgagaaaactgagggttgcattgcaggctgttcaaagagacgccccatccagacgagaagcaaagacagcagctgagcaagcaattagggctggctcctcgccaggtcaaattctggttccaaaaccgccgcacccagatcaaggtatgtatatcgacgtacgtgatgatgatgatatatatggatttcttaagacaaaaagactattcgcttggagctacatatgtatatagttatagtgaaatactgaaatgtaactgaacaggctattcaagaacggcacgagaactcgctgctgaaagcggaactagagaagctgagggaggaaaacaaaggcatgagagagtcttttgccaaggctaattcttgctgcccaaactgcggaggaggcaccgatgatgtccacatcgagaactccaaactgaaggcggagctggataagcttcgtgcggctctcggacgcactccctacccactccaggcctcatgctccgatgatcaaccacaccgtctcgacttctacacgggcgtctttgccctcgacaagtcccgcatcgtggagattgccagccgagccacccttgagctccagaagatggcctcctccggccaacctctttggctccgcagccttgagactggccgtgacattctcaactacgacgagtatctcaaggacttccctcaagctcaggcctctcccctccatgcaaggagatccatcgaagcatccagggatgtggggatcgtgtttatggacgcacacaaacttgctcagagttttatggacgtggtactctttttctttcatttcctccaaatatttacgaatatacttttgtgtatcacatgtaggcaatataaagatatatatacaacgtgcaggggcaatggaaagagatgtttgcgtgcttgatctcaaaggcggcgacggttgatgtaatccggcagggtgaagggccttcaaggatcgacggtgcgattcagttggttagtgaatcaccttttgatagatagtgatgacacgcgagagatgagagctaatataatacattgatggacatattggcagatgtttggggagatgcaactgctcactccggttgtccccacaagagaagtgtacttcgtgagaagctgccggcagcttagccctgagaaatgggccatcgtggacgtatcagtctctctggaggaagacgacaacaacaacaacacggaggacaaggaggcttcgctgcttaaatgccggaaacgcccctcaggttgcatcatcgaggacacctccaacggccactccaaggtcacctgggtggagcacctcgacttgtctgcctccaccgttcagcctctcttccgctcctttgtcaacaccggtttggcctttggggctcgacactgggtcgccaccctccagctccactgcgaacgcctcgtcttcttcatggctaccaacgtccctaccaaggactctctcggtccgtccattatttacactctctctctccctctctctctttctccctctcaccttttcttaaccccaatcctcctctcaggagttacaacgcttgccgggagaaagagcgtgctcaagatggcccagaggatgacacaaagcttctaccgcgccattgctgcttccagctaccaccaatggaccaaaatcaccaccaaaactggacaagacatgagggtttcttccaggaagaacctccatgatcctggtgagcccaccggagtcatcgtctgcgcttcttcctccctctggttacctgtttctcccactctcctcttcgatttctttagagatgaagctcgtcgccatgaggtaccttgtggcatacacttccttcgcacacacagaaccaataaaaccgttttaaatctaactatacatacgtattattatcatcagtgggatgctttgtcaaacggagctcatgttcagtctatcgcaagcttatccaagggacaagacagaggcaactcagtgtctatccagacagtgaaatcgagagaaaagagcatatgggtgctgcaggacagcagcacaaactcatatgagtcggtggtcgtatacgctcccgtagatataaacacgacacagctggtgattgcaggacatgatccaagcaacatccaaatcctgccttgtggattctcaatcatacccgatggagtagaatcaagaccactggtaatcacgtctgcacaagaggacagaaacagccaaggagggtctctgctcacactggccctccaaacgctcatcaacacttctcctgcagcaaagctgaatatggagtccgtggaatccgtcacaaacctcgtctctctcaccctccacaacattaagagaagcctccaaatcgaagattgttgatgacaactcacagcaggtgtgatgattgttgttacatatataagtatatcataatgtatagcagtgcattaagttttgtacaaaaacaaccctctctctctctcccgcaatcatactgttatccaacactttttgcagcattaagagagcatcatactcgactaagaacccaatacacaaaactttaccgaaacaaaagtgggatcagatgaaccaaatgcataaccctgatttagatacacagtaattggatcagaaacgaaggcctgatcaaattccacaacttaaacaatacgcaattcgagcaggaaaacaaaatgcattccataaacagagagaattacacttgattgcaatacacaacaaacagaaacgaaaaacagtaaaaaagacagctttttttttttaccaaaacaaacaaacactcagtgagtcgcattctcctctacgccggctgctgagattccaagggaatgccgaggtcgttcccagcttctcctccgccttccgctttcctgctgctccttgagacgacagcaagcgccacgaatgacttagtcttactgatgggtctgctcttctccagcctcaccacatcgcccaccttgaactgattatccgggtcatgcgcctggtacttcttcttcttcctcacgcgcctcttgtacttgggatgcggagccagcctcaccacctccaccgccacggtcttgtcgttggttgcgcacaccacgcgcccctgcatcgttttcatggctctgatgaccggaaccaatgccggccttcgagggttcgggaataaattgggcttagagagagatgagagtggagtcgagccatgggcgaatggagacgaaagcttcagagcttgcagagatgaggttattagcgacgtcatcgttatccccctcctctatgggatcgatttggaagacgatgaagaagataaggcgatagatcatgttattataatattggcttttgctaaatgggttaacaa

SEQ ID NO: 18 - DNA, 2007 bp, Thlaspi arvense
atggctactacgtataagcctaagaacattctcatcactggagctgctggattcattgcctctcatgttgccaacagattaatccgtagctatccagattacaagatcgttgtgttggacaagcttgattactgttcagatctgaagaatctcgatccttcgttttcttctccaaatttcaagtttgtgaaaggagatatcgcgagtgatgacctcgttaactacctcctcatcactgaaaacatcgacaccatcatgcactttgctgctcaaacccatgttgataactcctttggtaatagctttgagttcaccaagaacaacatttatggtactcatgtcctcttggaagcctgtaaagtaacaggacagatcaggaggtttattcatgtgagcaccgatgaagtctatggagaaaccgatgaggatgctgctgtaggaaaccatgaggcgtctcagcttttacccacaaacccatactcagccactaaggctggtgctgagatgcttgtgatggcttacggtagatcatacggactgccggttattacaactcgtgggaacaatgtttacggtcctaaccagtttcccgaaaaactgattcctaagttcatcttgttggctatgagtgggaagccgcttccgatccacggagatggatctaacgtaaggagttacttatactgtgaagacgttgctgaagcgtttgaggttgttcttcacaaaggagaagtcggtcacgtctacaacatcgggacaaagagagaaagaagagtgatcgatgtggcgacagacatctgcaaacttttcgggaaagatcctgagtcgagcatcgagttcgtggagaatcgaccgtttaacgatcaaaggtacttccttgatgatcagaagctgaagaatctgggttggtcagagcgaaccgcgtgggaagatggactgaagaagacaatggaatggtacattcagaatcctgagtggtggggtgatgtttctggagctttgcttcctcatccgagaatgcttatgatgcccggaggaagagttcctgacggctccgatgagaagaatgactcgtcaagcaacgcggtccagacattcacggttgtaacaccgaacaacaagactggtggttctagtgacaaagctttcttgaagtttttgatctacggtaagactggttggatcggtggtctcttagggaaactatgtgagaagcaagggattacttatgagtatgggaaaggacgtttagaagatagagcctctctcgtcgcggatattcgcagtatcaaaccgacccatgtgtttaacgctgctggtttaactggcagaccaaacgttgactggtgtgaatctcacaaaccagagaccattcgtgtcaatgtcgctggtactttgactctcgctgatgtttgcagagagaatgatctcttgatgatgaacttcgccaccggttgcatattcgagtacgatgctgcacatccagagcgttcgggtattggtttcaaggaagaagacaagccgaatttcactggctctttctactcaaaaaccaaagccatggtcgaggagcttctgagagaatttgacaatgtgtgtaccttgagagtgcggatgccgatctcatcagacctaaacaacccgagaaacttcatcacgaagatctcgcggtacaacaaagtggtgaacatcccgaacagcatgaccatactggacgagcttctgccgatctccatcgagatggcgaagagaaacctaagagggatatggaacttcaccaacccaggggtggtgagccacaacgagatactggagatgtacaagagttacatcgagccagggtttaaatggtccaacttcacagtggaagaacaagcaaaggtcattgttgctcctcgaagcaacaatgaaatggatgggactaaactaagcaaggagttcccagagatgctaccaattaaagaggcgctgatcaaatacgtcttcgaacctaacaagagaacctga

SEQ ID NO: 19 - protein, 668 aa, Thlaspi arvense
MATTYKPKNILITGAAGFIASHVANRLIRSYPDYKIVVLDKLDYCSDLKNLDPSFSSPNFKFVKGDIASDDLVNYLLITENIDTIMHFAAQTHVDNSFGNSFEFTKNNIYGTHVLLEACKVTGQIRRFIHVSTDEVYGETDEDAAVGNHEASQLLPTNPYSATKAGAEMLVMAYGRSYGLPVITTRGNNVYGPNQFPEKLIPKFILLAMSGKPLPIHGDGSNVRSYLYCEDVAEAFEVVLHKGEVGHVYNIGTKRERRVIDVATDICKLFGKDPESSIEFVENRPFNDQRYFLDDQKLKNLGWSERTAWEDGLKKTMEWYIQNPEWWGDVSGALLPHPRMLMMPGGRVPDGSDEKNDSSSNAVQTFTVVTPNNKTGGSSDKAFLKFLIYGKTGWIGGLLGKLCEKQGITYEYGKGRLEDRASLVADIRSIKPTHVFNAAGLTGRPNVDWCESHKPETIRVNVAGTLTLADVCRENDLLMMNFATGCIFEYDAAHPERSGIGFKEEDKPNFTGSFYSKTKAMVEELLREFDNVCTLRVRMPISSDLNNPRNFITKISRYNKVVNIPNSMTILDELLPISIEMAKRNLRGIWNFTNPGVVSHNEILEMYKSYIEPGFKWSNFTVEEQAKVIVAPRSNNEMDGTKLSKEFPEMLPIKEALIKYVFEPNKRT

SEQ ID NO: 20 - DNA, 5240 bp, Thlaspi arvense
acccttattttcaatcacagctccccaagatagatcagttaagcaacagcaacacacatatggccattgatgctaagctgttgcaggcgcaatcacagttcggtccagcgggagcagcagcggttgcggtagcggcacaccggaacattggcacaattagttacggcgcagcatcgtagactcatcaaacaaacagcattttcagacacatctttaacttacatcaccctccaaatccaggcaacgcgaaaccaggtgattccggtctcggtctctttatgtaagtattattcagccaggctctgatttaaacaactttgcagtgatattaataaaagactttcagttgtaactcaccagaacaagatcgcttagatcagtctgatcccgggttatcaccggtgattgtttcggttatcttgtttgctccatagtctttgaatttgttataagcgtagttcatcgaagagaagaaaaccgtcgtgattatatacttcttaaacttcaagatcggtcccattactccttaattgttcttcaacaatgatgaatctctttgtctatcagaaaattgattgatctatttggctatatagagagaatcattaggccgaaaattgtggaagtcaacaaaagtcattggtccgtagatctttctcatccgtaaatcaatcttttgcacattataattagccattttattcaatggttaccagtaaaaaagatatgtaaaagataatttcgaattcttgacgccattaaagtgtctatataatttacccgccaatttaagataaccggttttatgggcctgaactcagcacattaaaggttaacatttactataataattcaatgaacttaactccttttcttcaattacatgaaaaagtgcatttttgtctacttgattttttaattgatgaaaaaggaagtaaattaattattccgttacgtgaccttaagcatcagcattgaatcatctgttatgtttaatttcaggtcttttcttgttgaactgatgattgatatcaggttgacatgtgatatttctattcagtctagaattatttgtttttctaactgaacatatgtacgttttatcataaacaaatcagggattttattaaatcccaagtttaaccttccaataaaagaaatcatatttttattcagtttaaatcattttaagaaatatatatcagacaaaaatgcaaaatattttgtttacttcttccacaattaattaatctccttaattatacaaattttattctctttttattttttggaattttcttctattagtatagattttgtgtgaaaaaataaacaaaaaaaagacatcaaatttttatgtcggacgctaagctcacgtaaaatccgtaatatctaagacaagtaagggtaaatttgtcaattgacccctacggttctccgtaactgtctcaggatatatgaggcgcactgttcagagacgctccgtagaccgtagattccctcttcttcctcctctctctctctctctctctctctctctctcttctcatagaagtgtctctctctctctcttaggattcttctctgattctaacctgaattgtgtcggtacgtgatatgttgctctctttttgttgctgctgaaatttccataatgctttaagttaattttgcgaaatgctatacgtgagtaacggacaagtgtacaacatcagacaactgatcttgtttttgttcttttttttagatttctgtgttgtcggtttatgatcccatatgaaaagttcattatttttgttcgtataagatctggctactgaatttattcggttttggcgattggatctggatctgcctttattctgatttcctttcatatgatccgttctgaattttcgaatgatactgtgacgttattgttgttgttgttgcagatacttgatttcaaatggctactacgtataagcctaagaacattctcatcactggagctgctggattcattgcctctcatgttgccaacagattaatccgtagctatccagattacaagatcgttgtgttggacaagcttgattactgttcagatctgaagaatctcgatccttcgttttcttctccaaatttcaagtttgtgaaaggagatatcgcgagtgatgacctcgttaactacctcctcatcactgaaaacatcgacaccatcatgcactttgctgctcaaacccatgttgataactcctttggtaatagctttgagttcaccaagaacaacatttatggtactcatgtcctcttggaagcctgtaaagtaacaggacagatcaggaggtttattcatgtgagcaccgatgaagtctatggagaaaccgatgaggatgctgctgtaggaaaccatgaggcgtctcagcttttacccacaaacccatactcagccactaaggctggtgctgagatgcttgtgatggcttacggtagatcatacggactgccggttattacaactcgtgggaacaatgtttacggtcctaaccagtttcccgaaaaactgattcctaagttcatcttgttggctatgagtgggaagccgcttccgatccacggagatggatctaacgtaaggagttacttatactgtgaagacgttgctgaagcgtttgaggttgttcttcacaaaggagaagtcggtcacgtctacaacatcgggacaaagagagaaagaagagtgatcgatgtggcgacagacatctgcaaacttttcgggaaagatcctgagtcgagcatcgagttcgtggagaatcgaccgtttaacgatcaaaggtacttccttgatgatcagaagctgaagaatctgggttggtcagagcgaaccgcgtgggaagatggactgaagaagacaatggaatggtacattcagaatcctgagtggtggggtgatgtttctggagctttgcttcctcatccgagaatgcttatgatgcccggaggaagagttcctgacggctccgatgagaagaatgactcgtcaagcaacgcggtccagacattcacggttgtaacaccgaacaacaagactggtggttctagtgacaaagctttcttgaagtttttgatctacggtaagactggttggatcggtggtctcttagggaaactatgtgagaagcaagggattacttatgagtatgggaaaggacgtttagaagatagagcctctctcgtcgcggatattcgcagtatcaaaccgacccatgtgtttaacgctgctggtttaactggcagaccaaacgttgactggtgtgaatctcacaaaccagagaccattcgtgtcaatgtcgctggtactttgactctcgctgatgtttgcagagagaatgatctcttgatgatgaacttcgccaccggttgcatattcgagtacgatgctgcacatccagagcgttcgggtattggtttcaaggaagaagacaagccgaatttcactggctctttctactcaaaaaccaaagccatggtaaaatactaatatctataactcatgacagtctcgaaacaaagaagagtgtctttgtttataatctggttctgcttttttctcttcttctttgttcaccaggtcgaggagcttctgagagaatttgacaatgtgtgtaccttgagagtgcggatgccgatctcatcagacctaaacaacccgagaaacttcatcacgaagatctcgcggtacaacaaagtggtgaacatcccgaacagcatgaccatactggacgagcttctgccgatctccatcgagatggcgaagagaaacctaagagggatatggaacttcaccaacccaggggtggtgagccacaacgagatactggagatgtacaagagttacatcgagccagggtttaaatggtccaacttcacagtggaagaacaagcaaaggtcattgttgctcctcgaagcaacaatgaaatggatgggactaaactaagcaaggagttcccagagatgctaccaattaaagaggcgctgatcaaatacgtcttcgaacctaacaagagaacctgagacctgaacagcactcttcgccacaagtgcttacctataactgtttccttttctttctttctctttcaacagaaatgtctttttatgtttactcatcgtcttatgatccttgtaggtagtttcactatattgattctactaaaatatgatttatcattattatttatagagactaaagttttttttttctttctcaaattctacatttcccctcggattttacttactaagagacagtagtacacttataaaaatgaagagccacttactggttgtgatcattagggattccaccaaggcaggttcaaaacacttgaacttgattattaagctatagcctgagaagagaagcaaacaacaagtgttgatttgaaataaaccgaagtatatgatgtgaatttggtcaatattcagggttatagttttcttacgtgaacagttgagggcgggaacgagagagctgagagcgtttaataggggagagaataaggtttcgtagagttgactggggattagcagcgccaccaccaccgccaaatacaggatgtcctcctcctcctgctcttctgtttccaaggtctgttggaattgcgggtgagtcgttggagatgtcgaatggacctgagtttgaactgttctgtcttgctggccaaatctcatctttaggtcctggtgttgcaggagagtaaaacgaccggtctgcgccaaataagtcaacttgatttggagatattaaccaacaatagacttggaatcaaaagaagcactaggctcaaggtagttcattaacctttgcgagggggctctctgttctccatcatgttaactggtgggtttgagaaaaagtcaggttcgtggtgtcgtgggtagaaattgtttgctggttggatggctgtacgtttacatgactcgtattcacttcttagctggtcatacatctcatcgagcttcctcttctgtctggtgtttgaaacaataattacagctgagttagagataaggaacagaaccaggcaaacaaagcgtgtgttaaatcactgaccttgatttctcggagaacttctcttggagctcttgtttatccttggtcaagttttctacctcttgctccatcatctgacacctcttgcccatcttctggtatgctgtatgcacctgctccattttctcgctaaactttgct

SEQ ID NO: 21 - DNA, 1995 bp, Thlaspi arvense
atggctacatataagcccaagaacatcctcatcactggggctgctggattcatagcgtcccatgtcgccaacaggcttgttcgaagctaccctgactacaaaatcgttgtgcttgacaagcttgattactgctcaaacctgaaaaacctcaatccttcgaaatcctctccaaacttcaagtttgtcaagggagacatcgccagtgctgacctcgtcaactaccttctcatcactgaaaacatcgacacgattatgcactttgctgctcagacccatgtcgacaattccttcggtaacagcttcgagtttaccaagaacaatatttacggcacccatgtccttctggaagcttgcaaagtcactgggcagatcaggaggttcatccatgtgagtaccgatgaggtctatggagagactgatgaggatgcttcagtgggaaaccatgaggcttctcagttgctccctacaaacccttactctgccactaaagctggagctgagatgcttgtgatggcatacggtagatcatacgggttgccagttataacgactcgcgggaacaatgtctatggtccgaatcagtttcctgaaaagttgatccctaagttcattctgttggctatgagtgggaagccactgccgatccacggagatggatctaacgtgaggagttacctctactgcgaagatgttgctgaggcgtttgaggttgttctacacaaaggggaagtcaaccatgtctacaatatagggacaacgagagaaaggagagtgattgatgttgccaacgacatctcaaaactctttggaatagaccctgactccaccattcagtttgttgagaaccggccttttaatgaccagaggtacttcctcgatgaccagaagctgaagaagttgggatggtctgaacgaaccacttgggaagaaggactgaaaaagacaatggattggtacactgcgaaccctgagtggtggggagatgtctccggagctctgctgcctcatccacggatgttgatgatgcctggtgatagactctctgatggctctgacgagcgcaaggatgcagacggtaatcagacattcacggtggttactcccaccaaggccggtggttccgcagacaaaacatccttaaagttcctcatctatggcaaaactgggtggctcggtggtctcctaggaaagatatgtgagaagcaagggattccgtacgagtatggaaaagggagactagaagacagagcttcaatcatggcggatattcgcagcgtcaaacctacccatgtcttcaatgccgcgggcttaacaggcaggcctaatgttgactggtgtgagtctcacaaaaccgagactatccgagtcaacgtcgctggtactttgactctggcagatgtttgcagagagaatgatctgttgatgatgaactttgccaccggttgtatatttgagtatgacgctgcacatccagaaggttcagggattggcttcaaggaagaagacaaaccgaatttcaccggttccttctactcaaagacaaaggcaatggtcgaagagcttctaagagagtttgacaacgtatgcaccttgagagtgaggatgccaatctcatccgacttgaacaacccgcgaaacttcatcacaaagatctcgcgttacaacaaagtggtgaacatcccaaacagcatgaccatactcgacgagctcttaccaatctcaatcgagatggcgaagaggaacctacgggggatttggaatttcaccaacccaggagtggtgagtcacaacgagatactagagatgtacaagagctacatcgagccaggtttcaaatggtccaacttcactttagaggaacaggctaaggtcattgtcgcaccacggagcaacaacgagatggatggttttaagctcagcaaggagtttccagagatgctttccatcaaagattcgttgatcaaatacgtcttcgaacccaacaagagaacgtaa

SEQ ID NO: 22 - protein, 664 aa, Thlaspi arvense
MATYKPKNILITGAAGFIASHVANRLVRSYPDYKIVVLDKLDYCSNLKNLNPSKSSPNFKFVKGDIASADLVNYLLITENIDTIMHFAAQTHVDNSFGNSFEFTKNNIYGTHVLLEACKVTGQIRRFIHVSTDEVYGETDEDASVGNHEASQLLPTNPYSATKAGAEMLVMAYGRSYGLPVITTRGNNVYGPNQFPEKLIPKFILLAMSGKPLPIHGDGSNVRSYLYCEDVAEAFEVVLHKGEVNHVYNIGTTRERRVIDVANDISKLFGIDPDSTIQFVENRPFNDQRYFLDDQKLKKLGWSERTTWEEGLKKTMDWYTANPEWWGDVSGALLPHPRMLMMPGDRLSDGSDERKDADGNQTFTVVTPTKAGGSADKTSLKFLIYGKTGWLGGLLGKICEKQGIPYEYGKGRLEDRASIMADIRSVKPTHVFNAAGLTGRPNVDWCESHKTETIRVNVAGTLTLADVCRENDLLMMNFATGCIFEYDAAHPEGSGIGFKEEDKPNFTGSFYSKTKAMVEELLREFDNVCTLRVRMPISSDLNNPRNFITKISRYNKVVNIPNSMTILDELLPISIEMAKRNLRGIWNFTNPGVVSHNEILEMYKSYIEPGFKWSNFTLEEQAKVIVAPRSNNEMDGFKLSKEFPEMLSIKDSLIKYVFEPNKRT

SEQ ID NO: 23 - DNA, 5650 bp, Thlaspi arvense
cctttcgtttgcatttttgtgttacggtgtgatatctggtgaggatgtacatatgtggtaaagtggcaataatagtagctatttataaaattttatcataaatattattttttacatgaaactatatataatacaaaatttttaggcaaacaaaaattattagtcaaaaagtataattcaaaactcacttgattcaaatatcggaatcagcgcgctagatggggtgataagatttaccatctcaactaaatgaccatatatatgactccatataaatataatcaaatagttttgatttaataaaacgtttactattatatacgtttaataaaaaagtactttaccagcttttacgtgagttatggaaaaattatgaaatccaagatgtaatcaagggttgctgtccaaaaaaataaaaaaaaaacattagttaagggttgataagacgtagaaataaatagatcgttacgtaaaacatctgcaggaagtgtattgatttgtaaacgttaaaatacttctctctgaccatttattatatgtcagtcgttataagagaaaacaaaacgcacatgttatattgacatgtggacgataatgtatattgacatgtgaagaagccaactccgtacgtaaagcgccatttgcgctgcaaatactgatcctcaactacagtggattcttttctcacaaaaacatagaccgtttcaaatatatgttcccaaacacttgtgagacattctatacaaagtttatcatgcacccttcctttttttttaacgtcaaaatgatcatgtacttctgtcacattatttttgtacattatgaatatatagacatttgtattctctctttcgccgaatacacacatctatatatttgtaaatgtagcaggtttaaattttggagtaaaagaatagttgattttgaccacatagagaactaatggatcaattctcactaatacaaatatttggtgaaagccttagaggtgagaaagtccaaggcccataaaggcctattacggccacccccggtcacgtaaaaccaagcctcgttctcgttgatgaggccgaatataaaaggcatcatcaaatcaaacatgtgcgtaacgtgatatttaatttagcatttgcaagtaatgatcacttctgttttttcttttagtatttagttcttcacttaagttttccacgttatttattaatatacaggaactgctttttcttattttattggaaaaatcatgttttatgtttgttcaattaaaatttcagcacaatttctttttcatttttttatatgaaaactttaaggtagaaatgggaaattgcgaaaccgaatcatgcggacaaaacgaaatttctgcgttgcctatattttttgttggtaatttttaaaacaataaacaattaatttgacgtgataaaaacaaagggacatgaaaaaactctaaaagcgtagtaatggtaatttggtaatttcaaagtccgctggttctccgtaactgtctcaaattaaaaagagggcttactgttttctgacgctcgttagattccctctctttcttcttcattttctcctcttcgtcttcactgctaattcccttgatctctctccctgtcctccaattttccctctctacaaatatcgactccttcttcaatattagattgatcctgatccgattcgagccggtacgtacctgaactgtttctgtttctctgagctaattcgtgaatgtacgaggttctgctgcgttttattttttttgatggtatagttgacatgttttcaggattttttgttgtatactctgatctttgatgcttgtttatcgttttgccattggatctgctgctcgatctgggcaatttctcgcatttgattgctacatttgtcataacttcgggatctggatctaccttttttttctgatcatttagaatttcgctaacagctttagattttcgtacttatcgcgtggatttggcttcccgctacttgttcagctgtatctgttaaaatctcacaaatttttattgaactgaatcatggggttttcaataggatagatctggttgagttgttctcctcagtagctgtttccttccacatttgagcttaatcgatttcatggagtaatacgggtgatcgtgatttcgttaatcacatctgatccgatgacgttcatgatatatatactagccattatttacctgtttgctggatcttttgtccttcgattaaatctggctgtttcgtcattgacgagtgtactgaaagcttttccgaatgcaaatataatgttttgtgttgttgcagattatatatttatcatcacatggctacatataagcccaagaacatcctcatcactggggctgctggattcatagcgtcccatgtcgccaacaggcttgttcgaagctaccctgactacaaaatcgttgtgcttgacaagcttgattactgctcaaacctgaaaaacctcaatccttcgaaatcctctccaaacttcaagtttgtcaagggagacatcgccagtgctgacctcgtcaactaccttctcatcactgaaaacatcgacacgattatgcactttgctgctcagacccatgtcgacaattccttcggtaacagcttcgagtttaccaagaacaatatttacggcacccatgtccttctggaagcttgcaaagtcactgggcagatcaggaggttcatccatgtgagtaccgatgaggtctatggagagactgatgaggatgcttcagtgggaaaccatgaggcttctcagttgctccctacaaacccttactctgccactaaagctggagctgagatgcttgtgatggcatacggtagatcatacgggttgccagttataacgactcgcgggaacaatgtctatggtccgaatcagtttcctgaaaagttgatccctaagttcattctgttggctatgagtgggaagccactgccgatccacggagatggatctaacgtgaggagttacctctactgcgaagatgttgctgaggcgtttgaggttgttctacacaaaggggaagtcaaccatgtctacaatatagggacaacgagagaaaggagagtgattgatgttgccaacgacatctcaaaactctttggaatagaccctgactccaccattcagtttgttgagaaccggccttttaatgaccagaggtacttcctcgatgaccagaagctgaagaagttgggatggtctgaacgaaccacttgggaagaaggactgaaaaagacaatggattggtacactgcgaaccctgagtggtggggagatgtctccggagctctgctgcctcatccacggatgttgatgatgcctggtgatagactctctgatggctctgacgagcgcaaggatgcagacggtaatcagacattcacggtggttactcccaccaaggccggtggttccgcagacaaaacatccttaaagttcctcatctatggcaaaactgggtggctcggtggtctcctaggaaagatatgtgagaagcaagggattccgtacgagtatggaaaagggagactagaagacagagcttcaatcatggcggatattcgcagcgtcaaacctacccatgtcttcaatgccgcgggcttaacaggcaggcctaatgttgactggtgtgagtctcacaaaaccgagactatccgagtcaacgtcgctggtactttgactctggcagatgtttgcagagagaatgatctgttgatgatgaactttgccaccggttgtatatttgagtatgacgctgcacatccagaaggttcagggattggcttcaaggaagaagacaaaccgaatttcaccggttccttctactcaaagacaaaggcaatggtaatatactactacatcacataaccaaatcacatgtgatcctcaaactgtgcaactctgttcataaatcctctgtttctattttcgccaggtcgaagagcttctaagagagtttgacaacgtatgcaccttgagagtgaggatgccaatctcatccgacttgaacaacccgcgaaacttcatcacaaagatctcgcgttacaacaaagtggtgaacatcccaaacagcatgaccatactcgacgagctcttaccaatctcaatcgagatggcgaagaggaacctacgggggatttggaatttcaccaacccaggagtggtgagtcacaacgagatactagagatgtacaagagctacatcgagccaggtttcaaatggtccaacttcactttagaggaacaggctaaggtcattgtcgcaccacggagcaacaacgagatggatggttttaagctcagcaaggagtttccagagatgctttccatcaaagattcgttgatcaaatacgtcttcgaacccaacaagagaacgtaataccctcagtaacacatacacacacacacacttcctctttatctgttcattgttatattattatcttgcaggtagtttcaccactataatgattctactataattttattttgtcatatgattcatttactctttttttggctttctacgtcgaacatgtagctctcttgacgcattctacgtcacaacacattttgttttcattaatattatttattaaacgataaaattgcttgaagtttattactttcactattgattcctccttttagttttcatctcaaaagagcagaggacagagattaagaacgaaacagcattgactgataacttatttccctatgcttttaaacttgaggtttctatttgttacaaaacaatgtctttcataaagttaaatctttctattgcataaatcgaaactgcaaactcaaaatgtaatataaattaaaccttctgtacttcctgtccccaaatcttcaccatacgaccatctaaaagcagaatttttcacactacgaacaacattccataatctgatcatccttgcaacaaagcataccgattcgtaagccttcaatttgaatgaagacgtaaaatgatgaataaaaggtaagagagaggaacagaaaaagctcagcaccttgaaatttgttgttctcttcacatagcttgagcgtattgttgtctagacaatggtggaatttcttgtcccgtcataaaatttaaagtcaaaagtcagtagtagttggtgattgattggctcctgagttcttacaaaggaggagaacacttaaaaaacagagtatgagaatataccttctgcctctgtagacaaccaatcatgtgcacagaacagagcctgtctaatatcagggctcaaggaactctggctatcatcgatcaccggtctcccggagttgaacgttgaatcaggcgcaaggatcgacatcggcgtccccaagatatcgcgtgccatcatagagaggatagggtatctcggcgtatggaccttccagtaattcagaatgttgaactcgccactacgaggaaagattggttcagacaagtacttgtccaagtccgatgttgtgttctggctctgagatgtctcgtggagaaacttgtcgaatcctttcaacctgtctctagtgtccatacctgctctacctaagccagagccagagtaggaagagtcgtccccaacaatggctgagcatatc

SEQ ID NO: 24 - DNA, 1092 bp, Thlaspi arvense
atgggtagacattcttgctgttacaaacaaaagctgaggaaagggctttggtctcctgaagaagacgagaagcttctcaatcacatcacaaatcacggccatggctgctggagctctgtccctaaactcgctggtttgcagagatgcggaaagagttgcagactgagatggatcaattacttgagacctgatttaaagagaggagctttctctccagaggaagaaaatctcatcgtcgagcttcacgctgtcctcggaaacagatggtcacagattgcagcaaggcttccgggaagaaccgataacgagatcaagaatctgtggaattcaagtatcaagaagaaactgaaacaaagaggcattgatccaaacacacacaaacccatctctgaagttgagggctttagcgacaaagacaaaccagcaacaagcgacaataaaagaagcagcaacgatcataagtctccgagttcctcctctgcaaccaaccaagacttcttcctagaaaggccatctgatttctccgactacttcggttttcagaagcttaacttcaactccaacctcggactctctgctgcaactgattcttcactctgctccatcattccggcgcagtttagccccggaaacatgtctggttctgtcttccagactccggtatgcgtaaagccttcaattagtcttcctccggacaacagttcgagcaccgtctccggaggagatcatgtgaaactggctgcacctaattgggaatttcagacaaacaacgcctccagtttcttcgacaatggcggattctcatggtcaatcccaaattcttcttcttcactagtcaaacccaatcataacttcgaagaaatgaaatggtcagagtatttgaacacaccgttcttcaatgggagcactgtacagagtcaaagctcacaaccgatctacatcaaatcagaggcagattacttagccaatgtttcgaacatgacagatccttggagccaaacccagaacgagaatttgggcacaaatgaagctactgacgtgttctccaaggatcttcagagaatggccgtctcctttggtcagtccctttag

SEQ ID NO: 25 - protein, 363 aa, Thlaspi arvense
MGRHSCCYKQKLRKGLWSPEEDEKLLNHITNHGHGCWSSVPKLAGLQRCGKSCRLRWINYLRPDLKRGAFSPEEENLIVELHAVLGNRWSQIAARLPGRTDNEIKNLWNSSIKKKLKQRGIDPNTHKPISEVEGFSDKDKPATSDNKRSSNDHKSPSSSSATNQDFFLERPSDFSDYFGFQKLNFNSNLGLSAATDSSLCSIIPAQFSPGNMSGSVFQTPVCVKPSISLPPDNSSSTVSGGDHVKLAAPNWEFQTNNASSFFDNGGFSWSIPNSSSSLVKPNHNFEEMKWSEYLNTPFFNGSTVQSQSSQPIYIKSEADYLANVSNMTDPWSQTQNENLGTNEATDVFSKDLQRMAVSFGQSL

SEQ ID NO: 26 - DNA, 4198 bp, Thlaspi arvense
aaaataattaattctaacttatgacttaaaaaccttgtatacgtctagctaaatcttattttcgacgatcttttttaggattgggtcccaataaacaaatggataaacggtaagagtctaattacgagaggccatgtccagataacgtaagaaaactacaaaaattcaacatgtgaatatttgagggaaagtttgggtaaatggacaaagaatataccctctctattatgactggcttaaaggcaaaaaaagggagaaaattgccaaagagaagtgagtccatttaaatttaaaaatgtataaagcaaacaaaagagagacttaattattctcattcatctgcaaaagaaaccatgtatttaaagcaaaatttctaaattccgttatgtagacatttaattccatttaatcatttctggaaacattaaccaatgatgacaatttcttgctggttataaacctttcccattatttcctttaattgatgcgttcatcttcacaaagatttagtccacatttagcatttgcttttaattcattgcagaagtctttcatgacgacaacaatcaactcttctttgtccacattcttatctagctatacgatctacctcgtgtgttattttaattcttccgttctcactgtaaatcatttttgtatagcgcttccaccgctaactattgaatatcacttttcaatacattaatcgttacaataagtttgtagctgcaagaaaaaatttagactcggatgcatttggtaacatagatatcatataaaacttttaaactttttctcgtcatgcatcactcaaagagtgctatatccttgtcacataccaaaaacgttttaggagcacgcattgcttcaaactctcgtctatgtgcgatttcgatacatttttctaattactctcaagtctcaactaagcacacttaattatggatttcttttttaaaaatagcctatttctcgatttacaccactgtaaatatatttccataaattctatatcgaaccatatactacatgagtatttttaagtgaaaactaattattttgtgacataaaaaacctgatatacgtctaccaaaaaaggttttttttgtaaaccatgacttacgtgaatctccgaaataaaaatctttagaaaagttgttgaggtcacgctggcttttggctgcgtacgtatagagtggtccgtaacatcttcgaggacaaactgaacataaatgagcatgtctccactacttagaaccacacttactattaattttaaaagaagtttttttttttttttatcaattgttgcatttgtatgtatgatcataatgggtccatttggagatgacgaatgtatgatgattagagtgatgtaaaggtcaaaactacatgaactccatctcttaaccctgattattttaccattggtgtgaaccaatctgatgtggaccaatcatattgtttttacaaaagctaaaaaagatgtacatactttttgctatttaatctttaaagagagtatagaatttcaacaaacccttccgaagaaagtgacttttcttagtcctattaatactctctctctctctggagatctgttatttcgttttctccacctttctcttcagattccattaaccttcaaaagttttaaatacatgctctctgctcaaagcgtttttctttcgttacttgtaaagtaaaacacagagctctcttctctttcatcgttcctttgctcagcattgcagctttaataaaccaaaatgggtagacattcttgctgttacaaacaaaagctgaggaaagggctttggtctcctgaagaagacgagaagcttctcaatcacatcacaaatcacggccatggctgctggagctctgtccctaaactcgctggtaacattttcttccttaattcatgggatacaaaacatgaacttaaaaaggctaccttttttgtaataacaattcacaaatctgagtctactacaggtttgcagagatgcggaaagagttgcagactgagatggatcaattacttgagacctgatttaaagagaggagctttctctccagaggaagaaaatctcatcgtcgagcttcacgctgtcctcggaaacaggtaataattcatagaaaacagaggatcatgtttgtgtcttaagcttcctctgtttttaacagaggatcatgtatatcttttaaccttcctctgtttttttatcagatggtcacagattgcagcaaggcttccgggaagaaccgataacgagatcaagaatctgtggaattcaagtatcaagaagaaactgaaacaaagaggcattgatccaaacacacacaaacccatctctgaagttgagggctttagcgacaaagacaaaccagcaacaagcgacaataaaagaagcagcaacgatcataagtctccgagttcctcctctgcaaccaaccaagacttcttcctagaaaggccatctgatttctccgactacttcggttttcagaagcttaacttcaactccaacctcggactctctgctgcaactgattcttcactctgctccatcattccggcgcagtttagccccggaaacatgtctggttctgtcttccagactccggtatgcgtaaagccttcaattagtcttcctccggacaacagttcgagcaccgtctccggaggagatcatgtgaaactggctgcacctaattgggaatttcagacaaacaacgcctccagtttcttcgacaatggcggattctcatggtcaatcccaaattcttcttcttcactagtcaaacccaatcataacttcgaagaaatgaaatggtcagagtatttgaacacaccgttcttcaatgggagcactgtacagagtcaaagctcacaaccgatctacatcaaatcagaggcagattacttagccaatgtttcgaacatgacagatccttggagccaaacccagaacgagaatttgggcacaaatgaagctactgacgtgttctccaaggatcttcagagaatggccgtctcctttggtcagtccctttagctttttttttttcttcttttctttattctaacagatgtagagaacaaaaaaatatacaatacatacatacgtacagtggatttaagtctgtatattccatgagctgtctttatttttacattttttaagtgtgttttatacgtcaaatattcttctattttttgcaaacctttcagtctcatactatatatacacttttatttcttttgttttgttataaagattatgatgcatagaattctcgatgatttcagaggcctgtgtttgcaattaatctgttgaagaacaatgatgaaagtaataaatcagtttctgtctgtttccgtgaacgagttgtaatccagagtcacatccttcaccatttttcagacctgtaatgaattaaaagacaaaaaaggacaaaaacataaaactaaagcaaatcataataaataaactaaagtgggaattagctcaactaataagaagggacacttttttcgaaaggacccgagttttaatacgatgtaaattttttaaaaaaaaagatttctcttttctgaaatcaatgactgatcacatatttgagagattagaaatcgaatacccctaatttcttcgggctattataaactttgaaaaaggtacgtatgtcgtttttgcttagtcttatcagagaactggaattgtccccattgacggcgtcggaatattctttagcggtagaaaattcggaacagttcgagaattttctatttttttgtctgttaaataaaatagttatatgatttgaccttaataaacatgaaggaggtgatgactgatgagaaggtgacttcatttttaatcctaaaaagtcaattgatttattttataacccatatttttttttttagattctaatccaaaacaattacttattacttttttagaaataacctaacgcaataactcgactgataggtaaaactaaggtactataatatgtttgttttgactttaaatttaaagacgatgctatatttttttgaaaatgaaaagaaattgatctatcaaacacataagtctagattcaacagtaattataaaaatagaataaagagagaaaagttaatattttcttggcattatgagaaatcaaatatatttaacctata

SEQ ID NO: 27 - DNA, 939 bp, Thlaspi arvense
atgttctcatcactctccaaccacaattcaccacaatcaatggagtcaccacaatacgagatctcttcaagctcttcttctgaaaaacctagatactactttcaatcatctgatatattccccaacctcactcaaaaccctagtaacagcaatacccaaatcgagtcgttaccgcttatcgatgggataaatttaaactcaaaccttaacctaaaccttaagccaccgtatgttgaaaaagaagaggaagagaaagaagaggaggaagatcacgttgatctgagcttatacatcggccttcctagctctgataattcgagaaacggtgttaaactgccgaagaagaaaaatgggaaggacatcatcactcatgacgctggaaaacagatggagaatgaactttccggcaaagcatactggattccggcggtggagcaaattataataggcttcactcatttttcttgccatgtatgcttcaagacattcaatcgctacaacaatcttcagatgcacatgtggggccacggttcacaatacaggaaaggaccagagtcacttaaagggacgcagccacgagcaatgctagggatcccttgttactgctgcgtcgaagggtgtaggaaccacattgaccatcctcgatccaagccgcttaaagacttccgaacgctccaaacacactacaaacgcaaacacggccaaaagccctatgcgtgtcgcatctgcggtaagctgttggctgtcaaaggcgattggcgcacacacgagaagaattgtgggaaacgctgggtttgcgtttgcggttctgactttaaacacaaacgctcccttaaggaccatgttaaggcttttgggcctggtcatgggtcttatctaaccggtttgcttgacgagcaggcctctcattcttctctctctgagaatttgttcttttaa

SEQ ID NO: 28 - protein, 312 aa, Thlaspi arvense
MFSSLSNHNSPQSMESPQYEISSSSSSEKPRYYFQSSDIFPNLTQNPSNSNTQIESLPLIDGINLNSNLNLNLKPPYVEKEEEEKEEEEDHVDLSLYIGLPSSDNSRNGVKLPKKKNGKDIITHDAGKQMENELSGKAYWIPAVEQIIIGFTHFSCHVCFKTFNRYNNLQMHMWGHGSQYRKGPESLKGTQPRAMLGIPCYCCVEGCRNHIDHPRSKPLKDFRTLQTHYKRKHGQKPYACRICGKLLAVKGDWRTHEKNCGKRWVCVCGSDFKHKRSLKDHVKAFGPGHGSYLTGLLDEQASHSSLSENLFF

SEQ ID NO: 29 - DNA, 4025 bp, Thlaspi arvense
ttattgtttatcaccagtttggttgtcattaattaataagtaagatttgtgtttagtgacggctgattccgtttctagtgagtcagatgcgagatgattgaaaaccgagaagacgatgactccacaaaataagattttgtttaagttttataattgagttttagcgaaattcgttttcaatttttttttttagctttattttttttattgagaatttaagaattataaaagttttttaggtaaaatttgaagaaattttgattaataaattatttaatgaaatagctttaaattattggttgtagaagatgacataacagttttgaactctactattgattaattatttttgctgatgtggcatattgttttattcttattagttagttttttcataatttaatgatgtggtaatttgttatattcttattaactgattattttgatgattatttttgcttatgtgacaccttttagagagcaggaaatctatccttttatataaaggagattagattttaccgatcatgtattatttagtagccaattccatacgtaaaaaaaaagatttttacaatttggttataaatagcctgcatgttttatcggtcctatcttgattgtatatcgtaaaaaaagatgctgactctaagaaaacgaatttcatatggaccgtagtaacagggcccacgagtaattagggttttaacggctgacattttgatctctcatacatctaagtatctaactagaagtgttgaccgttagagaagaattaaataacttacatacatacaaaaacataagtcgaagaataatcataacagtgcatcttctacaataatgataacaaaaaaagtaaattagaaattagcatttattccaattaatacccatattcgaaaatgcacatggtagaaaagcaaaaaaagcttacgtaaattccaaatattgtcaaacccctgcaatgacaaagttgccaaaaattgaagaggttggtccacacaatttaaggttctttgcttcacactctatttataggcaaagagatgaaacagaggagattaaattgcttcttaacaaaggttgttttcactcaaccacatgccttctcaagtgtctgctgctcacattccccgagattctcatttactttttcctctatttggtacgtactttatattacaattctatttgtttctttgattattcgttttgttcatacttagttatcataaacatacatagttgatcttatattatacagtaaatttgataaatgtttctcttaattaatttactcacgcaatttaaaggagacgattgatacgcgggcctacttacgcacctgcatgattattagttataaaagttattgcaaacattaaattactttgatagctagagagcaattattatataaagctaatttttaattgtagatatacatttagtcgaaagttaaaaagaaaaatgaaatccctaaacaaacgttcccaaatgttctcatcactctccaaccacaattcaccacaatcaatggagtcaccacaatacgagatctcttcaagctcttcttctgaaaaacctagatactactttcaatcatctgatatattccccaacctcactcaaaaccctagtaacagcaatacccaaatcgagtcgttaccgcttatcgatgggataaatttaaactcaaaccttaacctaaaccttaagccaccgtatgttgaaaaagaagaggaagagaaagaagaggaggaagatcacgttgatctgagcttatacatcggccttcctagctctgataattcgagaaacggtgttaaactgccgaagaagaaaaatgggaaggacatcatcactcatgacgctggaaaacagatggagaatgaactttccggcaaagcatactggattccggcggtggagcaaattataataggcttcactcatttttcttgccatgtatgcttcaagacattcaatcgctacaacaatcttcaggtacaaaccaatgttatctcatgcgcattacgtgcatgcataaccaaataaaatcttaattcatatttgaatttgtttgttagagaacaaacggagaaaatcctattcgatttatatgtttataacccccttatctaatgttatgagttagaatgaatttatacatacataatcaaaccctaagttgactaactatatattattttgtagaataattgttaatatagatctgtttggatgcatggttgagatttaattaaaatatactgttaaataaacccaaatttaaaatgaatttaatagtttttctccatataattaattaacgtttcctttaaaatttcatccaaattaataattaatagattacttcagtgaaacaatatgatcgatcaacaataagattgtaatgattaatgaaccattttattagttgttaaacttatatttgattaaaaaaaggtggggggtatttgttatgaaaatttatcttgaaatcgtcagtctaaccattgttatccatttcattttttgttattacatatactgatatacaaatctttgttgacaccaaatatgaattcagatgcacatgtggggccacggttcacaatacaggaaaggaccagagtcacttaaagggacgcagccacgagcaatgctagggatcccttgttactgctgcgtcgaagggtgtaggaaccacattgaccatcctcgatccaagccgcttaaagacttccgaacgctccaaacacactacaaacgcaaacacggccaaaagccctatgcgtgtcgcatctgcggtaagctgttggctgtcaaaggcgattggcgcacacacgagaagaattgtgggaaacgctgggtttgcgtttgcggttctgactttaaacacaaacgctcccttaaggaccatgttaaggcttttgggcctggtcatgggtcttatctaaccggtttgcttgacgagcaggcctctcattcttctctctctgagaatttgttcttttaaaactttgtgcatctatcagtcttttgacgtgtgttgtccgtttatttagtctagaataatgtggtatctaataattctcgtagtgaataatatcataatctacttgatatgagaggtcaacatatttagtcccgcagttaataatatcataatttggtgcaccaactaagggaaatgactatcagccacacttagggattactcattaatcgtagactcataaaagctatatgtttaaaaatgctagtttgtatacatatcattagccacacttagggattacgcataaaccgtagactcataaaatctatatgtttaaaaatgttagtttgtataaaaggagatatatatgaaatgagtaaggaagtcacattcaagagcaagtgtagtgtgctttccgagaaatttcctccacatgtccagacggtacgaaatgccagttaattccaattctatcattattgatctgaatgtgatcgcaaaacatgatttgattagtttcctctctttataatttactaaaataaaatgacgaccatataacatcatttttcagaaggaaattaaaacatatcaagaatattcatgtaaaatagttaaaatatcagttaaaaatgttaccattctatacatattatattttatatacatggactgaattcgacaatattggtaaatatcaataaatccaaaatcctgattatttgtaaatcaataaaatagtattatgatacaaaccaattcatatacggtgattcgaaatttcagtacatcatgaacatggaacaatggattttatgaactgatgagttgtccaacgttcgttacgtgcatgcattcaatgcctcggtgccacattactcaccttttatgtatcctctctccattgtttttttttttttatctaacttattgggtatccaaattcatttttgatccttattttagtgaaaccatgcatgtcctacgtactatcgctcgtcatatttaaaggaacagg

SEQ ID NO: 30 - DNA, 966 bp, Thlaspi arvense
atgttctcatcactctccaaccacgattcaccacattcaatggagtcaccagactcaccacaatatgagatctcttcatgctcttcttctgaaaaacctagatactactttcaatcccttgatctcttccccaacctcactcaaaacgcttgtaacaacaataacctaatcgagcctttaccacttatcgatcggatagactcaagctcaaaccttaaccttaaccgtaagccaaaggcattgtatgttgaggaaggagaggaagaggaagaacaggaggaagaggacgtggatgtgagcttacgcatcggccttcctggctctgataatttgagcaacggtgctaaattttcgaagaaaaatgggaaggagatcatcactcacgatgccggaaaacaatcagagaatgaactttccggcaaggcatactggattccagcagtggagcaaattataataggcttcactcatttttcttgtcacgtctgtttcaagacattcaaccgctacaacaatcttcagatgcacatgtggggccacggttcacagtacaggaaaggaccagattcacttaaagggacgcagccacgagccatgctagggatcccttgttactgctgcgtcgaaggctgtaagaaccacattgaccatcctcgctccaagccgctcaaagactttcgaacgctccaaacgcactacaaacgcaaacacggccaaaagccctatgcgtgtcgcatctgcggtaagcttttggctgtcaaaggtgattggcgtacgcatgagaagaattgcgggaaacggtgggtttgcgtttgcggttccgattttaaacacaaacgctccctgaaggatcacgttaaagcttttgggcctggtcatgggtcttatccgaccggtttgtttgatgagcaggcctctaattcttctgtctttgaaagtttgttctgtgtgatcggtgagtattag

SEQ ID NO: 31 - protein, 321 aa, Thlaspi arvense
MFSSLSNHDSPHSMESPDSPQYEISSCSSSEKPRYYFQSLDLFPNLTQNACNNNNLIEPLPLIDRIDSSSNLNLNRKPKALYVEEGEEEEEQEEEDVDVSLRIGLPGSDNLSNGAKFSKKNGKEIITHDAGKQSENELSGKAYWIPAVEQIIIGFTHFSCHVCFKTFNRYNNLQMHMWGHGSQYRKGPDSLKGTQPRAMLGIPCYCCVEGCKNHIDHPRSKPLKDFRTLQTHYKRKHGQKPYACRICGKLLAVKGDWRTHEKNCGKRWVCVCGSDFKHKRSLKDHVKAFGPGHGSYPTGLFDEQASNSSVFESLFCVIGEY

SEQ ID NO: 32 - DNA, 3923 bp, Thlaspi arvense
cacgaaacaagttcaattaaatttaacggaaataaatggtaattaatgaaagtttgaattgtattaattactgcttccacgaaacaaccaaaaaaatcatttgacaaagtaatttgtgtacggtattagccacatggggccaatcctctatgtatatcggagttgttttgccaaatgcccaattcttactctagtaaatattaaaccattttgtagatcctaatcttgagtcaactcaaagtcctatgtttggaaactaaaaataagtttaaatcctctagactacgactaagttgtaaaaagaaatgttcaaaattccttagacattgaaattgaatacttcaattaaagaaaattttaccagcatgttcatagtagtagaccaccacagaacaaaattaatagtttttacattgcattcttatataataattttggagtataattgtaattataaacaaaataactaaaagaaaaggaaagtattcttgacatatttataggtactaatttgctagtacgactattaattatggagattaaatctagtatttgactaaccagaaacattttaaaggtaagtgataagttgataacctcgcaattatttttgaaagctattaatcactttagcagaatgtatacaagttctatattaacaagtttatctcaaaatcttgagatcctactaataaatcataacttttctcttattggtatgtcgaatctagtgtttaccaaactagaggtgttgaccgttagagacaattaaacaacttacatacatacaaaagtacaagccgaagaataatagtaataacagtgcattttctacaataattaaaacaaaaaagtatattaaaaattagcatttattccaattaataccaatattcgaaaattaatatggtagaaaagcaaaaagcttacgtaaattccacagattgtcaaaaccctgcaatgaaaaagttgccaaaaattgacgaggttggtccacaaaatttaaggttctttgcttcacactctatttataggcgaagagatgaaacagaggaaattaattactccttaacaaaggttgttttcactcaaccacatgccttctcaagtgtctgctgctcacattccccgagattctcatttacttactcctctatttggtacgtcctttatattacaattctagtattttttttttcattattcgttttgttcatacttcgtttcataaacatatatagttaatcttatattatacagtaactttgataaatatgtatcttaatttactcacgcagtttagagagacgattgatacgtggggactacttacgtacctgcatgattatataagttataaaagttattgcagaacattaaattactttgatagctcgagagcaatcattatataaagctatatttttaatcacaaatatacatctactcgaaagttttttttttaaaaaaaagatgaaatccctaaacaaacgttcccaaatgttctcatcactctccaaccacgattcaccacattcaatggagtcaccagactcaccacaatatgagatctcttcatgctcttcttctgaaaaacctagatactactttcaatcccttgatctcttccccaacctcactcaaaacgcttgtaacaacaataacctaatcgagcctttaccacttatcgatcggatagactcaagctcaaaccttaaccttaaccgtaagccaaaggcattgtatgttgaggaaggagaggaagaggaagaacaggaggaagaggacgtggatgtgagcttacgcatcggccttcctggctctgataatttgagcaacggtgctaaattttcgaagaaaaatgggaaggagatcatcactcacgatgccggaaaacaatcagagaatgaactttccggcaaggcatactggattccagcagtggagcaaattataataggcttcactcatttttcttgtcacgtctgtttcaagacattcaaccgctacaacaatcttcaggtaccaatgttatctcaaccaaattaaaaccagaattcaaattcgtttttttgtttctttatttaataaaaatagactttaatatatatatgtttggatgcatggtaaagaaaatatttattgaatagaccatggtttaaattcaaattacaagtttgattggctatcgttttaatagtttttcctcttataattaactcttcctttaatagttattcaaagagatttcaaccaaattaatacacagatttcttcaatgaaacagtatgatcgatctctaacaagattgtaatgattgatgaaccatgttattattagttaaaataaaattggagtcaaagatatgtgtatttgctgtgaacatttatcttgaatacggcagtcaaaccattttttatcaatttcattttttgtttttacgtatgcaaatctttgttgactccaaatatgaatgcagatgcacatgtggggccacggttcacagtacaggaaaggaccagattcacttaaagggacgcagccacgagccatgctagggatcccttgttactgctgcgtcgaaggctgtaagaaccacattgaccatcctcgctccaagccgctcaaagactttcgaacgctccaaacgcactacaaacgcaaacacggccaaaagccctatgcgtgtcgcatctgcggtaagcttttggctgtcaaaggtgattggcgtacgcatgagaagaattgcgggaaacggtgggtttgcgtttgcggttccgattttaaacacaaacgctccctgaaggatcacgttaaagcttttgggcctggtcatgggtcttatccgaccggtttgtttgatgagcaggcctctaattcttctgtctttgaaagtttgttctgtgtgatcggtgagtattagagtaactgagaggaatgtaactgagagaaaaaagaaaagtaataattaaaataattgaaaataataagtaagagcatctagatagtccttaccaaaaaaaagatcatctagatagtctttccatagtatctgatttatataatactaatataatgtatttatataattaaattataaattaataaagagatgaaccaattcttaacagacatttgcctagagacatatctttattcttaacaaacatttggctagaaacatatctaatagtttcttgtttcaaaaatgtcttcgctttttttctgtttttctcccttcctttttccttattttttttatttttcttattcactaaatatactcccataatatctgctatataatattaatataatatatttatataattaaattaaaaattcataaagagatgaaccaattcttaatagatatttggctaaatacatatttaatatttttttgtttgaaagatatctttgctatttttttctgtttccttctcttcttttcttcttatatttcttattttttttattcaataaatatattttaaaaaacaccaattttcttataagaatatctgaaaataattgagaataattaaattaaatattttcttttagtaaaacttataattatatatatgctaaaaagatatgtgatatttattattctatctttaaagatttttttatcgtgaatcactattttcagttatccaacctaaaatgaatactcagagagcaaccacatcgaaagtgttagagattgaatgaatacagttcttaaaaggtttatttcacattaatgaagtctatcaaaacaaaatttatctaattacatctctataacaaaaatgataattctaaagttaaatgaaaaaaaaaaacaaaaaaatagagagaatttttctttaaaaaaaagataagaaagatcaataaaaccgacttcctcacattataaatagaaaagtcttcat

SEQ ID NO: 33 - DNA, 1707 bp, Thlaspi arvense
atgtcacaatattccttcttctatttcttcctaatctctcttttcctctacgaaaattgcattgcgtatcgctacacattcacggttattgaagctccatatagcaaactgtgtagcacgaagaagattttgaccgttaatggtcagtttcctggaccagtgttaagggcttacaaaggtgacaccatttacgttaacgttcgtaaccaagctagtgaaaatatcacattgcattggcatggtgtagagcagccgagaaacccgtggtcagatggacccgaatacatcacacaatgcccgattcaacccgggtcagattttacgtacaaaattttactttccatcgaagacgcgactgtttggtggcatgcgcatagctcgtggacacgtgccaccgtacacggtctgattttcgtgtatcctcggcctcctgataccctgccttttccagaaccggactacgaagtccccttagtttttggagagtggtggaagagggatgtgagagaagtagtggaggatttcatgaggaacggaggtgaacctaatgtgtccgatgctttgactatcaatgggcatcctggtttcttgtatccttgctctcaatcagatacattcaagctcgtggtagagaagggcaaaacctaccgcattcggatggtaaacgccgcgatgaacctaattctcttcttcgccatcgcgaaccacaaactcaccgtggtcgccgccgatggccactacaccaaacctctaaccgctagttatatcaccatatctcctggccaaacgctagacctgttactatacgccgaccaaagtccagagagcacttataacatggcggccagagcttaccatagcaaccccaacgttgggttcaacaactctaccaccgtcgggatcttacgttactactcttcaaacgacgccggaacgtcttcatcagaacgttacccgtaccttcctggctacaatgacacctcagcagctttcgatttcttcacaaaaatcaaaggcttatactccagagtagctcccgccaaagtttcacgtaggataatcacgacggtttcgataaatctcctcaagtgtcccaacgactcgtgtgcaggcccaaacgggtcgaggttagcggcgagtatgaacaacatatcgttcgtcacaccgagccacgtggacatactaagagcttattaccttcacattaacggcgtttacggaacgcggtttccggagttcccaccgcggatattcaatttcacagcggacgaccaaccgctgtttttgcagactccgaggctggcgacggaggtaaagaagtttcagtacggggagacggttgagattgttatacaagggacgagtttggtaggtggtggaatcgatcatcctatgcatctccatggttttagcttctacgtggttggtttagggtttgggaattttaacgcacgtaaagatccctccaactataatctagacgatcctccttacagaaacacggcgactgtgcccaggaacggttggatcgctatcagattcgtagctgacaatccaggggtttggttcatgcactgtcactttgatagacatcaaacgtggggtatgaatgttgtcttcattgttaagaatggaataaaaccaaatcagaagattctacctccaccgcctggcttaccaccttgtgaccaatttgagaatctataa

SEQ ID NO: 34 - protein, 568 aa, Thlaspi arvense
MSQYSFFYFFLISLFLYENCIAYRYTFTVIEAPYSKLCSTKKILTVNGQFPGPVLRAYKGDTIYVNVRNQASENITLHWHGVEQPRNPWSDGPEYITQCPIQPGSDFTYKILLSIEDATVWWHAHSSWTRATVHGLIFVYPRPPDTLPFPEPDYEVPLVFGEWWKRDVREVVEDFMRNGGEPNVSDALTINGHPGFLYPCSQSDTFKLVVEKGKTYRIRMVNAAMNLILFFAIANHKLTVVAADGHYTKPLTASYITISPGQTLDLLLYADQSPESTYNMAARAYHSNPNVGFNNSTTVGILRYYSSNDAGTSSSERYPYLPGYNDTSAAFDFFTKIKGLYSRVAPAKVSRRIITTVSINLLKCPNDSCAGPNGSRLAASMNNISFVTPSHVDILRAYYLHINGVYGTRFPEFPPRIFNFTADDQPLFLQTPRLATEVKKFQYGETVEIVIQGTSLVGGGIDHPMHLHGFSFYVVGLGFGNFNARKDPSNYNLDDPPYRNTATVPRNGWIAIRFVADNPGVWFMHCHFDRHQTWGMNVVFIVKNGIKPNQKILPPPPGLPPCDQFENL

SEQ ID NO: 35 - DNA, 5054 bp, Thlaspi arvense
catgcacgtaagaaactaaatcaacacataaggtaacgaggctcggaatagttgggtttcggatttttatttttaaaaagaaagcatcacctaaccaaaactcataagggcatctccatattaaaaaatacaaattaatagaatggaaaaagaaagatagagacgtatctcgtttgaactttgaaatatgtttagcaacgtatctaattaagtgtcatattctgattagtttatattatttttagatactctatttaagatatgcaccgttaaaggtgttctaaagcatcttcatttactctgatagtatatccaaaacttattataataatataatttatttgtgtaataaaatattaaattattaaaagtgtgatgcatatattaaaaatgacagatattgagaaacatatctcatgtcatgctcttttctttgaaaaacagttcgtaatttctctcattctctctctttctttctaattaatttttttattatccagatattctctgaaataccgttgttgcaaatacttttagaacacctttaacagtgtataatctcaaatagaatatctaagatttttttttattaatataaaaaaattaaactaactaatacttgacacttggtcagatacatttctagataggattctctatctctctccatcctttccattattttgtacattttaattattataaattggtcatatatgactttcagatattattctcgaattttccatcacttaccaacatttgttaaaataattttccgtttaaaatagtttaatagtatatattaacaggttacaggtatgaaaatgactttagtatgagatagggagtcgagagtttttaaaatattcgaatactttagacttctcaaattacccatttaaaaatattcaataacttagacttctcgcattacccaaaataccaaatttgtctgaaaccaagctatatctgaattcttttgtcctgtattttaattactatacttcgaacagtatattcagatatctgaacaattcgttctcacctcttaccttctattactggtttcaatactcgaaataaatgctattgctaaaaagtctgtttgttacttttacactataaatttagaatgttatttcccttaagttgaaagttacgtttgaccgagagatgtcaagtattttcaagagtattacgattcttttcagacatagatattctaattaacttttaaagcttacgatacgaagacaggatttgtgtatgaacatcgatggcataacaacatatcttgaatcttgtccaccagagttatctggggggcagttttgaaaatataaaagatctgtaaggttaataaaaaaaacattatcttgtaattccgtagttcttatatcgaaactgttactaatttgagaaagacgtggagagctagaggcgtctataaatatatattcctctctcagaaatcataatatacctaatttattaaaaaagtctctcaaaatgtcacaatattccttcttctatttcttcctaatctctcttttcctctacgaaaattgcattgcgtatcgctacacattcacggtgagttcaaaattaattaatcaatttagtcaggcgtgagtaaactaacttaaaactgatggtatataggttattgaagctccatatagcaaactgtgtagcacgaagaagattttgaccgttaatggtcagtttcctggaccagtgttaagggcttacaaaggtgacaccatttacgttaacgttcgtaaccaagctagtgaaaatatcacattgcattggtatttcatccaaaaccctttttttcgtcttcttaattatgtaaccattttaaatacaagaacataaacgaaatttcgatggttgaataaaaacaggcatggtgtagagcagccgagaaacccgtggtcagatggacccgaatacatcacacaatgcccgattcaacccgggtcagattttacgtacaaaattttactttccatcgaagacgcgactgtttggtggcatgcgcatagctcgtggacacgtgccaccgtacacggtctgattttcgtgtatcctcggcctcctgataccctgccttttccagaaccggactacgaagtccccttagtttttggtacaaaccaggacatataacaaaagatcagtgaagttgcttttttttttttttttttttttatctctcttaaattaaaattaatttcataaaaacttgacaggagagtggtggaagagggatgtgagagaagtagtggaggatttcatgaggaacggaggtgaacctaatgtgtccgatgctttgactatcaatgggcatcctggtttcttgtatccttgctctcaatcaggtttcttttactttttccctttctcctattaatttcttattttgtttttaatatacagttgtgggataaaaactaattgtggagatgaaataaaatttagggatattgatcattgaaacaaattgtgaaatgattcaaacgagcattttttttttcaagtcaactgtttttaatttgtttttcctcgttttttcaaaagtttcttactaatttagttagttaaacataattaatgtttgatcaaattgtccaaaaattagttaagaacttacgagtggttgataaaaaaaaaatcacgaggcatattaattcaaaccaaaatagttgtgtttgtatttattagttcttaaaaattgtgctcataaatttgaaactagcatttgcatgcatatttatgtttaaaacctagttagtaaagtccgttattgacatgcatacgttacgtatacgtatgtttaacagatacattcaagctcgtggtagagaagggcaaaacctaccgcattcggatggtaaacgccgcgatgaacctaattctcttcttcgccatcgcgaaccacaaactcaccgtggtcgccgccgatggccactacaccaaacctctaaccgctagttatatcaccatatctcctggccaaacgctagacctgttactatacgccgaccaaagtccagagagcacttataacatggcggccagagcttaccatagcaaccccaacgttgggttcaacaactctaccaccgtcgggatcttacgttactactcttcaaacgacgccggaacgtcttcatcagaacgttacccgtaccttcctggctacaatgacacctcagcagctttcgatttcttcacaaaaatcaaaggcttatactccagagtagctcccgccaaagtttcacgtaggataatcacgacggtttcgataaatctcctcaagtgtcccaacgactcgtgtgcaggcccaaacgggtcgaggttagcggcgagtatgaacaacatatcgttcgtcacaccgagccacgtggacatactaagagcttattaccttcacattaacggcgtttacggaacgcggtttccggagttcccaccgcggatattcaatttcacagcggacgaccaaccgctgtttttgcagactccgaggctggcgacggaggtaaagaagtttcagtacggggagacggttgagattgttatacaagggacgagtttggtaggtggtggaatcgatcatcctatgcatctccatggttttagcttctacgtggttggtttagggtttgggaattttaacgcacgtaaagatccctccaactataatctagacgatcctccttacagaaacacggcgactgtgcccaggaacggttggatcgctatcagattcgtagctgacaatccaggtacgtacacttacataaacctctaactttgatttggttcaaatctctttttaatattttgtgtttttgtaggggtttggttcatgcactgtcactttgatagacatcaaacgtggggtatgaatgttgtcttcattgttaagaatggaataaaaccaaatcagaagattctacctccaccgcctggcttaccaccttgtgaccaatttgagaatctataaatgattttatagcatgttgcagtattgtgtttgatgtaataaactactgcatatttacaaaaaaaaatataatcttaaattttgtttttatttaattaattttcacaagtttttctatcgtagcagtcataataaggaaagatactcccaagacaaaacagtgtctgaagtcattattttaaccctgagcctttctttctcataatatcttcaaaagctatagatgtggtgaagtttacctcgctcacactgataagtccatgtcttgtaccatatcatcataatcttgagggacctctgcgtgatggaaacgccctgtgcaagtggagtgatgcatctgtgtaatgtgactctgttgaagtgctatagccttgtggcttctactccagtctcttcggctccaaaggtataacggtggcggcatattgttccactgctctatcgtttgatcatttacatctatcgatccaggcaagtagaacgactacagagcaaaaaaacaaaggaatgtgattgaaatgtattggttatactaaacgagagtttgattcattagtgaacgtacttaccatgccagaaagtaatctcgtgtcttcccaaatcaagtcatactcagctatctcgtcgaccctgtgattgtagaggaaaacaaaggttatgaaaagtttgtaactgacactctatatttgctatttacctttttgtttcacttggtacgatgaggattagaatcttgggtctaaactcgagggccttcctgatgaaaatgttagcaagactggatttgtaaccgaaaggcgggtttaatcccattatctgtttttactcacgaccaagtaatatctcagttagtgaattcaaaaagtgtatttcacctttaggatgttggttgcgttttttaccagtcgagagccatcgggtaactcttgtttcttcacactcaaccaatctctcttctcaaagttgaagttatactgccatggaaacatagtgtttcagaaacatcttcaaacacaacaataaaagagtagtg

SEQ ID NO: 36 - DNA, 1524 bp, Thlaspi arvense
atgagctccacggagacatatgagcctctattgagacggctccactcagattctcagttaaccgtaggttcttcaccggagatagaggagtttctcggccgtcgtagatccacggtgacgccacggtggtggctaaggctggccgtatgggaatcaaagcttctttggacgctctctggagcctccatagtggtctctgtgctgaattacatgctcagcttcgtcaccgttatgttcatcggccatcttggctctcttcagctcgccggcgcatccatcgccaccgtcggtatccaaggcctcgcttacggtatcatgttgggaatggcgagcgcggtccagacagtgtgtggtcaagcgtacggcgcgaggcagtactcatcaatgggaataatttgccaacgagccatggtcttgcacctcgcagctgcggtcctcctcacgttcctctactggtactcgggtccgatcctaaaggcgatgggccaatccgcagccatcgcacgcgagggtcaggtctttgcacgtgggattattccgcagatttatgcttttgccctcgcttgccctatgcagaggttcctccaggctcaaaaaattgtaaaccctttggcttacatgtcactaggagttttcgtgctacacacgctactaacctggctggtaaccaacgtcctgcatttcggcttgctcggtgcagctctggtgctgagtttttcgtggtggcttctcgcggctgtgaatggtctgtatatcgtgatgagcccgagttgcaaggaaacttggaccgggttctcagctagggctttaagagggatttggccttacttcaagctcacgatagcttcagcagtcatgctatgtttggagatatggtacgtccaagggctagtgattatttccggtttactcaccaatcccacaattgccctagacgcaatttcgatttgcatgtattactggaattgggatatgcagttcatgcttggtctaagtgcggcaatcactgtccgagtgagcaacgagctaggagcgggaaacccacgagtggctaagttatcagtggtagtggttaacatcacgacggttgtcatcagcttattcctctgtgtcgttgtgctcgtgttccgcattggccttagtaaagccttcaccagcgacgcagaggttatagctgcagtctctgatctctttcccctgctcgccgtttccattttcttaaacggaatccaaccaattctctctggtgttgccattggaagtgggtggcaagcagtggtggcttatgtgaatcttgttacttactatgtcattggtcttcctattggctgtgttcttggcttcaaaaccagtcttggagttgcggggatctggtgggggatgattgcaggagttatacttcaaaccctaactttgattgttcttacactcagaactaactggaattccgaggtggagaatgcagctcataggttaaaagcttcagcaaatgagagtcaagaaatggctaccgaaggaatctaa

SEQ ID NO: 37 - protein, 507 aa, Thlaspi arvense
MSSTETYEPLLRRLHSDSQLTVGSSPEIEEFLGRRRSTVTPRWWLRLAVWESKLLWTLSGASIVVSVLNYMLSFVTVMFIGHLGSLQLAGASIATVGIQGLAYGIMLGMASAVQTVCGQAYGARQYSSMGIICQRAMVLHLAAAVLLTFLYWYSGPILKAMGQSAAIAREGQVFARGIIPQIYAFALACPMQRFLQAQKIVNPLAYMSLGVFVLHTLLTWLVTNVLHFGLLGAALVLSFSWWLLAAVNGLYIVMSPSCKETWTGFSARALRGIWPYFKLTIASAVMLCLEIWYVQGLVIISGLLTNPTIALDAISICMYYWNWDMQFMLGLSAAITVRVSNELGAGNPRVAKLSVVVVNITTVVISLFLCVVVLVFRIGLSKAFTSDAEVIAAVSDLFPLLAVSIFLNGIQPILSGVAIGSGWQAVVAYVNLVTYYVIGLPIGCVLGFKTSLGVAGIWWGMIAGVILQTLTLIVLTLRTNWNSEVENAAHRLKASANESQEMATEGI

SEQ ID NO: 38 - DNA, 4858 bp, Thlaspi arvense
accgtttctttttgttgcgtgtcgagaataatagtcatctatgtgttttatatatagagagtcatagactatagaaaaaatgttataagaggacaaaatttcaataaattgaattagtttaaatttgatcaacaatttttttatcatcttatttaattcttagatgattatagtaaacaactaagatatcccagtatcaatatattcatgcataaatagaatgaaattgtattgggggggggggggaatatacattatttaattatatagattgtcatcaagtaattaaataaaataccaaaatgacattaaccataacaaagtgaatatgctgctgcatatttgtaagaaatcaaaagaaactttgcagcatataattactcgatgactaatacaagtatattgtgttgaaatttgatgtagtgtggaatagttaagattatttagaaaataaaaccacttttaataattacctgaaaatgagtaataatcttctaatttggtggggccatccgacctaatagacaactcattgatttcatcttacgtcagggacagttcataaaatgcaaataattgtctttttttttggtaatgattgtctttaatctttattttgtagattaacagattatattattcctttttctttcttactgttcttcagattatttggatggtttcagttgggcctcaggagcagaccggtaaatgggttggaggactattggtgggccacatttctgaaaagcatttcttcctctcaaaagctcattattatgagtatctttttatacggtagaaaggagtacataagtggtaacataaaatatattctgccaaaaaagttagttgattcttcttaatcactactccttttcttgataattatctacgtgggaaacactatttgtcctccccccatttaatttggttgaaagtcttgagactagaggttggctcaatccaaaatcgttgacgaacgttaggtatcgttatcaactacaactctttttttcactgaggtaccgttatatttatatacctacctagttttactcttgtgcacaaggatatttcggttcggtttgatatctttctcgatcttgaagaaatattaccaatttggagcttatacattcctcggtctggtatcattcaacaaagtttttggtttggtttgtttaacaaataatatgaatgtgtgtttagtcgtcccttaggtatttctcaatctctttcttttaagcttcactttcttaataagccattaagtaacgtaactagagaatggttgttacactatacactaacaaaaatcagaccaaacagtcatgaaagatcttaaccatcaattccgtttcggtcaacgactcgaaccctcagcataaccaaaacaaacagtcgtaatataaacacgcccggtctataactataacaaaataacggcaaaagaaagaaaatacgagaaaaagaagaagacgaacaaacaaacggaccatgagctccacggagacatatgagcctctattgagacggctccactcagattctcagttaaccgtaggttcttcaccggagatagaggagtttctcggccgtcgtagatccacggtgacgccacggtggtggctaaggctggccgtatgggaatcaaagcttctttggacgctctctggagcctccatagtggtctctgtgctgaattacatgctcagcttcgtcaccgttatgttcatcggccatcttggctctcttcagctcgccggcgcatccatcgccaccgtcggtatccaaggcctcgcttacggtatcatggtatgtgctttagagagtaaacgacgttgacgtcgttcgatgttatagcttcacattcatttgcttatcattttgtaatatagtaaatccgggttttgaattaggtttctcaatattttgaccattttatgaataccagcaaccataataaaaatacaaactgtcggatcagttttgttctccatttgagatccgattttggtctttcagatgcaaaccatattaggatacagttcggttttcatgtcggctattttggtccggtttatcatttttgatcaatcttagccttaggcatctcccaactgtttttatgtatcaaatgtactagttgggaatggcgagcgcggtccagacagtgtgtggtcaagcgtacggcgcgaggcagtactcatcaatgggaataatttgccaacgagccatggtcttgcacctcgcagctgcggtcctcctcacgttcctctactggtactcgggtccgatcctaaaggcgatgggccaatccgcagccatcgcacgcgagggtcaggtctttgcacgtgggattattccgcagatttatgcttttgccctcgcttgccctatgcagaggttcctccaggctcaaaaaattgtaaaccctttggcttacatgtcactaggagttttcgtgctacacacgctactaacctggctggtaaccaacgtcctgcatttcggcttgctcggtgcagctctggtgctgagtttttcgtggtggcttctcgcggctgtgaatggtctgtatatcgtgatgagcccgagttgcaaggaaacttggaccgggttctcagctagggctttaagagggatttggccttacttcaagctcacgatagcttcagcagtcatgctatggtaaatgtctttaatctaaacacaaatctgtatgatttgaccggttaaaatttatggtttgaagaaagctgatatataccaatttaaaatgaaatatctgcagtttggagatatggtacgtccaagggctagtgattatttccggtttactcaccaatcccacaattgccctagacgcaatttcgatttggtactcctttcacccgagatttatcatatgccgacgaacctcaacggttacgtcttaacccggttaagtgattttgcagcatgtattactggaattgggatatgcagttcatgcttggtctaagtgcggcaatcacgtaacaaaacaaaattaaaaatggcatgtagtttttaatttaaatgatccatttgcaaaaaccgtgccgtttttgtgtgttttgtgttagtgtccgagtgagcaacgagctaggagcgggaaacccacgagtggctaagttatcagtggtagtggttaacatcacgacggttgtcatcagcttattcctctgtgtcgttgtgctcgtgttccgcattggccttagtaaagccttcaccagcgacgcagaggttatagctgcagtctctgatctctttcccctgctcgccgtttccattttcttaaacggaatccaaccaattctctctggtaaaaacacacacaagaaaaagaggctcttttgtgaattttggtttgttgattgatctttgctctatggattcaaaggtgttgccattggaagtgggtggcaagcagtggtggcttatgtgaatcttgttacttactatgtcattggtcttcctattggctgtgttcttggcttcaaaaccagtcttggagttgcggtataatctcttttactctttctttgtgtttatatgtattgtatgcatcataagagatgggaggtatttcattacaggggatctggtgggggatgattgcaggagttatacttcaaaccctaactttgattgttcttacactcagaactaactggaattccgaggtaaaacaatcaccaaatctctctttttttctctaaatactccaaagtccttacctttactctgcatctcttacaggtggagaatgcagctcataggttaaaagcttcagcaaatgagagtcaagaaatggctaccgaaggaatctaacagcaactctgttcttttctcctctcttttgttggcaagagatatgaaataaataccttctgtttattaggattcagtaacatatttcatttcgttaaactacagacaaaaaataatggacaaactacttaatcctcttctgcaaaatctttcttctgcctttagatgattacaaaaatcaaaactttctcgttgttttcataaccccacaagtttttccgtctgtgagctaacataagccaaagacttttcttgtgttttatcatacaacacagtttctcttgcatcatcatcaccatctccttcatagtcctcctcatcctcatcctcatcctcatcatcactactcacatcgacatcatcatcatcatcatcatcatcatcagatctgtagactccagcaatgatggttgtagtctcatctctgagaccagtaagttctttagcttcctctagctcatcttgagttgaagccaatgacaaaagcacattcttcgctttctgatcaggtggtaccccacaactctccatctccttgtaccaactaagagcgctcccgaaatccttgcacctcccagacgcatccatgatagtcgttatgatggtttgattcgctttgatgccacttaacctcattttctcatatacctccataattttatcaagatcgtttgctttcgcatagccttttatcattgtcccataggtgactatattcggctcaaaaccatctacctttatcctcttgaagaatttctcagcaccctccatgtccgaagcattcacatacgctgataacatagttgtgtaagaccagagatccgggaaaaatctgcaaagggaattatgttttgttaccaatctaaaacagagaagcaacacagttcacatgatagaattattctttacctgtcacgtcgcatgctttgaaaaacggtctttgcttgatccaccattccagaaatagcgaatgcatcaagcaaaatgttataagctttat

SEQ ID NO: 39 - DNA, 2214 bp, Thlaspi arvense
atgcttccattaatggcgataccacttgcgacttgcaggagcatcaactggtcagccacggaaaggattcctgtttcgcttctgttccggagtattcttctccaagacgacgaagtttgtagcgctgtgccactataccggatcctcgatcagaatgacgggcaacttggtcctataagtatggccgaggaatcagacaaaccattgctggatcctgatactctcaacagagaaggaattgacttgggtctgttgccattggaggaggtttttgaatacctaagaacatctccacgggggcttttatctggagatgctgaagaaagattgacgatatttggtcctaacagccttgaagagaaacgggagaacaagtttctgaagttcctaggttttatgtggaatcctttgtcatgggttatggaagctgcagcattgatggccatcgccctagcagatagtgaagtagagactatcagtcttttgctataccatttctgctcagtgctgaccggagaatcgctacctgtgaccaagaagaagggtgagcaagtcttctctggctctacttgtaagcaaggtgagatagaagctgttgtgatagccaccggttcgagcactttctttggtaaaacagcatctttggtggacagcacagatgcaactggacattttcagcaggttctaagcttgtgccagcagaaaaatgagattgcgcaaagagtttatgccatcataaatagatttgcagaaaaaggtttgaggtctcttgctgttgcttatcaggaaattccagagagaagcagcaacagtcctggaggaccatggttgttctgtggtctgttgccactgtttgatcctccaaggcatgacagtgctgaaaccatactgagagctcttaaccttggagtttgtgttaagatgatcaccggtgatcagttggcgattgcaaaggagacaggaaggcgacttgggatgggaaccaatatgtatccttcttcctctttgttaggccacaacaacgatgatcacgaagccattccattggatgagcttattgaaatggcagatggatttgctggagtgttccctgaacacaagtatgagattgtaaagatattacaagaaaagaagcatgtggttggaatgaccggagatggtgtgaatgatgctcctgctctgaaaaaggctgacattggaatagctgtcgctgatgcaacagatgccgcaagaagttctgctgacattgtactaactgagcctggcttaagtgtaattatcagtgctgtcttgaccagcagagccattttccagcgtatgaagaactatacagtatatgcagtctcgatcaccatacgaatagtgctcggttttacacttttagcgttgatatgggaatacgactttccacctttcatggttttgataatcgcaatactcaatgacgggaccatcatgactatctctaaagatcgagtaaggccatctcctacacccgagagttggaagctcaaccagatatttgcgactggaattgtcattggaacataccttgcattggtcactgtcctattctactggatcattgtctctaccaccttcttcgagaaacacttccatgtaaaatcaatcggcaacaacagtgaacaagtctcatccgctctgtatctccaagtaagcatcatcagtcaagcactcatatttgtaacacgtagtcgaagctggtcttttcttgaacgtcccgggactctcctgattttcgccttccttgttgcccaacttgccgctacattgattgctgtctatgccaacatcagctttgctaacatcaccggcattggatggggatgggcaggtgttatatggttatacagtttgattttttacatacctcttgatattataaagttcttcttccactacgcattgagtggagatgcttggaaccttgtatttgaccgtaagacagcatttactaataagaaagattatagaaaagatgacggagcgtccaatgtaaccatctctcagagaagtcactctgcagaagaactcagtggaagtcgttctcgcgcatcttggatcgctgagcagaccagaaggcgtgcagaaaccgccaggctcttggagggacactcggtgtcaaggcatttggaatcagtaatgaagctcaaacaaattgaccccaagatgattcgtgcagacactgtctaa

SEQ ID NO: 40 - protein, 737 aa, Thlaspi arvense
MLPLMAIPLATCRSINWSATERIPVSLLFRSILLQDDEVCSAVPLYRILDQNDGQLGPISMAEESDKPLLDPDTLNREGIDLGLLPLEEVFEYLRTSPRGLLSGDAEERLTIFGPNSLEEKRENKFLKFLGFMWNPLSWVMEAAALMAIALADSEVETISLLLYHFCSVLTGESLPVTKKKGEQVFSGSTCKQGEIEAVVIATGSSTFFGKTASLVDSTDATGHFQQVLSLCQQKNEIAQRVYAIINRFAEKGLRSLAVAYQEIPERSSNSPGGPWLFCGLLPLFDPPRHDSAETILRALNLGVCVKMITGDQLAIAKETGRRLGMGTNMYPSSSLLGHNNDDHEAIPLDELIEMADGFAGVFPEHKYEIVKILQEKKHVVGMTGDGVNDAPALKKADIGIAVADATDAARSSADIVLTEPGLSVIISAVLTSRAIFQRMKNYTVYAVSITIRIVLGFTLLALIWEYDFPPFMVLIIAILNDGTIMTISKDRVRPSPTPESWKLNQIFATGIVIGTYLALVTVLFYWIIVSTTFFEKHFHVKSIGNNSEQVSSALYLQVSIISQALIFVTRSRSWSFLERPGTLLIFAFLVAQLAATLIAVYANISFANITGIGWGWAGVIWLYSLIFYIPLDIIKFFFHYALSGDAWNLVFDRKTAFTNKKDYRKDDGASNVTISQRSHSAEELSGSRSRASWIAEQTRRRAETARLLEGHSVSRHLESVMKLKQIDPKMIRADTV

SEQ ID NO: 41 - DNA, 5382 bp, Thlaspi arvense
atgcttccattaatggcgataccacttgcgacttgcaggagcatcaactggtcagccacggaaaggtggtttcaattttcattcgtggaccctttttaaggattcctgtttcgcttctgttccggagtattcttctccaagacgacgaagtttgtagcgctgtgccactataccggatcctcgatcagaatgacgggcaacttggtcgtaacatagtggtttaagttcgtgtgtagctcgtactatgttttgatggtttgctattaccttagaattttaaataattatcttatgtacatcgacgaagttacggtttttgctattgttcactagttccaaggtgtggatcgaatctaggaatgtgggctttgaagtggtacttgtaccgtggattttgaagctataagtatggccgaggaatcagacaaaccattgctggatcctgatactctcaacagagaaggaattgacttggtaaatgatgtgtggttcctttacttttattaaaattcttggattctttagtggcaaaaatggttttgacgcttgagctggacagggtctgttgccattggaggaggtttttgaatacctaagaacatctccacgggggcttttatctggagatgctgaagaaagattgacgatatttggtcctaacagccttgaagagaaacgggtaataaaaagcttatcgtcaaagtttttccatagtgttcctgcctaagacaggagagaagcttactagttctgagatcttattcattatgaacactcttcatttctttttcacatattatccttaggccacacactgatttttctgccaagttgtggttctttacattagctcttgtataatatgttagtgttgtcctaatgacactgaaaacgaaacgatacaggagaacaagtttctgaagttcctaggttttatgtggaatcctttgtcatgggttatggaagctgcagcattgatggccatcgccctagcagatagtgaagtagagactatcagtcttttgctataccatttctgcgtacatgagagtttatgaaatcgtttctgctcttgaaactcatggtgaaaaatgtttattacagagcttaggtcctgactgggaagactttgttggaatcgtttgccttttactgatcaacgcaacaatcagcttctttgaagaaaacaatgctgggaatgctgctggagctcttatggctcgcctggctccaaaaacaagagtctgcttcttcaccttatgcattttcactcttattaccttaaatctgatcaagatccactcttgataggttcttagagatggacagtggcaagagcaagacgcgtctatcttggtacctggtgatattattagcataaagcttggggatatcattcctgcagatgctcgccttcttgaaggagaccccttgaaaattgatcaggcacgcacagattatatttagcgctaagtcacatttcttctctcttagtacattatgtaaagactgtatctgacagaatattcctgcagtcagtgctgaccggagaatcgctacctgtgaccaagaagaagggtgagcaagtcttctctggctctacttgtaagcaaggtgagatagaagctgttgtgatagccaccggttcgagcactttctttggtaaaacagcatctttggtggacagcacagatgcaactggacattttcagcaggttctttattgttccttaactcccttttctggttgaaacagtctgactggtaaaagaccaaaccttgtaaagctgtgaatacctttgcaagaacatgacatgtttctgtgacatgttttccttataggttcttacgtcaattgggaacttctgcatttgctcaattgctgttggaatggttcttgaaatcattgtcatgttccctatacaacatcgctcatacagaattgggatcaataaccttcttgtactactgattggagggatacccattgccatgcccactgtactatctgtcacgcttgccattggatctcatcgactctcacaacaggtgtcgtttctcttgactgattaactgtaacagagtgaaccaagaagaatccaacttttaagcttctgtagaactttttgttagcaatataatatgtgtttcttgttgttttaaaagggtgccatcacgaaaaggatgacggcgatagaggaaatggctgggatggatgtcctctgctgtgataaaactggaacccttaccttgaacagtctcaccgttgatagaaatcttattgaggtaccaaccaatacttcccatgtgacttgcatttcaaagtccaaagagtacagttaacaacagttgcctccatctttacaggttttcgatgactacatggacaaggacacaattttgctgcttgcaggcagagcttcacggttagaaaaccaggatgccatagatgcagcaattgttagcatgcttgctgatccgaaagaggtggagatgtttcttttacataaactctgttttatgaaaatattgtcatcttctttagaagttttacttattagaaaaggttgtttatctttaggcacgtgcaaacattaaagaaattcatttcttgccattcaatcctgtggacaaacgtacagcaataacatatattgactccgatggaaaatggtatcgcgctagcaaaggagctcccgaacaggtaacaaagaatcaccctatactacttggcactttcaaaactgactctagatgtaaaaaaatgaaagttcttttatatataggtccataaaagatatatcatcactgattcaattccaactgtactgtatacataggttctaagcttgtgccagcagaaaaatgagattgcgcaaagagtttatgccatcataaatagatttgcagaaaaaggtttgaggtctcttgctgttgcttatcaggtaaaatatttctgttatcccttttctctcttgatatggtttttattgtaagtgtactatttggggaagaagcttataatgacattagttatactcattcaatcattttaatcattgtttctaggaaattccagagagaagcagcaacagtcctggaggaccatggttgttctgtggtctgttgccactgtttgatcctccaaggcatgacagtgctgaaaccatactgagagctcttaaccttggagtttgtgttaagatgatcaccggtaattctgaaccctagagcaggcttgcttgggaccacagaggaacagacacgctctcatggtgaaaatctgataagtttggataaaaaaaatgtaggtgatcagttggcgattgcaaaggagacaggaaggcgacttgggatgggaaccaatatgtatccttcttcctctttgttaggccacaacaacgatgatcacgaagccattccattggatgagcttattgaaatggcagatggatttgctggagtgttccctggtcatactcacaacacagcgcttatatcttaccgagtttcagattttctctcttttactgatcccagtttcttttgatggctctcatgtttcagaacacaagtatgagattgtaaagatattacaagaaaagaagcatgtggttggaatgaccggagatggtgtgaatgatgctcctgctctgaaaaaggctgacattggaatagctgtcgctgatgcaacagatgccgcaagaagttctgctgacattgtactaactgagcctggcttaagtgtaattatcagtgctgtcttgaccagcagagccattttccagcgtatgaagaactatacagtaagtactaaagacaactatcatctgattccacattgctaaagataagcaaatccatgtaatataggatatgaatttcaagtagtttaatgaaattctgaagtttcttttggtttcctctgcaggtatatgcagtctcgatcaccatacgaatagtggtaaggagcttcaagatacacgatctaacttgctaagttacatctacttgagccttctcttcttatcattgtttcatgcagctcggttttacacttttagcgttgatatgggaatacgactttccacctttcatggttttgataatcgcaatactcaatgacggtaatcttttaatcctctcaatagcttcatgtttgaattgttgatgttaaaaactctaaattcttaacactttcaagtgctcttgtttatctcctacgcaacagggaccatcatgactatctctaaagatcgagtaaggccatctcctacacccgagagttggaagctcaaccagatatttgcgactggaattgtcattggaacataccttgcattggtcactgtcctattctactggatcattgtctctaccaccttcttcgaggtatcttcccgtcgctcgaaagtaatcaaattcgatttgcttaccgagaaaaacgcataaccatgaccatccctgaatcttaaatggctgcagaaacacttccatgtaaaatcaatcggcaacaacagtgaacaagtctcatccgctctgtatctccaagtaagcatcatcagtcaagcactcatatttgtaacacgtagtcgaagctggtcttttcttgaacgtcccgggactctcctgattttcgccttccttgttgcccaacttgtaagaactcttcatgtttaacctttttccatcacagaatactacatacagcatacataggtcttggttttgatttgtccgttttcatgtacacaggccgctacattgattgctgtctatgccaacatcagctttgctaacatcaccggcattggatggggatgggcaggtgttatatggttatacagtttgattttttacatacctcttgatattataaagttcttcttccactacgcattgagtggagatgcttggaaccttgtatttgaccgtaaggttagtgcatgtcttgtcctctgtctcagactttaactctgtttttttcttaaaagacaaagagtgttggttttgtcttgcagacagcatttactaataagaaagattatagaaaagatgacggagcgtccaatgtaaccatctctcagagaagtcactctgcagaagaactcagtggaagtcgttctcgcgcatcttggatcgctgagcagaccagaaggcgtgcagaaaccgccaggttctcttttgtctatacgactttttttgggtttctctttcatttcacatactaccagaaccatctctggtccacagaaaatagaaacttagtttttttgttcatttgataggctcttggagggacactcggtgtcaaggcatttggaatcagtaatgaagctcaaacaaattgaccccaagatgattcgtgcagacactgtctaa

SEQ ID NO: 42 - DNA, 1857 bp, Thlaspi arvense
atggagagtagtgtagttaatcatccattgcaagaagatgagaagggtttttctgatgaagataatgctgtaaataatgagaaagagagtttattgcaaacatctggctctgtagagaatgctcctgaaggttctggtcgttcttcggattggcgtaggggactagaccactgcataactgcacctgttggtctctatggagatatggtaatcgatgacaatgaggttaagtactctcggtccataacagagagattgtcccctgcgagtcataattcaaaattagatcgattatcggagcgggaaaagcaaaaactcattgttgagctagtcagaatacaaaatgacgggaccgtggaagttgatatagataacggtacaccggtatcggagttattggagtttcagccaaccaaagggcagccaacaatcacatatgaaaagtcatttgctgattcctttagatcaattccaagattaaaaattgtgatacttgtggttggaactcgcggtgatgtgcagcctttcttggccatggcaaagcgcctccaggagtttggtcatcgtgttaggttggcaactcatgcaaatttctgctcttttgtacgatctgctggagtagagttctatcccttgggtggtgatcctcgagaactagctggatatatggctagaaataaaggtctgattccttctgggcctggagaaatagcaaaacagagaaaacagttgagggcaattatagagtctcttcttccggcttgcacagagcctgatatgcaaactgctgcctctttcagagctcaagcaataattgcaaaccctcctgcgtatggacatgtgcatgttgctgaagctctaggagtaccaattcacatttttttcacaatgccttggacgccaactcatgaatttccccaccctttggcccgagttcctcaaagtcctgcgtattggctatcatatatagttgttgatctgatggtatggtggagcataaggacatacataaatgattttaggaagaggaagctaaaccttgcacctttcgcatatttcagcacataccatggctcaatttctcacttgcctactgcttacatgtggagtccccatgttgtgccaaaaccaagtgattggggtcctttagttgatgttgttgggtattgtttcttgagccttggatcgaagtaccaacctcgtgaagattttatccactggatagaaagaggatcaccgcccgtatatattggtttcggaagcatgcctcttgacaatccgaaaaaaacaatggatattatactggaaacactgagagatacagaacacagagggatagttgatcgaggttggggtggccttggaaaccttgctgaagttcctgaaaatgtattcctcttggaggactgtcctcatgattggttgtttcctcaatgttcagctgtgattcatcatggaggtgctggaaccacagcgactggactaaaagctgggtgtccaacaacaatcgtgccgttctttggggatcagttcttctggggtgacaggatctatgagaaaggacttgggcctgcgccaataccaatagctcagctcaatgttgagaacctctgcaattccataagattcatgcttcaaccagaggtgaaatcacgagtgatggaactagcgaaagtactggagaacgaggacggtgtagctgcagctgttgatgcattccacaggcatttgccactggctctgccactcccggagtcctcgccggagaaaagacacgaagatgatcgaccagacctgttacagtggttcttcatccagattggtaaaaagtgttgccttccatgtggtggtgtgtga

SEQ ID NO: 43 - protein, 618 aa, Thlaspi arvense
MESSVVNHPLQEDEKGFSDEDNAVNNEKESLLQTSGSVENAPEGSGRSSDWRRGLDHCITAPVGLYGDMVIDDNEVKYSRSITERLSPASHNSKLDRLSEREKQKLIVELVRIQNDGTVEVDIDNGTPVSELLEFQPTKGQPTITYEKSFADSFRSIPRLKIVILVVGTRGDVQPFLAMAKRLQEFGHRVRLATHANFCSFVRSAGVEFYPLGGDPRELAGYMARNKGLIPSGPGEIAKQRKQLRAIIESLLPACTEPDMQTAASFRAQAIIANPPAYGHVHVAEALGVPIHIFFTMPWTPTHEFPHPLARVPQSPAYWLSYIVVDLMVWWSIRTYINDFRKRKLNLAPFAYFSTYHGSISHLPTAYMWSPHVVPKPSDWGPLVDVVGYCFLSLGSKYQPREDFIHWIERGSPPVYIGFGSMPLDNPKKTMDIILETLRDTEHRGIVDRGWGGLGNLAEVPENVFLLEDCPHDWLFPQCSAVIHHGGAGTTATGLKAGCPTTIVPFFGDQFFWGDRIYEKGLGPAPIPIAQLNVENLCNSIRFMLQPEVKSRVMELAKVLENEDGVAAAVDAFHRHLPLALPLPESSPEKRHEDDRPDLLQWFFIQIGKKCCLPCGGV

SEQ ID NO: 44 - DNA, 7708 bp, Thlaspi arvense
ctaaaagagcatgagcagcaccgcgatcatcatcggaatagtccgccaccaacgcaattgaactaagaaaggctacaaaactgctttaaatccatcctgctgcttattccttttgcgtgtggccgccagaagaagatgagaaaacttactttcaccattagaaattagaataaagagtcaccgaaagtgaaagtgaataggatattcaccagaccgcctttgagaagcgccagttctgcagatcctgcatctcaatcactcaagataactcccaaatctcaaatcaactccgctaaagaaacttcctcttcgcaatcacgacgatttattaacagaaaagagaaggaattgctctttcgggagaagatccagcataactaacggaaagagtttcatcaaattcgtctggaataaagatgaaaacaagcaaaaggaaaaccgaacgttgtcggagaacttagaatcctataaacggaaaataaaatccgatcaacggaaaagaagatccgattgacggaactataagacagccaaaaagccgatcaaatcggatcaaagaaagaactctctcgctctgaaagattttaaagagagaagagagagagagcccttcaccttgtgccacccgtacttttaagagcatctccaaccatattctattttcaactccaaatgctattttgaagtaaaatcctctccaaccctagtctattttcaactttaaaatagagtaaacctaaattttactctatatttggagtaaatctaaactttactccatcttggaattagacttttttatttgcaaattaatccttgagatttattataattatattttatactatttaatatttataacaaatattataaaactgataattatgaatatttaaatactgcaattattcctacaaaattaaaaaatataataaactttaaaatacaaaataagggctaaaattaagataaacaacataaataaatttaagacaacaaatactaaaaatattaatgataatttttttttattatagtaatgtttaaataaaaattgcatatgcttttttgtgatgttatgtaatttttattatttgataaatatttaagttatagtttttcaaagaaattgtaaataataaaataagtgggatttatttataaattttaaaactaaaaaatatttataataaaatcaaataagattctatttagaatatttctttttagagtaaaaaataaagaaatacattagagtaaaacacaactctattttagagttactctatttttctattttggagtagaaaatgaagaaataattgaagatggtataacaaacgaaaagtcgcattatcttactgttaaattactataattcataatcaattggttttgtttcggtggcatccggcatcccctaatatgattgatttttatcgctgcatttattaaaatatatatatcttcatcctcgatcaccacaattcattgattcaaaagtctccaaaccccttggaagctcaacattacaatctcgccaaattcctcaaaaccagaattttccacagacccagaaacatttctcatcaaagttctctcctttcctgtctcttgaactttctctcctactcactcagttcaagaacaatctttcgatcattgatcagtgatggtagattcaattgttgggtttcatttacttgggcaatggcttttcttttcttttctcttctcttttcgattgattgattggttaattctgtgtctctgtacagtttcgaattgtgtctttcaagttaaagctggatcatttttctagttgatctcatcctcgcgcttaacgtgagagactctctgctctgtaatctttccctgcgttttcttgttttatctgaaacggttaatatagagataaaaaaacccaatttctctgacttttttttctttctttaatatatcatttcttctcccttttgctttttgtataaagtgcagctaactttccttaaggattcactggttggttcaagcactgattcgccgcgtacagcttttggcaggagccatttgcatctctgatcgacatggattagaatagtgtgcagttgtgttgtgtacaactcgctgcatagatgttactttgtggagttcaattcatatgtagtatgtttgttgtttaagaagctgatctttgtgggggcattgggtagtgagatctgttaaattgaagtcggtgatggagagtagtgtagttaatcatccattgcaagaagatgagaagggtttttctgatgaagataatgctgtaaataatgagaaagagagtttattgcaaacatctggctctgtagagaatgctcctgaaggttctggtcgttcttcggattggcgtaggggttagtcctctattggaacacgtgtatttatcttattccaagctttgccatcaaaaccataacttagagcataacaacttatcaagattgtatgttcttgaaggactagaccactgcataactgcacctgttggtctctatggagatatggtaatcgatgacaatgaggttaagtactctcggtccataacagagagattgtcccctgcgagtcataattcaaaattagatcgattatcggagcgggaaaaggtaggaatctgaaccttcattgcaatggatatgttcttcatttgattacaaatttttttggtaacttgaaaacttcttgttattccagcaaaaactcattgttgagctagtcagaatacaaaatgacgggaccgtggaagttgatatagataacggtacaccggtatcggagttattggagtttcagccaaccaaagggcagccaacaatcacatatgaaaagtcatttgctgattcctttagatcaattccaagattaaaaattgtgatacttgtggttggaactcgcggtgatgtgcagcctttcttggccatggcaaagcgcctccaggtagtttcgaaattgctttctcattctttgtatccttttgcgaaattaagattcacagagggaatcattgtgactttacatatgtatattttgtggatgcatgcatatagtacactgcaattgaacaggctcgtatcaaagtgttggcatgtgcctatatcatgtgttctcgtcattttaaatttgtttcatttcttcatcctatcgtcatatgtgttcttgacgcttttcttagcatttggtgagagatttggaactgattggcattgagagaggttaaagttagatattgtttttctctgttgcaggagtttggtcatcgtgttaggttggcaactcatgcaaatttctgctcttttgtacgatctgctggagtagagttctatcccttgggtggtgatcctcgagaactagctggatgtaagaagtcctccttgaaaagattcgtttatattttagtttctcgagttttttttgtttgatgatgaaagctgtcataaattctctctttagcttcatgtgggtatttttgaatgtagatatggctagaaataaaggtctgattccttctgggcctggagaaatagcaaaacagagaaaacagttgagggcaattatagagtctcttcttccggcttgcacagagcctgatatgcaaactgctgcctctttcagagctcaagcaataattgcaaaccctcctgcgtatggtatatccttcgttaactttaaaactctttgatccatcagaacctcattgtttgtaaacctttcttaagcactttttctatgaaactgatggtatggtttttggttctaattataggacatgtgcatgttgctgaagctctaggagtaccaattcacatttttttcacaatgccttggacgtgagttgacttctctgcttttaaacttgccttaacgtgttatttggtttcctgttctcttacatcatcttcatgtaggcaggccaactcatgaatttccccaccctttggcccgagttcctcaaagtcctgcgtattgggtaatgttattctttcttatgaccatatactctctcgaagataatgaggcttattgtttcacaacatttttttgtctcagctatcatatatagttgttgatctgatggtatggtggagcataaggacatacataaatgattttaggaagaggaagctaaaccttgcacctttcgcatatttcagcacataccatggctcaatttctcacttgcctactgcttacatgtggagtccccatgttgtgccaaaaccaagtggtgagattcccgctgcatccccagtacatatattccgctgaggtttatcatatgtattgtagcttcattctggcttctagattaatgttgttcttctggctttgtcaattggcaagaccataatgggttgtcaattttaggctgagctctttatctttccttcggtagatatctgaaagattttgctttttgtttgactaatttgcagattggggtcctttagttgatgttgttgggtattgtttcttgagccttggatcgaagtaccaacctcgtgaagattttatccactggatagaaagaggatcaccgcccgtatatattggtttcggaagcatggtaaactgatgatccttagaaaatatgctcttccttgctttggtgatattcagttataatgcatagtactgatattgttgtttcttctcttttacacaaccaagcctcttgacaatccgaaaaaaacaatggatattatactggaaacactgagagatacagaacacagagggatagttgatcgaggttggggtggccttggaaaccgtaagcagcttctgtaccttctcttttgatgctctgtgtcctgattcctgaactacttttcttctttgcttatacataattttttttatcttcaaacatcttgcagttgctgaagttcctgaaaatgtattcctcttggaggactgtcctcatgattggttgtttcctcaatgttcagctgtggtaacccctttttagattaactacatcatgtctccaaagacattatcttctaatccaggctatttcttgtgttgtggatatgaagattcatcatggaggtgctggaaccacagcgactggactaaaagctggggtaaaacattttgctttcacagaaatgtcctgtagtgaaatcagttttcttgaccatatgaaacctaatggttcctatattcttttgaattctatgatatgtctccagtgtccaacaacaatcgtgccgttctttggggatcagttcttctggggtgacaggatctatgagaaaggacttgggcctgcgccaataccaatagctcagctcaatgttgagaacctctgcaattccataagattcatgcttcaaccagaggtaaacaaacttaaattttccttctttttttccatgtatctcatgcccatgtaggatgtttgagtaaagaaccacagtagaagttaaacacaaacactctttcttgcaaaattaaacaaactaaacaaaacccaaaacctaaagctgtccttttgagttcaaaaaagtagaaagatgtaatcttgtatatacacttaaatattgcttatacagttcatacaaatagaaaatgtcatctttatagttcatagaagtagaaagatgtaatctttatatatacacttagaaattgcttatatagttcatacaaatagaaaaatgtcatctttatagttcatacaaatagaaagatttaatctttatagttcatacaaatagaaagatgtaacttttatgtatatgcgtggatatcgctttatcagttttttaatatgtgaaggccctcgcacaaaaaaaaaaatattatgtgaaagaaagctcggtgcttaatatttgaactatgaagcaactttctatatatatacacaaaactgacattgctttatagttcatacaaaaaaaaagatgtaatcgttatagttagttcatacaaaagaaagatgtgatctttctattttcgttcagtgatgttatgtgaagaaaaattcggtgtttagatttgaactatgaagcatctttctatttatatacacaaaactgatattgttttatactcatacaaatagaaagatgtatgaactataaaaatagaaagcatcatacaaatacaaatagttcatacaaacatcacacacaatgcacactagctcaaagctttttcctctgtttaaaactcataaaacttccaaaggtctctctctagctttgttgtatctcacaaacggaactggaatcggtagaatatgtaaaaccaatcatggcctatccaggtgaaatcacgagtgatggaactagcgaaagtactggagaacgaggacggtgtagctgcagctgttgatgcattccacaggcatttgccactggctctgccactcccggagtcctcgccggagaaaagacacgaagatgatcgaccagacctgttacagtggttcttcatccagattggtaaaaagtgttgccttccatgtggtggtgtgtgataacaaactcccttagatattttgatcttgtctctgcaactcgtttcatttcattcagttgtcaagaatatgattagatttttaacacagctgcaaaagatgggtttggggcatctttataagtttgttgttcagtgagaataagatgatatttgtgtgagtttgtcttaagaacaaagtaccgatctcctttattgtatacttaaaacccattcgaaacagaatctcccacgtcaaactacatttctcagcttgtaggcattggatttcatcagctcctgagcatgtgccagatgacccttcatatgatctgttaagtttcagtggctcaaaacggcacctttaagagaagcttgaagtatcaaaacgtgagattaaaacggaagttgcagaaacttgcagaaagcagagtatgagagattgagagaagaagaagggagaagggaacacatacaaatatttaacgagttcacgcccataacacgctatatctcaccaagactaagctggaaatccactagatatcagagagaatacatatttagagacgaacaagtgaccgttttaatatctttcactagcacttaaaattcactatgttaaatcaattaaaaccagaaaaaaaacaatagctaaacttatgctaagatgtgtttttctctccactctcactagcgactacattgtgtctatctcgttctcttcctcatgtgtactacaatctctctcacgtcttcagcttcactttatagtgacaacaacattagacctaaagcaccttgccaaacgccaaaacagcttcctatagatgcgtttgcttttttatcatatcttagaggcaaatactccttagcttttaaattcacaacaagacaaaagcaagaggctctccttgtggtcccaaaagtaactcaatccaatatgaactcaccaaagtaatcatagttatgccttgagttacttgacttgaatttgcttgagcgacaagttctcgtcttcacaaatctccacctgagaacatgatgttcaagccaaacgacatacactcttgagaaagatatagaacgccttcttctagcttatggattctaatcttggtttctgagtatgattacccagtcttgatactaagcagatttaaataccataaaactgatagatccttgctggatttaa

SEQ ID NO: 45 - DNA, 732 bp, Thlaspi arvense
atgggaagagggaagatagagataaagaagatagagaatcagacagcgaggcaagtgaccttctgcaagaggagaactggtcttatcaagaagactaatgagctctctgttctctgcgatgctcacattggtctcatcgtcttctcctccaccggaaagctctcgcagtactgttccgaacccctcaggatgcctcagctcattgaccgatacttgaagaccagtggaatgcgacttcctgatcctaatgacggccgggaggaattgtaccaagagatggaagtactaaaaagagagacatgtaagcttgagcttcgtctgcgtccataccatggacatgacttaacctcccttcctccacacgagctcgatggtctcgagcaacagctcgaacattctgtccttaaagtccgcgagcgtaagaatgagttgatgcagcaacagttggagaatctaagcagaaagaggcggatgctagaagaagataacaacaatatgtaccgtttgcttcatgagcatcgtaacgcggttgaatttcagcaagctgggatagagacgaaaccaggggagtatcaacagtttctagagcagcttcagtactataatgatcatcagcaacaaccaaacagtgttcttcagcttgctacgcttccttctgagattgatcctaattaccatctccagcttgctcagcctaatcttcaaaacgatccaacggccaagattgattag

SEQ ID NO: 46 - protein, 243 aa, Thlaspi arvense
MGRGKIEIKKIENQTARQVTFCKRRTGLIKKTNELSVLCDAHIGLIVFSSTGKLSQYCSEPLRMPQLIDRYLKTSGMRLPDPNDGREELYQEMEVLKRETCKLELRLRPYHGHDLTSLPPHELDGLEQQLEHSVLKVRERKNELMQQQLENLSRKRRMLEEDNNNMYRLLHEHRNAVEFQQAGIETKPGEYQQFLEQLQYYNDHQQQPNSVLQLATLPSEIDPNYHLQLAQPNLQNDPTAKID

SEQ ID NO: 47 - DNA, 5332 bp, Thlaspi arvense
ttacatttcaaacagatttgacataacatgtaatattgcttaggacatttgtgttcatcacgtccgtctttcaatgaccaattaatgctgttttgtttgtttgttttaaccacgttttagcaaaagtacatttatacaggacttttttaatccgctcgttacttaatcgacaaatatataatgtccctcaatactatttggtatatattttttacaaaacatgccactgaaaatgattcagttgtatatgttcatatcatcacataattgtgttcaacctgatgtagcggctgattactctatgcacaatgttagaaaatctgaatattaactcgatgatctaaataccaatttcttttccagaattttaatacgttcgagtttcagcataaaagcttttactcacaccacttgtttccccttgcgttgtgtggcaatgtcgctgtataaatgtacatattccttttgttttcctccaaaaagtttattaatgaaattcagattctacgatataataataaataatgttacttcaaaaataaaagagtgtgccaatatggactgtgcttttaccatgagggatttaaactcgattttttttttgttacactgaagttgatgaatatagacattaaattaactcgaatagacaggaaaaatccgatgtccaaaaaaaaagacaggaaagagatatcacaaataatctaacaaaactattatggctaagtatcacatttttagatatatcaacggttcaaagcccgatccatactgtcatacgtaaaaaaatattgttttggcaaaactacatataaggtgatgttactatagaaataaaaccaaattaagaggaaggtgggtaagaaaaaataagagagagtcactttcaagtattgttacattttgtcttttcccatttggctatctctctcttttgccttttcccttttgtggtaactttattttccctataacattttttcattaagtttccatttatggattattttctagttgcgtcaagcatggaatatcaaagaaattagttcgagatttgactaaaaagggtcatttctgctaaataaattactaacactgccattaggccaatcacatgtctagtaacaatttgacatttcacttactattgtaacttttgatagatattgagactttacaaaaaaatattttaagaaaattttgttgaagaaaaaaacttgaatatcattcactataaaaaaaaggaaaaaatgtataggtttttgttacaatactgaacgtaaattgtgaccatgattccataaagcagtaacatttcaaactctaaaaattgttgatattaaaaacttgaatatcatccactataaaaaaaaggaaaaaatgtataggtttttgttacaatactgaacgtaaattgtgaccatgattccataaagcagtaacatttcaaactctaaaaattgttgatattaatctagtttacagaaaaagtagaagaaagaaaaaatgaaattagaaaatgttgagctgacatcacacgccacacacagaattgtatagaaaagaggaagtgtaattaagcatattcttccgcattaacctctctcctctctgtgtcatccaacctcatatactactgatctccatttccagatccccaagaacacaactcatcaacaagtactttaaatactctatctctctctttagagatctctctttctctctctctctctctctctctctctctctctctttctctctgtttctcactaattactctctacctctcttacatacacaaacacaatctctctcgcttctctctaattcacacatcaagataaaagaatcaaaccatccttgaaatgaatcctgtaattaattataggatttcagtttttgagttttttgttcttaatttggttttgtagttaattagggtttctttatagtttatctaccttgcatatatatatgtatgacatagacttacatgacactgaatcaggaggaagaggaaggaacgaataagaggaagaggagagagatgggaagagggaagatagagataaagaagatagagaatcagacagcgaggcaagtgaccttctgcaagaggagaactggtcttatcaagaagactaatgagctctctgttctctgcgatgctcacattggtctcatcgtcttctcctccaccggaaagctctcgcagtactgttccgaacccctcaggttaacttcttcttcctctccctctctcgaattagggtttcagagatctatacatacatgtgtatgtattatctaattaaatgagtaaataagagatatatagctcgtgcttgtgaacagacaattctcatcattagtttctgaagttagcaggtatcatgaatactatgtttcagattttaatttgacccagaagttaagaatctctctgatgctatatatatatatatatatatatatatatatttacttttgcagtatttgatttgtatatatctgtagatgcatgtatataatcattgtttattgatatcggtcaaattctgtaatttctacacctgccaagcaaagagatgttttttcaaagatttttcatttcttgatcaaccttttttcccatataatgtttacgacatatatatatatatacctagtatatatataagtcttatttgaatcattcgatataagtaccattaattataaaggatttttattaaaagttgtaaatctaagtcatgaaccagaagacgaatttattcacatctagcctaacaatataagaagaaaggtatgctgatatagtttgaattttgctatcataaaacaaaaatggggaaaatgtatactctctccgtttttttatataaaatattttatgaattgttttttgttcaaaaatagttgatgttctcacatatctatgcagaaattaattgcattttattgattttaagtgtttaaattttgtatattgtttttttattggttgaattgttttggaattaatgactaaaacatgttttgttttggaaatatacaaaattaaatgatttcttaatctatataaaaaaaccttaaacatcgtatataaaaaaacggagggagtatgttatttgatttttgtgttcctccaatgatgattaaagtcttgacgatgtacgattaaagatactatttgataacaatttattattaccaatgttgaataggatgcctcagctcattgaccgatacttgaagaccagtggaatgcgacttcctgatcctaatgacggccgggtaatatatatatacacgcatacttattcctttgtcttagccaattcaaaacaaagaatataacattctcacaaaaatcaataatcatttggagttttttgtgtgtatatataggaggaattgtaccaagagatggaagtactaaaaagagagacatgtaagcttgagcttcgtctgcgtccataccatggacatgacttaacctcccttcctccacacgagctcgatggtctcgagcaacagctcgaacattctgtccttaaagtccgcgagcgtaaggtaacgtaatatatgttcacatcaatatacatattctcttaaaactatagtgattattacacttttgtttgatctctcttttctatctctactgttaataaattgaagaatgagttgatgcagcaacagttggagaatctaagcagaaaggtcgctctctaattaatcattcttttgataagtactcttaattttattttcctctaattagtcatcttttataccgcggatttaatgatcattaccgtgtctatataaatatatgatcagaggcggatgctagaagaagataacaacaatatgtaccgtttggtaagtttggttactagagaacgtttaatttggttgcacattttcggtttgtgtgacataattattcaacgtattaattgcagcttcatgagcatcgtaacgcggttgaatttcagcaagctgggatagagacgaaaccaggggagtatcaacagtttctagagcagcttcagtactataatgatcatcagcaacaaccaaacagtgttcttcagcttgctacgcttccttctgagattgatcctaattaccatctccagcttgctcagcctaatcttcaaaacgatccaacggccaagattgattagtcctcaaaagtgaatcatttatgtcttttattactacctattttgattatagccaatgccttcttctgtgtctgttttgtgtggttatggaaacctaatattgtttgaagtacaattcacttgaaaagcgtttatggtctttctttgattaaataatttaatcttcattatcacacatttgccaactagagatcaactgtttatgtaatcgcagattttgagatacatttttggccatagaaagagtgggagacacatgagtaaactattcttaggttgttgacaaaaggaagaaccaacacctcagaatcttaataatgtgtgatcgacaagcttatcaaggaccttcactgaaaatagattttatatatttcagacagattagatcgcaatcccaaaaatagctcttataaactcagccaagattgcaaaaattcaatcaacttctgtagggtattgcaagggacgatcaagaagcaggaaaagagttctggaagaagaatcttcctttcctcttttcctcttcaatctgttttcatcataaagacgagaaaaaattgaatacttggcttcttgatcgctcgaataaccatcatcatcatctagatcccccaaacgctgcgttttttgttggctgaaccgtctacatccatgacaggaggatattttatatccgagagtggccatggaaaagagtaccaagaaggccgtgttactgcttttgtcgtgatctcctgcattgtggctgcaatgggaggtctcctcttcggttacgatatcggtatctcaggtttgtttcttcccaaccaagaaaccccaagatttctccttctctcttcttctttctcttctcatcatggcgggatatatttttttcaggaggagtgacatcaatggatgagtttctaacgagattcttccccgacgtgcaacgccaaaggcaacacaatacagggcatgaaacagagtattgcaaattcgacaatgagcttctcactctcttcacctcctctctctacctcgcggctctattcgcttccttcctcgcttcaacgatcacaaggctttttggccggaaaatctcaatgaagatcggaggtctcgcttttctctccggagctcttctcaacggt

SEQ ID NO: 48 - DNA, 1071 bp, Thlaspi arvense
atggctgcagtagaaagagtggagagtttagccaaaagcggaatcaaatctatcccaaaagattacgttcgtccgaaagaagagctcgagagcatcaacgacgttttccaagaagagaagaaagaagaaggtcctcaagtccccaccatcgatctacaagacatcgagtcagaagacgaaacgatccgcgagaagtgcacagaggagctgaggaaggcggctatggattggggagtgatgcatttgatcaaccatggtataccggtcgatctaatggagcgtgtgaagaaaaccggagaagagtttttcggttctcctgtggaagtgaaggagaagtatgccaacgatcaagccacagggaagattcaagggtatggaagtaagttggctaacaacgcgagcggacagttggagtggcaagattacttcttccatcttgtttatcctgaagataagagagatctaacactttggcccaagacaccaagtgattacattgaagcaacgagtgagtacgcgaagtgtcttcgtttgctagcgacaaaagtcttcaaggctctttctatcggtctagggttagagcctgaccgtttagagagagaagtgggtggtttagaagagcttcttctacagatgaagatcaattattacccaaaatgccctcagcctgagctagcacttggcgtggaagctcacaccgacgttagcgccttaaccttcattctacacaacatggttccaggtttgcagctattctacgagggcaaatgggtcattgcaaaatgtgtccccgactcgattgtgatgcacattggagacactctagagattcttagtaatggcaagtataagagtatacttcatcgtgggttggtgaacaaggagaaggttagggtttcttgggctgtgttttgtgagccaccaaaggaaaagattgttcttaaaccgttgccggagttggtgactgttgagtctccggctaagtttcctccaaggacatttgcacaacatgtcgagcataagttgtttaggaaggaacaagaggaattggtgtctgagaaaaaaagttga

SEQ ID NO: 49 - protein, 356 aa, Thlaspi arvense
MAAVERVESLAKSGIKSIPKDYVRPKEELESINDVFQEEKKEEGPQVPTIDLQDIESEDETIREKCTEELRKAAMDWGVMHLINHGIPVDLMERVKKTGEEFFGSPVEVKEKYANDQATGKIQGYGSKLANNASGQLEWQDYFFHLVYPEDKRDLTLWPKTPSDYIEATSEYAKCLRLLATKVFKALSIGLGLEPDRLEREVGGLEELLLQMKINYYPKCPQPELALGVEAHTDVSALTFILHNMVPGLQLFYEGKWVIAKCVPDSIVMHIGDTLEILSNGKYKSILHRGLVNKEKVRVSWAVFCEPPKEKIVLKPLPELVTVESPAKFPPRTFAQHVEHKLFRKEQEELVSEKKS

SEQ ID NO: 50 - DNA, 4065 bp, Thlaspi arvense
gtaaagtagacagctttttggaatttgcagagattatggtacaggaataaacactgaatcgagattatagccactgaatcaatcaaagccttgagcaaatgcgattgagagctgaaatttaacagggtttcgagccacaatactataaactagtgactgaaaaacttcgatcactaaagcttcagctagatttggtggaagaagaaatctaccactaaattctaaaaggctccatctttgtagaatcaattgtgaacggattctaggtaaaggatgaaaattgaagacctgattgctctgtggtggcttttgcaggcaataagaaggatcttcttctcaaggaaatcgatcttccagggctgagctgatcccattgagtcctcggcgacgacgacgacggaggagaaggagaagagaaagaagtggtgggtttgcgagaaacggcggagaaaagtcgagggcttgtcaaattgaacaacatcttgctacccattttccccgggagaagcaaggagagatccttttcctctgttttccgggaaggaacctgtggttgaagatgagttactgtgagcttcaggttccttctgatttttttattttattttaattcaatattttattatttatttatttaatttagtagagaggatttggagggaagaaattaggaaagataagagaggtgtggagatgaattcctaggcagatctctgatattttttccccctctcatcttaaagaaaaagaatatccacgtcagcaataaatatcccacctttctgtattttttgtaactttataagaattttatttactttaatattttttaaatgatacagtgatttctctttgtatataaaaaactttgaagtactaatttactttagacaaacaaatgtgatattattatttcctttgttcagttgatcttttatacaattagtctttttgaaactgaaaccagtcaaatactcaaaatgtttttagtgatgctaaaaattacagaaattatgataaaatgtggacattaaaaataaaataaaaaggtggataatgtacagacacctatattgattgaactatttaaaggtggacacgtggagatacgatttaggcacgtgcacacggacgcagaagaaacgccaccaaaagtctgacgttgatagtcatcggtttaactctattgggcttcttttttatgggcttttaaatccaaagcccttaccaagctaggacatactgtagtaacttctcttccagaattaaaagaaaacttttttgaccgttggatctcaaggatggtgaaaccatcagtcaacctctctcgttgacctgaccgtgaagtgtgttgtcactcactcacctgttcttcctccctacccaaccggtagctccacacttcctaattccttgattaattcttaattctaatggaaaattaatataattatctttgttatataagaaagcctctgcatatatttcatttgacatgcaacaaaatcggcaagaagaatagtagaacaaagtatttattcgttagttatcttacacactgttttttcctctgctttattaagtttctttacttacttactctgtttctttgctctgttttagcttttaaaagaagacaataaagatggctgcagtagaaagagtggagagtttagccaaaagcggaatcaaatctatcccaaaagattacgttcgtccgaaagaagagctcgagagcatcaacgacgttttccaagaagagaagaaagaagaaggtcctcaagtccccaccatcgatctacaagacatcgagtcagaagacgaaacgatccgcgagaagtgcacagaggagctgaggaaggcggctatggattggggagtgatgcatttgatcaaccatggtataccggtcgatctaatggagcgtgtgaagaaaaccggagaagagtttttcggttctcctgtggaagtgaaggagaagtatgccaacgatcaagccacagggaagattcaagggtatggaagtaagttggctaacaacgcgagcggacagttggagtggcaagattacttcttccatcttgtttatcctgaagataagagagatctaacactttggcccaagacaccaagtgattacatgtaagcttttgattcgtttgttttatcatttataaaacaaagttcttgctttggttatagtaacgttttttggatgattgtagtgaagcaacgagtgagtacgcgaagtgtcttcgtttgctagcgacaaaagtcttcaaggctctttctatcggtctagggttagagcctgaccgtttagagagagaagtgggtggtttagaagagcttcttctacagatgaagatcaattattacccaaaatgccctcagcctgagctagcacttggcgtggaagctcacaccgacgttagcgccttaaccttcattctacacaacatggttccaggtttgcagctattctacgagggcaaatgggtcattgcaaaatgtgtccccgactcgattgtgatgcacattggagacactctagagattcttagtaatggcaagtataagagtatacttcatcgtgggttggtgaacaaggagaaggttagggtttcttgggctgtgttttgtgagccaccaaaggaaaagattgttcttaaaccgttgccggagttggtgactgttgagtctccggctaagtttcctccaaggacatttgcacaacatgtcgagcataagttgtttaggaaggaacaagaggaattggtgtctgagaaaaaaagttgaagtttgagtctaatatgagtaaaaactccatgttaaagtttctcgtttcttttgtgtttatgtctttatcctgtatttgatgcgtcttgttgaagatgacacgaaatatttctaccgattgtgaaattgttaaaaatttcactctattataagttggttttatgtatcgccgaagtgacagatgttggaagaaatctagtcattggaaactgtattacattcgtgctaattgcatttcttttcaagtttaaaccaaattagtggaacgtctccggttctagtctgtgtgacttagttatagcttggtgaatagtaaaggaagctcagtaaatacgagtaacatagaaagatatttatgaaccacattgttgtattaaggacttgagaatattctgatttacatttccagtttgttcttttttgttatgctactaactgtaaaaaaactactcttctccctcctttaatgataattggcattccctgcttggaaagagttcactctattttccttgaagaccttaaaaccaagaatagattgcacaactcaatgattagtgttggaaaatagaaaaaaaaaaatcaaaaattgagtttcaagtttcacaaggctgcacctttggttgacgaaatcttgtgagagatccattgttttgctggagctccgatttgatagagagctgcacaggtttaatacgggtcaagagagcgtatacaaataaactagagtgtgtttaagaaagatccattacatcaaaccatgagctgtaccttgctgaaaagatctgttggtaaatctggctgaactctcttttccgaatgaaaactaaactcctgtgtttgcattcccaaaacagtttgcatcctcatcaggtaactcaattttacagacatacagaagatcaagcgcaaaaagaataattggtaaagactaccataccaaaggtactgttgtttctcgcttgctgtttttgaaaatgcccatgtctcctctgcttgagagtatctgttttgcaggagtgtgaaactatgtaaggtgtgacacgtataattaacgcaagcgaaatgagactcgagaaaggataataccttcttgttcagaggacgagctttaaaaacgtgttttccctccgagacatcatgcttaggtatatccataacgcttggtctgcaagaaaaaaatacacttttatgtttacattcacttcaaccacaagttgaagtgagaaatcaagcaatccttcttaatgttccatgtgactttat

SEQ ID NO: 51 - DNA, 645 bp, Thlaspi arvense
atggttgtgaagctatacgggcaggtaacggcagcttgtccacagagggtcttgctttgttttctggagaaagaaattgaatttgagattgttcatatcgatcttgatacatttgagcagaaaaaaccagaacatcttcttcgtcagccatttggtcaagttccagccatagaagatggagatttcaagctttttgaatcaagagccattgcgagatactacgcgaccaagtactcggaccaaggcacgaaccttttgggcaagtctctagagcaccgagccatcgtggatcagtgggccgatgttgagacccattacttcaacgttctggcccaccccattgtgattaacctagtcatcaagcctaggttaggcgaagaatgtgacgtcgttttggtcaaggacctcaaggtgaagcttgaggaagttttggacatatacgagaaccggcttgcttcgaaccggtttttggctggtgatgaattcaccatggctgatttgacgcacatgccagctatgcggtatttgatgggtataatcgatataaaccggatggtcaaggctcgggtgaatatgaaccggtggtgggaagagattacggctagaccggcttggaagaagcttatggtgatggctggttcttga

SEQ ID NO: 52 - protein, 214 aa, Thlaspi arvense
MVVKLYGQVTAACPQRVLLCFLEKEIEFEIVHIDLDTFEQKKPEHLLRQPFGQVPAIEDGDFKLFESRAIARYYATKYSDQGTNLLGKSLEHRAIVDQWADVETHYFNVLAHPIVINLVIKPRLGEECDVVLVKDLKVKLEEVLDIYENRLASNRFLAGDEFTMADLTHMPAMRYLMGIIDINRMVKARVNMNRWWEEITARPAWKKLMVMAGS

SEQ ID NO: 53 - DNA, 3574 bp, Thlaspi arvense
ttaaatgtcggattccaattgagttaagtaagtctcatctatatgtaaatgggtttttggaatagtatcatcttataatcattttacacagaatcaaagttattagccttgctaaatctaggttgtattgatcgaatgatcttcgaaaaaactcagttagctgtaaatgctttgcagggtatgttaatgaatgaaaatctacataatcacatccctcttgaactaatatgtctgtttatagatcaaaaacaagttaggcatgtgaaagttttgtaatcttgttctggttatggtatttgtgcaagctttcgaactcgtgtataaaggttttcttctcattttcatgttacaacaacgcagagatctcaggtcaaggttaccaccacttcagatccactcacacgatgctcttatccaagaagtccagctttggatctcggcttcacttcagctatttttctaatgatggctcagataatcgtcagcgtcggaagcggctgtctctgttgtagaaaaggtcctgctccttccagatctaattggattatcgccttaacctgcttcgttgtttcctggtaatcctcatcatttctttctcctatcgagctttcctacttcacaattttgctggacagacacaagtgacgaatctttgtgtttactcttaggttcacttttgtgatagctttcctcttgctgctaaccggagctgcactcaacgatgaacacactgaggagtcaatgtatgccggttactactcctgctacattgtgaaaccgggagttttctctaccggttctttgctttcgcttctcactgttgccctcgggattgtctactatttgtgtttgacttcgagtaaacaaaacgttgctgacacagcgacgacggcgaaccgaggaggaggtatagcaatgggacagcctcagattccggagagagtggaagatcctgtctttgttcatgaagatacttacatgagaagacagttcacttaaaaacagaacatggctttctttggatacacgttaggttttaggatgataattagataaacaagagatgctgttttttttttttggggattttatctttgtgattttagtatgtgaaactaagaccatgaaacttggtagctggtaatgatgattaatgatgattgataacgtacagaaaaccaaacaaacgtctccttttacttatctatgtgaatttaaagtggttgttgggaagtgttcacaaaaatcagaaattgaaataaataattaacctatccaccggtccgaccaaacacgggacatctaatagaaatcaattttgtttatctcgaatcataagacgaaaactactgaaatttttatgttaataagtttgtagagcaactttggatgatatccaccgttagtggaacaaccaccacatgctctacccaaccagcacaacaaccagctccttttaaatgtttttgagtctaataaaatgccaacacatctactactctcacttcttcacatttataaataagatccagagaagcaattttaaaataacacattgaaattgtttcaaagcttatttttttttaaatttatatcaataaaaatttggttgcaaagttattgtaacgcttatagaatggttgtgaagctatacgggcaggtaacggcagcttgtccacagagggtcttgctttgttttctggagaaagaaattgaatttgagattgttcatatcgatcttgatacatttgagcagaaaaaaccagaacatcttcttcgtcaggtcaaacattttatattttctaattttgaaaagtcatgaattgtatttaatatcattaatgttttcttttagccatttggtcaagttccagccatagaagatggagatttcaagctttttggtaagatcctaataacagcattgtaaaacattctttaatacttgttttatatcattaatatgtagattgtgttttgaaatttggcgtgtgtgctcagaatcaagagccattgcgagatactacgcgaccaagtactcggaccaaggcacgaaccttttgggcaagtctctagagcaccgagccatcgtggatcagtgggccgatgttgagacccattacttcaacgttctggcccaccccattgtgattaacctagtcatcaagcctaggttaggcgaagaatgtgacgtcgttttggtcaaggacctcaaggtgaagcttgaggaagttttggacatatacgagaaccggcttgcttcgaaccggtttttggctggtgatgaattcaccatggctgatttgacgcacatgccagctatgcggtatttgatgggtataatcgatataaaccggatggtcaaggctcgggtgaatatgaaccggtggtgggaagagattacggctagaccggcttggaagaagcttatggtgatggctggttcttgaattatttcgaatttatggtgatctgaaccaaataagcttcatattttctgtactattttctttatctatgttttgtaagtttcaattgataaaataaatttacttttaaagatttaaattcgttaatattttctttatctatgttttgtaagtttcaattgataaaataaatttacttttaaagatttaaattcgttaattctcaattttaaaggggactatagatttacagttatcattttgttacgtattactacaaattgctgaattgttatagaactttttttccaattgtttgtgaacctaatactttaaatctgaatagacatcatgtatttaattatttcccatgttatattttcatctagtatatatagttcattcatttgtagccatgcagatgcacaatgaatctcgattttttttttttttgtgcgagcacaatgaatctcgatctcttagtgtttttgaattcagtaacttctttgcatctttcactaaactatctctccaaccaaaaaaattcatatttcttcagcagccaagagagaaataaaaaatttcaaaaattactttttacatagagaaaaagaagggaacatccgcccatttatatgtatattagttaacatgataaaaaatccgaccctaagttttttcattaatcacaaaagccctctctttggttgtttttcttggcttctctcattcatgtcgacttagaagaagaagctaatcttgagcttgaagtctttagcactgattttgcataagccaatggcaaagctgcaattttcttggctttccctacataagctctctttgtaaaattgttgtaatcattcgcttcaatctcgtccagtatcctcctgtataatagcagcgatgcccatacctgaaaaaattgcacagccaagtgtaagggggttaaatcgatccaaacaaaaaagctttggggcgaaaacaaaacaaaaatgtaaacggtaaagtgtaaacgtgggggcttaagagtgttgttagagacacttaccggccatctgcttgcggcgtcgagctccgtgacgcctttctcagcttcgtcgaagaacattcttgctcgtttaagctgcattttcatgaagttt

SEQ ID NO: 54 - DNA, 1155 bp, Thlaspi arvense
atggttagtcacaaagagaccgtgtgtgtaacaggcgcatcgggattcatcggttcatggcttgttatgcgattattggagcgtggttactttgtccgtgccactgttcgcgaccccggaaatttgaagaaagtgcaacatcttgttgatttacctaacgccaagacgcaactcactctatggaaagccgatttatctgatgaaggaagctacgatgacgccataaacggatgcgacggcgttttccatgtagcaactcccatggattttgaatcaacggatccggaaaacgaagtgataaaaccaacagtgaatggagtgttggggataatgaaagcttgtgataaggcaaaaacagtacgaagaatcatctttacttcttctgccggaactgttaatgtcgaggaacatcagaaaaatgtctacgttgaaaatgattggagtgatcttgactttatcatgtccaaaaagatgaccggatggatgtatttcttgtcgaaaactttagccgagaaagcagcgtgggattatgcgaaggaaaatggattagacttcattagtataattcctacattggtgatcggtccattcataacaacatctatgccgcctagcctcatcaccgcgctctctcctatcactcggaacgaggcacattactcgatcataagacaagggcagtacgtgcatttggacgacttatgcaatgctcatatattcttgtacgaacaagctgatgccaagggacgttatgtttgttcctctcacgatgccacgattcttagtatctctgaatttattaggaaaaagtaccccgagtataacgtgccttcaacgtttgaaggtgtggatgaaaatctagagagcattgtgttcagttcgaagaagctgattgatatgggatttagctttaagtatagtctcgaggagatgttggtcgaatcgattgagacatgtcgtcaaaagggttttctcccggtttctttaccagatccatcaatatttgaggacaaagttccgactagtgatgacaagattgagcacaaaaccggagctggtttacccgatgatgtggtgccctgtaagaagacagaaccggtggtaatccgcgagaaaaccgatgcttgcatgccggcagagcagatgtgtgcttag

SEQ ID NO: 55 - protein, 384 aa, Thlaspi arvense
MVSHKETVCVTGASGFIGSWLVMRLLERGYFVRATVRDPGNLKKVQHLVDLPNAKTQLTLWKADLSDEGSYDDAINGCDGVFHVATPMDFESTDPENEVIKPTVNGVLGIMKACDKAKTVRRIIFTSSAGTVNVEEHQKNVYVENDWSDLDFIMSKKMTGWMYFLSKTLAEKAAWDYAKENGLDFISIIPTLVIGPFITTSMPPSLITALSPITRNEAHYSIIRQGQYVHLDDLCNAHIFLYEQADAKGRYVCSSHDATILSISEFIRKKYPEYNVPSTFEGVDENLESIVFSSKKLIDMGFSFKYSLEEMLVESIETCRQKGFLPVSLPDPSIFEDKVPTSDDKIEHKTGAGLPDDVVPCKKTEPVVIREKTDACMPAEQMCA

SEQ ID NO: 56 - DNA, 4705 bp, Thlaspi arvense
cctccgttattatggagccttgtaattagtgttcagaaaatcaatcccaacaatattatctaatattttctatagaaaaaatatagtttaacaagtgtttagatgcctcatatcaaactctctaagattgtgtttctaatctagtactaagtacaagtccaatgactccaaccacaatcatatttattctacacatgaggggtgaaattttaattgttaaataaaaaaatatagatacaattattctattctatagtttatatgttgacaaagaaatctttggtaaattttatttttaaaagtcaaaaagatatttgttaaaagtattgttgtttgaggaaatgctccaaaataatccagaataagaaaataatatgaaacggtactccattgagaaaaaactgtgaaaataacccatattttatgattttttttaaataccagtgctacatttctaactatttttacttgtagtctaatggcatactgaatgcagagtactggcagactgattggtcttacaattgaatatagactattggcagactaaatgcaaattactgacagactaacgacagattaaaagcatattagtggatcctgcttatggatcatttgaaaaaggttcatgtttggtaacaaaattaccaaatgaataatttcaaaaattatcccatttgagtaaagtatatttttatttttggctaatttcttctttgaattaacccaaattatggtgtttgtaaattgtaactgtgatttttttttacatcaagaagtgaatggttgacaaaaaaaaaagaatgattaaggtttaaatactaaactcgtatatttaaattataaacttttcgaattcattttttttaattttatcaatctttagaaaaatattatatgtttctagaaagtttctataaattctaatgtgtttaccattaaaaatatattatttattttcctcatttgaaatatcaatttatttatatataactcataattttaaaaatttatatatcaactcatgtcaaaattttaatttcatatcagtttatttcaataatgtttttacacgtattaaaatctaatcaattacactcttttattattaacaaatttgacgtattaaattttatatgataaattttgttaacgtattaaaataatataaactcttcttgtagtttagtaacaaaataaaaaaattacaaaaaacaataagtaagaaaaggaaacttcaactcttgtcgctatctcactaaacaaacaagcaaacccattcggcgtagttcacccaccagtacaactaaaactatatcctaaaaaataataaaatcaaacttaccagtttgtcacgtaccacacaacccagtccttcgccaaccaacgttcctcacgtgcttcgccggttggtactcacgtgaccggcagctttctaatagcaattctcaatacatatataatctcttcataccaaagctacatatatagtctcttcataccaaagctacatagcaaagtctatcccaaagcacagtccatctttataatacacaaaaatggttagtcacaaagagaccgtgtgtgtaacaggcgcatcgggattcatcggttcatggcttgttatgcgattattggagcgtggttactttgtccgtgccactgttcgcgaccccggtacgtatatatgttcttacaaactaactcgttaattaatttttcctaagattaattaaatctatgtgtggctaatttacgggttttattgggttatttatataggaaatttgaagaaagtgcaacatcttgttgatttacctaacgccaagacgcaactcactctatggaaagccgatttatctgatgaaggaagctacgatgacgccataaacggatgcgacggcgttttccatgtagcaactcccatggattttgaatcaacggatccggaagtaagttataatatgaacctcttttaggtttcatatcaaccctaaaagatcttgttggttaaatttttttttttttttaatcagaacgaagtgataaaaccaacagtgaatggagtgttggggataatgaaagcttgtgataaggcaaaaacagtacgaagaatcatctttacttcttctgccggaactgttaatgtcgaggaacatcagaaaaatgtctacgttgaaaatgattggagtgatcttgactttatcatgtccaaaaagatgaccggatgggtaaatatatataaattatatatcaaacatcacactaaccctaagtttattcttcttcatagttatttatgttttaataaaatgtttttggcagatgtatttcttgtcgaaaactttagccgagaaagcagcgtgggattatgcgaaggaaaatggattagacttcattagtataattcctacattggtgatcggtccattcataacaacatctatgccgcctagcctcatcaccgcgctctctcctatcactcgtgagctctcacttaatttctactctttttgtaaactaagagatttcttgaccttaggccaggtcttgctcataaaatcaatgtccactgagcaatattctattttataagcctaataatcataaatggcaaggaaaacaacctatttttttttaaagaaccttaacgtctaaccaaaaattacaaaaagttatatggacccaatgcaaatacatctttggcacatgccaagaaccggatcgtaggaagatctttctggctagcgactagagcatgtcaactagtctcttctatcttccatcttcttttgttggaatttgaaatgttaattttttttaaaaacggtgaaaatgtttcagggaacgaggcacattactcgatcataagacaagggcagtacgtgcatttggacgacttatgcaatgctcatatattcttgtacgaacaagctgatgccaagggacgttatgtttgttcctctcacgatgccacgattcttagtatctctgaatttattaggaaaaagtaccccgagtataacgtgccttcaacgtaagatttatagatttaaattacggagtttaagccttgttttgcttaagcaatcaagatcgtttgctgaaaaactatttggaacaggtttgaaggtgtggatgaaaatctagagagcattgtgttcagttcgaagaagctgattgatatgggatttagctttaagtatagtctcgaggagatgttggtcgaatcgattgagacatgtcgtcaaaagggttttctcccggtttctttaccagatccatcaatatttgaggacaaagttccgactagtgatgacaagattgagcacaaaaccggagctggtttacccgatgatgtggtgccctgtaagaagacagaaccggtggtaatccgcgagaaaaccgatgcttgcatgccggcagagcagatgtgtgcttagagatttaaccggtatctattatatatcaattgtcgtatcgttttagtattggatgtgtgttttgaatttgttactttctgaatcgtagattattattgaagggtggtatggactgattctgatagtaacatgattgagtgtaacattatgaacttttacatatttaagaagcagagtgatatttaaacaatgttgccttgagtcaaattagtcgtgtaatgtcgcttgaatgcttccataatctataattagacaatttcaacatctcaatcgcaggcatgcatttcttaacaaagagttatatattcggtggtcactggaaatattttatacatatataatataatttaactactatgcagattacagagtataagaaaacaattcttggctaaatagattttcagttacaaaataaagaaaaaccaaatgactgaactttttttatttgaagaacaaaaaatgaaaatttagtcgttcgagttaatttacggatcctatcagctaaaaataatttagttctgttgagatgtccatgctttttttggaatttggattttcctttttccatatgtgaaacctttccatataccaaaaactctatcatcaaactacccagcctttgtatctctatgccaaaaaaaaaaaattaaacaaaatctttaatttgaagtcggactgtcggagtatatggtttttcttgtacgtacgttttccaaatgcttcagtaaattgctcttcgaagtctttcatcgtcagctggaaagaaatacaaaagtgattcctcttgtgcctcaaatgttcttttgtagcttaggagaggatattgggagatgggttttaaagaatttttcaaattttgagattctattgtttataaatttttaaaatcttaatagttaatattgttattggttgaaagattttaaaattctatccaaaatcctttgttatttaaaaaatttagcttttaaagattttatgatttattaaaatcttgtgttattggaacatgaattttaaacaatctaacttataaaataattctttcaaaatactacctatatagcttagattctcaaagtcattataataaaatattttgatagattttttaaatataaaaactctttccaaatttaacaaatattttttacaagtttaacaaatctcccaactcttgaaatcaatcaaaactttataatttcatctcttaatgaccctcccttactctttgctttttgttgtttgtttctcaattc

SEQ ID NO: 57 - DNA, 1188 bp, Thlaspi arvense
atggtgatgggtacacaaccgtcgttggaagagatcagaaaggcacagagagcggatggccccgcaggcatcttggggataggcacggccaaccctgcgaaccatgtgatccaggcagagtatccggactactacttccgcatcaccaacagtgagcacatgactgacctcaaggagaagttcaagcgcatgtgcgacaagtcgatgatacggaaacggcacatgcacctgacggaggagttcctgaaggagaatccggacatgtgcgcctacatggctccttctcttgatgtgaggcaggacatcgtggtggtcgaggtccctaagctagggaaagaggcggcagtgaaggccatcaaggagtggggtcagcccaagtccaagatcacccacgtcgtcttctgcactacatccggagttgacatgcctggtgctgactaccagctcaccaagctcctcggtcttcgcccttccgtcaagcgtctcatgatgtaccagcaaggttgctacgccggcggcactgtcctccgactcgccaaggacctcgctgagaataaccgtggtgctcgtgtccttgtcgtctgctccgagatcacagccgtcaccttccgtggcccctctgacacacacctcgactccctcgttggtcaggctctcttcagtgacggtgctgccgcgctcattgttggtgcggaccctgatgcctccgtgggagagaagcctatcttcgagatggtgtctgctgcacagaccatcctcccagactcggacggagccatagatggacacttgagggaagttgggctcaccttccatctcctcaaggacgtccctgggctcatctcgaagaacatagagaagagtctagaagaagcgtttaaaccgctcgggataagtgactggaactctctcttttggatagctcaccctggaggtcctgcgatcctggaccaggttgagttaaagctaggactcaaggaagagaagatgagggccacgcgtcacgtgctgagcgagtacggaaacatgtcgagcgcgtgcgttctcttcattatggacgagatgaggaggaagtccaaggaggatggtgtggccacgacaggagaagggttggagtggggtgtcttgtttggtttcggaccaggtctcaccgtagagacagtcgtcttgcacagcgtccctgtttga

SEQ ID NO: 58 - protein, 395 aa, Thlaspi arvense
MVMGTQPSLEEIRKAQRADGPAGILGIGTANPANHVIQAEYPDYYFRITNSEHMTDLKEKFKRMCDKSMIRKRHMHLTEEFLKENPDMCAYMAPSLDVRQDIVVVEVPKLGKEAAVKAIKEWGQPKSKITHVVFCTTSGVDMPGADYQLTKLLGLRPSVKRLMMYQQGCYAGGTVLRLAKDLAENNRGARVLVVCSEITAVTFRGPSDTHLDSLVGQALFSDGAAALIVGADPDASVGEKPIFEMVSAAQTILPDSDGAIDGHLREVGLTFHLLKDVPGLISKNIEKSLEEAFKPLGISDWNSLFWIAHPGGPAILDQVELKLGLKEEKMRATRHVLSEYGNMSSACVLFIMDEMRRKSKEDGVATTGEGLEWGVLFGFGPGLTVETVVLHSVPV

SEQ ID NO: 59 - DNA, 4151 bp, Thlaspi arvense
cgaatccgcatagagaagctgaagctcaggtttctcaattatttcttctttctttttcaaaaggcttatcattgacttgtctctgtttttttttttttttttttgtgatcattgattcagtctctccaacttgatgaaaaagataaccatccaagagcccacctttgagagaattattgtagtatacaggtacaagagtagagtaatggtgaaatctttggagggatgtgagtttgattctcattttggctttggattcacatacacgcaggagagtttcagggaagagagaatcagaaaggaacatatatgtgaaacacttcaagagcattcctatggctgatatggaaattgtgcttgtaagcatccattaaccaacactttgtgctcaaatgtatcttactaattataaattaactgattgctcataacggcacagccagagaagaaaaatccaggtcttacgccactggactgggtcaagtttcttgtctctgctgccattggactggtcagttctgctacactattctaaagactttaataatcagactctgaaaattttgatttctcaaactctgcttttacaggtcacagtggttagttcagtgagcctaaaaaaaactgacatcagagtcattgctgccatacttagcacggtcgtggcctactgcgttaaaacatatttcacgtaatctacactcaataatcagacaacaccctcgcttatagctaaattaatccttaattagctctgtctcttcctctgtatgaaatgtaggttccagagaaacttggtagattatcagagccttatcacaagatctgtgtatgataagcagctagacagtggaagaggcactctgcttcacctctgcgatgaagtcatccaacaagaggtgctaataaatagtccttttttcttatttttcttatgtcatattcttgtgttttgctaattaaaaaactgatcaaacgcaggttaaagaggtcattatttccttcttcatgctgataaagcaagggcgtcccacgagcaaggaggagcttgacatgcaaagtgaagcattcatcaaagaagaattcaacgaaagttgcaatttcgatgtggatgatgctgtcaagaagcttgagaagcttggacttgtctctcgtgtgagtctccttcatctctcttctataatcttttctttttctccacgcatatgcttgtatatactcagtaagtaaactaatattgtgaaaatggaaagggttggtcaggattcagaagacaagtatagatgcgtgaatatgaaggaagcaaacgagataatgggaacaacgacggaagagatggtactcaaggcaagaagaggtggtgaatatgaagatgaagaggcagcagagactgagccacggatgaatcctcaagatgaactcacagcaaaggaagaacgttatcaatctcaattagacgagttcgagaccttgtggttgtaaaaagatttgacgtcattcaagacaaataaatttgatattgtattaaagaaaaagaaaaaaagacataaaggcagacaaattaattgaaaggacccatcaacaatgagtccaccacatttcacatttcacactaaatgaattctcccttaattatttcatacataatttatattaaaatgaaaaacataagactcgatgatggaaagtatgtgtaggtaggtaggcatataagaggagagcgctctgtatggtgatgggtacacaaccgtcgttggaagagatcagaaaggcacagagagcggatggccccgcaggcatcttggggataggcacggccaaccctgcgaaccatgtgatccaggcagagtatccggactactacttccgcatcaccaacagtgagcacatgactgacctcaaggagaagttcaagcgcatgtgtgagtatccctcttaatactccctattttgtatctcttcatttcttttggcatatggttcccatagttaacaattactgtaacaggcgacaagtcgatgatacggaaacggcacatgcacctgacggaggagttcctgaaggagaatccggacatgtgcgcctacatggctccttctcttgatgtgaggcaggacatcgtggtggtcgaggtccctaagctagggaaagaggcggcagtgaaggccatcaaggagtggggtcagcccaagtccaagatcacccacgtcgtcttctgcactacatccggagttgacatgcctggtgctgactaccagctcaccaagctcctcggtcttcgcccttccgtcaagcgtctcatgatgtaccagcaaggttgctacgccggcggcactgtcctccgactcgccaaggacctcgctgagaataaccgtggtgctcgtgtccttgtcgtctgctccgagatcacagccgtcaccttccgtggcccctctgacacacacctcgactccctcgttggtcaggctctcttcagtgacggtgctgccgcgctcattgttggtgcggaccctgatgcctccgtgggagagaagcctatcttcgagatggtgtctgctgcacagaccatcctcccagactcggacggagccatagatggacacttgagggaagttgggctcaccttccatctcctcaaggacgtccctgggctcatctcgaagaacatagagaagagtctagaagaagcgtttaaaccgctcgggataagtgactggaactctctcttttggatagctcaccctggaggtcctgcgatcctggaccaggttgagttaaagctaggactcaaggaagagaagatgagggccacgcgtcacgtgctgagcgagtacggaaacatgtcgagcgcgtgcgttctcttcattatggacgagatgaggaggaagtccaaggaggatggtgtggccacgacaggagaagggttggagtggggtgtcttgtttggtttcggaccaggtctcaccgtagagacagtcgtcttgcacagcgtccctgtttgacttttacaattcaagtcttttagagtttgatcgatgagtgagattgtgtactatgcaagttatgtatatttgatggcaagcggagagtgggagtttatattaacgagagaaagggagaagagagagtgtggtaggttagatggacgggcagatgaagcactacgtgtctatgtgttagctcccttttatgtggttctccttcttgcttcccttttatttcgttacttaccaagaatattgaatggtggtttttttattgattttacgtatattcgcaacaacaagtcatattaatttctatgtgcgtaattattatatattcgatgtatatacatgtaaagatacgtacggcctactggagaggttagttgtatagattttcccacacgtgcatacttaactccatcattagctcctactaatctaattttccttcttaatatacctgataatcctataactaactaaaaattacattaggtacgtctcgttttctctctcccaccccatcatgatgatagtttgaatctgctcctttttcggcttccaacaacgcaagatgcatttcgcatcccatcataatgatatttgtgttgttgctgttctttatgttagactaataaaagatgcatttgtaagcttttgcctcattaattttattcggaaaaaaattgaatatgcgtaatatcacatcgttttttgttagtattcatttattcaattcatgtcttaataatgttgtagatatttttattggaaaaataatatcaatgggcccataaaagaaggtgggccctagagctggttatgcttagccatgtgggcagaatataaccagagtgtgttgtcattgtggtaagtaggggcactccaatgcgggtgtttttatcaacccggcccggcccaaagcctatccgtcgaaaacccgtgtccatcaaaaactcgccaaactagcggttatatttagggttgggcaaattatccgttatatttgattcgatctgctatttgtttcgattcgattcgaaaaatccagatatccatagctttacggagcaaagcaaatactaaattttgatattcgttaaaaacggagcaaatcacaaatattaaaattttaagagtcggatatccgatctgctctaata

SEQ ID NO: 60 - DNA, 759 bp, Thlaspi arvense
atgtcttcttccgcatgtccgtcaccgttaccctcagtcagcaaacttcatgtcgattccgttacttttccaccgtccgtcaattcaccggcttcctccaatcccctattcctcggtggcgcaggggtgcgagggttagatattcaaggaaagtttgtgattttcaccgtcatcggagtttacctagacgctgtcgccgtcccgtcactctctgttaagtgggagggcaaaactacagaagagttaacggaatccgtcccttttttccgtgaaatcgtcacaggtgcgtttgagaaattcataaaggtgacgatgaaactgccgttaacgggacagcagtattcggagaaagtaacggagaattgtgtggcgatttggaaatcgttagggatttacacagagagtgaagctaaagctgtggagagatttttggaagtcttcaaggaccaaactttcgctcctggtgcatccatcctcttcgctctctcccctaacggctccctcacggttgcgttttcgaaagacgatagcattcctgaaaccggaaaagcggtgatcgagaataaattgttggcagaggcagttcttgaatcaataattggaaagaagggtgtgtctcctgggactaggctgagtatagcagagaggttagctaagctgatgaagaagaagaaggtcgaagaagatgcatcatcactgactgatcaagaggaagctacagatctctccctcggagataaattggccaaagagaactga

SEQ ID NO: 61 - protein, 252 aa, Thlaspi arvense
MSSSACPSPLPSVSKLHVDSVTFPPSVNSPASSNPLFLGGAGVRGLDIQGKFVIFTVIGVYLDAVAVPSLSVKWEGKTTEELTESVPFFREIVTGAFEKFIKVTMKLPLTGQQYSEKVTENCVAIWKSLGIYTESEAKAVERFLEVFKDQTFAPGASILFALSPNGSLTVAFSKDDSIPETGKAVIENKLLAEAVLESIIGKKGVSPGTRLSIAERLAKLMKKKKVEEDASSLTDQEEATDLSLGDKLAKEN

SEQ ID NO: 62 - DNA, 3963 bp, Thlaspi arvense
ttccccacaaacaatgtgtgtgtcagctatatatttatgggaaggctgaaacgtttaaatactagcctctgcatcgtttgttgtaattttgtgataaaattgtaacatatttaatcgttttatctctaggtacttttatggaatattgtaaaagaattctatttttgtgtaaaatccaaattagcgtattatacttgaatacacaagcatttcggcacatagttcaattggggttaattcatgaatcatttttaattcaaaaatttcgacccatcaaaattagacaatgaccaaagaaattataaaaaatgagatgatgtttgaaaatgtttagtgaggaagtgaaggtatagattatagacgtttattgtcaaatttcaacggatgttatatacgttgttaaatttaaaacaactttagaatatatatggcgcgtgattttgttaaatcgactttggtaggaaaatgttattttgcgattttgtcaagaaaacgtaattttgtgattttgaccaaaaaaaatgttatttacagtaatagaaaaaaataattttataatttaaaaaacatgatttttgattttattgaaattttttttttttaattttagtgagaagtgattgcacatttttaatgggaaaattttctacaattttaattaaaaaaatgatttcagcataattttagtaaaaaaattgtgattttacagttttataaaaaaatatacgtttttatttttttgaaataattgaaaaatctcatttatattatgttgatttattcatctgaaatttgcatttaaatattctatctaaataaaagtattttaattatttgttattttaaaatagattatttccattttttatcaataaacaaccccatatgttgttaaacaaagaaagaaaggacaatctatatttcttagttatttttattattatattttctttattctttattctctttatttatattatttttataatgttcattaattaaaacctacctcttacagaacttttttgggttgttttaaaaggatcagacatagtgtaaactaaaaaattaaactgaaccaaaccaaactatgtcttatacttatcaagtaatatacactacatgataagcttaaactagattctatctttatcataaattaattttatctttatcacattgtggtctacataaatcctcattacataagtatcttaattaaatcttctagattcttccttaacagtaaaccaagattaaaaatgatctgatttgaactgataaaacctaaactaaaaagaaattggcatacctaccgactctaaagcggtcagagttcccgcaaccaccaaaattataaaccactgaatcttccaatcaacaaaaccacgtgtttacccatccaacactcgtaagctattgctagttgctacctacctccatcttctcttataattaccaatctccatcaaattcttttttacttttttttacattataatcaaacctaacaccctcaaagtcaaaaccatgtcttcttccgcatgtccgtcaccgttaccctcagtcagcaaacttcatgtcgattccgttacttttccaccgtccgtcaattcaccggcttcctccaatcccctattcctcggtggcgcaggttcgagtgctgtttaattcatttgctcttgcagcattcttttttttttttttaaatgcgttttttgttgcctctttgagtttctctgtttcttgctaacttacgcaggggtgcgagggttagatattcaaggaaagtttgtgattttcaccgtcatcggagtttacctagacgctgtcgccgtcccgtcactctctgttaagtgggagggcaaaactacagaagagttaacggaatccgtcccttttttccgtgaaatcgtcacaggtgcttgtcatgcaacaaactgttttaagtcaaaaagggattttaatttgtttagaccaaactatttgaccgtcattaatttattattaccatttttagttaattatgatttttttttgtttttgggcacgattaggtgcgtttgagaaattcataaaggtgacgatgaaactgccgttaacgggacagcagtattcggagaaagtaacggagaattgtgtggcgatttggaaatcgttagggatttacacagagagtgaagctaaagctgtggagagatttttggaagtcttcaaggaccaaactttcgctcctggtgcatccatcctcttcgctctctcccctaacggctccctcacggtacttcttgtcctatcacacagctttgcgtttgcgtttacattactattacgaactgtttacaatgaaacgcaaattaatgtagaaatagcgtttaaaacgaactgtgcccaaaacatgtatttttaagtaagatttggttttaaaaattgttttacgtgtattaaacgcaattgacgttagaaaaacagtcgtaggttgtaaaatgtctttgttgtgaaaaaaaaatcgttttgcaggttgcgttttcgaaagacgatagcattcctgaaaccggaaaagcggtgatcgagaataaattgttggcagaggcagttcttgaatcaataattggaaagaagggtgtgtctcctgggactaggctgagtatagcagagaggttagctaagctgatgaagaagaagaaggtcgaagaagatgcatcatcactgactgatcaagaggaagctacagatctctccctcggagataaattggccaaagagaactgatcctatgccgagatttttcttggtttctgagggattttatgtttctgttatatttaatcctattccatcgcatgtttaatttatctctgttcgtaagaataattaaataacctcatggtattggatcaaagtttccaaacaaaacaaaattgtattgtcaaatatttaatacaagccaaacttgataaacatttagttctaggcttgatcacacggatccgcaaggttaagtaattggttaaccgaagggaagggaaaacacctacacgaatcccggaccgggcctaaattcttttaactagaacacggcccaatctgtagaccagttcggcccattgtagtatcaaaaatattccataaacgaaatcatttgatttcaaatggaggaaatcattaaattagcagacgcggaaaaccactatctcatcaaaataaattgcgaaatttattgaataaactaatgaatcaataaataaatgaaatggtccaaccatctaaaaattgattttctaagatgtcactgtatcaatatcacccattcatgttcatataaaccctacccgccagcataatgcatattgagtattgacgacttataaacaaaagaagaaatcacttacagaaaaatgatttcttgaggaaatagatcacaggatgtgtatgttgattaatgacctagggtacaataatgcagtttgattcactactagacccataattttttttttttaaaaataaaaagggctttcatgacccataaaaattattattatctttttttcccataaaaattatttgataattgtttacgtgtttgtttgttttctcgttcatattgatatttctctcatccgaattcttgcattttcaacgtgtcaattatctttttaaaactacgtaaatactattatgataccttgtaggcttgtactgaatatttgtgagtattttaggctttataaattcttatgccgactttgttatcaagccttcgacacattttctgtggcgttcttgagactataaaatttgggagacgattgaaccattttgtttttatctataatggtttttcttttgtatcctttatttgattttttttcttctttttttggctggttctagagaccttcttagccacagtgattcttctgtcatcagttcatcaaatcctgaaaagagcatcatagc

SEQ ID NO: 63 - DNA, 1239 bp, Thlaspi arvense
atggctccagggactctcaccgagctcgccggagaggctaagctcaactctaaattcgtccgggacgaggacgaacgtcccaaggtggcatacaacaagtttagcgacgatatcccggtgatatctctcgccggactcgacgatgttggtgggaaaagaggagagatctgccgtaagatcgttgaggcttgcgagaattggggcgtgttccaggtggtcgatcatggtgtcgataccaatttggtagaggatatgactcgcctcgctcgcgacttctttgctttaccacccgaagagaaacttagtttcgacatgtctggtggtaagaaaggcggcttcatcgtctctagtcaccttcagggagagactgtgcaagattggagagagatcgtgacgtacttctcgtacccggtgagaaacagagactactcacggtggccagataagccggaagggtgggtgaaagtgacggaggagtacagcgacaaactgatgggtttagcttgtaagcttcttgaggttttgtctgaagctatggggctcgagaaagaagcacttaccaatgcttgcgtcgatatggaccaaaagatagttgttaattattaccctaaatgccctcagcctgatctcaccctcggactcaagcgtcacactgatcctggaaccatcactttgctgctccaagaccaggtcggtggattacaagccacacgcgacgatggcaaaacatggataacggttcagccaattgagggagcttttgtcgtgaatctcggcgaccatggtcactatttgagcaacgggaggttcaagaacgcggatcatcaggcggtggtgaattccaactcgagcaggctatctatagccacgtttcagaatccggcgcaggatgcaaccgtgtatccgcttaaagttagagaaggagagaagccgatcttggaggagccaatcacttttgcagagatgtataagagaaagatgggaaaagatctggagctggctcgcctcaagaagcttgcgaaagaagaaaatgaccagaagctggccaaagaagaacatgacaagaacctggccaaagaagaaaatgatcagaagctggctaaagaagaacatgaccagaagctggccaaagaagaacatgacaagagccttgccaaagaagaaaattaccaaaagctggccaaagatgaacatagccacacggaagctgttaagcgtctcggccaaatcctcgcttag

SEQ ID NO: 64 - protein, 412 aa, Thlaspi arvense
MAPGTLTELAGEAKLNSKFVRDEDERPKVAYNKFSDDIPVISLAGLDDVGGKRGEICRKIVEACENWGVFQVVDHGVDTNLVEDMTRLARDFFALPPEEKLSFDMSGGKKGGFIVSSHLQGETVQDWREIVTYFSYPVRNRDYSRWPDKPEGWVKVTEEYSDKLMGLACKLLEVLSEAMGLEKEALTNACVDMDQKIVVNYYPKCPQPDLTLGLKRHTDPGTITLLLQDQVGGLQATRDDGKTWITVQPIEGAFVVNLGDHGHYLSNGRFKNADHQAVVNSNSSRLSIATFQNPAQDATVYPLKVREGEKPILEEPITFAEMYKRKMGKDLELARLKKLAKEENDQKLAKEEHDKNLAKEENDQKLAKEEHDQKLAKEEHDKSLAKEENYQKLAKDEHSHTEAVKRLGQILA

SEQ ID NO: 65 - DNA, 4251 bp, Thlaspi arvense
aaaatgtagggaaaaaaaaacagagagaatcagatacagagagacgaaatccgaatcggagtctatctatctacttgaaattggtgacagaagaggaacagagaattgctaataaaattctaagataggcacaaaaaaacaagaacaagtttcatttggaacaagaagatgactgaaagaaactgcaagaagagaatcatggaaagacaaaacatacctaatgaaaagggaattttagagtcagaatcagagttactgattgaaaagatagcctgcgatctagtgactcttcttgctgatgatggagtctccattaggatcttgatcgtcttgcaagcaacaacggctaaagatcaagtgaaagaatttctgggaaaatcaatctgaatttcaatatctgagatatcaataaagaagagaaaggggataaacaattgcgaatctcttaggtagcagtattataggtatggggaaaaggttaccgtttgaaataaactagccgttgcgtctaaacggaaggaaggagccgtaatactagccgttgggtccattctctcatggaaagaaatcaagaatggttaaagacttaaagtagctgtttgggttgaaatctcagtacgttaggggcttttacggattaagaaggctgcgattaatagctcggcccatttatctctctgttgcgagttgcaagctgctaaaagttttataagcttttttattcggttatttgccaatcgtttaaattactcctatgatttataaatcttggaatgtgtgtatgagacgaagtattcattgttttcaatctatggtgtctgttttatgttttgcttttttttttttaattaaatatacaactcacaattcacaagccatgacaaaacatatcaaaatgttgataagagtaatgaaaactaaatacactagaaaagtcagatccaacatttcgtcttctcggattaaggacgatataaatataatatatatagtgaaaaaaaggtttttcttctctgatctcaatgggattatgtacaaataaccatgcaaaattgatgatcatttggatttttgtagtgcaaacccgtaacgtaacaatttttgccatgtgaattcaccgagaacgaccattttttttctttttttaataaaaaaatatgcaacccattttttaagacgtggcattaaattcaccgtaaaaaacatttaactatattgggcatggtgttaaagcaactttactagaaacgatttatgtacacaatggaatgtagcgcagaaaatatgatttattagaaagaaattaaagacagaagcacgtataggaagttgagtaactgcgtgtttctagaaacagaacggacggtatagtactgtggtaggtagcgagcgacctcttcgttcgtcagtcttcacaacctttgaaaggtttttcagctaccagtcatctccttatatattggttacctcttttatctctctttataaacttaattagtcttttgcctttgtaaccaaacactcacaaaaaaatataaaaatggctccagggactctcaccgagctcgccggagaggctaagctcaactctaaattcgtccgggacgaggacgaacgtcccaaggtggcatacaacaagtttagcgacgatatcccggtgatatctctcgccggactcgacgatgttggtgggaaaagaggagagatctgccgtaagatcgttgaggcttgcgagaattggggcgtgttccaggtggtcgatcatggtgtcgataccaatttggtagaggatatgactcgcctcgctcgcgacttctttgctttaccacccgaagagaaacttagtttcgacatgtctggtggtaagaaaggcggcttcatcgtctctagtcaccttcaggtaaagccacacaatttacgttacgttttcatgcgactcaaacttttatactgtagacttaattagacctataatcacatttcgggccgcaaaaatacgaattatgttttgatcttgtagttaaatacgaaataatgatgataaacgcagggagagactgtgcaagattggagagagatcgtgacgtacttctcgtacccggtgagaaacagagactactcacggtggccagataagccggaagggtgggtgaaagtgacggaggagtacagcgacaaactgatgggtttagcttgtaagcttcttgaggttttgtctgaagctatggggctcgagaaagaagcacttaccaatgcttgcgtcgatatggaccaaaagatagttgttaattattaccctaaatgccctcagcctgatctcaccctcggactcaagcgtcacactgatcctggaaccatcactttgctgctccaagaccaggtcggtggattacaagccacacgcgacgatggcaaaacatggataacggttcagccaattgagggagcttttgtcgtgaatctcggcgaccatggtcacgtacgtcagtatactctctcaatctctctgcttatatttttctccgtttgtgattttgacttggccaaacttgcttgtctattgaagtatttgagcaacgggaggttcaagaacgcggatcatcaggcggtggtgaattccaactcgagcaggctatctatagccacgtttcagaatccggcgcaggatgcaaccgtgtatccgcttaaagttagagaaggagagaagccgatcttggaggagccaatcacttttgcagagatgtataagagaaagatgggaaaagatctggagctggctcgcctcaagaagcttgcgaaagaagaaaatgaccagaagctggccaaagaagaacatgacaagaacctggccaaagaagaaaatgatcagaagctggctaaagaagaacatgaccagaagctggccaaagaagaacatgacaagagccttgccaaagaagaaaattaccaaaagctggccaaagatgaacatagccacacggaagctgttaagcgtctcggccaaatcctcgcttagagtccttgttgctccgctgtgttggtttcggtttggttttgtaatttgttttatcgtcaagttaacgaacgtggtgtgtttgagtttcttctcaatatagaaataatgacaagtaatgcaattgtacttgctctgtttgtttggttactttttatgtcagaagcacatacattactttctcgctattcgtgtggatgtaaatttaataagataatgacggttaaaccggtagtaggaccattttatttctttatggtttctttacgccacgtgtccgtctaaaagaaacttaccttgaaaaagtgaataattcatccctctttttcaagtttcgatttttttttctcttttcgagtcattttgttctaatcaacgacgacgcgacggagatgaatccttttcacggtgccgacgggaagcaaagaccggcgatgtatccggacatcgatcaatcaattccggataatcctttcgctcagacaaacccttatgccgcttctgcccctaatctctacccttctccctcctcgaacaatctcgggcctaatcttttcccggaccacggagatgcatccaacaaccagtcaccgtctgctccgcctcaagcgacggaggaggttctcatccgtgtcccgggctccattctcaaccttatcgacaaatcctacagcgtcgaactcgcgtgcggtgacttcaccatcgttcgaatcgtccagggccagaacatcgtcgccgttctcgccaacgtcgccgatgagattcaatggccgttgaacaagagcgaggtagcagcgaaggtcgatgggtcgcactatttcttttcaatccacccgccaaaggaagagggtcacggatctgggtccgactccgatggtgagaagcaggggaaaaagagcaatccgaaaccggaggacgaaattctcaattacggattgaccattgcttcgaaagggcaagagaacgtattaaacgagctcgaccgggttctccgggactattgctgcttcacggagcagaggatgtctgaaaaggcgaaggagacgggagaggaggtgctgggaaactccatggctgcggcgacttcgccggaggagctgaagggtgagaggaaagacatcgtggagggtcaatgcgcggcgtattggaccacactcgcgcctaacatcgaggattacagtagcaagactgctaagttgatagcttccgggtcaggtcagctgatcagagggatactt

SEQ ID NO: 66 - DNA, 1545 bp, Thlaspi arvense
atggccactctcttactcacaatcctcctccccactttcctcttcctcctcgtcctcctcctttctctccgccgcaaccacaaccgcagtagccgtctcccaccaggcccaaaaccatggcccatcctcggaaacctccctcacatgggtcctaaaccccatcgaaccctagccgccatggtaaccacctacggtccaatcctccacctccgattagggttctccaacgtcgtggttgctgcgtctaaatccgtggccgaacagttcttcaaaatccatgatgccaatttcgctagccgaccaccaaattcaggagccaaacacatggcatataactatcaagatcttgtctttgcgccttacggacaacgatggagaatgttgaggaagattagttctgttcatttattttcagctaaagctcttgaagattacaagcatgttcggcaggaagaggtaggaacgctcacgcgcgagctagtggatgcaggcacgaaacccgtaaacttaggccagttggtgaacatgtgtgtggtcaacgcgcttggaagagagatgatcggacggcgtctgttcggcgccggagctgatcacaaagcggaggagtttcgatcgatggtgacggaaatgatggctctcgccggagtattcaacctcggagatttcgtgccggctctggattggttagatttacaaggcgttgctggtaaaatgaaacggctacacaaaagattcgacacttttctatcgtcgattttgaaggagcacgagatgatgcacggtcaagatcaaaagcataaagatatgctcagcactttaatctcgctcaagggaactgattttgacggtgacggcggaagcctaacggatactgagatcaaagccttgctcttgaacatgtttacggctggaactgacacgtcagcaagtacggtggactgggccatagctgaactgatacgacacccggatgcaatgaccagagcccaagaagaacttgattcagttgtaggccgcgataggcccattaacgagtcagacctttctcggcttccttatcttcaggcggttatcaaagagaatttcaggcttcatccgccgacaccactctcgttaccacacatcgcatcagagagctgtgagatcaacggctaccatatcccgaaaggatcgactcttttaacaaacatatgggccatagcccgtgacccggaacaatggtccgacccgttatcgtttcgacccgagagatttttacagggtggagaaaaatccggcgtcgatgtgaaaggaagcgatttcgagcttataccgttcggagccgggaggagaatctgcgctgggctcagtttagggctacggatgattcagttactgacggcgacgctggttcacggatttgattgggaattggccggaggaattccgccggagaagctgaatatggaggagacttatgggattactctgcaaagagcagttcctttggtggtgcatcctaagccaaggttggctcccagtgtttacgaactcgggtcgcgctaa

SEQ ID NO: 67 - protein, 514 aa, Thlaspi arvense
MATLLLTILLPTFLFLLVLLLSLRRNHNRSSRLPPGPKPWPILGNLPHMGPKPHRTLAAMVTTYGPILHLRLGFSNVVVAASKSVAEQFFKIHDANFASRPPNSGAKHMAYNYQDLVFAPYGQRWRMLRKISSVHLFSAKALEDYKHVRQEEVGTLTRELVDAGTKPVNLGQLVNMCVVNALGREMIGRRLFGAGADHKAEEFRSMVTEMMALAGVFNLGDFVPALDWLDLQGVAGKMKRLHKRFDTFLSSILKEHEMMHGQDQKHKDMLSTLISLKGTDFDGDGGSLTDTEIKALLLNMFTAGTDTSASTVDWAIAELIRHPDAMTRAQEELDSVVGRDRPINESDLSRLPYLQAVIKENFRLHPPTPLSLPHIASESCEINGYHIPKGSTLLTNIWAIARDPEQWSDPLSFRPERFLQGGEKSGVDVKGSDFELIPFGAGRRICAGLSLGLRMIQLLTATLVHGFDWELAGGIPPEKLNMEETYGITLQRAVPLVVHPKPRLAPSVYELGSR

SEQ ID NO: 68 - DNA, 7303 bp, Thlaspi arvense
ctctttttcgtttaaaaataaatataaaatcagttctttatgaaattcaaatgcggtctatgatccataaacgtggccttggcatttacccgaatcccatccgtctccatcatttgcctttcgatcgtatatggaagttggaacgacgtcgacgccaattctgcggtaatcgtaatagtattaaaattgtggagccaacggaaacacaatgcatttttgcatttccatgcacacctttgtttaattttctaaagagaaattagtatatatataatttgtattgatctaatttttttaaatccagttcgactttgaaggaatttaagttcgacttgtatataattcttgtcaagacctcgatcccgcatccagtaataaaataataatgattgcaaaggacaacactaataaagaaaatgctataacgagaaagaattctgaaagacgtactaacgaaaattgtgtcctagtgaccataacaggagtatcatccaacactatgaaccacatatcttacctacccttcacgagtactctccagctaccacgattaacgataaatatatggtccagagaatttccgaatgatccgctaatattcgaataactgaaattatcaagcagtgagtttaattttttgtaaccgtatatctttttagccttttaaaatgataaactcatttatgaattaattgaatatatattacgtttaacccatccattcatattgtcacatatttttgaattttgttaacttcctttttatttcttttcgtattttctcaaaatcatatgtagtcattatatatacacacaaaaaaaagagatagatattgactaaaaggtagtgaaaaattacaaatctatagacattacaccataaaaaccatttttcaatagacaaatatatggttttactatgtgttgcgggaatcaacggaatcaacttgatgttagtatttacaaatagacgataaatcttctaaaattaattataaacacgtgaaagcttaaagacattgtgtaatatcttctgataatttttaatgttcaagacagtattttgattatgaagcttggtcgaaaccaaaaacaaaaatcaaaagacaagaagaattgaagaagtgaagaacacaacgtttcgttttaaaccatacaaaaaagtggttcacgatgtgatcttaaatgtatatctctttaataatcacttttccgttgaaaaggagaggaaaaaatcactgtagacttagtttttggaaagtatttctcatccccttttcgcaaggggattgtgtttttttttatcgaaaatacatggtccatggttaaatgggtcaagagtataatttagtactataattttataatcaaaatgttctaagttctatcttatatttatataaaaatagaagaagatgttctaacttatatcatattaattagtggctttacttaaccaaaagattgttacttatatttttcaacctacgttctactaacgactaagtattcagtaagatatatagctacctttcatagtattaatcaaatcttacgaaccagaaagctcacctaccattcgactctctttcgcttccaacttattctacataagataagattttctcatctacatattcgtatgtttgacgtcgtggtgggatccatgatttatccactttaacaatagaaaacaaaaacctaatcagagaaatataagctcttatgttttaaaaggaaaaaagcaatggaaattgaagctttttaaccaacaaaaaaaccagagaaatatacattattataattttatatattctgtcaagacgataattatcaatgtatatgtgtactaataatgttattactcgattacacccgtagttaataagccacttaaaattaactatttacaaaaaaaaaaaatcttttggtgactttgatttgatggtgtgaaaatctacatctcattcttcagtattcagatgattataacaaaatgttttttttctaaacttgcatttccgataatctaatactaaaaaatgtatcggcagaaagaatactagcttgaaaaacctttttataaaaaagaaaagtaaatatactagctaatggtgcccaacaggagatcgaagtggtgatgtttaattagttaaaggtaaaagaaaacctatttctaacttttgatgaaacaataaaaacaaaaaaatctttctaacctaaccgagacatgcatagatagattattggatttcgcaaaaaaaaaaaaatcaccctttatttatagcttatgtttgttattcctcatttctcacttaccattcaaacccaacactatggccactctcttactcacaatcctcctccccactttcctcttcctcctcgtcctcctcctttctctccgccgcaaccacaaccgcagtagccgtctcccaccaggcccaaaaccatggcccatcctcggaaacctccctcacatgggtcctaaaccccatcgaaccctagccgccatggtaaccacctacggtccaatcctccacctccgattagggttctccaacgtcgtggttgctgcgtctaaatccgtggccgaacagttcttcaaaatccatgatgccaatttcgctagccgaccaccaaattcaggagccaaacacatggcatataactatcaagatcttgtctttgcgccttacggacaacgatggagaatgttgaggaagattagttctgttcatttattttcagctaaagctcttgaagattacaagcatgttcggcaggtaacagtattagttataaacgttattctcatttcctaacgctataactcacctatatatagagatagtcatgccgttaatttttatatttatgattagtttattttatatcattatttaactgtggtacgaactctagaatttaataaaataaatttagagaagtacgtatagagatttttaatggtggagtggcgtttttttgtttagtattatgttttcagtgttgataaaataaccaaaaaataataatgttagtaatcgttaaaacacaaaacaaattttgttgataaaacgagatttatgactttttatcaacagattttgttttgaaaaacgagaactagaacataatactataacaagttccaatcctgtagaactagtcaccaagtcataaaactggaacttttttatcaaaaaatattgtttcgtttttcacgatttgcaacctttttcgttattttaacaatattggaaacattgcaacctataaaccccaatttaaacgagtaaaacaaaaaaaaaatactaaagtaggcctaagtgcaactgtgcaatactgtcgttgccatagacgtacagtacgatgtatccttgataataccatggaaaaatggaaagttcatcagaaacccaaggacaaaatacttcaatatgtatggaccacatttttccttaaataagatgtatcaacgagtcaccacgagacacgagtgattcactttcagtagtataagattgtttttgcattttcgtttaaaaaaatgtagatgaacatacaagatgatcctgacaatttatttataggtagattacttttcattgatggaacaattgaatatacaaaaatgtaaactagacttcagaattttaagtttaggggttaaagtaacttaactagggtctaaagtgtatataggctttatatttgagcttaggatttagatattggttaattagtggattttaatcgatttaaatttagaagcaagattatttgttattaagttattactttttaaaatcatagttaaagtcatgtgttaggggtttaataaattctaaatattagttgaaatttaatgttattaatttttataagaaatcgattttacattcgattttagtttttaacatctttgtaagtgcttttgagttactaaagcaactttcttatttaaaaacaggcttattgaattttttttaaaaattacgttttgaaagcatttgagtaattgtaaatcttaagtaaatttataaatcaattataaccctaactaaaatttattaatcaactaaacttcatacaccaataatcctacttagagttttataaggtttttgctgttaatcaaacatcaagatttaaaaatgagtaaaataaattccaaaatcaactaatatacccaaaattttccatttatagtttaagtagagcaaaattgaattttacaggaagaggtaggaacgctcacgcgcgagctagtggatgcaggcacgaaacccgtaaacttaggccagttggtgaacatgtgtgtggtcaacgcgcttggaagagagatgatcggacggcgtctgttcggcgccggagctgatcacaaagcggaggagtttcgatcgatggtgacggaaatgatggctctcgccggagtattcaacctcggagatttcgtgccggctctggattggttagatttacaaggcgttgctggtaaaatgaaacggctacacaaaagattcgacacttttctatcgtcgattttgaaggagcacgagatgatgcacggtcaagatcaaaagcataaagatatgctcagcactttaatctcgctcaagggaactgattttgacggtgacggcggaagcctaacggatactgagatcaaagccttgctcttggttcgtataacgatcaattaattgtagtattaatttcatactttatgaaaagttattgattccttcttaaatacagaacatgtttacggctggaactgacacgtcagcaagtacggtggactgggccatagctgaactgatacgacacccggatgcaatgaccagagcccaagaagaacttgattcagttgtaggccgcgataggcccattaacgagtcagacctttctcggcttccttatcttcaggtatacccttaaccgggaattaggaattgtcttggttaacgagctctattgttaatccggtttaaacggttttgttttaaaaacaggcggttatcaaagagaatttcaggcttcatccgccgacaccactctcgttaccacacatcgcatcagagagctgtgagatcaacggctaccatatcccgaaaggatcgactcttttaacaaacatatgggccatagcccgtgacccggaacaatggtccgacccgttatcgtttcgacccgagagatttttacagggtggagaaaaatccggcgtcgatgtgaaaggaagcgatttcgagcttataccgttcggagccgggaggagaatctgcgctgggctcagtttagggctacggatgattcagttactgacggcgacgctggttcacggatttgattgggaattggccggaggaattccgccggagaagctgaatatggaggagacttatgggattactctgcaaagagcagttcctttggtggtgcatcctaagccaaggttggctcccagtgtttacgaactcgggtcgcgctaaacctaagtttgcttgccagcaaaggtaggtcttgcacggaggttaaaaagcttgtttctggaatttcctcaaataaagtttaaaatagcgtaatgtggtccggagtataaggctatgttatctgcgtcgtcgatccgatgccgaggaagaagacgatggctctcgaaagcaaacctgatccgcggacccgacccgttttatacgactaagattttcattcataatagtatatgataattttaaattttaaatttttatcgtgtaatttttacagtactgaattttgtattaaagcatcttccttactgtaccagatgcatttacaactctagatttttttctgccagcaaaatcagatttttccatcttttttatatatattaaagtggaacaccactacaacctgcaattctgcaacacatgttacattacacattcatttggcgttttccaataagttataaacagtgaatgtttgtagacaatagacaattataaacagtaaatcatgtttcccctctgttttcaaaagtgaaaaagtttctaaatatgtatatgtattatactttaataactcgtcggaccatactattcccaccttctaattaaccttgtatacactggtttaccaacaccatgtctcttccttgttcaaaaaaactccatgtctctttaattactttttttcttcttctcgaaatttgttgataatagaaactagtcgaagtttctctttaattctgttttcatttaatataagcgtcgttgttataatttcaaatttcaaaaaggtacttacaagttcacacggagagctacaataatggaaaagctgactcaagaagggctagaaaagaaacaagagtcacggaacaagtagtcactttcaatctcagtatacagtacactagtgtctgcttgcatctctctctctctctctctctctctcttggtctaaaaatatcagaagagaaaatctctctatctatttatctctctttccctttctctttcaacaagacaatagtgacgacatttgtgtttccatggctgttctggttctctatctcctcggtttcctcatggctggccactgtagtaagaaactctcgctcttcactacattacttatctctctcttttttttaaatgtgtctattgatgggaactaaatttcaataaaattctttcggctcttagctagttatcactacatctcttaagttcacgaccctcaaaaagaaggtttcctcaaatcttcttggcttcacacttacaatttgtttcatttggtaggcgcgacgtggtgtgtgtgcaaaacaggactgagtgactcagtgctacaaaagacattagactatgcttgcgggaatggagctgactgtaacccaactcacccaaaagggtcttgcttcaaccccgacaatgttagggctcattgtaactatgctgtcaatagcttctatcaaaagaaaggtcaagcttctgaatcttgtaatttcactggaactgccactcctaccacaactgatcccagtaagtttccctcagaaatctgatgcttttactgtgattgtttacaactctaaatagtttttggagtcacagaaagtccaccgtcattttggttacttaaaatgatttggtattagagattagtgaatattaaagtttaaagtaacaatttggttttagtaatgtatgaggaggatctgatttggttacagtacactaaatgtttttttttttgtgtgtgtgcttttttgctttgatgggtgaacattttgtcacaggctactcag

SEQ ID NO: 69 - DNA, 1581 bp, Thlaspi arvense
atggatgaatcaagtatttttacggcagagaaagtgatcggagctgagaaaagagagcttcaagggctgcttaaggcggcggtgcaatctgtggagtggacttatagtctcttctggcaactttgtcctcaacaaagggttttgctgtgggagaatggatactacaacggtgcaataaagacgaggaagacaactcagccggcggaagtgacggcggaagaggctgcgttagagaggagtcagcagctaagggaactttacgaggcccttttggccggagagtcctcatcggaagctagggcatgcacggcattatcgccggaggatctgacggagactgaatggttttatctaatgtgtgtctctttctctttccctcctccttccgggatgccaggaaaggcgtatgcgaggaggaaacacgtatggctatgtggtgcaaatgaggttgacagtaaaatcttttctagggctattctcgcaaagagtgccaaaatccagcagacagtggtttgcattcccatgcttgatggcgttgtggaactaggcacaacgaacaaggtaaaagaagatatagcgtttgttgagctcataaagagttttttccataaccaccccaagtcaaacccaaaagctgctctttctgaacactccatcaacgaagagcacgaagaagacgaagaacaagaagaagaagaagaagaagaagtagaagaagaaatgacaatgtcagaggagataaggcttggctctcctgatgatgatgacgtctccaatcaaaacctactctctgatttccatgtagaatcaacccacactttagacacacacatggacatgatgaatctaatggaggagggtggaaactattctcagacagtatcaacacttcttatgtcacaacccacgagtcttttttcagattcagtttccacatcttcttacatccaatcatcatttgccacatggaaggctgataattttaaagagcatcagcgagtggaaactaaatcgacgtcgtcgtcgcaatggatgctcaaacacataatcttgagagttcctttactccacgaccacactaaagaaaagaggctgcctcgagaagagcttaatcacgtggtggcagagcgccgcaggagagagaagctgaatgagagattcataacactgagatcattggttccctttgtgaccaagatggataaagtctcaattcttggagacaccatcaactacgtaaaccatcttcgaaatagggtccaagagctggagactaatcatcacgaacaaaaacataagcggatgcgtagctgtaagggaaaaacgtgggaagaggtcgttgaggtttccatcatagagagtgatgttttgttagagatgagatgcgagtaccgagatggtctattgctcgacatccttcaggttcttaaggaacatggtatagagactactgcagttcataccgcggtgaacgagcgtgatttcgaggccgagataagggctatggtgagagggaagaaaccaagcattgctgaggtcaaaagagccatccatcaaactatatccaatattaaactatag

SEQ ID NO: 70 - protein, 526 aa, Thlaspi arvense
MDESSIFTAEKVIGAEKRELQGLLKAAVQSVEWTYSLFWQLCPQQRVLLWENGYYNGAIKTRKTTQPAEVTAEEAALERSQQLRELYEALLAGESSSEARACTALSPEDLTETEWFYLMCVSFSFPPPSGMPGKAYARRKHVWLCGANEVDSKIFSRAILAKSAKIQQTVVCIPMLDGVVELGTTNKVKEDIAFVELIKSFFHNHPKSNPKAALSEHSINEEHEEDEEQEEEEEEEVEEEMTMSEEIRLGSPDDDDVSNQNLLSDFHVESTHTLDTHMDMMNLMEEGGNYSQTVSTLLMSQPTSLFSDSVSTSSYIQSSFATWKADNFKEHQRVETKSTSSSQWMLKHIILRVPLLHDHTKEKRLPREELNHVVAERRRREKLNERFITLRSLVPFVTKMDKVSILGDTINYVNHLRNRVQELETNHHEQKHKRMRSCKGKTWEEVVEVSIIESDVLLEMRCEYRDGLLLDILQVLKEHGIETTAVHTAVNERDFEAEIRAMVRGKKPSIAEVKRAIHQTISNIKL

SEQ ID NO: 71 - DNA, 5726 bp, Thlaspi arvense
atctaatcaagagaagctagctaacaatatcgaagggaagacatgaacacatcctcacttttgcctaatcgaatgaaagctaaaaatggatctagggtttaagggatctaacgatggaaagcaaaggactcaagagaacggcggctaggaacggcggaacgacggcggctctcctcagcggcggcggtcggcggcgaaaacgaacggcggcggcggcttgctcggttagggttcctaggttatatctctgagtgctttgggagttatgatggaaaacctaattctctaactctgtttatatagggaagactcaggaaaaatcctaatatccttttctcttgggcttctgacacatgaacctttccttttcctattgagcctagatccaggacgttacaactagaatcagaatcgaacaacaagcgtatgcgcttaagaaatgatttttactcacactatatgggcgcgcatggcattgtcgtaagaattaaataagcttcgtcccactccttaatggatttacgcacacagtcaatccacgtggttgtcataactaaatataattggtgaaaaaactaatttaaagacaaagtaagaagcggaaaccgaaggaaaagccaaacaacattatgtttatcgacaaaaaagccaaaacaacatttaatgttaatttttgtccaaaccaggaatacatcactcatacggtcatatataccataccccaaattgtatgtactacatgtgtacgtaactgatttatgtatatctatctatttctcttttattgtaggggtcaaaatctacctatcgatatttataaataggattttataagacattgttaaaatggaaaacatggtagctacttggccagcgattaacatcaataattaaaaatacgaattgtgaaacatctcactctcttccttttatcacaccaaaccacttctctttctttacttaccggtcaggtcaacaattctaccattccctttatttagtttttttttttcatctatctctcttttcatttttaacttttaaaaaatattagtccgaaaatcgcactcttttatattcgttgatgggcattaaaatattgtaaaaattaaaaaaaatgtgtaaattaaaacgcaatttgtttgcacctgcagcagtagtaacacacaagtcaaagcaatgtctgttttctcttgtatgtcggttagctattttatgtactgaaatatgttattctttctgaccaaaacatattaagaaatttgcattctgtaatttgatttatccaatcagtagaggacacgtaaccaagataattagatatttttattctatctgtatactactaattcatccaacgtctgttggacgaccaaccagtcaaaactcataaaagtcaacttttactacatcgtgaattttttggtcatgcatttatatacacatacatggaagaaaaaacaatactttacctatgtcaaaatgctgcaaaagcattaagatggtatgtatacatacatattgatataacagtggtcccatatatcattttaaatcatcataaagagtatccatcttctttcatattaacatccccttcaaagttataagatttttctctcttcattagagagagagagagagagaattaacacaagttttaatctccgggaaagatggatgaatcaagtatttttacggcagagaaagtgatcggagctgagaaaagagagcttcaagggctgcttaaggcggcggtgcaatctgtggagtggacttatagtctcttctggcaactttgtcctcaacaaaggttcttttttttttttaataaatttcatcgatctctcacaataaaaaccctaaattttatatcatttattattatatgtttaactacataattatcagtattttaaccgtccatgtgctttatttggttccatttctgtctcatattttacttgaggttcagactgccgagcacatctctcgtttgtctcgaatctgtgagactttttcgtttattggcacttctgtgtcaattgagttatactgaagtaattatatgtttaaatgaattagggttttgctgtgggagaatggatactacaacggtgcaataaagacgaggaagacaactcagccggcggaagtgacggcggaagaggctgcgttagagaggagtcagcagctaagggaactttacgaggcccttttggccggagagtcctcatcggaagctagggcatgcacggcattatcgccggaggatctgacggagactgaatggttttatctaatgtgtgtctctttctctttccctcctccttccgggtacccaactctctctctctctctctctctctctctctctctctctctctctctctctctcttttgtctatactgaagtttcttaatttatctttttatcatctcctactgaagacaaaaatagtattgtgtgttaaatgcgaatcacgaatattgtggaagcattaaaaacaaactgaggaggttgagttactgaaagaagaaatgtattggagttgatgaaacgtacactccattttagtgaacataattggaccgttgagattcttatttttttgctgattgattatctaaagtagaagcataaatagataatacataaatgcataacaaattgtgttagttatgggtatagttaatgctttttctctatgagaggaaaaaaaaaaaaatatataaatgtggaagtaataattttgtaggatgccaggaaaggcgtatgcgaggaggaaacacgtatggctatgtggtgcaaatgaggttgacagtaaaatcttttctagggctattctcgcaaaggtctatttcctttttcatttaccactactctatgcatctacttctctacctatttatatatctcatctttcaaattaattaattttctgtctttattttcttggatgctccttctacatcggtcggttccttaatggttagagtgccaaaatccaggtaaacgttgtctttattgattaattctaattttgagtaatattttacatttattttacatgtttgaaaattgttttgtgataaaaaaaaagcagacagtggtttgcattcccatgcttgatggcgttgtggaactaggcacaacgaacaaggtacggcgtagttatctttttatatatgcataaccaaatggttaagaaaaaggttagaagagaaatagatcatgcttaagttttatcagttaaattaaaaatgtaaaaataagatattatgttcattaataatgtatagtccctgttagttaaaaaaaagaataaaatatttaaccatttgaagtcataatataaaaatattgtttttggagatagtacataattctcacaataaaaaaaataacaaagggatgattaagggaaggagttggatacatgttgtttgtctgtgtgtgtgaaggtaaaagaagatatagcgtttgttgagctcataaagagttttttccataaccaccccaagtcaaacccaaaagctgctctttctgaacactccatcaacgaagagcacgaagaagacgaagaacaagaagaagaagaagaagaagaagtagaagaagaaatgacaatgtcagaggagataaggcttggctctcctgatgatgatgacgtctccaatcaaaacctactctctgatttccatgtagaatcaacccacactttaggtatacacttatacattaaattagttaacgatatcattacacgtatctatttattttgttaacaagaaatttaaaaatattcgccatttctttgttatgtctaaagaaaatctataaaattttatgaatagacacacacatggacatgatgaatctaatggaggagggtggaaactattctcagacagtatcaacacttcttatgtcacaacccacgagtcttttttcagattcagtttccacatcttcttacatccaatcatcatttgccacatggaaggctgataattttaaagagcatcagcgagtggaaactaaatcgacgtcgtcgtcgcaatggatgctcaaacacataatcttgagagttcctttactccacgaccacactaaagaaaagaggctgcctcgagaagagcttaatcacgtggtggcagagcgccgcaggagagagaagctgaatgagagattcataacactgagatcattggttccctttgtgaccaagatggataaagtctcaattcttggagacaccatcaactacgtaaaccatcttcgaaatagggtccaagagctggagactaatcatcacgaacaaaaacataagcggatgcgtagctgtaagggaaaaacgtgggaagaggtcgttgaggtttccatcatagagagtgatgttttgttagagatgagatgcgagtaccgagatggtctattgctcgacatccttcaggttcttaaggaacatggtatagagactactgcagttcataccgcggtgaacgagcgtgatttcgaggccgagataagggctatggtgagagggaagaaaccaagcattgctgaggtcaaaagagccatccatcaaactatatccaatattaaactatagtttaagactctaacaatattgatgccaactctagaaaaggacaactgaacttattttgttttaagccttggctatattacattatcagttttacacttctacgtatacacaactttaatttttctatattactacatgcatactagatgttagaaatatcttatataagcatacatattaaattagttatgcgatatttaaaattaatgtatataaatattcagtttcaaagcttacgaatacgtaaaattaatcaatacaaaccgaaaccaaaaagccacttctcatctcaaaatgttaattacaaatttacaataagccgaatcactatctaaaaagcttttgggatcccgagacccaaaacatttcttcgtataagtgcaacaattatcgagtgtgatgagacacgtaaaaagcaaggatcgggacaacgattttcggctatatagtagtttctcatatctgactttattagcaaattactacataaaattgcttttaagtatgattaacggaacaagtataatgcgtttatttaattacagatctggctaaatgtaatatggtatcaaagctggaaagacaaatagtctaaggtttggaatttttcatctgtctataaaattcttaagacactgatagatcattaacttattttggagtcaccaatggacaaatcaataactattgatgtccaaaacccacaagacaagcctattttttttgcacgtgcaagtacaccggtggaagaattcatttgtatactgaatctgaaattataaaagattagaattggttgaagaatttacttcaaaacaagctagaagatggtgttatttaaataaacaatgttaaattatatcaatgactttcaaattttatcaaaacattttttgaaagagaatcacgcacaaagtatttcgaattacaaaacaattttttgcaataaattttatagttaaagcaaattttgtcaattattgaaaaaaattacttagataaaatatctaatttttttttttaaacaatgtctctataaaagatggattagccaagaaaatctgatggatgctacaacgcagggttggagatatggtgctgacactacat

SEQ ID NO: 72 - DNA, 2583 bp, Thlaspi arvense
atggaagggaactctttaagttcatcttccttagtttcagccaatcgggtgggtcaatgtgacaatcttgagcatagtagaatgacttgttctcgaaatttcattgagatgcatttgactgaccagctgagaaaaactcagatagtgaacgagaccaataaggatcttgttgtcgaggcactgagatcaatcgcggagatattgacttatggcgatcagcacgaccctttattctttgaattttttatggagaagcaagtaatgggagagtttgtacgtattttgagggttagcaagacagtaacagtttccgttcagttgttgcaaaccatgagtattatgatccagaacctaaaaagtgaacaagccatctactacttgttcagtaacgaatatgtaaattatttgataacatatacatttgacttccaacatgaagagcttctatcttactacatatccttcctaagagctgttagtgggaaactaaaccagcatacaatatcgttgcttttgaagaccgagaacgatgtagtagtttcttttcccctttacgtcgagggcataaaatttgcatttcatgaagagaacatgatacgcactgcagttcgtgccctgactcttaatgtgtatcatgttggcgatgaatctgtgaatgattatgtagttagtccaccgcacactgagtacttttcaaaattagttacatttttccaaaagcaatgcatggatctaagtgcaatggtgttgaacactctaaagagcccatcccgagactcaggtggaaaattgtttgctgccgttgatgggatcgaggacacgctgtactactttagtgatgttatctctgctggcatacctgatatcgggaggctgataacagatcacattctacagcatctaactctcccacttcttctcccgtctttgtgctctgaggctgataaatcagttgatcctgtgacttctctctatctgctctgttgcatcgtgcggatagttaaaatcaaagatttggcgaatttgactgctgctacttttttctgccctgtagaagctttcatttcaagttccctagtgaaacctaatagtagcttggctcctgaacgtcttacatatggaaatgggcatccagacaatggtgttgctgaggaaacagttcaacagtgtccaagcactgcagtctcgagtgaatatggaaattcccacgtttgcagtgaaaatactacgaaaagcatcttcaacaattcacgtattacgtttagggatactttacttcaatatatttctgagggagatgatgtgcaagctcagggttccttgtttgtgctagccacgttgttgcagacaaaagaacttgaagagtcaatgctagatgcttttggcattcttcctcagcgtaagcagcacaaaaagcttttgctgcaatctttggttggggaagacactggtgaagaacaactgttttcaccacaaaatggttccatgagagatggcttaagcagcgaacttgattggtatctacggaggttggaggagcagtttggagtatgctgttcactgcctggggctgcaatgtgcccgcgtgtacatagacatcaggtggtggatgcattggtcattcttctctgccgtgaaaacatatctgcagaaacattatgggatggagggtggcttttacggcagttgcttccttatagcgaggcagagtttaatcgtaaacatctcaaaatgctgaatgattcatatgagaagtgcacaagtgcactaatccgggaggttaaaggtacctggcctgatctactcatcacggtgctgcttgatgagtggaaaaagttgatcgaagctccatcccctcaaaaagagcctaaatctgttcttctccagctggataaatcctcttctagtggtaacactgttagcgaatcatcattcacagccggtgaaaaactgtgcgaggtggtgaaggtttttgtgcttcttcaccaactccagatcttctcgcttggtaggcccttgccagagcagcctcctatccatcctcctgcagacagatctgaaacgtctcgcgccacaagtgctggtttggatgtttcagtccccaaaactggcaccgaagtgaagctagttgatgctgtacactgtaggattgcctttgaaagaggcaaggagcggaatttctcgtttctagcattatcatctggtgtgtctgggtggattgtccttgctgaagaatcgctttcgaagccagatcacggaaccgtccgtgttaccgcacctttagccggctgcaaaccccggatagatgaaaagcacccaagatggctacacttgaagatccggccatcgacgttaccattcttggatccaacaaagcgaggagtctatgagaagctcaagtccaaaggtctagtagacgggagatggacattagcattcagagacgaagagtcttgttactctgcttactcaatggttgtacatgagatcgatctacaatgcagcgaggttgaaaggaggttaaagccattgttcgaccttgagagaaaccagcaagatcaatcaaacgttgcttctctatag

SEQ ID NO: 73 - protein, 860 aa, Thlaspi arvense
MEGNSLSSSSLVSANRVGQCDNLEHSRMTCSRNFIEMHLTDQLRKTQIVNETNKDLVVEALRSIAEILTYGDQHDPLFFEFFMEKQVMGEFVRILRVSKTVTVSVQLLQTMSIMIQNLKSEQAIYYLFSNEYVNYLITYTFDFQHEELLSYYISFLRAVSGKLNQHTISLLLKTENDVVVSFPLYVEGIKFAFHEENMIRTAVRALTLNVYHVGDESVNDYVVSPPHTEYFSKLVTFFQKQCMDLSAMVLNTLKSPSRDSGGKLFAAVDGIEDTLYYFSDVISAGIPDIGRLITDHILQHLTLPLLLPSLCSEADKSVDPVTSLYLLCCIVRIVKIKDLANLTAATFFCPVEAFISSSLVKPNSSLAPERLTYGNGHPDNGVAEETVQQCPSTAVSSEYGNSHVCSENTTKSIFNNSRITFRDTLLQYISEGDDVQAQGSLFVLATLLQTKELEESMLDAFGILPQRKQHKKLLLQSLVGEDTGEEQLFSPQNGSMRDGLSSELDWYLRRLEEQFGVCCSLPGAAMCPRVHRHQVVDALVILLCRENISAETLWDGGWLLRQLLPYSEAEFNRKHLKMLNDSYEKCTSALIREVKGTWPDLLITVLLDEWKKLIEAPSPQKEPKSVLLQLDKSSSSGNTVSESSFTAGEKLCEVVKVFVLLHQLQIFSLGRPLPEQPPIHPPADRSETSRATSAGLDVSVPKTGTEVKLVDAVHCRIAFERGKERNFSFLALSSGVSGWIVLAEESLSKPDHGTVRVTAPLAGCKPRIDEKHPRWLHLKIRPSTLPFLDPTKRGVYEKLKSKGLVDGRWTLAFRDEESCYSAYSMVVHEIDLQCSEVERRLKPLFDLERNQQDQSNVASL

SEQ ID NO: 74 - DNA, 7185 bp, Thlaspi arvense
cgtggatggaggaagggtttctcgtcgtgttcgtcgcgaaagatggttcctcttctgcgccgccaccgccggagatcgaggagaatcgcaacgtgagagtcgtggaaatcaccggtgatgaatgaatgaataattatgtctttaaaacttcaaaatctgtgtattatatgaacagagtaatcatgttgtgatcgtgctgctgttttcgtatgtaatagtgaaagttgcataaaagcccttaaactaatcaaagttttcaaaataacccatcatttaagaaaactataaaacgatcaaaattaatgtaaaatctacatttgagcttccgactacaacatttattcgattcaatttcccttttaataatctaacaaattttccaaatttcaacaaatctcgaaccgaatgattatttgattcaaagacaaactattatgttttcgctacaacccaaaacgatgaatttaagtgtacagtcggaattgtattactgtatagattttaaattagatgggacatttgtttaaacaatttaattaagtgagggttattttacaactttgctatattttgaggggttttgttataattttgtgacttaatagcaagagtcgtctttgaaggaaccgttgtgacgtggcggtcttcaacactcgaatggtcgatcgtaaaaataaatgttttccctaattaaaatgccatagacggatccccccattctaaagattctttctttgaattcgatattgaacccgacccggatccgaatctggatacttgacccaacgccagctcaacgccccacttcggtgcttgcttctattcgtctctccgtcaacaattctgttgtttaccggaatacctagagccttcgagaaattcaaacacgacgcagatatcattctttcgcttacgctattgatttgtatgattttgtcgtcggtgaagcaatccgaaccggaactggaatcggatttcatcaggacttgtggggttccctttaatcgaggagcaaccatggaattggggttttcgcgggagtgaaggatgatccagagaagactggattcagaggattgatccgataatcatgtggttctccttcttaagacccagagatcgattctccttggtcgaactcaggttaaatttttttttgtttgatcgggtcgatcccgcaacaagttccatttgcgatatatatctctgtttcgtttgatccctattgtgactaagattagcggatttttgtgaattctggccttaaaatgtgtcttttaagggtggttgagaggtttttcgtcgtaatctctttggtgtgaatgacttgttctcgaaatttcattgagattttagtgtacgacaagtatttgttcggtgattgtaagcgttgaaattttgagttttttcgtcgtagtctcttcggaattagaatgggcagtttgcagttatctgttagggttttcgagaatttgaacatttgatcgcttgaatggtgtcatggaagggaactctttaagttcatcttccttagtttcagccaatcgggtgggtcaatgtgacaatcttgagcatagtagaatgacttgttctcgaaatttcattgagatgttagtgtacgacaagtatttgttcggtgattataccagatgatgaagcataaacgttgaaactttgggttttgtttttgtaggcatttgactgaccagctgagaaaaactcagatagtgaacgagaccaataaggtcagtgggataaaagtctttttcactttagcaactttgtcttggcattactgttctgttttttccttgtggattcgatctttgtttaccgttttgaaggatcttgttgtcgaggcactgagatcaatcgcggagatattgacttatggcgatcagcacgaccctttattctttgagtgagagtctttatgtcaattatcagtcaatgcccttcattttcttattggcatatatgctaataatactttgcgctcgttgcagattttttatggagaagcaagtaatgggagagtttgtacgtattttgagggttagcaagacagtaacagtttccgttcagttgttgcaaaccatgagtattatgatccagaacctaaaaagtgaacaagccatctgtgagttcatcagaagcagtgtatattttgtctttgataattcgtaatgattatagcctattgatgatcttcttttgaaactacttgcagactacttgttcagtaacgaatatgtaaattatttgataacatatacatttgacttccaacatgaagagcttctatcttactacatatccttcctaaggtacattcttctgttgttgacctcggcttcaggaagtacatgttgactgtatctggtaactgttttgttttctttttgtagagctgttagtgggaaactaaaccagcatacaatatcgttgcttttgaagaccgagaacgtgagtattctttaagttgcatcttccttaaacttctataatagtcctttatggattttttttttctgccatattttaattctgcgtttctgcgtctaggatgtagtagtttcttttcccctttacgtcgagggcataaaatttgcatttcatgaagagaacatgatacgcactgcagttcgtgccctgactcttaatgtgtatcatggtaagtcactcagtcctttcgatttgtcactttaatgactcagaagcttttagcaatgtttctgatgcctttagttttttttttcttttcgcagttggcgatgaatctgtgaatgattatgtagttagtccaccgcacactgagtacttttcaaaattagttacatttttccaaaagcaatgcatggatctaagtgcaatggtgttgaacactctaaagtaagattcactgcatcttcatttcccagggcaataatatcgtgttaaatacgtatcatatccccttttcatctattgactcattagttatattcttctgaaagatttccatttactttgtctaaaggagcccatcccgagactcaggtggaaaattgtttgctgccgttgatgggatcgaggacacgctgtactactttagtgatgttatctctgctggcatacctgatatcgggaggctgataacagatcacattctacagcatctaactctcccacttcttctcccgtctttgtgctctgaggctgtaaatgtataacatatctactttttcgatttattttgtccttttgtgctaattttgtaagccttgttagttttttctatgcaagagtacaatttctaatgtcagtatactgtttgttctgtggttatttcaggataaatcagttgatcctgtgacttctctctatctgctctgttgcatcgtgcggatagttaaaatcaaagatttggcgaatttgactgctgctacttttttctgccctgtagaagctttcatttcaagttccctagtgaaacctaatagtagcttggctcctgaacgtcttacatatggaaatgggcatccagacaatggtgttgctgaggaaacagttcaacagtgtccaagcactgcagtctcgagtgaatatggaaattcccacgtttgcagtgaaaatactacgaaaagcatcttcaacaattcacgtattacgtttaggtaacatgttatctaacaacctgagtgaatttgagatagttgctttttacactccttaagctgtcttaatcataatatattcctatatctctccgaagctgatgttccttttgtaaatagggatactttacttcaatatatttctgagggagatgatgtgcaagctcagggttccttgtttgtgctagccacgttgttgcagacaaaaggtattggtagtggctttgtgcatctccttattttatttctagttttgacagggaaattcgcatctcacgcttacattctctttgtggtagaacttgaagagtcaatgctagatgcttttggcattcttcctcagcgtaagcagcacaaaaagcttttgctggtgagtatctgtcattattctttatcttctgctcttttccagcaaattccaaggcagattgccagggaaattcgcatctcatggtttatggaccgtctactatagtctggaccaaaaatataagctttacttcttggatagctaaacttaatttggtggtcatctctgacagcaatctttggttggggaagacactggtgaagaacaactgttttcaccacaaaatggttccatgagagatggcttaagcagcgaacttgattggtatctacggaggttggaggtacttcagtcactgcatatcttagaattttgcaaacacgttctacttctccatctctttggtgttgtgttaaattgtgattgacttactcattcaagtaccctcaacaggagcagtttggagtatgctgttcactgcctggggctgcaatgtgcccgcgtgtacatagacatcaggtaaattacgaatgtttgtaaacctaaattattagcctcgcttcttctgaaaagtgaaaattccatctgcttgagttaggttctttcttcatcacagagcaagttcttgtcttgaatcaatgaaaaaattgtggtataggtggtggatgcattggtcattcttctctgccgtgaaaacatatctgcagaaacattatgggatggagggtggcttttacggcagttgcttccttatagcgaggcagagtttaatcgtaaacatctcaaaatgctgaatgtatgtgtgttgcttttaagatgttgacactgttacactctccctttcgtcattatttaccagtttcctgctgatgtcaggattcatatgagaagtgcacaagtgcactaatccgggaggttaaaggtacctggcctgatctactcatcacggtgctgcttgatgagtggaaaaagtgtaaaagaggcaagtaaagaagcaaaatgtttggattttgattctaaatttacatgttcagtgaatctaataccaaatctcttgtgacagtgatcgaagctccatcccctcaaaaagagcctaaatctgttcttctccagctggataaatcctcttctagtggtagaatttttgttttacaatcaatgtgaatgatatagacactcccttgttcagttcctgctaatgcaaaccgttaacaactgaacttttacaggtaacactgttagcgaatcatcattcacagccggtgaaaaactgtgcgaggtggtgaaggtaagtccattgtgttccctctgtattttcaatcagcgcttgtcgttgatgtgtaaatgctacagaaatctgagaatggagcattttactccttaggtttttgtgcttcttcaccaactccagatcttctcgcttggtaggcccttgccagagcagcctcctatccatcctcctgcagacagatctgaaacgtctcgcgccacaagtgctggtttggatgtttcagtccccaaaactggcaccgaagtgaagctaggttagcacatgatgctctttatgcttgcttagttcaacatctaccaaaccgacaccatgtccgtagttaaactgatgtttgaaatttcccggtgcagttgatgctgtacactgtaggattgcctttgaaagaggcaaggagcggaatttctcgtttctagcattatcatctggtgtgtctgggtggattgtccttgctgaagaatcgctttcgaagccagatcacggaaccgtccgtgttaccgcacctttagccggctgcaaagtacgtgctcacctacattgtctttttttttgtaacgatattgcttgtgaacaccacttacaaggacagatataatcatgatgttggcatagagaaatgagctatcttttgtttggtattcagccccggatagatgaaaagcacccaagatggctacacttgaagatccggccatcgacgttaccattcttggatccaacaaagcgaggagtctatgagaagctcaagtccaaaggtctagtagacgggagatggacattagcattcagagacgaagagtcttgttactctgcttactcaatggttgtacatgagatcgatctacaatgcagcgaggttgaaaggaggttaaagccattgttcgaccttgagagaaaccagcaagatcaatcaaacgttgcttctctatagctcttgggtttgtttttgttttattcattaaattttttgtttcttctttgtaatgttgctataatgtgataatatcgttgtatatttgaaagtgatagtgaatttcagtttttatcacacaaaaatatgactagtgtgagtgtcgagaactctgcttactcttataattctgtgattctgcgtctcttcttgttgaatatgaaaccctaaaacaaatgaacccttactcttctttatgcatcctgtagctgtcaacgagagcagttttgtatgagttacggacactctgtttccagatggagagagaagcaatcaccgtccgtattttgagcaatcctctttttaacgcagctaatggatgcaacattggcttttagacttgtaactatgtctctctctctctctctcttccttcagccgcagtttaaaagacccacatacagtaccacatcatacctcagatgtgaatggtttgtcttcactaaaaggtttgctggaaccaaaacctaaacaggaaacataactccttgacccacagtaaattaaactaccagaatcactctgaaagaagttcctcgaccagaaatatccaaaagccacataaacagggtctggtcagacataacagtggcaacatcgtaataagaaagatgccaagaagttgcagaggctaatgtttgaaaaaaaaagaagccatgagagaccaaaattaagagaatttgtaattaatacagtactcaggaaaagagtttcaaccacttgcgccaacaaactagatagacattgttatccaacacacaaactcatgtccaaccaaaagatagagagataaagagacattatccaacacaacacatgtccaaataaaagagataacagataaaagatagaagagtgggttctccttttcttactacaaacacccatgaattcgattccctactttcggccaagtaccctgaaacacaacacaaaactgaattgttatacaaaactatgt

SEQ ID NO: 75 - DNA, 1026 bp, Thlaspi arvense
atggataactcagctccggattctttgtccagatcggaaaccgccgtcacctacgattctccttacccactctacgccatggccttctcttccatcggtactccctccggccaccgaatcgccgtcggaagcttcctcgaggattacaacaaccgcatcgacattctctccttcgattccgactccatgacggtgaagcctctcccgaatctctccttcgatcatccttatcctcccacaaagctgatgttcagccctccctccctccgtcgtccctccgccggcgatctcctcgcttcctccggcgatttcctccgtttatgggagatcagtgaagattcctccaccgtcgagcctgtctcggtgctcaacaacagcaagacgagcgagttctgcgcgccgttgacctccttcgactggaacgacgtcgagccgaaacgcctgggaacctgcagcatcgacacgacctgcacgatttgggacatcgagaagtgcgtggtggagacgcagctcatagcgcacgataaggaggtccacgacatcgcttggggagaagctagggttttcgcgtcggtctccgccgacggatccgtcaggatcttcgatctacgcgacaaggagcattccaccatcatctacgagagtcctcagcccgatacgcctctcctaagactcgcctggaacaaacaagacctgaggtacatggcgacgatcctgatggattcgaataaggtcgtgattctcgacattcgctcgccgacgatgcctgtcgccgagctcgaacggcaccaggctagcgtcaacgccatagcttgggctccacagagctgcaaacacatctgctctgctggtgacgacacgcaggctctcatctgggagctcccgactgtagctggacccaacggcattgatccgatgtcggtttactcagccggctcggagataaaccagttgcagtggtcctcttcacagcctgattggattggcatcgctttcgctaacaaaatgcagctccttagagtttga

SEQ ID NO: 76 - protein, 341 aa, Thlaspi arvense
MDNSAPDSLSRSETAVTYDSPYPLYAMAFSSIGTPSGHRIAVGSFLEDYNNRIDILSFDSDSMTVKPLPNLSFDHPYPPTKLMFSPPSLRRPSAGDLLASSGDFLRLWEISEDSSTVEPVSVLNNSKTSEFCAPLTSFDWNDVEPKRLGTCSIDTTCTIWDIEKCVVETQLIAHDKEVHDIAWGEARVFASVSADGSVRIFDLRDKEHSTIIYESPQPDTPLLRLAWNKQDLRYMATILMDSNKVVILDIRSPTMPVAELERHQASVNAIAWAPQSCKHICSAGDDTQALIWELPTVAGPNGIDPMSVYSAGSEINQLQWSSSQPDWIGIAFANKMQLLRV

SEQ ID NO: 77 - DNA, 4435 bp, Thlaspi arvense
acacatatctaatactataaaaaaaggtgtatagcgtccgcgaaactcatgtcttccataatcattaatcaaaaaccgatatctctaatcaagatgcatttgacaagaaaaaagaatcaaaatgcattgccaagaaaaaaagaatcaagatgcatgattgtttggtgagtaaacgagacatcttaattttaatataacaattcgttccttgtttttttttttcctgtatcgtacgtgattcatgtgttcaactgttttgttgtcatctcatgtgttagttaaattctatcttattgattttaatacatagatatttcggtgcagcgcaaaaacattattatatttcggtgtagccgcatttagcacaatcatacctaaatattaccaaattgtgctccactatcttacgtgattcatgtgttaaactgttttttctttcctgtggtctaccaaaattaagtttttaattgcaaagacgattgccaattttaattgacgatctaatttgtcacagataacataattatctgatggcgtataagttataagctcttttattttttgaacaaaatatttttgttcttagctgagctgggaaatgtcgtatttaaagtattaaacctataatctcttcggtaatatgttaaataaatctgttttttcaggtcgttagtaaattatttcggctacagacgccatatcaaataatatatcaggttgctgtgaatgagtatctcaatttgcatgctaagaactatataaactgtattaacttttatcttaataccatgagtaagtcgaattatcgatctatctattatttttatttttaaacgtgtggcctgattgataaaataaacttgtggtcatatcaaatctgaaactggagtaaacgtgggattggggatgaagaaattagggcatgtcaacgtcttgggacttaccgtcatgtcccttcactgtaatattggacctatcattttcttccttatcatcttagttttttttgtcgtctcatcctctttaaaataaagtaaaagtaattaacactattatattttctcacaaaattagatattatatgctcttttcaaaaaaatgttaggcatctaacatgatatttttgagatagaaaatgacacaaatactcttcaccccaacctcacgcatatctctatatttattacatcgctattacacacattacacatagtattcatgtacatgtctatttacgcaaaggatcacacgttccacaaaccatttgctaaatcctaaatgagtagtaacaagatattgtccgtctcaaaacaaaatatatatttgtagagaatatcataattttagtatcgtcttcaaaatggtttgaaaatgttattgactttttgtagacaacattttaatctgtgtgtttgggaaagaaatgtggaaagctcgcttagcgttgaaaaggcctactatgtaaagacacaaggcccaaaaatgcgttgaaaggcccactatcaatagatattgattgacacagagggtttagcatgcagtcaaaatatcgcactggacactgaccatagaactttctgtcattttcctctgaaaaacggagatgtcgccgtgaagaatccaaaaatcgaatcgaatcagatcaaaccattccacattttcgtgcagagataatggataactcagctccggattctttgtccagatcggaaaccgccgtcacctacgattctccttacccactctacgccatggccttctcttccatcggtactccctccggccaccgaatcgccgtcggaagcttcctcgaggattacaacaaccgcatcgacattctctccttcgattccgactccatgacggtgaagcctctcccgaatctctccttcgatcatccttatcctcccacaaagctgatgttcagccctccctccctccgtcgtccctccgccggcgatctcctcgcttcctccggcgatttcctccgtttatgggagatcagtgaagattcctccaccgtcgagcctgtctcggtgctcaacaacagcaagacgagcgagttctgcgcgccgttgacctccttcgactggaacgacgtcgagccgaaacgcctgggaacctgcagcatcgacacgacctgcacgatttgggacatcgagaagtgcgtggtggagacgcagctcatagcgcacgataaggaggtccacgacatcgcttggggagaagctagggttttcgcgtcggtctccgccgacggatccgtcaggatcttcgatctacgcgacaaggagcattccaccatcatctacgagagtcctcagcccgatacgcctctcctaagactcgcctggaacaaacaagacctgaggtacatggcgacgatcctgatggattcgaataaggtcgtgattctcgacattcgctcgccgacgatgcctgtcgccgagctcgaacggcaccaggctagcgtcaacgccatagcttgggctccacagagctgcaaacacatctgctctgctggtgacgacacgcaggctctcatctgggagctcccgactgtagctggacccaacggcattgatccgatgtcggtttactcagccggctcggagataaaccagttgcagtggtcctcttcacagcctgattggattggcatcgctttcgctaacaaaatgcagctccttagagtttgaggttaggttttatatttaactatgaagtcgatgatatgaatgatatcacctggttaggcctaatgaattcgcaaagaaagttgaactgaaaactcacttgaatgctttcatggctggctattacagattgtcttgtagctataagagaactttgttagtaaatgatctcacagttgctgtaatggctgataaaatgatattcatgtagacgatgattgggtacaaaacacctttgtactttgtgcttcaggtttttgcaactcatatagagaatctagattgaacaataacattgcacatgtagaaaatcaaataacatttccttattatatacatctcgcttgatgtcagatgcagatggtgaagtggtcaaaatcagatttagcatagacccgatgtgacaagtaggttcggtgcacgcgcactctcgcgtcttgggtcagcaagcaatgcctctgtatctacctgattgtaactaaaactgatttcatttgatgaaccaaatgccactgttatctttctgttttgtgtataaaccccaaccagaatttattgcggtttctggtgtttagatttgaagtggaagcttattacagtataatgcaccctgtctttcctttgttgggtattcttcggataaaacagctacttgtcatcggttatttagcatctaaacaaagcaattataaaatatgtgttacaggttccaacttcgaacacctgtttttagtcagagttttttttttgtattttgcaaattaacttcaagtgacaagcaaattctcaatttattataccttcttcgtttgagaaaacctctgaacgtccgactgttatatttctctatctcattctttacaaagagataaatttatgttaaacttctctatttaccatttttaaaatttcatataaccaatttacataactttggagaacgttgatattcatattttccatttaataaaatgaataaaaatagaaaatttagcttaagggaaaggaaaatatgtgtcagattcttgatttcacaaaaccctacaagcaaccccctctacatataaatagcaacgtccttgtaacttaaaaggcaagtgataataatagtgcaaaaagatttgaaaaaaaaggttagagagaatgtccaccagcgagcttgcctgcacatatgccgctctaatcctccacgatgatgggattgacatcaccgttagttttctcttctctctaattctcaattttaacctctttttgatctagtttctactctttttctttgctcttcatgcatgtacttatatatgttgtagttgcgaatttcgtttatatagtttcatgtcggtaactttcttgtttattgtggatttactaggccgagaagatatcaaagctggtgaaagcagccaacgtgaatgttgaatcatactggcctagcctctttgctaagctatgtgcgaagaagaatattgacgatctcatcatgaatgttggagccagtggtggtggtgaggcagctccggttgcaaccaacgttcctccaactgctcaagcagctccagcagttgaggagacaaagaagaagaaggtatatcctattgtctttctaacagtcttagcgttattgcaatccaaatcatcaactatataatttaacaagcttatgattaaaactaaccaatgggaatattgttttaaaaattctcaggaggaggtgaaggaagagagtgaagatgaca

SEQ ID NO: 78 - DNA, 1275 bp, Thlaspi arvense
atggaggtgaaagagagtgaaagagtggtaatagccaaaccagtggcttcaaggccttcatgctctagcttcaggactttcactgagcttctgactgattcagctactgtgtctcctcaatcgaattgccacgagattgtagacgctgccattagaccaaagactctcaggtttaaccagccagctgcagctgcggtctcatgtccacgggctaaagaaaatggcaatggaaagtcttgtgatgacacagatggcggaaactacgtcgtttacaaacctaaagcaaagcttgtctccaaagcaaccgtctctgtgttggctaacatggggaatcgtcaacagacttggagacaacccgaagcagtagcgtatgggaagagtgtgagtcaaggtactggtcctaatctagtccagagagtttcatcctttacagaaacagagacatcggtcggggacagatcatctgtggacggatacaactggaggaaatacggacagaagcaagttaaaggaagtgagtgtccaagaagctattacaaatgcacacacccgaaatgtccggtgaagaagaaagtagagaggtcattgggaggtcaggtctcagagattgtgtatcaaggtgagcataatcactcgaagccgtcttgtccacttccacggcgcgcttcgtcatcatcctcttcagggtttcagaaaccaccaaaagggcttgtctctgaaggatcaatgggacaagaccctaatagtaatgccttttatcatcatcctctttggagcaatcaaagcaatgactcgtctaagatgtatgagggttgtgttgtaactccattcgagttcgctgttccaagatcggcgaattcaaccggcggaacttcggattccggttgtcgaagtagccagtgtgatgaaggcagcaatggaggagagcttgatgatccaagcagaagcaaaagaagcaggaagaacgagaagcaatcaagtgaagcaggagtatcgcaaggttcggtggaatcagacagtcttgaagatggatttaggtggagaaaatacggacagaaagttgttggaggcaatgcgtatccaagaagttattacagatgcacgagcgcgaattgcagagcaaggaaacacgtcgagagagcgagtgatgatccaagagcttttattacaacctacgaaggtaaacacaatcaccatttgctcttgagacctccaccttcgtctacggttcttcttccctttaactccacacaacattctaatcaagccatttga

SEQ ID NO: 79 - protein, 424 aa, Thlaspi arvense
MEVKESERVVIAKPVASRPSCSSFRTFTELLTDSATVSPQSNCHEIVDAAIRPKTLRFNQPAAAAVSCPRAKENGNGKSCDDTDGGNYVVYKPKAKLVSKATVSVLANMGNRQQTWRQPEAVAYGKSVSQGTGPNLVQRVSSFTETETSVGDRSSVDGYNWRKYGQKQVKGSECPRSYYKCTHPKCPVKKKVERSLGGQVSEIVYQGEHNHSKPSCPLPRRASSSSSSGFQKPPKGLVSEGSMGQDPNSNAFYHHPLWSNQSNDSSKMYEGCVVTPFEFAVPRSANSTGGTSDSGCRSSQCDEGSNGGELDDPSRSKRSRKNEKQSSEAGVSQGSVESDSLEDGFRWRKYGQKVVGGNAYPRSYYRCTSANCRARKHVERASDDPRAFITTYEGKHNHHLLLRPPPSSTVLLPFNSTQHSNQAI

SEQ ID NO: 80 - DNA, 5443 bp, Thlaspi arvense
  misc_feature (887)..(887): n is a, c, g, or t
ttgaatgtgatatatgatattgcggctggccgagctggctggtttaagtactcaaccagacagtaaagtaaaacagccgcatagattgaaatctcgtggaacgtataaccagctcctgtctgtcctagaattggcggttcgggatagaactgttccttacatctcttggaatctccggttgagttgatgctaattgtatcactacttgtgatgtgatctagaaacaaacatagcttatgttttgcgtttgcggtctctgagaaatcgttggggttctatgattcttctggcctgacaattaaaatcattttatggacccaattgaaagactaaaccggacgcagcctattgcaatttaaagaacaataacgagcatgtaggttagaaaccggtttgtagttccacttgagtcgaaactgtactacttgaaaaatttgggttttagacttaaactggtttcaagctccttttatctagggtggagagaacttgttaggaaaaaaaacaaattgttgtaatgcgcggaacggatcgacttatgctctataaaagtctgcggacgcagccaatattaaaggcatgttattataagaaaatgtcttgcggatgcaaaattaaggtaaaataaaacttctgttttaaactgtaactgtgtgtacattgattatgctcaaacaaaccaccttcttaacgaatctttaaggaggtgttattggttcttatattttaatggatttgagaatctaaaccaaattcagtattattggtttttgtattttaaaatttatattgaaatatagtgttattagttttatgattttaaaattcataatgaaatacagtgttattggttctattattttagaatctaaatattataaggattnaagaaaatgtcttgcggatgcaaaattaaggtaaaataaaacttctgttttaaactgtaactgtgtgtacattgattatgctcaaacaaaccaccttcttaacgaatctttaaggaggtgttattggtttttatattttaatggatttgagaatctaaaccaaattcagtattattattttaaaatttatattgaaatatagtgttattagttttatgattttaaaatccataatgaaatacagtgttattgtatctatcattttagaatctaaatattataaggatttgagttttaattgaatttgaatggatttggaaggattttcatgactaaaatataaagatccaaatacaaagtctaattttggtatttaaatagatttgattttttttttattttattgattttgaaatcaataaatttatcaaatccaaaaaagatttataaatctaccaaaatacaagaaccaataacccctagtaagtaatccagcaaactgtttgtataatgtcacctctaatagtagttgaaaattacaaactaataattgtttaactttcataaatgtttctgttaatggataattcataatattttttgtattgtgatactttattatattcatgcgaataataatattttagtttcggttcaatataaacttctgaaattgggacaacagcaacgtgataatattatatatcttcttatttctgacaatggagaggggtgaaatcgagaatgaaccggtttaaatttcggtacggttcagttcactttgtctaaacgagttggtatggttcacgcgtgctttacttctaacaagacaagctcgcgcgcgtgtgtcaacaaccaaccaaagtcactttggccgctggagcctcaaccaaaattcgaaacgacgccgtttctttggccgcgtttccaactaactttcaaaggcctataaaactcaactaacgttcaaccaaaactatctgtctcttctctgtctttcattttcatcgccttctttcatcactatagactagctcatctaaagtacggaccttgatccatccaacgtaccctaccttgacacgtgtcccttgacagtgtgtcggcaagactcaacgaactgaaccgatacgacggatacatcaacgcccaccttaatgaaaaacccgaattcggatcttcctaaagggttttgcctcaaactccttttttgaacttcagattctgcatcatcatctctctcaccgtgagtaacttacttatgtcctctcttttgcgtcacttatggttttacatttgtattcatcttttgggtttttgatttggaatgattcagaacctaatcacaactgtatcggcgcatgtgggtatcatcaagtttcttttttttttttttccggcatcatcaagtttctttctttttgctatagtttgcatcaaactttccaaggctctatatatagatcgagattatgtattgttggatttgatgcttctcaccgtccaaatccaatcttttgttcctctccttttaaaaccttctcgatacttgacttaagactctagaaaatgagctccgattcagaatctgaatctcttataaatttgattgaggctatgtgaagctaatgtgttgatttttaatctgtggaacatttttcaggttgaatcaaagctttttgactggaaacaattttgggtggtaaggttggaacaatggaggtgaaagagagtgaaagagtggtaatagccaaaccagtggcttcaaggccttcatgctctagcttcaggactttcactgagcttctgactgattcagctactgtgtctcctcaatcgaattgccacgagattgtagacgctgccattagaccaaagactctcaggtttaaccagccagctgcagctgcggtctcatgtccacgggtgattcatcttattaatctcttggcaatataatatatcttcttatttctgaatcttctgcattttagcactgactcgtataagtttttctcataatcttaggctaaagaaaatggcaatggaaagtcttgtgatgacacagatggcggaaactacgtcgtttacaaacctaaagcaaagcttgtctccaaagcaaccgtctctgtgttggctaacatggtaagttgtttctagtgctacaaagatcaagaatttctcggaattagtttcttaactctgtttttgttttagcttcaggggaatcgtcaacagacttggagacaacccgaagcagtagcgtatgggaagagtgtgagtcaaggtactggtcctaatctagtccagagagtttcatcctttacagaaacagagacatcggtcggggacagatcatctgtggacggatacaactggaggaaatacggacagaagcaagttaaaggaagtgagtgtccaagaagctattacaaatgcacacacccgaaatgtccggtgaagaagaaagtagagaggtcattgggaggtcaggtctcagagattgtgtatcaaggtgagcataatcactcgaagccgtcttgtccacttccacggcgcgcttcgtcatcatcctcttcagggtttcagaaaccaccaaaagggcttgtctctgaaggatcaatgggacaagaccctaatagtaatgccttttatcatcatcctctttggagcaatcaaagcaatgactcgtctaagatgtatgagggttgtgttgtaactccattcgagttcgctgttccaagatcggcgaattcaaccggcggaacttcggattccggttgtcgaagtagccagtgtgatgaaggcagcaatggaggagagcttgatgatccaagcagaagcaaaagaaggtataatattagagagctttgaatagtttcaaaacaccaatcttcttcgtttactgttacattgacttttatgaataataatatacagcaggaagaacgagaagcaatcaagtgaagcaggagtatcgcaaggttcggtggaatcagacagtcttgaagatggatttaggtggagaaaatacggacagaaagttgttggaggcaatgcgtatccaagaagttattacagatgcacgagcgcgaattgcagagcaaggaaacacgtcgagagagcgagtgatgatccaagagcttttattacaacctacgaaggtaaacacaatcaccatttgctcttgagacctccaccttcgtctacggttcttcttccctttaactccacacaacattctaatcaagccatttgatgaatgatggtatattgatacattacttcttcaatcttcatagcaacattagttcatcattttcttgttgttgcactgtgaatttatttattttacatcaaaattgtaaggagaagcaaaatagttgttatttaacaaacgaaaaaaaaagcaaataaaaagagtgttatattttaggtttaacaacttatgttcccatgttgtagctttcttctgttagtatattgggtttgatctacagtagtggtaaaaagaaactacttttactaatcacaaaaacagtaaatgtaaaacgcaacacacacttaccgcttaataaatcatttgaagcttaaccaccaattagttgaaatacaaacatgaaaggtttggttacaattgatttcatggcaataaacaatttttatttaggaaaatagcagaaaatcggaatatttaatttggagttaagaaccattgaagatggaaaccatatcactttaatgtatcagctttctaattagaaatataaagatgaaatattcttaaatatgaaaccgtttgatcaaagatcccaagtcgataaagcgtcaaaacttgattaaaggtagagaaattttctgaaacatatccaaagctaacgaaaacagcacaaaaaaaatgtctttggagatataatgcaaactcagggcaaaggaagatcccttaacgattggccttggcaacacgctcaatctcatctttcttcttgatagcatagctgcaaagacaagacaaagatgcatctcatcagctactaaagtaacacaaatgtgaagccatttaatagacaagacgatgtagagaatttgttttataaaacctgttggaagatcccttggcagcattgatgagttcatcagcaaggcactcagcgattgtcttgacgtttctaaacgcagcctcacgtgcaccagtggtgatcaagaagattgcttggttcacacgtcttagaggagagatatcaacggcctgcctcctaaccacaccagcagatccaatcctggtagcatcttctctcggaccactgtctcaccaaaaataaacgaacatcatgagaaaagaggttcataacaacacaacaagaaagtgagagggtttcagtatcaccacatgtttgatttacttacctgttaacaatggcatcaatgataacctgaatcgggttctggtcagacaagagatggatgatctccatggcgtgcttgatgatcctgacggccatcagcttcttaccgttgttccttccgtgcatcatgagagagttcgtgagcctctc

SEQ ID NO: 81 - DNA, 404 bp, Thlaspi arvense
caaacacacgctcggacgcatattacacatgttcatacacttaatactcgctgttttgaattgatgttttaggaatatatatgtagctatctgatcggtcagtattttcacaggtcgtgatatgattcaattagcttccgactcattcatccaaataccgagtcgccaaaattcaaactagactcgttaaatgaatgaatgatgcggtagacaaattggatcattgattctctttgataatactcaccgatcagacagctctcttttgtattccaattttcttgattaatctttcctgcacaaaaacatgcttgatccactaagtgacatatatgctgccttcgtatatatagttctggtaaaattaacattttgggtttatctttatttaaggcatcgccatg

SEQ ID NO: 82 - DNA, 404 bp, Thlaspi arvense
caaacacacgctcggacgcatattacacatgttcatacacttaatactcgctgttttgaattgatgttttaggaatatatatgtaggaacgtattacctacacattttcacaggtcgtgatatgattcaattagcttccgactcattcatccaaataccgagtcgccaaaattcaaactagactcgttaaatgaatgaatgatgcggtagacaaattggatcattgattctctttgataatgtgaaggtaatacgctcctctcttttgtattccaattttcttgattaatctttcctgcacaaaaacatgcttgatccactaagtgacatatatgctgccttcgtatatatagttctggtaaaattaacattttgggtttatctttatttaaggcatcgccatg

SEQ ID NO: 83 - DNA, 404 bp, Thlaspi arvense
caaacacacgctcggacgcatattacacatgttcatacacttaatactcgctgttttgaattgatgttttaggaatatatatgtagtcagctccgagttatcaattttcacaggtcgtgatatgattcaattagcttccgactcattcatccaaataccgagtcgccaaaattcaaactagactcgttaaatgaatgaatgatgcggtagacaaattggatcattgattctctttgataattgaaaactcggagccgactctcttttgtattccaattttcttgattaatctttcctgcacaaaaacatgcttgatccactaagtgacatatatgctgccttcgtatatatagttctggtaaaattaacattttgggtttatctttatttaaggcatcgccatg

SEQ ID NO: 84 - DNA, 404 bp, Thlaspi arvense
caaacacacgctcggacgcatattacacatgttcatacacttaatactcgctgttttgaattgatgttttaggaatatatatgtaggaacttgacagtataatcttttcacaggtcgtgatatgattcaattagcttccgactcattcatccaaataccgagtcgccaaaattcaaactagactcgttaaatgaatgaatgatgcggtagacaaattggatcattgattctctttgataagattttactgtcaagctcctctcttttgtattccaattttcttgattaatctttcctgcacaaaaacatgcttgatccactaagtgacatatatgctgccttcgtatatatagttctggtaaaattaacattttgggtttatctttatttaaggcatcgccatg

SEQ ID NO: 85 - DNA, 1998 bp, Thlaspi arvense
ctataaaatataatatttagcaccttgacaggattgtcagttattatattgttagagtgataaagatcatcatcacgtacatataaagagattataagataaaaataattttcggtactgtaggttttctgcaatttaaattatttaaaatatgtaattgagaaaatattcggtcgcctggtttatatagtcaagtgttacgaaaacatgtttgttttgtatgcaatttttgttttacttatttgagacataaatgagttattttataatgggctgttacagatatgtttaattaatataaattattggtttttaacttgttgattttttatttttatttttcaagctttagaaactgatgccacgtggcattgtgggagagagttttttttgcttaggtggatagcctaagaagccccaaataatcctttttatttagtatagattagtcacggcttccacgaaacaagttcaattaaatttaacggaaataaatggtaattaatgaaagtttgaattgtattaattactgcttccacgaaacaaccaaaaaaatcatttgacaaagtaatttgtgtacggtattagccacatggggccaatcctctatgtatatcggagttgttttgccaaatgcccaattcttactctagtaaatattaaaccattttgtagatcctaatcttgagtcaactcaaagtcctatgtttggaaactaaaaataagtttaaatcctctagactacgactaagttgtaaaaagaaatgttcaaaattccttagacattgaaattgaatacttcaattaaagaaaattttaccagcatgttcatagtagtagaccaccacagaacaaaattaatagtttttacattgcattcttatataataattttggagtataattgtaattataaacaaaataactaaaagaaaaggaaagtattcttgacatatttataggtactaatttgctagtacgactattaattatggagattaaatctagtatttgactaaccagaaacattttaaaggtaagtgataagttgataacctcgcaattatttttgaaagctattaatcactttagcagaatgtatacaagttctatattaacaagtttatctcaaaatcttgagatcctactaataaatcataacttttctcttattggtatgtcgaatctagtgtttaccaaactagaggtgttgaccgttagagacaattaaacaacttacatacatacaaaagtacaagccgaagaataatagtaataacagtgcattttctacaataattaaaacaaaaaagtatattaaaaattagcatttattccaattaataccaatattcgaaaattaatatggtagaaaagcaaaaagcttacgtaaattccacagattgtcaaaaccctgcaatgaaaaagttgccaaaaattgacgaggttggtccacaaaatttaaggttctttgcttcacactctatttataggcgaagagatgaaacagaggaaattaattactccttaacaaaggttgttttcactcaaccacatgccttctcaagtgtctgctgctcacattccccgagattctcatttacttactcctctatttggtacgtcctttatattacaattctagtattttttttttcattattcgttttgttcatacttcgtttcataaacatatatagttaatcttatattatacagtaactttgataaatatgtatcttaatttactcacgcagtttagagagacgattgatacgtggggactacttacgtacctgcatgattatataagttataaaagttattgcagaacattaaattactttgatagctcgagagcaatcattatataaagctatatttttaatcacaaatatacatctactcgaaagttttttttttaaaaaaaagatgaaatccctaaacaaacgttcccaaatgttctcatcactctccaaccacgattcaccacattca

SEQ ID NO: 86 - DNA, 1978 bp, Thlaspi arvense
agtaactgagaggaatgtaactgagagaaaaaagaaaagtaataattaaaataattgaaaataataagtaagagcatctagatagtccttaccaaaaaaaagatcatctagatagtctttccatagtatctgatttatataatactaatataatgtatttatataattaaattataaattaataaagagatgaaccaattcttaacagacatttgcctagagacatatctttattcttaacaaacatttggctagaaacatatctaatagtttcttgtttcaaaaatgtcttcgctttttttctgtttttctcccttcctttttccttattttttttatttttcttattcactaaatatactcccataatatctgctatataatattaatataatatatttatataattaaattaaaaattcataaagagatgaaccaattcttaatagatatttggctaaatacatatttaatatttttttgtttgaaagatatctttgctattttttttctgtttctttctcttcttttcttcttatatttcttattttttttattcaataaatatattttaaaaaacaccaattttcttataagaatatctgaaaataattgagaataattaaattaaatattttcttttagtaaaacttataattatatatatgctaaaaagatatgtgatatttattattctatctttaaagatttttttatcgtgaatcactattttcagttatccaacctaaaatgaatactcagagagcaaccacatcgaaagtgttagagattgaatgaatacagttcttaaaaggtttatttcacattaatgaagtctatcaaaacaaaatttatctaattacatctctataacaaaaatgataattctaaagttaaatgaaaaaaaaaaacaaaaaaatagagagaatttttctttaaaaaaaagataagaaagatcaataaaaccgacttcctcacattataaatagaaaagtcttcataatttgaagattcaatccgaaaatccctaaaattctagaaagtaagaccaaatgttcaaagttttctagtttaattttttcaagtgttcttacacacagtttagcaaaacgtgattgttaagctatctttgtaatcactctgagcttttgagtaataatgagatttaattttttaaacacacaaccttatattgctttttttctttgagtgatatcttggttaacaattgacgtcgtctgtagaaaataaagaataaattcttaagcaaaacaaggtttagagatgagctctccgaataagagcaatcaacacactcaaatccctacctttgatgagcacagcaacccccattgtcattggaaatcaaacaccacctccaccactagccacatgaacattgacccttgtctctaccggtgatcttgctgctgcaattcaacccgccctaaaaatcgatcacctaagaccttagttccaaattcgataacttgcaagctcagcaagcaagggatcaggaacaactcaacctcatggcaacctcggccactaaacaagttgcaccacttggacgaagacttgtctttgagacacccaccgtccacatcgtagcaagagccacaacagacacccaagcaaacaagacgaatgtcccagccctaactaatgaagcgttacatgccaaggtgggttatgaagtctcacctgccaaggtgggttagacgaatgtctctctgttagacacctccacttgaccacttgtttgaggatggtaaggagtagcaaccttatgcttaacaccatgcttccttagcagattctcaaaaactttgttgatgaagtggcttcctccatcacttataacacaccttggaacaccaaaccttgggaagatgattatcttgaaaagtttcagcacaaccctagcatcatttgttggactggctatggcttcaacccactttgagacatagtctac

SEQ ID NO: 87 - DNA, 1424 bp, Thlaspi arvense
tgctttgggagttatgatggaaaacctaattctctaactctgtttatatagggaagactcaggaaaaatcctaatatccttttctcttgggcttctgacacatgaacctttccttttcctattgagcctagatccagaacgttacaactagaatcagaatcgaacaacaagcgtatgcgcttaagaaatgatttttactcacactatatgggcgcgcatggcattgtcgtaagaattaaataagcttcgtcccactccttattggatttacgcacacagtcaatccacgtggttgtcataactaaatataattggtgaaaaaactaatttaaagacaaagtaagaagcggaaaccgaaggaaaagccaaacaacattatgtttatcgacaaaaaagccaaaacaacatttaatgttaatttttgtccaaaccaggaatacatcactcatacggtcatatataccataccccaaattgtatgtactacatgtgtacgtaactgatttatgtatatctatctatttctcttttattgtaggggtcaaaatctacctatcgatatttataaataggattttataagacattgttaaaatggaaaacatggtagctacttggccagcgattaacatcaataattaaaaatacgaattgtgaaacatctcactctcttccttttatcacaccaaaccacttctctttctttacttaccggtcaggtcaacaattctaccattccctttatttagtttttttttttcatctatctctcttttcatttttaacttttaaaaaatattagtccgaaaatcgcactcttttatattcgttgatgggcattaaaatattgtaaaaattaaaaaaaatgtgtaaattaaaacgcaatttgtttgcacctgcagcagtagtaacacacaagtcaaagcaatgtctgttttctcttgtatgtcggttagctattttatgtactgaaatatgttattctttctgaccaaaacatattaagaaatttgcattctgtaatttgatttatccaatcagtagaggacacgtaaccaagataattagatatttttattctatctgtatactactaattcatccaacgtctgttggacgaccaaccagtcaaaactcataaaagtcaacttttactacatcgtgaattttttggtcatgcatttatatacacatacatggaagaaaaaacaatactttacctatgtcaaaatgctgcaaaagcattaagatggtatgtatacatacatattgatataacagtggtcccatatatcattttaaatcatcataaagagtatccatcttctttcatattaacatccccttcaaagttataagatttttctctcttcattagagagagagagagagagaattaacacaagttttaatctccgggaaag

SEQ ID NO: 88 - DNA, 1982 bp, Thlaspi arvense
tttaagactctaacaatattgatgccaactctagaaaaggacaactgaacttattttgttttaagccttggctatattacattatcagttttacacttctacgtatacacaactttaatttttctatattactacatgcatactagatgttagaaatatcttatataagcatacatattaaattagttatgcgatatttaaaattaatgtatataaatattcagtttcaaagcttacgaatacgtaaaattaatcaatacaaaccgaaaccaaaaagccacttctcatctcaaaatgttaattacaaatttacaataagccgaatcactatctaaaaagcttttgggatcccgagacccaaaacatttcttcgtataagtgcaacaattatcgagtgtgatgagacacgtaaaaagcaaggatcgggacaacgattttcggctatatagtagtttctcatatctgactttattagcaaattactacataaaattgcttttaagtatgattaacggaacaagtataatgcgtttatttaattacagatctggctaaatgtaatatggtatcaaagctggaaagacaaatagtctaaggtttggaatttttcatctgtctataaaattcttaagacactgatagatcattaacttattttggagtcaccaatggacaaatcaataactattgatgtccaaaacccacaagacaagcctattttttttgcacgtgcaagtacaccggtggaagaattcatttgtatactgaatctgaaattataaaagattagaattggttgaagaatttacttcaaaacaagctagaagatggtgttatttaaataaacaatgttaaattatatcaatgactttcaaattttatcaaaacattttttgaaagagaatcacgcacaaagtatttcgaattacaaaacaattttttgcaataaattttatagttaaagcaaattttgtcaattattgaaaaaaattacttagataaaatatctaatttttttttttaaacaatgtctctataaaagatggattagccaagaaaatctgatggatgctacaacgcagggttggagatatggtgctgacactacatactattaattggttgatagaatcggtaaatatagatatgaatatcgaaatggagacaacaggaaactcaaccgtatggaaggaataaaatagaggaactttaaagagaacttgaggatatacaaacagatgactcacgtatgcaagagaagcttaatgagataacaaataactaaaggatgcgtatcgggatgagaaacaattctggcaacagaagagcagaaacttatggaacaaatgtggagattttaatacataattttataatacttcaacaaagcaacggaggactataaacagaatagtgggactacatgatagtcagggtgtatggataacttaggttgcatggaaactccctccgaggtacgtttctcgcttccgaaacgtttcggaaaccgaaactctcggaagctcgtcggaaacacaaaaatcacgtttcctaaaaattctaatttgtgaatactttggaaacacgtttccattttaaaaacacatgtttccattttggaaagaagataaaaactaattttttttgttttatgaaataaatagataattataaaaattagatttaaatgatcaatttaattatttatagtaaataataattgatttggtaactaaaattaattttgatattattaagtttgaaaattattctttccatgaattagaattagagatagtttggttaatgaaactaataaaattgataataaagaaaatcttctaaatttttgactttacatattttaatttttatagtttaataattatgtaaaaattatatattagattttgttgatttaaatattctacttataacataattagatctttaataattaatatatatatatacacatttcc

SEQ ID NO: 89 - DNA, 24 bp, Thlaspi arvense
attgtatatcatgatccatggcga

SEQ ID NO: 90 - DNA, 24 bp, Thlaspi arvense
aaactcgccatggatcatgatata

SEQ ID NO: 91 - DNA, 24 bp, Thlaspi arvense
attgatctgatggatttggaaggt

SEQ ID NO: 92 - DNA, 24 bp, Thlaspi arvense
aaacaccttccaaatccatcagat

SEQ ID NO: 93 - DNA, 24 bp, Thlaspi arvense
attgttcgtgctgatgaatcttct

SEQ ID NO: 94 - DNA, 24 bp, Thlaspi arvense
aaacagaagattcatcagcacgaa

SEQ ID NO: 95 - DNA, 24 bp, Thlaspi arvense
attgacaacggtgcaataaagacg

SEQ ID NO: 96 - DNA, 24 bp, Thlaspi arvense
aaaccgtctttattgcaccgttgt

SEQ ID NO: 97 - DNA, 24 bp, Thlaspi arvense
attggcatgccctagcttccgatg

SEQ ID NO: 98 - DNA, 24 bp, Thlaspi arvense
aaaccatcggaagctagggcatgc

SEQ ID NO: 99 - DNA, 24 bp, Thlaspi arvense
attgatgcacggcattatcgccgg

SEQ ID NO: 100 - DNA, 24 bp, Thlaspi arvense
aaacccggcgataatgccgtgcat

SEQ ID NO: 101 - DNA, 24 bp, Thlaspi arvense
attgagtttcctggaccagtgtta

SEQ ID NO: 102 - DNA, 24 bp, Thlaspi arvense
aaactaacactggtccaggaaact

SEQ ID NO: 103 - DNA, 24 bp, Thlaspi arvense
attgccatcgaagacgcgactgtt

SEQ ID NO: 104 - DNA, 24 bp, Thlaspi arvense
aaacaacagtcgcgtcttcgatgg

SEQ ID NO: 105 - DNA, 24 bp, Thlaspi arvense
attggttctctgcgatgctcacat

SEQ ID NO: 106 - DNA, 24 bp, Thlaspi arvense
aaacatgtgagcatcgcagagaac

SEQ ID NO: 107 - DNA, 24 bp, Thlaspi arvense
attggaccgatacttgaagaccag

SEQ ID NO: 108 - DNA, 24 bp, Thlaspi arvense
aaacctggtcttcaagtatcggtc

SEQ ID NO: 109 - DNA, 20 bp, Thlaspi arvense
cggaagaggctgcgttagag

SEQ ID NO: 110 - DNA, 20 bp, Thlaspi arvense
gcagctaagggaactttacg

SEQ ID NO: 111 - DNA, 20 bp, Thlaspi arvense
cggaagaggctgcgttagag

SEQ ID NO: 112 - DNA, 20 bp, Thlaspi arvense
caggaaaggcgtatgcgagg

SEQ ID NO: 113 - DNA, 20 bp, Thlaspi arvense
cgccgtcggaagcttcctcg

SEQ ID NO: 114 - DNA, 20 bp, Thlaspi arvense
caaacaagacctgaggtaca

SEQ ID NO: 115 - DNA, 20 bp, Thlaspi arvense
agcattccaccatcatctac

SEQ ID NO: 116 - DNA, 20 bp, Thlaspi arvense
tcgactggaacgacgtcgag

SEQ ID NO: 117 - DNA, 1188 bp, Thlaspi arvense
atggtgatgggtacacaaccgtcgttggaagagatcagaaaggcacagagagcggatggccccgcaggcatcttggggataggcacggccaaccctgcgaaccatgtgatccaggcagagtatccggactactacttccgcatcaccaacagtgagcacatgactgacctcaaggagaagttcaagcgcatgtgcgacaagtcgatgatacggaaacggcacatgcacctgacggaggagttcctgaaggagaatccggacatgtgcgcctacatggctccttctcttgatgtgaggcaggacatcgtggtggtcgaggtccctaagctagggaaagaggcggcagtgaaggccatcaaggagtggggtcagcccaagtccaagatcacccacgtcgtcttctgcactacatccggagttgacatgcctggtgctgactaccagctcaccaagctcctcggtcttcgcccttccgtcaagcgtctcatgatgtaccagcaaggttgctacgccggcggcactgtcctccgactcgccaaggacctcgctgagaataaccgtggtgctcgtgtccttgtcgtctgctccaagatcacagccgtcaccttccgtggcccctctgacacacacctcgactccctcgttggtcaggctctcttcagtgacggtgctgccgcgctcattgttggtgcggaccctgatgcctccgtgggagagaagcctatcttcgagatggtgtctgctgcacagaccatcctcccagactcggacggagccatagatggacacttgagggaagttgggctcaccttccatctcctcaaggacgtccctgggctcatctcgaagaacatagagaagagtctagaagaagcgtttaaaccgctcgggataagtgactggaactctctcttttggatagctcaccctggaggtcctgcgatcctggaccaggttgagttaaagctaggactcaaggaagagaagatgagggccacgcgtcacgtgctgagcgagtacggaaacatgtcgagcgcgtgcgttctcttcattatggacgagatgaggaggaagtccaaggaggatggtgtggccacgacaggagaagggttggagtggggtgtcttgtttggtttcggaccaggtctcaccgtagagacagtcgtcttgcacagcgtccctgtttga

SEQ ID NO: 118 - protein, 395 aa, Thlaspi arvense
MVMGTQPSLEEIRKAQRADGPAGILGIGTANPANHVIQAEYPDYYFRITNSEHMTDLKEKFKRMCDKSMIRKRHMHLTEEFLKENPDMCAYMAPSLDVRQDIVVVEVPKLGKEAAVKAIKEWGQPKSKITHVVFCTTSGVDMPGADYQLTKLLGLRPSVKRLMMYQQGCYAGGTVLRLAKDLAENNRGARVLVVCSKITAVTFRGPSDTHLDSLVGQALFSDGAAALIVGADPDASVGEKPIFEMVSAAQTILPDSDGAIDGHLREVGLTFHLLKDVPGLISKNIEKSLEEAFKPLGISDWNSLFWIAHPGGPAILDQVELKLGLKEEKMRATRHVLSEYGNMSSACVLFIMDEMRRKSKEDGVATTGEGLEWGVLFGFGPGLTVETVVLHSVPV

SEQ ID NO: 119 - DNA, 1188 bp, Thlaspi arvense
atggtgatgggtacacaaccgtcgttggaagagatcagaaaggcacagagagcggatggccccgcaggcatcttggggataggcacggccaaccctgcgaaccatgtgatccaggcagagtatccggactactacttccgcatcaccaacagtgagcacatgactgacctcaaggagaagttcaagcgcatgtgcgacaagtcgatgatacggaaacggcacatgcacctgacggaggagttcctgaaggagaatccggacatgtgcgcctacatggctccttctcttgatgtgaggcaggacatcgtggtggtcgaggtccctaagctagggaaagaggcggcagtgaaggccatcaaggagtggggtcagcccaagtccaagatcacccacgtcgtcttctgcactacatccggagttgacatgcctggtgctgactaccagctcaccaagctcctcggtcttcgcccttccgtcaagcgtctcatgatgtaccagcaaggttgctacgccggcggcactgtcctccgactcgccaaggacctcgctgagaataaccgtggtgctcgtgtccttgtcgtctgctccgagatcacagccgtcaccttccgtggcccctctgacacacacctcgactccctcgttggtcaggctctcttcagtgacggtgctgccgcgctcattgttggtgcggaccctgatgcctccgtgggagagaagcctatcttcgagatggtgtctgctgcacagaccatcctcccagactcggacggagccatagatggacacttgagggaagttgggctcaccttccatctcctcaaggacgtccctgggctcatctcgaagaacatagagaagagtctagaagaagcgtttaaaccgctcgggataagtgactgaaactctctcttttggatagctcaccctggaggtcctgcgatcctggaccaggttgagttaaagctaggactcaaggaagagaagatgagggccacgcgtcacgtgctgagcgagtacggaaacatgtcgagcgcgtgcgttctcttcattatggacgagatgaggaggaagtccaaggaggatggtgtggccacgacaggagaagggttggagtggggtgtcttgtttggtttcggaccaggtctcaccgtagagacagtcgtcttgcacagcgtccctgtttga

SEQ ID NO: 120 - protein, 300 aa, Thlaspi arvense
MVMGTQPSLEEIRKAQRADGPAGILGIGTANPANHVIQAEYPDYYFRITNSEHMTDLKEKFKRMCDKSMIRKRHMHLTEEFLKENPDMCAYMAPSLDVRQDIVVVEVPKLGKEAAVKAIKEWGQPKSKITHVVFCTTSGVDMPGADYQLTKLLGLRPSVKRLMMYQQGCYAGGTVLRLAKDLAENNRGARVLVVCSEITAVTFRGPSDTHLDSLVGQALFSDGAAALIVGADPDASVGEKPIFEMVSAAQTILPDSDGAIDGHLREVGLTFHLLKDVPGLISKNIEKSLEEAFKPLGISD

SEQ ID NO: 121 - DNA, 1239 bp, Thlaspi arvense
atggctccagggactctcaccgagctcgccggagaggctaagctcaactctaaattcgtccgggacgaggacgaacgtcccaaggtggcatacaacaagtttagcgacgatatcccggtgatatctctcgccggactcgacgatgttggtgggaaaagaggagagatctgccgtaagatcgttgaggcttgcgagaattggggcgtgttccaggtggtcgatcatggtgtcgataccaatttggtagaggatatgactcgcctcgctcgcgacttctttgctttaccacccgaagagaaacttagtttcgacatgtctggtggtaagaaaggcggcttcatcgtctctagtcaccttcagggagagactgtgtaagattggagagagatcgtgacgtacttctcgtacccggtgagaaacagagactactcacggtggccagataagccggaagggtgggtgaaagtgacggaggagtacagcgacaaactgatgggtttagcttgtaagcttcttgaggttttgtctgaagctatggggctcgagaaagaagcacttaccaatgcttgcgtcgatatggaccaaaagatagttgttaattattaccctaaatgccctcagcctgatctcaccctcggactcaagcgtcacactgatcctggaaccatcactttgctgctccaagaccaggtcggtggattacaagccacacgcgacgatggcaaaacatggataacggttcagccaattgagggagcttttgtcgtgaatctcggcgaccatggtcactatttgagcaacgggaggttcaagaacgcggatcatcaggcggtggtgaattccaactcgagcaggctatctatagccacgtttcagaatccggcgcaggatgcaaccgtgtatccgcttaaagttagagaaggagagaagccgatcttggaggagccaatcacttttgcagagatgtataagagaaagatgggaaaagatctggagctggctcgcctcaagaagcttgcgaaagaagaaaatgaccagaagctggccaaagaagaacatgacaagaacctggccaaagaagaaaatgatcagaagctggctaaagaagaacatgaccagaagctggccaaagaagaacatgacaagagccttgccaaagaagaaaattaccaaaagctggccaaagatgaacatagccacacggaagctgttaagcgtctcggccaaatcctcgcttag

SEQ ID NO: 122 - protein, 124 aa, Thlaspi arvense
MAPGTLTELAGEAKLNSKFVRDEDERPKVAYNKFSDDIPVISLAGLDDVGGKRGEICRKIVEACENWGVFQVVDHGVDTNLVEDMTRLARDFFALPPEEKLSFDMSGGKKGGFIVSSHLQGETV

SEQ ID NO: 123 - DNA, 1239 bp, Thlaspi arvense
atggctccagggactctcaccgagctcgccggagaggctaagctcaactctaaattcgtccgggacgaggacgaacgtcccaaggtggcatacaacaagtttagcgacgatatcccggtgatatctctcgccggactcgacgatgttggtgggaaaagaggagagatctgccgtaagatcgttgaggcttgcgagaattggggcgtgttccaggtggtcgatcatggtgtcgataccaatttggtagaggatatgactcgcctcgctcgcgacttctttgctttaccacccgaagagaaacttagtttcgacatgtctggtggtaagaaaggcggcttcatcgtctctagtcaccttcagggagagactgtgcaagattggagagagatcgtgacgtacttctcgtacccggtgagaaacagagactactcacggtggccagataagccggaagggtgggtgaaagtgacggaggagtacagcgacaaactgatgggtttagcttgtaagcttcttgaggttttgtctgaagctatggggctcgagaaagaagcacttaccaatgcttgcgtcgatatggaccaaaagatagttgttaattattaccctaaatgccctcagcctgatctcaccctcggactcaagcgtcacactgatcctggaaccatcactttgctgctccaagaccaggtcggtggattacaagccacacgcgacgatggcaaaacatggataacggttcagccaattgagggagcttttgtcgtgaatctcggcgaccatggtcactatttgagcaacgggaggttcaagaacgcggatcatcaggcggtggtgaattccaactcgagcaggctatctatagccacgtttcagaatctggcgcaggatgcaaccgtgtatccgcttaaagttagagaaggagagaagccgatcttggaggagccaatcacttttgcagagatgtataagagaaagatgggaaaagatctggagctggctcgcctcaagaagcttgcgaaagaagaaaatgaccagaagctggccaaagaagaacatgacaagaacctggccaaagaagaaaatgatcagaagctggctaaagaagaacatgaccagaagctggccaaagaagaacatgacaagagccttgccaaagaagaaaattaccaaaagctggccaaagatgaacatagccacacggaagctgttaagcgtctcggccaaatcctcgcttag

SEQ ID NO: 124 - protein, 412 aa, Thlaspi arvense
MAPGTLTELAGEAKLNSKFVRDEDERPKVAYNKFSDDIPVISLAGLDDVGGKRGEICRKIVEACENWGVFQVVDHGVDTNLVEDMTRLARDFFALPPEEKLSFDMSGGKKGGFIVSSHLQGETVQDWREIVTYFSYPVRNRDYSRWPDKPEGWVKVTEEYSDKLMGLACKLLEVLSEAMGLEKEALTNACVDMDQKIVVNYYPKCPQPDLTLGLKRHTDPGTITLLLQDQVGGLQATRDDGKTWITVQPIEGAFVVNLGDHGHYLSNGRFKNADHQAVVNSNSSRLSIATFQNLAQDATVYPLKVREGEKPILEEPITFAEMYKRKMGKDLELARLKKLAKEENDQKLAKEEHDKNLAKEENDQKLAKEEHDQKLAKEEHDKSLAKEENYQKLAKDEHSHTEAVKRLGQILA

SEQ ID NO: 125 - DNA, 1545 bp, Thlaspi arvense
atggccactctcttactcacaatcctcctccccactttcctcttcctcctcgtcctcctcctttctctccgccgcaaccacaaccgcagtagccgtctcccaccaggcccaaaaccatggcccatcctcggaaacctccctcacatgggtcctaaaccccatcgaaccctagccgccatggtaaccacctacggtccaatcctccacctccgattagggttctccaacgtcgtggttgctgcgtctaaatccgtggccgaacagttcttcaaaatccatgatgccaatttcgctagccgaccaccaaattcaagagccaaacacatggcatataactatcaagatcttgtctttgcgccttacggacaacgatggagaatgttgaggaagattagttctgttcatttattttcagctaaagctcttgaagattacaagcatgttcggcaggaagaggtaggaacgctcacgcgcgagctagtggatgcaggcacgaaacccgtaaacttaggccagttggtgaacatgtgtgtggtcaacgcgcttggaagagagatgatcggacggcgtctgttcggcgccggagctgatcacaaagcggaggagtttcgatcgatggtgacggaaatgatggctctcgccggagtattcaacctcggagatttcgtgccggctctggattggttagatttacaaggcgttgctggtaaaatgaaacggctacacaaaagattcgacacttttctatcgtcgattttgaaggagcacgagatgatgcacggtcaagatcaaaagcataaagatatgctcagcactttaatctcgctcaagggaactgattttgacggtgacggcggaagcctaacggatactgagatcaaagccttgctcttgaacatgtttacggctggaactgacacgtcagcaagtacggtggactgggccatagctgaactgatacgacacccggatgcaatgaccagagcccaagaagaacttgattcagttgtaggccgcgataggcccattaacgagtcagacctttctcggcttccttatcttcaggcggttatcaaagagaatttcaggcttcatccgccgacaccactctcgttaccacacatcgcatcagagagctgtgagatcaacggctaccatatcccgaaaggatcgactcttttaacaaacatatgggccatagcccgtgacccggaacaatggtccgacccgttatcgtttcgacccgagagatttttacagggtggagaaaaatccggcgtcgatgtgaaaggaagcgatttcgagcttataccgttcggagccgggaggagaatctgcgctgggctcagtttagggctacggatgattcagttactgacggcgacgctggttcacggatttgattgggaattggccggaggaattccgccggagaagctgaatatggaggagacttatgggattactctgcaaagagcagttcctttggtggtgcatcctaagccaaggttggctcccagtgtttacgaactcgggtcgcgctaa

SEQ ID NO: 126 - protein, 514 aa, Thlaspi arvense
MATLLLTILLPTFLFLLVLLLSLRRNHNRSSRLPPGPKPWPILGNLPHMGPKPHRTLAAMVTTYGPILHLRLGFSNVVVAASKSVAEQFFKIHDANFASRPPNSRAKHMAYNYQDLVFAPYGQRWRMLRKISSVHLFSAKALEDYKHVRQEEVGTLTRELVDAGTKPVNLGQLVNMCVVNALGREMIGRRLFGAGADHKAEEFRSMVTEMMALAGVFNLGDFVPALDWLDLQGVAGKMKRLHKRFDTFLSSILKEHEMMHGQDQKHKDMLSTLISLKGTDFDGDGGSLTDTEIKALLLNMFTAGTDTSASTVDWAIAELIRHPDAMTRAQEELDSVVGRDRPINESDLSRLPYLQAVIKENFRLHPPTPLSLPHIASESCEINGYHIPKGSTLLTNIWAIARDPEQWSDPLSFRPERFLQGGEKSGVDVKGSDFELIPFGAGRRICAGLSLGLRMIQLLTATLVHGFDWELAGGIPPEKLNMEETYGITLQRAVPLVVHPKPRLAPSVYELGSR

SEQ ID NO: 127 - DNA, 1581 bp, Thlaspi arvense
atggatgaatcaagtatttttacggcaaagaaagtgatcggagctgagaaaagagagcttcaagggctgcttaaggcggcggtgcaatctgtggagtggacttatagtctcttctggcaactttgtcctcaacaaagggttttgctgtgggagaatggatactacaacggtgcaataaagacgaggaagacaactcagccggcggaagtgacggcggaagaggctgcgttagagaggagtcagcagctaagggaactttacgaggcccttttggccggagagtcctcatcggaagctagggcatgcacggcattatcgccggaggatctgacggagactgaatggttttatctaatgtgtgtctctttctctttccctcctccttccgggatgccaggaaaggcgtatgcgaggaggaaacacgtatggctatgtggtgcaaatgaggttgacagtaaaatcttttctagggctattctcgcaaagagtgccaaaatccagcagacagtggtttgcattcccatgcttgatggcgttgtggaactaggcacaacgaacaaggtaaaagaagatatagcgtttgttgagctcataaagagttttttccataaccaccccaagtcaaacccaaaagctgctctttctgaacactccatcaacgaagagcacgaagaagacgaagaacaagaagaagaagaagaagaagaagtagaagaagaaatgacaatgtcagaggagataaggcttggctctcctgatgatgatgacgtctccaatcaaaacctactctctgatttccatgtagaatcaacccacactttagacacacacatggacatgatgaatctaatggaggagggtggaaactattctcagacagtatcaacacttcttatgtcacaacccacgagtcttttttcagattcagtttccacatcttcttacatccaatcatcatttgccacatggaaggctgataattttaaagagcatcagcgagtggaaactaaatcgacgtcgtcgtcgcaatggatgctcaaacacataatcttgagagttcctttactccacgaccacactaaagaaaagaggctgcctcgagaagagcttaatcacgtggtggcagagcgccgcaggagagagaagctgaatgagagattcataacactgagatcattggttccctttgtgaccaagatggataaagtctcaattcttggagacaccatcaactacgtaaaccatcttcgaaatagggtccaagagctggagactaatcatcacgaacaaaaacataagcggatgcgtagctgtaagggaaaaacgtgggaagaggtcgttgaggtttccatcatagagagtgatgttttgttagagatgagatgcgagtaccgagatggtctattgctcgacatccttcaggttcttaaggaacatggtatagagactactgcagttcataccgcggtgaacgagcgtgatttcgaggccgagataagggctatggtgagagggaagaaaccaagcattgctgaggtcaaaagagccatccatcaaactatatccaatattaaactatag

SEQ ID NO: 128 - protein, 526 aa, Thlaspi arvense
MDESSIFTAKKVIGAEKRELQGLLKAAVQSVEWTYSLFWQLCPQQRVLLWENGYYNGAIKTRKTTQPAEVTAEEAALERSQQLRELYEALLAGESSSEARACTALSPEDLTETEWFYLMCVSFSFPPPSGMPGKAYARRKHVWLCGANEVDSKIFSRAILAKSAKIQQTVVCIPMLDGVVELGTTNKVKEDIAFVELIKSFFHNHPKSNPKAALSEHSINEEHEEDEEQEEEEEEEVEEEMTMSEEIRLGSPDDDDVSNQNLLSDFHVESTHTLDTHMDMMNLMEEGGNYSQTVSTLLMSQPTSLFSDSVSTSSYIQSSFATWKADNFKEHQRVETKSTSSSQWMLKHIILRVPLLHDHTKEKRLPREELNHVVAERRRREKLNERFITLRSLVPFVTKMDKVSILGDTINYVNHLRNRVQELETNHHEQKHKRMRSCKGKTWEEVVEVSIIESDVLLEMRCEYRDGLLLDILQVLKEHGIETTAVHTAVNERDFEAEIRAMVRGKKPSIAEVKRAIHQTISNIKL

SEQ ID NO: 129 - DNA, 1581 bp, Thlaspi arvense
atggatgaatcaagtatttttacggcagagaaagtgatcggagctgagaaaagagagcttcaagggctgcttaaggcggcggtgcaatctgtggagtggacttatagtctcttctggcaactttgtcctcaacaaagggttttgctgtgggagaatggatactacaacggtgcaataaagacgaggaagacaactcagccggcggaagtgacggcggaagaggctgcgttagagaggagtcagcagctaagggaactttacgaggcccttttggccggagagtcctcatcggaagctagggcatgcacggcattatcgccggaggatctgacggagactgaatggttttatctaatgtgtgtctctttctctttccctcctccttccgggatgccaggaaaggcgtatgcgaggaggaaacacgtatggctatgtggtgcaaatgaggttgacagtaaaatcttttctagggctattctcgcaaagagtgccaaaatccagcagacagtggtttgcattcccatgcttgatggcgttgtggaactaggcacaacgaacaaggtaaaagaagatatagcgtttgttgagctcataaagagttttttccataaccaccccaagtcaaacccaaaagctgctctttctgaacactccatcaacgaagagcacgaagaagacgaagaacaagaagaagaagaagaagaagaagtagaagaagaaatgacaatgtcagaggagataaggcttggctctcctgatgatgatgacgtctccaatcaaaacctactctctgatttccatgtagaatcaacccacactttagacacacacatggacatgatgaatctaatggaggagggtggaaactattctcagacagtatcaacacttcttatgtcacaacccacgagtcttttttcagattcagtttccacatcttcttacatctaatcatcatttgccacatggaaggctgataattttaaagagcatcagcgagtggaaactaaatcgacgtcgtcgtcgcaatggatgctcaaacacataatcttgagagttcctttactccacgaccacactaaagaaaagaggctgcctcgagaagagcttaatcacgtggtggcagagcgccgcaggagagagaagctgaatgagagattcataacactgagatcattggttccctttgtgaccaagatggataaagtctcaattcttggagacaccatcaactacgtaaaccatcttcgaaatagggtccaagagctggagactaatcatcacgaacaaaaacataagcggatgcgtagctgtaagggaaaaacgtgggaagaggtcgttgaggtttccatcatagagagtgatgttttgttagagatgagatgcgagtaccgagatggtctattgctcgacatccttcaggttcttaaggaacatggtatagagactactgcagttcataccgcggtgaacgagcgtgatttcgaggccgagataagggctatggtgagagggaagaaaccaagcattgctgaggtcaaaagagccatccatcaaactatatccaatattaaactatag

SEQ ID NO: 130 - protein, 316 aa, Thlaspi arvense
MDESSIFTAEKVIGAEKRELQGLLKAAVQSVEWTYSLFWQLCPQQRVLLWENGYYNGAIKTRKTTQPAEVTAEEAALERSQQLRELYEALLAGESSSEARACTALSPEDLTETEWFYLMCVSFSFPPPSGMPGKAYARRKHVWLCGANEVDSKIFSRAILAKSAKIQQTVVCIPMLDGVVELGTTNKVKEDIAFVELIKSFFHNHPKSNPKAALSEHSINEEHEEDEEQEEEEEEEVEEEMTMSEEIRLGSPDDDDVSNQNLLSDFHVESTHTLDTHMDMMNLMEEGGNYSQTVSTLLMSQPTSLFSDSVSTSSYI

SEQ ID NO: 131 - DNA, 1581 bp, Thlaspi arvense
atggatgaatcaagtatttttacggcagagaaagtgatcggagctgagaaaagagagcttcaagggctgcttaaggcggcggtgcaatctgtggagtggacttatagtctcttctggcaactttgtcctcaacaaagggttttgctgtgggagaatggatactacaacggtgcaataaagacgaggaagacaactcagccggcggaagtgacggcggaagaggctgcgttagagaggagtcagcagctaagggaactttacgaggcccttttggccggagagtcctcatcggaagctagggcatgcacggcattatcgccggaggatctgacggagactgaatggttttatctaatgtgtgtctctttctctttccctcctccttccgggatgccaggaaaggcgtatgcgaggaggaaacacgtatggctatgtggtgcaaatgaggttgacagtaaaatcttttctagggctattctcgcaaagagtgccaaaatccagcagacagtggtttgcattcccatgcttgatggcgttgtggaactaggcacaacgaacaaggtaaaagaagatatagcgtttgttgagctcataaagagttttttccataaccaccccaagtcaaacccaaaagctgctctttctgaacactccatcaacgaagagcacgaagaagacgaagaacaagaagaagaagaagaagaagaagtagaagaagaaatgacaatgtcagaggagataaggcttggctctcctgatgatgatgacgtctccaatcaaaacctactctctgatttccatgtagaatcaacccacactttagacacacacatggacatgatgaatctaatggaggagggtggaaactattctcagacagtatcaacacttcttatgtcacaacccacgagtcttttttcagattcagtttccacatcttcttacatccaatcatcatttgccacatgaaaggctgataattttaaagagcatcagcgagtggaaactaaatcgacgtcgtcgtcgcaatggatgctcaaacacataatcttgagagttcctttactccacgaccacactaaagaaaagaggctgcctcgagaagagcttaatcacgtggtggcagagcgccgcaggagagagaagctgaatgagagattcataacactgagatcattggttccctttgtgaccaagatggataaagtctcaattcttggagacaccatcaactacgtaaaccatcttcgaaatagggtccaagagctggagactaatcatcacgaacaaaaacataagcggatgcgtagctgtaagggaaaaacgtgggaagaggtcgttgaggtttccatcatagagagtgatgttttgttagagatgagatgcgagtaccgagatggtctattgctcgacatccttcaggttcttaaggaacatggtatagagactactgcagttcataccgcggtgaacgagcgtgatttcgaggccgagataagggctatggtgagagggaagaaaccaagcattgctgaggtcaaaagagccatccatcaaactatatccaatattaaactatag

SEQ ID NO: 132 - protein, 322 aa, Thlaspi arvense
MDESSIFTAEKVIGAEKRELQGLLKAAVQSVEWTYSLFWQLCPQQRVLLWENGYYNGAIKTRKTTQPAEVTAEEAALERSQQLRELYEALLAGESSSEARACTALSPEDLTETEWFYLMCVSFSFPPPSGMPGKAYARRKHVWLCGANEVDSKIFSRAILAKSAKIQQTVVCIPMLDGVVELGTTNKVKEDIAFVELIKSFFHNHPKSNPKAALSEHSINEEHEEDEEQEEEEEEEVEEEMTMSEEIRLGSPDDDDVSNQNLLSDFHVESTHTLDTHMDMMNLMEEGGNYSQTVSTLLMSQPTSLFSDSVSTSSYIQSSFAT

SEQ ID NO: 133 - DNA, 1582 bp, Thlaspi arvense
atggatgaatcaagtatttttacggcagagaaagtgatcggagctgagaaaagagagcttcaagggctgcttaaggcggcggtgcaatctgtggagtggacttatagtctcttctggcaactttgtcctcaacaaagggttttgctgtgggagaatggatactacaacggtgcaataaagaacgaggaagacaactcagccggcggaagtgacggcggaagaggctgcgttagagaggagtcagcagctaagggaactttacgaggcccttttggccggagagtcctcatcggaagctagggcatgcacggcattatcgccggaggatctgacggagactgaatggttttatctaatgtgtgtctctttctctttccctcctccttccgggatgccaggaaaggcgtatgcgaggaggaaacacgtatggctatgtggtgcaaatgaggttgacagtaaaatcttttctagggctattctcgcaaagagtgccaaaatccagcagacagtggtttgcattcccatgcttgatggcgttgtggaactaggcacaacgaacaaggtaaaagaagatatagcgtttgttgagctcataaagagttttttccataaccaccccaagtcaaacccaaaagctgctctttctgaacactccatcaacgaagagcacgaagaagacgaagaacaagaagaagaagaagaagaagaagtagaagaagaaatgacaatgtcagaggagataaggcttggctctcctgatgatgatgacgtctccaatcaaaacctactctctgatttccatgtagaatcaacccacactttagacacacacatggacatgatgaatctaatggaggagggtggaaactattctcagacagtatcaacacttcttatgtcacaacccacgagtcttttttcagattcagtttccacatcttcttacatccaatcatcatttgccacatggaaggctgataattttaaagagcatcagcgagtggaaactaaatcgacgtcgtcgtcgcaatggatgctcaaacacataatcttgagagttcctttactccacgaccacactaaagaaaagaggctgcctcgagaagagcttaatcacgtggtggcagagcgccgcaggagagagaagctgaatgagagattcataacactgagatcattggttccctttgtgaccaagatggataaagtctcaattcttggagacaccatcaactacgtaaaccatcttcgaaatagggtccaagagctggagactaatcatcacgaacaaaaacataagcggatgcgtagctgtaagggaaaaacgtgggaagaggtcgttgaggtttccatcatagagagtgatgttttgttagagatgagatgcgagtaccgagatggtctattgctcgacatccttcaggttcttaaggaacatggtatagagactactgcagttcataccgcggtgaacgagcgtgatttcgaggccgagataagggctatggtgagagggaagaaaccaagcattgctgaggtcaaaagagccatccatcaaactatatccaatattaaactatag

SEQ ID NO: 134 - protein, 99 aa, Thlaspi arvense
MDESSIFTAEKVIGAEKRELQGLLKAAVQSVEWTYSLFWQLCPQQRVLLWENGYYNGAIKNEEDNSAGGSDGGRGCVREESAAKGTLRGPFGRRVLIGS

SEQ ID NO: 135 - DNA, 1579 bp, Thlaspi arvense
atggatgaatcaagtatttttacggcagagaaagtgatcggagctgagaaaagagagcttcaagggctgcttaaggcggcggtgcaatctgtggagtggacttatagtctcttctggcaactttgtcctcaacaaagggttttgctgtgggagaatggatactacaacggtgcaataaacgaggaagacaactcagccggcggaagtgacggcggaagaggctgcgttagagaggagtcagcagctaagggaactttacgaggcccttttggccggagagtcctcatcggaagctagggcatgcacggcattatcgccggaggatctgacggagactgaatggttttatctaatgtgtgtctctttctctttccctcctccttccgggatgccaggaaaggcgtatgcgaggaggaaacacgtatggctatgtggtgcaaatgaggttgacagtaaaatcttttctagggctattctcgcaaagagtgccaaaatccagcagacagtggtttgcattcccatgcttgatggcgttgtggaactaggcacaacgaacaaggtaaaagaagatatagcgtttgttgagctcataaagagttttttccataaccaccccaagtcaaacccaaaagctgctctttctgaacactccatcaacgaagagcacgaagaagacgaagaacaagaagaagaagaagaagaagaagtagaagaagaaatgacaatgtcagaggagataaggcttggctctcctgatgatgatgacgtctccaatcaaaacctactctctgatttccatgtagaatcaacccacactttagacacacacatggacatgatgaatctaatggaggagggtggaaactattctcagacagtatcaacacttcttatgtcacaacccacgagtcttttttcagattcagtttccacatcttcttacatccaatcatcatttgccacatggaaggctgataattttaaagagcatcagcgagtggaaactaaatcgacgtcgtcgtcgcaatggatgctcaaacacataatcttgagagttcctttactccacgaccacactaaagaaaagaggctgcctcgagaagagcttaatcacgtggtggcagagcgccgcaggagagagaagctgaatgagagattcataacactgagatcattggttccctttgtgaccaagatggataaagtctcaattcttggagacaccatcaactacgtaaaccatcttcgaaatagggtccaagagctggagactaatcatcacgaacaaaaacataagcggatgcgtagctgtaagggaaaaacgtgggaagaggtcgttgaggtttccatcatagagagtgatgttttgttagagatgagatgcgagtaccgagatggtctattgctcgacatccttcaggttcttaaggaacatggtatagagactactgcagttcataccgcggtgaacgagcgtgatttcgaggccgagataagggctatggtgagagggaagaaaccaagcattgctgaggtcaaaagagccatccatcaaactatatccaatattaaactatag

SEQ ID NO: 136 - protein, 98 aa, Thlaspi arvense
MDESSIFTAEKVIGAEKRELQGLLKAAVQSVEWTYSLFWQLCPQQRVLLWENGYYNGAINEEDNSAGGSDGGRGCVREESAAKGTLRGPFGRRVLIGS

SEQ ID NO: 137 - DNA, 1582 bp, Thlaspi arvense
atggatgaatcaagtatttttacggcagagaaagtgatcggagctgagaaaagagagcttcaagggctgcttaaggcggcggtgcaatctgtggagtggacttatagtctcttctggcaactttgtcctcaacaaagggttttgctgtgggagaatggatactacaacggtgcaataaaggacgaggaagacaactcagccggcggaagtgacggcggaagaggctgcgttagagaggagtcagcagctaagggaactttacgaggcccttttggccggagagtcctcatcggaagctagggcatgcacggcattatcgccggaggatctgacggagactgaatggttttatctaatgtgtgtctctttctctttccctcctccttccgggatgccaggaaaggcgtatgcgaggaggaaacacgtatggctatgtggtgcaaatgaggttgacagtaaaatcttttctagggctattctcgcaaagagtgccaaaatccagcagacagtggtttgcattcccatgcttgatggcgttgtggaactaggcacaacgaacaaggtaaaagaagatatagcgtttgttgagctcataaagagttttttccataaccaccccaagtcaaacccaaaagctgctctttctgaacactccatcaacgaagagcacgaagaagacgaagaacaagaagaagaagaagaagaagaagtagaagaagaaatgacaatgtcagaggagataaggcttggctctcctgatgatgatgacgtctccaatcaaaacctactctctgatttccatgtagaatcaacccacactttagacacacacatggacatgatgaatctaatggaggagggtggaaactattctcagacagtatcaacacttcttatgtcacaacccacgagtcttttttcagattcagtttccacatcttcttacatccaatcatcatttgccacatggaaggctgataattttaaagagcatcagcgagtggaaactaaatcgacgtcgtcgtcgcaatggatgctcaaacacataatcttgagagttcctttactccacgaccacactaaagaaaagaggctgcctcgagaagagcttaatcacgtggtggcagagcgccgcaggagagagaagctgaatgagagattcataacactgagatcattggttccctttgtgaccaagatggataaagtctcaattcttggagacaccatcaactacgtaaaccatcttcgaaatagggtccaagagctggagactaatcatcacgaacaaaaacataagcggatgcgtagctgtaagggaaaaacgtgggaagaggtcgttgaggtttccatcatagagagtgatgttttgttagagatgagatgcgagtaccgagatggtctattgctcgacatccttcaggttcttaaggaacatggtatagagactactgcagttcataccgcggtgaacgagcgtgatttcgaggccgagataagggctatggtgagagggaagaaaccaagcattgctgaggtcaaaagagccatccatcaaactatatccaatattaaactatag

SEQ ID NO: 138 - protein, 99 aa, Thlaspi arvense; identical to SEQ ID NO: 134

SEQ ID NO: 139 - DNA, 1707 bp, Thlaspi arvense
atgtcacaatattccttcttctatttcttcctaatctctcttttcctctacgaaaattgcattgcgtatcgctacacattcacggttattgaagctccatatagcaaactgtgtagcacgaagaagattttgaccgttaatggtcagtttcctggaccagtgttaagggcttacaaaggtgacaccatttacgttaacgttcgtaaccaagctagtgaaaatatcacattgcattggcatggtgtagagcagccgagaaacccgtggtcagatggacccgaatacatcacacaatgcccgattcaacccgggtcagattttacgtacaaaattttactttccatcgaagacgcgactgtttgatggcatgcgcatagctcgtggacacgtgccaccgtacacggtctgattttcgtgtatcctcggcctcctgataccctgccttttccagaaccggactacgaagtccccttagtttttggagagtggtggaagagggatgtgagagaagtagtggaggatttcatgaggaacggaggtgaacctaatgtgtccgatgctttgactatcaatgggcatcctggtttcttgtatccttgctctcaatcagatacattcaagctcgtggtagagaagggcaaaacctaccgcattcggatggtaaacgccgcgatgaacctaattctcttcttcgccatcgcgaaccacaaactcaccgtggtcgccgccgatggccactacaccaaacctctaaccgctagttatatcaccatatctcctggccaaacgctagacctgttactatacgccgaccaaagtccagagagcacttataacatggcggccagagcttaccatagcaaccccaacgttgggttcaacaactctaccaccgtcgggatcttacgttactactcttcaaacgacgccggaacgtcttcatcagaacgttacccgtaccttcctggctacaatgacacctcagcagctttcgatttcttcacaaaaatcaaaggcttatactccagagtagctcccgccaaagtttcacgtaggataatcacgacggtttcgataaatctcctcaagtgtcccaacgactcgtgtgcaggcccaaacgggtcgaggttagcggcgagtatgaacaacatatcgttcgtcacaccgagccacgtggacatactaagagcttattaccttcacattaacggcgtttacggaacgcggtttccggagttcccaccgcggatattcaatttcacagcggacgaccaaccgctgtttttgcagactccgaggctggcgacggaggtaaagaagtttcagtacggggagacggttgagattgttatacaagggacgagtttggtaggtggtggaatcgatcatcctatgcatctccatggttttagcttctacgtggttggtttagggtttgggaattttaacgcacgtaaagatccctccaactataatctagacgatcctccttacagaaacacggcgactgtgcccaggaacggttggatcgctatcagattcgtagctgacaatccaggggtttggttcatgcactgtcactttgatagacatcaaacgtggggtatgaatgttgtcttcattgttaagaatggaataaaaccaaatcagaagattctacctccaccgcctggcttaccaccttgtgaccaatttgagaatctataa

SEQ ID NO: 140 - protein, 120 aa, Thlaspi arvense
MSQYSFFYFFLISLFLYENCIAYRYTFTVIEAPYSKLCSTKKILTVNGQFPGPVLRAYKGDTIYVNVRNQASENITLHWHGVEQPRNPWSDGPEYITQCPIQPGSDFTYKILLSIEDATV

SEQ ID NO: 141 - DNA, 1707 bp, Thlaspi arvense
atgtcacaatattccttcttctatttcttcctaatctctcttttcctctacgaaaattgcattgcgtatcgctacacattcacggttattgaagctccatatagcaaactgtgtagcacgaagaagattttgaccgttaatggtcagtttcctggaccagtgttaagggcttacaaaggtgacaccatttacgttaacgttcgtaaccaagctagtgaaaatatcacattgcattggcatggtgtagagcagccgagaaacccgtggtcagatggacccgaatacatcacacaatgcccgattcaacccgggtcagattttacgtacaaaattttactttccatcgaagacgcgactgtttggtggcatgcgcatagctcgtggacacgtgccaccgtacacggtctgattttcgtgtatcctcggcctcctgataccctgccttttccagaaccggactacgaagtccccttagtttttggagagtggtggaagagggatgtgagagaagtagtggaggatttcatgaggaacggaggtgaacctaatgtgtccgatgctttgactatcaatgggcatcctggtttcttgtatccttgctctcaatcagatacattcaagctcgtggtagagaagggcaaaacctaccgcatttggatggtaaacgccgcgatgaacctaattctcttcttcgccatcgcgaaccacaaactcaccgtggtcgccgccgatggccactacaccaaacctctaaccgctagttatatcaccatatctcctggccaaacgctagacctgttactatacgccgaccaaagtccagagagcacttataacatggcggccagagcttaccatagcaaccccaacgttgggttcaacaactctaccaccgtcgggatcttacgttactactcttcaaacgacgccggaacgtcttcatcagaacgttacccgtaccttcctggctacaatgacacctcagcagctttcgatttcttcacaaaaatcaaaggcttatactccagagtagctcccgccaaagtttcacgtaggataatcacgacggtttcgataaatctcctcaagtgtcccaacgactcgtgtgcaggcccaaacgggtcgaggttagcggcgagtatgaacaacatatcgttcgtcacaccgagccacgtggacatactaagagcttattaccttcacattaacggcgtttacggaacgcggtttccggagttcccaccgcggatattcaatttcacagcggacgaccaaccgctgtttttgcagactccgaggctggcgacggaggtaaagaagtttcagtacggggagacggttgagattgttatacaagggacgagtttggtaggtggtggaatcgatcatcctatgcatctccatggttttagcttctacgtggttggtttagggtttgggaattttaacgcacgtaaagatccctccaactataatctagacgatcctccttacagaaacacggcgactgtgcccaggaacggttggatcgctatcagattcgtagctgacaatccaggggtttggttcatgcactgtcactttgatagacatcaaacgtggggtatgaatgttgtcttcattgttaagaatggaataaaaccaaatcagaagattctacctccaccgcctggcttaccaccttgtgaccaatttgagaatctataa

SEQ ID NO: 142 - protein, 568 aa, Thlaspi arvense
MSQYSFFYFFLISLFLYENCIAYRYTFTVIEAPYSKLCSTKKILTVNGQFPGPVLRAYKGDTIYVNVRNQASENITLHWHGVEQPRNPWSDGPEYITQCPIQPGSDFTYKILLSIEDATVWWHAHSSWTRATVHGLIFVYPRPPDTLPFPEPDYEVPLVFGEWWKRDVREVVEDFMRNGGEPNVSDALTINGHPGFLYPCSQSDTFKLVVEKGKTYRIWMVNAAMNLILFFAIANHKLTVVAADGHYTKPLTASYITISPGQTLDLLLYADQSPESTYNMAARAYHSNPNVGFNNSTTVGILRYYSSNDAGTSSSERYPYLPGYNDTSAAFDFFTKIKGLYSRVAPAKVSRRIITTVSINLLKCPNDSCAGPNGSRLAASMNNISFVTPSHVDILRAYYLHINGVYGTRFPEFPPRIFNFTADDQPLFLQTPRLATEVKKFQYGETVEIVIQGTSLVGGGIDHPMHLHGFSFYVVGLGFGNFNARKDPSNYNLDDPPYRNTATVPRNGWIAIRFVADNPGVWFMHCHFDRHQTWGMNVVFIVKNGIKPNQKILPPPPGLPPCDQFENL

SEQ ID NO: 143 - DNA, 1708 bp, Thlaspi arvense
atgtcacaatattccttcttctatttcttcctaatctctcttttcctctacgaaaattgcattgcgtatcgctacacattcacggttattgaagctccatatagcaaactgtgtagcacgaagaagattttgaccgttaatggtcagtttcctggaccagtgtttaagggcttacaaaggtgacaccatttacgttaacgttcgtaaccaagctagtgaaaatatcacattgcattggcatggtgtagagcagccgagaaacccgtggtcagatggacccgaatacatcacacaatgcccgattcaacccgggtcagattttacgtacaaaattttactttccatcgaagacgcgactgtttggtggcatgcgcatagctcgtggacacgtgccaccgtacacggtctgattttcgtgtatcctcggcctcctgataccctgccttttccagaaccggactacgaagtccccttagtttttggagagtggtggaagagggatgtgagagaagtagtggaggatttcatgaggaacggaggtgaacctaatgtgtccgatgctttgactatcaatgggcatcctggtttcttgtatccttgctctcaatcagatacattcaagctcgtggtagagaagggcaaaacctaccgcattcggatggtaaacgccgcgatgaacctaattctcttcttcgccatcgcgaaccacaaactcaccgtggtcgccgccgatggccactacaccaaacctctaaccgctagttatatcaccatatctcctggccaaacgctagacctgttactatacgccgaccaaagtccagagagcacttataacatggcggccagagcttaccatagcaaccccaacgttgggttcaacaactctaccaccgtcgggatcttacgttactactcttcaaacgacgccggaacgtcttcatcagaacgttacccgtaccttcctggctacaatgacacctcagcagctttcgatttcttcacaaaaatcaaaggcttatactccagagtagctcccgccaaagtttcacgtaggataatcacgacggtttcgataaatctcctcaagtgtcccaacgactcgtgtgcaggcccaaacgggtcgaggttagcggcgagtatgaacaacatatcgttcgtcacaccgagccacgtggacatactaagagcttattaccttcacattaacggcgtttacggaacgcggtttccggagttcccaccgcggatattcaatttcacagcggacgaccaaccgctgtttttgcagactccgaggctggcgacggaggtaaagaagtttcagtacggggagacggttgagattgttatacaagggacgagtttggtaggtggtggaatcgatcatcctatgcatctccatggttttagcttctacgtggttggtttagggtttgggaattttaacgcacgtaaagatccctccaactataatctagacgatcctccttacagaaacacggcgactgtgcccaggaacggttggatcgctatcagattcgtagctgacaatccaggggtttggttcatgcactgtcactttgatagacatcaaacgtggggtatgaatgttgtcttcattgttaagaatggaataaaaccaaatcagaagattctacctccaccgcctggcttaccaccttgtgaccaatttgagaatctataa

SEQ ID NO: 144 - protein, 60 aa, Thlaspi arvense
MSQYSFFYFFLISLFLYENCIAYRYTFTVIEAPYSKLCSTKKILTVNGQFPGPVFKGLQR

SEQ ID NO: 145 - DNA, 1708 bp, Thlaspi arvense
atgtcacaatattccttcttctatttcttcctaatctctcttttcctctacgaaaattgcattgcgtatcgctacacattcacggttattgaagctccatatagcaaactgtgtagcacgaagaagattttgaccgttaatggtcagtttcctggaccagtgattaagggcttacaaaggtgacaccatttacgttaacgttcgtaaccaagctagtgaaaatatcacattgcattggcatggtgtagagcagccgagaaacccgtggtcagatggacccgaatacatcacacaatgcccgattcaacccgggtcagattttacgtacaaaattttactttccatcgaagacgcgactgtttggtggcatgcgcatagctcgtggacacgtgccaccgtacacggtctgattttcgtgtatcctcggcctcctgataccctgccttttccagaaccggactacgaagtccccttagtttttggagagtggtggaagagggatgtgagagaagtagtggaggatttcatgaggaacggaggtgaacctaatgtgtccgatgctttgactatcaatgggcatcctggtttcttgtatccttgctctcaatcagatacattcaagctcgtggtagagaagggcaaaacctaccgcattcggatggtaaacgccgcgatgaacctaattctcttcttcgccatcgcgaaccacaaactcaccgtggtcgccgccgatggccactacaccaaacctctaaccgctagttatatcaccatatctcctggccaaacgctagacctgttactatacgccgaccaaagtccagagagcacttataacatggcggccagagcttaccatagcaaccccaacgttgggttcaacaactctaccaccgtcgggatcttacgttactactcttcaaacgacgccggaacgtcttcatcagaacgttacccgtaccttcctggctacaatgacacctcagcagctttcgatttcttcacaaaaatcaaaggcttatactccagagtagctcccgccaaagtttcacgtaggataatcacgacggtttcgataaatctcctcaagtgtcccaacgactcgtgtgcaggcccaaacgggtcgaggttagcggcgagtatgaacaacatatcgttcgtcacaccgagccacgtggacatactaagagcttattaccttcacattaacggcgtttacggaacgcggtttccggagttcccaccgcggatattcaatttcacagcggacgaccaaccgctgtttttgcagactccgaggctggcgacggaggtaaagaagtttcagtacggggagacggttgagattgttatacaagggacgagtttggtaggtggtggaatcgatcatcctatgcatctccatggttttagcttctacgtggttggtttagggtttgggaattttaacgcacgtaaagatccctccaactataatctagacgatcctccttacagaaacacggcgactgtgcccaggaacggttggatcgctatcagattcgtagctgacaatccaggggtttggttcatgcactgtcactttgatagacatcaaacgtggggtatgaatgttgtcttcattgttaagaatggaataaaaccaaatcagaagattctacctccaccgcctggcttaccaccttgtgaccaatttgagaatctataa

SEQ ID NO: 146 - protein, 60 aa, Thlaspi arvense; identical to SEQ ID NO: 144

SEQ ID NO: 147 - DNA, 1700 bp, Thlaspi arvense
atgtcacaatattccttcttctatttcttcctaatctctcttttcctctacgaaaattgcattgcgtatcgctacacattcacggttattgaagctccatatagcaaactgtgtagcacgaagaagattttgaccgttaatggtcagtttcctggttaagggcttacaaaggtgacaccatttacgttaacgttcgtaaccaagctagtgaaaatatcacattgcattggcatggtgtagagcagccgagaaacccgtggtcagatggacccgaatacatcacacaatgcccgattcaacccgggtcagattttacgtacaaaattttactttccatcgaagacgcgactgtttggtggcatgcgcatagctcgtggacacgtgccaccgtacacggtctgattttcgtgtatcctcggcctcctgataccctgccttttccagaaccggactacgaagtccccttagtttttggagagtggtggaagagggatgtgagagaagtagtggaggatttcatgaggaacggaggtgaacctaatgtgtccgatgctttgactatcaatgggcatcctggtttcttgtatccttgctctcaatcagatacattcaagctcgtggtagagaagggcaaaacctaccgcattcggatggtaaacgccgcgatgaacctaattctcttcttcgccatcgcgaaccacaaactcaccgtggtcgccgccgatggccactacaccaaacctctaaccgctagttatatcaccatatctcctggccaaacgctagacctgttactatacgccgaccaaagtccagagagcacttataacatggcggccagagcttaccatagcaaccccaacgttgggttcaacaactctaccaccgtcgggatcttacgttactactcttcaaacgacgccggaacgtcttcatcagaacgttacccgtaccttcctggctacaatgacacctcagcagctttcgatttcttcacaaaaatcaaaggcttatactccagagtagctcccgccaaagtttcacgtaggataatcacgacggtttcgataaatctcctcaagtgtcccaacgactcgtgtgcaggcccaaacgggtcgaggttagcggcgagtatgaacaacatatcgttcgtcacaccgagccacgtggacatactaagagcttattaccttcacattaacggcgtttacggaacgcggtttccggagttcccaccgcggatattcaatttcacagcggacgaccaaccgctgtttttgcagactccgaggctggcgacggaggtaaagaagtttcagtacggggagacggttgagattgttatacaagggacgagtttggtaggtggtggaatcgatcatcctatgcatctccatggttttagcttctacgtggttggtttagggtttgggaattttaacgcacgtaaagatccctccaactataatctagacgatcctccttacagaaacacggcgactgtgcccaggaacggttggatcgctatcagattcgtagctgacaatccaggggtttggttcatgcactgtcactttgatagacatcaaacgtggggtatgaatgttgtcttcattgttaagaatggaataaaaccaaatcagaagattctacctccaccgcctggcttaccaccttgtgaccaatttgagaatctataa

SEQ ID NO: 148 - protein, 52 aa, Thlaspi arvense
MSQYSFFYFFLISLFLYENCIAYRYTFTVIEAPYSKLCSTKKILTVNGQFPG

SEQ ID NO: 149 - DNA, 1520 bp, Thlaspi arvense
atgagctccacggagacatatgagcctctattgagacggctccactcagattctcagttaaccgtaggttcttcaccggagatagaggagtttctcggccgtcgtagatccacggtgacgccacggtggtggctaaggctggccgtatgggaatcaaagcttctttggacgctctctggagcctccatagtggtctctgtgctgaattacatgctcagcttcgtcaccgttatgttcatcggccatcttggctctcttcagctcgccggcgcatccatcgccaccgtcggtatccaaggcctcgcttacggtatcatgttgggaatggcgagcgcggtccagacagtgtgtggtcaagcgtacggcgcgaggcagtactcatcaatgggaataatttgccaacgagccatggtcttgcacctcgcagctgcggtcctcctcacgttcctctactggtactcgggtccgatcctaaaggcgatgggccaatccgcagccatcgcacgcgagggtcaggtctttgcacgtgggattattccgcagatttatgcttttgccctcgcttgccctatgcagaggttcctccaggctcaaaaaattgtaaacccttttacatgtcactaggagttttcgtgctacacacgctactaacctggctggtaaccaacgtcctgcatttcggcttgctcggtgcagctctggtgctgagtttttcgtggtggcttctcgcggctgtgaatggtctgtatatcgtgatgagcccgagttgcaaggaaacttggaccgggttctcagctagggctttaagagggatttggccttacttcaagctcacgatagcttcagcagtcatgctatgtttggagatatggtacgtccaagggctagtgattatttccggtttactcaccaatcccacaattgccctagacgcaatttcgatttgcatgtattactggaattgggatatgcagttcatgcttggtctaagtgcggcaatcactgtccgagtgagcaacgagctaggagcgggaaacccacgagtggctaagttatcagtggtagtggttaacatcacgacggttgtcatcagcttattcctctgtgtcgttgtgctcgtgttccgcattggccttagtaaagccttcaccagcgacgcagaggttatagctgcagtctctgatctctttcccctgctcgccgtttccattttcttaaacggaatccaaccaattctctctggtgttgccattggaagtgggtggcaagcagtggtggcttatgtgaatcttgttacttactatgtcattggtcttcctattggctgtgttcttggcttcaaaaccagtcttggagttgcggggatctggtgggggatgattgcaggagttatacttcaaaccctaactttgattgttcttacactcagaactaactggaattccgaggtggagaatgcagctcataggttaaaagcttcagcaaatgagagtcaagaaatggctaccgaaggaatctaa

SEQ ID NO: 150 - protein, 207 aa, Thlaspi arvense
MSSTETYEPLLRRLHSDSQLTVGSSPEIEEFLGRRRSTVTPRWWLRLAVWESKLLWTLSGASIVVSVLNYMLSFVTVMFIGHLGSLQLAGASIATVGIQGLAYGIMLGMASAVQTVCGQAYGARQYSSMGIICQRAMVLHLAAAVLLTFLYWYSGPILKAMGQSAAIAREGQVFARGIIPQIYAFALACPMQRFLQAQKIVNPFTCH

SEQ ID NO: 151 - DNA, 1524 bp, Thlaspi arvense
atgagctccacggagacatatgagcctctattgagacggctccactcagattctcagttaaccgtaggttcttcaccggagatagaggagtttctcggccgtcgtagatccacggtgacgccacggtggtggctaaggctggccgtatgggaatcaaagcttctttggacgctctctggagcctccatagtggtctctgtgctgaattacatgctcagcttcgtcaccgttatgttcatcggccatcttggctctcttcagctcgccggcgcatccatcgccaccgtcggtatccaaggcctcgcttacggtatcatgttgggaatggcgagcgcggtccagacagtgtgtggtcaagcgtacggcgcgaggcagtactcatcaatgggaataatttgccaacgagccatggtcttgcacctcgcagctgcggtcctcctcacgttcctctactggtactcgggtccgatcctaaaggcgatgggccaatccgcagccatcgcacgcgagggtcaggtctttgcacgtgggattattccgcagatttatgcttttgccctcgcttgccctatgcagaggttcctccaggctcaaaaaattgtaaaccctttggcttacatgtcactaggagttttcgtgctacacacgctactaacctggctggtaaccaacgtcctgcatttcggcttgctcggtgcagctctggtgctgagtttttcgtggtggcttctcgcggctgtgaatggtctgtatatcgtgatgagcccgagttgcaaggaaacttggaccgggttctcagctagggctttaagagggatttggccttacttcaagctcacgatagcttcagcagtcatgctatgtttggagatatggtacgtccaagggctagtgattatttccggtttactcaccaatcccacaattgccctagacgcaatttcgatttgcatgtattactggaattgggatatgcagttcatgcttggtctaagtgcggcaatcactgtccgagtgagcaacgagctaggagcgggaaacccacgagtggctaagttatcagtggtagtggttaacatcacgacggttgtcatcagcttattcctctgtgtcgttgtgctcgtgttccgcattggccttagtaaagccttcaccagcgacgcagaggttatagctgcagtctctgatctctttcccctgctcgccgtttccattttcttaaacggaatccaaccaattctctctagtgttgccattggaagtgggtggcaagcagtggtggcttatgtgaatcttgttacttactatgtcattggtcttcctattggctgtgttcttggcttcaaaaccagtcttggagttgcggggatctggtgggggatgattgcaggagttatacttcaaaccctaactttgattgttcttacactcagaactaactggaattccgaggtggagaatgcagctcataggttaaaagcttcagcaaatgagagtcaagaaatggctaccgaaggaatctaa

SEQ ID NO: 152 - protein, 507 aa, Thlaspi arvense
MSSTETYEPLLRRLHSDSQLTVGSSPEIEEFLGRRRSTVTPRWWLRLAVWESKLLWTLSGASIVVSVLNYMLSFVTVMFIGHLGSLQLAGASIATVGIQGLAYGIMLGMASAVQTVCGQAYGARQYSSMGIICQRAMVLHLAAAVLLTFLYWYSGPILKAMGQSAAIAREGQVFARGIIPQIYAFALACPMQRFLQAQKIVNPLAYMSLGVFVLHTLLTWLVTNVLHFGLLGAALVLSFSWWLLAAVNGLYIVMSPSCKETWTGFSARALRGIWPYFKLTIASAVMLCLEIWYVQGLVIISGLLTNPTIALDAISICMYYWNWDMQFMLGLSAAITVRVSNELGAGNPRVAKLSVVVVNITTVVISLFLCVVVLVFRIGLSKAFTSDAEVIAAVSDLFPLLAVSIFLNGIQPILSSVAIGSGWQAVVAYVNLVTYYVIGLPIGCVLGFKTSLGVAGIWWGMIAGVILQTLTLIVLTLRTNWNSEVENAAHRLKASANESQEMATEGI

SEQ ID NO: 153 - DNA, 2214 bp, Thlaspi arvense
atgcttccattaatggcgataccacttgcgacttgcaggagcatcaactggtcagccacggaaaggattcctgtttcgcttctgttccggagtattcttctccaagacgacgaagtttgtagcgctgtgccactataccggatcctcgatcagaatgacgggcaacttggtcctataagtatggccgaggaatcagacaaaccattgctggatcctgatactctcaacagagaaggaattgacttgggtctgttgccattggaggaggtttttgaatacctaagaacatctccacgggggcttttatctggagatgctgaagaaagattgacgatatttggtcctaacagccttgaagagaaacgggagaacaagtttctgaagttcctaggttttatgtggaatcctttgtcatgggttatggaagctgcagcattgatggccatcgccctagcagatagtgaagtagagactatcagtcttttgctataccatttctgctcagtgctgaccggagaatcgctacctgtgaccaagaagaagggtgagcaagtcttctctggctctacttgtaagcaaggtgagatagaagctgttgtgatagccaccggttcgagcactttctttggtaaaacagcatctttggtggacagcacagatgcaactggacattttcagcaggttctaagcttgtgccagcagaaaaatgagattgcgcaaagagtttatgccatcataaatagatttgcagaaaaaggtttgaggtctcttgctgttgcttatcaggaaattccagagagaagcagcaacagtcctggaggaccatggttgttctgtggtctgttgccactgtttgatcctccaaggcatgacagtgctgaaaccatactgagagctcttaactttggagtttgtgttaagatgatcaccggtgatcagttggcgattgcaaaggagacaggaaggcgacttgggatgggaaccaatatgtatccttcttcctctttgttaggccacaacaacgatgatcacgaagccattccattggatgagcttattgaaatggcagatggatttgctggagtgttccctgaacacaagtatgagattgtaaagatattacaagaaaagaagcatgtggttggaatgaccggagatggtgtgaatgatgctcctgctctgaaaaaggctgacattggaatagctgtcgctgatgcaacagatgccgcaagaagttctgctgacattgtactaactgagcctggcttaagtgtaattatcagtgctgtcttgaccagcagagccattttccagcgtatgaagaactatacagtatatgcagtctcgatcaccatacgaatagtgctcggttttacacttttagcgttgatatgggaatacgactttccacctttcatggttttgataatcgcaatactcaatgacgggaccatcatgactatctctaaagatcgagtaaggccatctcctacacccgagagttggaagctcaaccagatatttgcgactggaattgtcattggaacataccttgcattggtcactgtcctattctactggatcattgtctctaccaccttcttcgagaaacacttccatgtaaaatcaatcggcaacaacagtgaacaagtctcatccgctctgtatctccaagtaagcatcatcagtcaagcactcatatttgtaacacgtagtcgaagctggtcttttcttgaacgtcccgggactctcctgattttcgccttccttgttgcccaacttgccgctacattgattgctgtctatgccaacatcagctttgctaacatcaccggcattggatggggatgggcaggtgttatatggttatacagtttgattttttacatacctcttgatattataaagttcttcttccactacgcattgagtggagatgcttggaaccttgtatttgaccgtaagacagcatttactaataagaaagattatagaaaagatgacggagcgtccaatgtaaccatctctcagagaagtcactctgcagaagaactcagtggaagtcgttctcgcgcatcttggatcgctgagcagaccagaaggcgtgcagaaaccgccaggctcttggagggacactcggtgtcaaggcatttggaatcagtaatgaagctcaaacaaattgaccccaagatgattcgtgcagacactgtctaa

SEQ ID NO: 154 - protein, 737 aa, Thlaspi arvense
MLPLMAIPLATCRSINWSATERIPVSLLFRSILLQDDEVCSAVPLYRILDQNDGQLGPISMAEESDKPLLDPDTLNREGIDLGLLPLEEVFEYLRTSPRGLLSGDAEERLTIFGPNSLEEKRENKFLKFLGFMWNPLSWVMEAAALMAIALADSEVETISLLLYHFCSVLTGESLPVTKKKGEQVFSGSTCKQGEIEAVVIATGSSTFFGKTASLVDSTDATGHFQQVLSLCQQKNEIAQRVYAIINRFAEKGLRSLAVAYQEIPERSSNSPGGPWLFCGLLPLFDPPRHDSAETILRALNFGVCVKMITGDQLAIAKETGRRLGMGTNMYPSSSLLGHNNDDHEAIPLDELIEMADGFAGVFPEHKYEIVKILQEKKHVVGMTGDGVNDAPALKKADIGIAVADATDAARSSADIVLTEPGLSVIISAVLTSRAIFQRMKNYTVYAVSITIRIVLGFTLLALIWEYDFPPFMVLIIAILNDGTIMTISKDRVRPSPTPESWKLNQIFATGIVIGTYLALVTVLFYWIIVSTTFFEKHFHVKSIGNNSEQVSSALYLQVSIISQALIFVTRSRSWSFLERPGTLLIFAFLVAQLAATLIAVYANISFANITGIGWGWAGVIWLYSLIFYIPLDIIKFFFHYALSGDAWNLVFDRKTAFTNKKDYRKDDGASNVTISQRSHSAEELSGSRSRASWIAEQTRRRAETARLLEGHSVSRHLESVMKLKQIDPKMIRADTV

SEQ ID NO: 155 - DNA, 2214 bp, Thlaspi arvense
atgcttccattaatggcgataccacttgcgacttgcaggagcatcaactggtcagccacggaaaggattcctgtttcgcttctgttccggagtattcttctccaagacgacgaagtttgtagcgctgtgccactataccggatcctcgatcagaatgacgggcaacttggtcctataagtatggccgaggaatcagacaaaccattgctggatcctgatactctcaacagagaaggaattgacttgggtctgttgccattggaggaggtttttgaatacctaagaacatctccacgggggcttttatctggagatgctgaagaaagattgacgatatttggtcctaacagccttgaagagaaacgggagaacaagtttctgaagttcctaggttttatgtggaatcctttgtcatgggttatggaagctgcagcattgatggccatcgccctagcagatagtgaagtagagactatcagtcttttgctataccatttctgctcagtgctgaccggagaatcgctacctgtgaccaagaagaagggtgagcaagtcttctctggctctacttgtaagcaaggtgagatagaagctgttgtgatagccaccggttcgagcactttctttggtaaaacagcatctttggtggacagcacagatgcaactggacattttcagcaggttctaagcttgtgccagcagaaaaatgagattgcgcaaagagtttatgccatcataaatagatttgcagaaaaaggtttgaggtctcttgctgttgcttatcaggaaattccagagagaagcagcaacagtcctggaggaccatggttgttctgtggtctgttgccactgtttgatcctccaaggcatgacagtgctgaaaccatactgagagctcttaaccttggagtttgtgttaagatgatcaccggtgatcagttggcgattgcaaaggagacaggaaggtgacttgggatgggaaccaatatgtatccttcttcctctttgttaggccacaacaacgatgatcacgaagccattccattggatgagcttattgaaatggcagatggatttgctggagtgttccctgaacacaagtatgagattgtaaagatattacaagaaaagaagcatgtggttggaatgaccggagatggtgtgaatgatgctcctgctctgaaaaaggctgacattggaatagctgtcgctgatgcaacagatgccgcaagaagttctgctgacattgtactaactgagcctggcttaagtgtaattatcagtgctgtcttgaccagcagagccattttccagcgtatgaagaactatacagtatatgcagtctcgatcaccatacgaatagtgctcggttttacacttttagcgttgatatgggaatacgactttccacctttcatggttttgataatcgcaatactcaatgacgggaccatcatgactatctctaaagatcgagtaaggccatctcctacacccgagagttggaagctcaaccagatatttgcgactggaattgtcattggaacataccttgcattggtcactgtcctattctactggatcattgtctctaccaccttcttcgagaaacacttccatgtaaaatcaatcggcaacaacagtgaacaagtctcatccgctctgtatctccaagtaagcatcatcagtcaagcactcatatttgtaacacgtagtcgaagctggtcttttcttgaacgtcccgggactctcctgattttcgccttccttgttgcccaacttgccgctacattgattgctgtctatgccaacatcagctttgctaacatcaccggcattggatggggatgggcaggtgttatatggttatacagtttgattttttacatacctcttgatattataaagttcttcttccactacgcattgagtggagatgcttggaaccttgtatttgaccgtaagacagcatttactaataagaaagattatagaaaagatgacggagcgtccaatgtaaccatctctcagagaagtcactctgcagaagaactcagtggaagtcgttctcgcgcatcttggatcgctgagcagaccagaaggcgtgcagaaaccgccaggctcttggagggacactcggtgtcaaggcatttggaatcagtaatgaagctcaaacaaattgaccccaagatgattcgtgcagacactgtctaa

SEQ ID NO: 156 - protein, 322 aa, Thlaspi arvense
MLPLMAIPLATCRSINWSATERIPVSLLFRSILLQDDEVCSAVPLYRILDQNDGQLGPISMAEESDKPLLDPDTLNREGIDLGLLPLEEVFEYLRTSPRGLLSGDAEERLTIFGPNSLEEKRENKFLKFLGFMWNPLSWVMEAAALMAIALADSEVETISLLLYHFCSVLTGESLPVTKKKGEQVFSGSTCKQGEIEAVVIATGSSTFFGKTASLVDSTDATGHFQQVLSLCQQKNEIAQRVYAIINRFAEKGLRSLAVAYQEIPERSSNSPGGPWLFCGLLPLFDPPRHDSAETILRALNLGVCVKMITGDQLAIAKETGR

SEQ ID NO: 157 - DNA, 2214 bp, Thlaspi arvense
atgcttccattaatggcgataccacttgcgacttgcaggagcatcaactggtcagccacggaaaggattcctgtttcgcttctgttccggagtattcttctccaagacgacgaagtttgtagcgctgtgccactataccggatcctcgatcagaatgacgggcaacttggtcctataagtatggccgaggaatcagacaaaccattgctggatcctgatactctcaacagagaaggaattgacttgggtctgttgccattggaggaggtttttgaatacctaagaacatctccacgggggcttttatctggagatgctgaagaaagattgacgatatttggtcctaacagccttgaagagaaacgggagaacaagtttctgaagttcctaggttttatgtggaatcctttgtcatgggttatggaagctgcagcattgatggccatcgccctagcagatagtgaagtagagactatcagtcttttgctataccatttctgctcagtgctgaccggagaatcgctacctgtgaccaagaagaagggtgagcaagtcttctctggctctacttgtaagcaaggtgagatagaagctgttgtgatagccaccggttcgagcactttctttggtaaaacagcatctttggtggacagcacagatgcaactggacattttcagcaggttctaagcttgtgccagcagaaaaatgagattgcgcaaagagtttatgccatcataaatagatttgcagaaaaaggtttgaggtctcttgctgttgcttatcaggaaattccagagagaagcagcaacagtcctggaggaccatggttgttctgtggtctgttgccactgtttgatcctccaaggcatgacagtgctgaaaccatactgagagctcttaaccttggagtttgtgttaagatgatcaccggtgatcagttggcgattgcaaaggagacaggaaggcgacttgggatgggaaccaatatgtatccttcttcctctttgttaggccacaacaacgatgatcacgaagccattccattggatgagcttattgaaatggcagatggatttgctggagtgttccctgaacacaagtatgagattgtaaagatattacaagaaaagaagcatgtggttggaatgaccagagatggtgtgaatgatgctcctgctctgaaaaaggctgacattggaatagctgtcgctgatgcaacagatgccgcaagaagttctgctgacattgtactaactgagcctggcttaagtgtaattatcagtgctgtcttgaccagcagagccattttccagcgtatgaagaactatacagtatatgcagtctcgatcaccatacgaatagtgctcggttttacacttttagcgttgatatgggaatacgactttccacctttcatggttttgataatcgcaatactcaatgacgggaccatcatgactatctctaaagatcgagtaaggccatctcctacacccgagagttggaagctcaaccagatatttgcgactggaattgtcattggaacataccttgcattggtcactgtcctattctactggatcattgtctctaccaccttcttcgagaaacacttccatgtaaaatcaatcggcaacaacagtgaacaagtctcatccgctctgtatctccaagtaagcatcatcagtcaagcactcatatttgtaacacgtagtcgaagctggtcttttcttgaacgtcccgggactctcctgattttcgccttccttgttgcccaacttgccgctacattgattgctgtctatgccaacatcagctttgctaacatcaccggcattggatggggatgggcaggtgttatatggttatacagtttgattttttacatacctcttgatattataaagttcttcttccactacgcattgagtggagatgcttggaaccttgtatttgaccgtaagacagcatttactaataagaaagattatagaaaagatgacggagcgtccaatgtaaccatctctcagagaagtcactctgcagaagaactcagtggaagtcgttctcgcgcatcttggatcgctgagcagaccagaaggcgtgcagaaaccgccaggctcttggagggacactcggtgtcaaggcatttggaatcagtaatgaagctcaaacaaattgaccccaagatgattcgtgcagacactgtctaa

SEQ ID NO: 158 - protein, 737 aa, Thlaspi arvense
MLPLMAIPLATCRSINWSATERIPVSLLFRSILLQDDEVCSAVPLYRILDQNDGQLGPISMAEESDKPLLDPDTLNREGIDLGLLPLEEVFEYLRTSPRGLLSGDAEERLTIFGPNSLEEKRENKFLKFLGFMWNPLSWVMEAAALMAIALADSEVETISLLLYHFCSVLTGESLPVTKKKGEQVFSGSTCKQGEIEAVVIATGSSTFFGKTASLVDSTDATGHFQQVLSLCQQKNEIAQRVYAIINRFAEKGLRSLAVAYQEIPERSSNSPGGPWLFCGLLPLFDPPRHDSAETILRALNLGVCVKMITGDQLAIAKETGRRLGMGTNMYPSSSLLGHNNDDHEAIPLDELIEMADGFAGVFPEHKYEIVKILQEKKHVVGMTRDGVNDAPALKKADIGIAVADATDAARSSADIVLTEPGLSVIISAVLTSRAIFQRMKNYTVYAVSITIRIVLGFTLLALIWEYDFPPFMVLIIAILNDGTIMTISKDRVRPSPTPESWKLNQIFATGIVIGTYLALVTVLFYWIIVSTTFFEKHFHVKSIGNNSEQVSSALYLQVSIISQALIFVTRSRSWSFLERPGTLLIFAFLVAQLAATLIAVYANISFANITGIGWGWAGVIWLYSLIFYIPLDIIKFFFHYALSGDAWNLVFDRKTAFTNKKDYRKDDGASNVTISQRSHSAEELSGSRSRASWIAEQTRRRAETARLLEGHSVSRHLESVMKLKQIDPKMIRADTV

SEQ ID NO: 159 - DNA, 733 bp, Thlaspi arvense
atgggaagagggaagatagagataaagaagatagagaatcagacagcgaggcaagtgaccttctgcaagaggagaactggtcttatcaagaagactaatgagctctctgttctctgcgatgctcacattggtctcatcgtcttctcctccaccggaaagctctcgcagtactgttccgaacccctcaggatgcctcagctcattgaccgatacttgaagacccagtggaatgcgacttcctgatcctaatgacggccgggaggaattgtaccaagagatggaagtactaaaaagagagacatgtaagcttgagcttcgtctgcgtccataccatggacatgacttaacctcccttcctccacacgagctcgatggtctcgagcaacagctcgaacattctgtccttaaagtccgcgagcgtaagaatgagttgatgcagcaacagttggagaatctaagcagaaagaggcggatgctagaagaagataacaacaatatgtaccgtttgcttcatgagcatcgtaacgcggttgaatttcagcaagctgggatagagacgaaaccaggggagtatcaacagtttctagagcagcttcagtactataatgatcatcagcaacaaccaaacagtgttcttcagcttgctacgcttccttctgagattgatcctaattaccatctccagcttgctcagcctaatcttcaaaacgatccaacggccaagattgattag

SEQ ID NO: 160 - protein, 80 aa, Thlaspi arvense
MGRGKIEIKKIENQTARQVTFCKRRTGLIKKTNELSVLCDAHIGLIVFSSTGKLSQYCSEPLRMPQLIDRYLKTQWNATS

SEQ ID NO: 161 - DNA, 733 bp, Thlaspi arvense
atgggaagagggaagatagagataaagaagatagagaatcagacagcgaggcaagtgaccttctgcaagaggagaactggtcttatcaagaagactaatgagctctctgttctctgcgatgctcacattggtctcatcgtcttctcctccaccggaaagctctcgcagtactgttccgaacccctcaggatgcctcagctcattgaccgatacttgaagacgcagtggaatgcgacttcctgatcctaatgacggccgggaggaattgtaccaagagatggaagtactaaaaagagagacatgtaagcttgagcttcgtctgcgtccataccatggacatgacttaacctcccttcctccacacgagctcgatggtctcgagcaacagctcgaacattctgtccttaaagtccgcgagcgtaagaatgagttgatgcagcaacagttggagaatctaagcagaaagaggcggatgctagaagaagataacaacaatatgtaccgtttgcttcatgagcatcgtaacgcggttgaatttcagcaagctgggatagagacgaaaccaggggagtatcaacagtttctagagcagcttcagtactataatgatcatcagcaacaaccaaacagtgttcttcagcttgctacgcttccttctgagattgatcctaattaccatctccagcttgctcagcctaatcttcaaaacgatccaacggccaagattgattag

SEQ ID NO: 162 - protein, 80 aa, Thlaspi arvense; identical to SEQ ID NO: 160

SEQ ID NO: 163 - DNA, 733 bp, Thlaspi arvense
atgggaagagggaagatagagataaagaagatagagaatcagacagcgaggcaagtgaccttctgcaagaggagaactggtcttatcaagaagactaatgagctctctgttctctgcgatgctcacattggtctcatcgtcttctcctccaccggaaagctctcgcagtactgttccgaacccctcaggatgcctcagctcattgaccgatacttgaagactcagtggaatgcgacttcctgatcctaatgacggccgggaggaattgtaccaagagatggaagtactaaaaagagagacatgtaagcttgagcttcgtctgcgtccataccatggacatgacttaacctcccttcctccacacgagctcgatggtctcgagcaacagctcgaacattctgtccttaaagtccgcgagcgtaagaatgagttgatgcagcaacagttggagaatctaagcagaaagaggcggatgctagaagaagataacaacaatatgtaccgtttgcttcatgagcatcgtaacgcggttgaatttcagcaagctgggatagagacgaaaccaggggagtatcaacagtttctagagcagcttcagtactataatgatcatcagcaacaaccaaacagtgttcttcagcttgctacgcttccttctgagattgatcctaattaccatctccagcttgctcagcctaatcttcaaaacgatccaacggccaagattgattag

SEQ ID NO: 164 - protein, 80 aa, Thlaspi arvense; identical to SEQ ID NO: 160

SEQ ID NO: 165 - DNA, 1005 bp, Thlaspi arvense
atggataactcagctccggattctttgtccagatcggaaaccgccgtcacctacgattctccttacccactctacgccatggccttctcttccatcggtactccctccggccaccgaatcgccgtcggaagcttcctcgaggattacaacaaccgcatcgacattctctccttcgattccgactccatgacggtgaagcctctcccgaatctctccttcgatcatccttatcctcccacaaagctgatgttcagccctccctccctccgtcgtccctccgccggcgatctcctccgtttatgggagatcagtgaagattcctccaccgtcgagcctgtctcggtgctcaacaacagcaagacgagcgagttctgcgcgccgttgacctccttcgactggaacgacgtcgagccgaaacgcctgggaacctgcagcatcgacacgacctgcacgatttgggacatcgagaagtgcgtggtggagacgcagctcatagcgcacgataaggaggtccacgacatcgcttggggagaagctagggttttcgcgtcggtctccgccgacggatccgtcaggatcttcgatctacgcgacaaggagcattccaccatcatctacgagagtcctcagcccgatacgcctctcctaagactcgcctggaacaaacaagacctgaggtacatggcgacgatcctgatggattcgaataaggtcgtgattctcgacattcgctcgccgacgatgcctgtcgccgagctcgaacggcaccaggctagcgtcaacgccatagcttgggctccacagagctgcaaacacatctgctctgctggtgacgacacgcaggctctcatctgggagctcccgactgtagctggacccaacggcattgatccgatgtcggtttactcagccggctcggagataaaccagttgcagtggtcctcttcacagcctgattggattggcatcgctttcgctaacaaaatgcagctccttagagtttga

SEQ ID NO: 166 - protein, 334 aa, Thlaspi arvense
MDNSAPDSLSRSETAVTYDSPYPLYAMAFSSIGTPSGHRIAVGSFLEDYNNRIDILSFDSDSMTVKPLPNLSFDHPYPPTKLMFSPPSLRRPSAGDLLRLWEISEDSSTVEPVSVLNNSKTSEFCAPLTSFDWNDVEPKRLGTCSIDTTCTIWDIEKCVVETQLIAHDKEVHDIAWGEARVFASVSADGSVRIFDLRDKEHSTIIYESPQPDTPLLRLAWNKQDLRYMATILMDSNKVVILDIRSPTMPVAELERHQASVNAIAWAPQSCKHICSAGDDTQALIWELPTVAGPNGIDPMSVYSAGSEINQLQWSSSQPDWIGIAFANKMQLLRV

SEQ ID NO: 167 - DNA, 1026 bp, Thlaspi arvense
atggataactcagctccggattctttgtccagatcggaaaccgccgtcacctacgattctccttacccactctacgccatggccttctcttccatcggtactccctccggccaccgaatcgccgtcggaagcttcctcgaggattacaacaaccgcatcgacattctctccttcgattccgactccatgacggtgaagcctctcccgaatctctccttcgatcatccttatcctcccacaaagctgatgttcagccctccctccctccgtcgtccctccgccggcgatctcctcgcttccttcggcgatttcctccgtttatgggagatcagtgaagattcctccaccgtcgagcctgtctcggtgctcaacaacagcaagacgagcgagttctgcgcgccgttgacctccttcgactggaacgacgtcgagccgaaacgcctgggaacctgcagcatcgacacgacctgcacgatttgggacatcgagaagtgcgtggtggagacgcagctcatagcgcacgataaggaggtccacgacatcgcttggggagaagctagggttttcgcgtcggtctccgccgacggatccgtcaggatcttcgatctacgcgacaaggagcattccaccatcatctacgagagtcctcagcccgatacgcctctcctaagactcgcctggaacaaacaagacctgaggtacatggcgacgatcctgatggattcgaataaggtcgtgattctcgacattcgctcgccgacgatgcctgtcgccgagctcgaacggcaccaggctagcgtcaacgccatagcttgggctccacagagctgcaaacacatctgctctgctggtgacgacacgcaggctctcatctgggagctcccgactgtagctggacccaacggcattgatccgatgtcggtttactcagccggctcggagataaaccagttgcagtggtcctcttcacagcctgattggattggcatcgctttcgctaacaaaatgcagctccttagagtttga

SEQ ID NO: 168 - protein, 341 aa, Thlaspi arvense
MDNSAPDSLSRSETAVTYDSPYPLYAMAFSSIGTPSGHRIAVGSFLEDYNNRIDILSFDSDSMTVKPLPNLSFDHPYPPTKLMFSPPSLRRPSAGDLLASFGDFLRLWEISEDSSTVEPVSVLNNSKTSEFCAPLTSFDWNDVEPKRLGTCSIDTTCTIWDIEKCVVETQLIAHDKEVHDIAWGEARVFASVSADGSVRIFDLRDKEHSTIIYESPQPDTPLLRLAWNKQDLRYMATILMDSNKVVILDIRSPTMPVAELERHQASVNAIAWAPQSCKHICSAGDDTQALIWELPTVAGPNGIDPMSVYSAGSEINQLQWSSSQPDWIGIAFANKMQLLRV

SEQ ID NO: 169 - DNA, 1026 bp, Thlaspi arvense
atggataactcagctccggattctttgtccagatcggaaaccgccgtcacctacgattctccttacccactctacgccatggccttctcttccatcggtactccctccggccaccgaatcgccgtcggaagcttcctcgaggattacaacaaccgcatcgacattctctccttcgattccgactccatgacggtgaagcctctcccgaatctctccttcgatcatccttatcctcccacaaagctgatgttcagccctccctccctccgtcgtccctccgccggcgatctcctcgcttcctccggcgatttcctccgtttatgggagatcagtgaagattcctccaccgtcgagcctgtctcggtgctcaacaacagcaagacgagcgagttctgcgcgccgttgacctccttcgactggaacgacgtcgagccgaaacgcctgggaacctgcagcatcgacacgacctgcacgatttgggacatcgagaagtgcgtggtggagacgcagctcatagcgcacgataaggaggtccacgacatcgcttgggaagaagctagggttttcgcgtcggtctccgccgacggatccgtcaggatcttcgatctacgcgacaaggagcattccaccatcatctacgagagtcctcagcccgatacgcctctcctaagactcgcctggaacaaacaagacctgaggtacatggcgacgatcctgatggattcgaataaggtcgtgattctcgacattcgctcgccgacgatgcctgtcgccgagctcgaacggcaccaggctagcgtcaacgccatagcttgggctccacagagctgcaaacacatctgctctgctggtgacgacacgcaggctctcatctgggagctcccgactgtagctggacccaacggcattgatccgatgtcggtttactcagccggctcggagataaaccagttgcagtggtcctcttcacagcctgattggattggcatcgctttcgctaacaaaatgcagctccttagagtttga

SEQ ID NO: 170 - protein, 341 aa, Thlaspi arvense
MDNSAPDSLSRSETAVTYDSPYPLYAMAFSSIGTPSGHRIAVGSFLEDYNNRIDILSFDSDSMTVKPLPNLSFDHPYPPTKLMFSPPSLRRPSAGDLLASSGDFLRLWEISEDSSTVEPVSVLNNSKTSEFCAPLTSFDWNDVEPKRLGTCSIDTTCTIWDIEKCVVETQLIAHDKEVHDIAWEEARVFASVSADGSVRIFDLRDKEHSTIIYESPQPDTPLLRLAWNKQDLRYMATILMDSNKVVILDIRSPTMPVAELERHQASVNAIAWAPQSCKHICSAGDDTQALIWELPTVAGPNGIDPMSVYSAGSEINQLQWSSSQPDWIGIAFANKMQLLRV

SEQ ID NO: 171 - DNA, 1917 bp, Thlaspi arvense
atgatggatggaatggttactgaacaaaacagaatatctgttccggagaatctgaaaaaacagctcgcagtttcagttcgaagaattcaatggagttacgcaatcttctggtctatttctgcttctcagcctggagtgttagaatggggagatggatactataatggagatatcaaaacgaggaagacgattctagcatcggagatcaaagctgatcagcttggtttacgaaggagcgagcaacttagggagctttacgagtctctttctgtcgctgaatcttcttcctccggcgtcgccgccggatctcaggtcactagacgagcttctgccgccgcactctcgccggaagatctcgccgacacagagtggtactacttggtttgtatgtctttcgtcttcaacatcggtgaaggaatgcctggacgaacgtttgcgaacagtgaaccgatatggttgtgcaacgctcacaccgcagatagtaaagtctttagccgctctcttctggcaaaaagtgcttcggttgtgacagtgatttgcttcccgtttcttggaggagtcgttgagatcggtactacagaacatatcatagaggacatgaatgtaatacaatgcgtgaagacatcattcctcgaagctccagatccatacgcttcactgttaccaacaagatccgattatcacatcgacaacgttctcgatccgcaacagatcctaggtgacgagatttacgcgcctatgtttggtactgagacttttccggcgacttctcctagcagaactaccagcaggttcgatcctgaacacgagcaagtagcagaagatcatgactcgttcatggccgaaggaatcaatggaggagcttctcaggttcaaagctggcagttcatggacgaagagcttagtaactgcgttcaccaatcgcttaattccagtgattgcgtctctcaaacgtttgttaaagcagcggctggacgagtttcttgcaacgcaagaaaaggaagggctcaaaggttagggcatattcaagagcggcagagaaatgtgaaaatgttgtcttttgatccaagaaacgatgacgttcattaccaaagtgtgatctccacaatttttaagaccaaccatcagttaattctcggaccgcagttccggaattgcgataagcggtcaagcttcacgaggtggaagaaattatcgtcatcatcatctggaaccgcgtcaatcgtatcaccgtcacaaggaatgttaaagaagattcttttcgaggttcctcgagtgcaccagaaagagaagttgttgttggattcaccagggatcggggatgaaaccacgaaccacgcggttttagagaagaaacggcgtgagaaattgaacgaacggttcatgatcttgagatcaatcattccatcaatcaataagatcgataaagtatcaattcttgacgatacgatagagtatcttcaagaactggaaagacgtgttcaagaactagaatcttgcagagaatcaaccgatacagaaacacgtgggacaatgacagtgaagaggaagaaatctcacgacgcaggggaaagaacttcagccaactgcacaaacaatgaaaccggaaacgggaagagagttcaggttggagaaaccgagccggcagagaccgattataccggtttaactgataatttaaggatcggttcgtttggtaatgaggtcgttattgagcttagatgtgcttggagagaaggagtattgcttgagataatggatgtcattagtgatctcaacttagattctcattcggtacaatcctcgacaggagatggtttactctgcttaaccgtcaactgcaagcacaagggttcaaaaatgacgacaacaggaatgatcaaagaggcacttcaaaaggttgcatggatctgttga

SEQ ID NO: 172 - protein, 638 aa, Thlaspi arvense
MMDGMVTEQNRISVPENLKKQLAVSVRRIQWSYAIFWSISASQPGVLEWGDGYYNGDIKTRKTILASEIKADQLGLRRSEQLRELYESLSVAESSSSGVAAGSQVTRRASAAALSPEDLADTEWYYLVCMSFVFNIGEGMPGRTFANSEPIWLCNAHTADSKVFSRSLLAKSASVVTVICFPFLGGVVEIGTTEHIIEDMNVIQCVKTSFLEAPDPYASLLPTRSDYHIDNVLDPQQILGDEIYAPMFGTETFPATSPSRTTSRFDPEHEQVAEDHDSFMAEGINGGASQVQSWQFMDEELSNCVHQSLNSSDCVSQTFVKAAAGRVSCNARKGRAQRLGHIQERQRNVKMLSFDPRNDDVHYQSVISTIFKTNHQLILGPQFRNCDKRSSFTRWKKLSSSSSGTASIVSPSQGMLKKILFEVPRVHQKEKLLLDSPGIGDETTNHAVLEKKRREKLNERFMILRSIIPSINKIDKVSILDDTIEYLQELERRVQELESCRESTDTETRGTMTVKRKKSHDAGERTSANCTNNETGNGKRVQVGETEPAETDYTGLTDNLRIGSFGNEVVIELRCAWREGVLLEIMDVISDLNLDSHSVQSSTGDGLLCLTVNCKHKGSKMTTTGMIKEALQKVAWIC

SEQ ID NO: 173 - DNA, 3577 bp, Thlaspi arvense
atgatgtaaagagttgcaggtttttcttttctttttttgtttgctataattttaaccccaaaaaaaaaactcactttttctaaatcaggacaaaaatgaaattgatccttttgttttctttttccattttgtatggtttcatgaaaatttagggatggaatggttactgaacaaaacagaatatctgttccggagaatctgaaaaaacagctcgcagtttcagttcgaagaattcaatggagttacgcaatcttctggtctatttctgcttctcagcctgggtgagtttcttaatcactatccttgaaactgatcagttttgttatttttgaaggttcaaatctctactagggggaaaaaaatgaatttcgaattttcattgctaaagcctttgtctgaagctagaagtgcttttggttctgccttaaaaattattaaaactttgataaaaagattactgatttaatttgggaaattttgatttattctgcttctaagttccatcaatgaagttcttcaactcaagacaatgttctaagtcgatttgagttttaggttgatactgtcttagagattattagaaattttataagtggaaatagtgagaccttattagttacaaaaaaaactcaaaacaaagattaattatggttttttttttcttaaaattcaattttcttttgtcttttttttgtgtgtggataattcgggccggaaaccgattaatctcagagtgtgcaagttcgttgggttcttgaagttcttcattagtttcttactgattcgattcgattttttgttttttattgtttgaaccaaaagagtgttagaatggggagatggatactataatggagatatcaaaacgaggaagacgattctagcatcggagatcaaagctgatcagcttggtttacgaaggagcgagcaacttagggagctttacgagtctctttctgtcgctgaatcttcttcctccggcgtcgccgccggatctcaggtcactagacgagcttctgccgccgcactctcgccggaagatctcgccgacacagagtggtactacttggtttgtatgtctttcgtcttcaacatcggtgaagggtaattgcgtctatttatctttcggcattgacatttactatgtgcgtcgtcatgttcggattgatcttgtcagtgaaataaataaaaaaaagacaaaatacccttttattacatgtatgtctggatattagactttttggtaaaaaactaaaaagttttaactagaaaccaaaaattattattttccacaatcgtttgaaatttcttttttttttcttttttttttggtttggtttggttcagtttagggtttttttggattttcagatttttaggtcctggagaaaagaagtccaagatcggtttggttaagtcaaattttaaaatgatttggataattggtcttggtttggtttttaattaaaaattaatcaaaatgaaaatatataattagatttaatcattattataaattttgtaaatgcttaatgaaatgaatttcgatttattcagttctgttacaccaaatatgcgtttggttttgctttttatgcatggcatttccgtcttttcacgtatctagctattcattcacagaatgcctggacgaacgtttgcgaacagtgaaccgatatggttgtgcaacgctcacaccgcagatagtaaagtctttagccgctctcttctggcaaaagttagttgtattatattgtagttgctatataacatttctttttttgcgactgcaaacgcttaaattaatcgttttttttgtgtgtttgtgtgttttgtgcctgtttagagtgcttcggttgtgacagtgatttgcttcccgtttcttggaggagtcgttgagatcggtactacagaacatgtaaggcaaaatttccattttctgtcacaatttgagaatagttataaaacaaccactagttaagtttataacagtgcgaactaattcatcagaccgacgaattaaggtataaagttatgatacaaaaagtttaaagacttatcttgttgtgtgttttatcccgtagatcatagaggacatgaatgtaatacaatgcgtgaagacatcattcctcgaagctccagatccatacgcttcactgttaccaacaagatccgattatcacatcgacaacgttctcgatccgcaacagatcctaggtgacgagatttacgcgcctatgtttggtactgagacttttccggcgacttctcctagcagaactaccagcaggttcgatcctgaacacgagcaagtagcagaagatcatgactcgttcatggccgaaggaatcaatggaggagcttctcaggttcaaagctggcagttcatggacgaagagcttagtaactgcgttcaccaatcgcttaattccagtgattgcgtctctcaaacgtttgttaaagcagcggctggacgagtttcttgcaacgcaagaaaaggaagggctcaaaggttagggcatattcaagagcggcagagaaatgtgaaaatgttgtcttttgatccaagaaacgatgacgttcattaccaaagtgtgatctccacaatttttaagaccaaccatcagttaattctcggaccgcagttccggaattgcgataagcggtcaagcttcacgaggtggaagaaattatcgtcatcatcatctggaaccgcgtcaatcgtatcaccgtcacaaggaatgttaaagaagattcttttcgaggttcctcgagtgcaccagaaagagaagttgttgttggattcaccagggatcggggatgaaaccacgaaccacgcggttttagagaagaaacggcgtgagaaattgaacgaacggttcatgatcttgagatcaatcattccatcaatcaataaggtatatataaccgaatcttcaaaaattcaaattcatattatgtaaccagagttaactaattctaggtttgacattttcaatagatcgataaagtatcaattcttgacgatacgatagagtatcttcaagaactggaaagacgtgttcaagaactagaatcttgcagagaatcaaccgatacagaaacacgtgggacaatgacagtgaagaggaagaaatctcacgacgcaggggaaagaacttcagccaactgcacaaacaatgaaaccggaaacgggaagagagttcaggttggagaaaccgagccggcagagaccgattataccggtttaactgataatttaaggatcggttcgtttggtaatgaggtcgttattgagcttagatgtgcttggagagaaggagtattgcttgagataatggatgtcattagtgatctcaacttagattctcattcggtacaatcctcgacaggagatggtttactctgcttaaccgtcaactgcaaggtacagcctttaacctaatttttgcttaaccgggataaggttaacatggattgatatattgtgaaatgttggtttcagcacaagggttcaaaaatgacgacaacaggaatgatcaaagaggcacttcaaaaggttgcatggatctgttga

SEQ ID NO: 174 - DNA, 1917 bp, Thlaspi arvense
atgatggatggaatggttactgaacaaaacagaatatctgttccggagaatctgaaaaaacagctcgcagtttcagttcgaagaattcaatggagttacgcaatcttctggtctatttctgcttctcagcctggagtgttagaatggggagatggatactataatggagatatcaaaacgaggaagacgattctagcatcggagatcaaagctgatcagcttggtttacgaaggagcgagcaacttaggaagctttacgagtctctttctgtcgctgaatcttcttcctccggcgtcgccgccggatctcaggtcactagacgagcttctgccgccgcactctcgccggaagatctcgccgacacagagtggtactacttggtttgtatgtctttcgtcttcaacatcggtgaaggaatgcctggacgaacgtttgcgaacagtgaaccgatatggttgtgcaacgctcacaccgcagatagtaaagtctttagccgctctcttctggcaaaaagtgcttcggttgtgacagtgatttgcttcccgtttcttggaggagtcgttgagatcggtactacagaacatatcatagaggacatgaatgtaatacaatgcgtgaagacatcattcctcgaagctccagatccatacgcttcactgttaccaacaagatccgattatcacatcgacaacgttctcgatccgcaacagatcctaggtgacgagatttacgcgcctatgtttggtactgagacttttccggcgacttctcctagcagaactaccagcaggttcgatcctgaacacgagcaagtagcagaagatcatgactcgttcatggccgaaggaatcaatggaggagcttctcaggttcaaagctggcagttcatggacgaagagcttagtaactgcgttcaccaatcgcttaattccagtgattgcgtctctcaaacgtttgttaaagcagcggctggacgagtttcttgcaacgcaagaaaaggaagggctcaaaggttagggcatattcaagagcggcagagaaatgtgaaaatgttgtcttttgatccaagaaacgatgacgttcattaccaaagtgtgatctccacaatttttaagaccaaccatcagttaattctcggaccgcagttccggaattgcgataagcggtcaagcttcacgaggtggaagaaattatcgtcatcatcatctggaaccgcgtcaatcgtatcaccgtcacaaggaatgttaaagaagattcttttcgaggttcctcgagtgcaccagaaagagaagttgttgttggattcaccagggatcggggatgaaaccacgaaccacgcggttttagagaagaaacggcgtgagaaattgaacgaacggttcatgatcttgagatcaatcattccatcaatcaataagatcgataaagtatcaattcttgacgatacgatagagtatcttcaagaactggaaagacgtgttcaagaactagaatcttgcagagaatcaaccgatacagaaacacgtgggacaatgacagtgaagaggaagaaatctcacgacgcaggggaaagaacttcagccaactgcacaaacaatgaaaccggaaacgggaagagagttcaggttggagaaaccgagccggcagagaccgattataccggtttaactgataatttaaggatcggttcgtttggtaatgaggtcgttattgagcttagatgtgcttggagagaaggagtattgcttgagataatggatgtcattagtgatctcaacttagattctcattcggtacaatcctcgacaggagatggtttactctgcttaaccgtcaactgcaagcacaagggttcaaaaatgacgacaacaggaatgatcaaagaggcacttcaaaaggttgcatggatctgttga

SEQ ID NO: 175 - protein, 638 aa, Thlaspi arvense
MMDGMVTEQNRISVPENLKKQLAVSVRRIQWSYAIFWSISASQPGVLEWGDGYYNGDIKTRKTILASEIKADQLGLRRSEQLRKLYESLSVAESSSSGVAAGSQVTRRASAAALSPEDLADTEWYYLVCMSFVFNIGEGMPGRTFANSEPIWLCNAHTADSKVFSRSLLAKSASVVTVICFPFLGGVVEIGTTEHIIEDMNVIQCVKTSFLEAPDPYASLLPTRSDYHIDNVLDPQQILGDEIYAPMFGTETFPATSPSRTTSRFDPEHEQVAEDHDSFMAEGINGGASQVQSWQFMDEELSNCVHQSLNSSDCVSQTFVKAAAGRVSCNARKGRAQRLGHIQERQRNVKMLSFDPRNDDVHYQSVISTIFKTNHQLILGPQFRNCDKRSSFTRWKKLSSSSSGTASIVSPSQGMLKKILFEVPRVHQKEKLLLDSPGIGDETTNHAVLEKKRREKLNERFMILRSIIPSINKIDKVSILDDTIEYLQELERRVQELESCRESTDTETRGTMTVKRKKSHDAGERTSANCTNNETGNGKRVQVGETEPAETDYTGLTDNLRIGSFGNEVVIELRCAWREGVLLEIMDVISDLNLDSHSVQSSTGDGLLCLTVNCKHKGSKMTTTGMIKEALQKVAWIC

SEQ ID NO: 176 - DNA, 1917 bp, Thlaspi arvense
atgatggatggaatggttactgaacaaaacagaatatctgttccggagaatctgaaaaaacagctcgcagtttcagttcgaagaattcaatggagttacgcaatcttctggtctatttctgcttctcagcctggagtgttagaatggggagatggatactataatggagatatcaaaacgaggaagacgattctagcatcggagatcaaagctgatcagcttggtttacgaaggagcgagcaacttagggagctttacgagtctctttctgtcgctgaatcttcttcctccggcgtcgccgccggatctcaggtcactagacgagcttctgccgccgcactctcgccggaagatctcgccgacacaaagtggtactacttggtttgtatgtctttcgtcttcaacatcggtgaaggaatgcctggacgaacgtttgcgaacagtgaaccgatatggttgtgcaacgctcacaccgcagatagtaaagtctttagccgctctcttctggcaaaaagtgcttcggttgtgacagtgatttgcttcccgtttcttggaggagtcgttgagatcggtactacagaacatatcatagaggacatgaatgtaatacaatgcgtgaagacatcattcctcgaagctccagatccatacgcttcactgttaccaacaagatccgattatcacatcgacaacgttctcgatccgcaacagatcctaggtgacgagatttacgcgcctatgtttggtactgagacttttccggcgacttctcctagcagaactaccagcaggttcgatcctgaacacgagcaagtagcagaagatcatgactcgttcatggccgaaggaatcaatggaggagcttctcaggttcaaagctggcagttcatggacgaagagcttagtaactgcgttcaccaatcgcttaattccagtgattgcgtctctcaaacgtttgttaaagcagcggctggacgagtttcttgcaacgcaagaaaaggaagggctcaaaggttagggcatattcaagagcggcagagaaatgtgaaaatgttgtcttttgatccaagaaacgatgacgttcattaccaaagtgtgatctccacaatttttaagaccaaccatcagttaattctcggaccgcagttccggaattgcgataagcggtcaagcttcacgaggtggaagaaattatcgtcatcatcatctggaaccgcgtcaatcgtatcaccgtcacaaggaatgttaaagaagattcttttcgaggttcctcgagtgcaccagaaagagaagttgttgttggattcaccagggatcggggatgaaaccacgaaccacgcggttttagagaagaaacggcgtgagaaattgaacgaacggttcatgatcttgagatcaatcattccatcaatcaataagatcgataaagtatcaattcttgacgatacgatagagtatcttcaagaactggaaagacgtgttcaagaactagaatcttgcagagaatcaaccgatacagaaacacgtgggacaatgacagtgaagaggaagaaatctcacgacgcaggggaaagaacttcagccaactgcacaaacaatgaaaccggaaacgggaagagagttcaggttggagaaaccgagccggcagagaccgattataccggtttaactgataatttaaggatcggttcgtttggtaatgaggtcgttattgagcttagatgtgcttggagagaaggagtattgcttgagataatggatgtcattagtgatctcaacttagattctcattcggtacaatcctcgacaggagatggtttactctgcttaaccgtcaactgcaagcacaagggttcaaaaatgacgacaacaggaatgatcaaagaggcacttcaaaaggttgcatggatctgttga

SEQ ID NO: 177 - protein, 638 aa, Thlaspi arvense
MMDGMVTEQNRISVPENLKKQLAVSVRRIQWSYAIFWSISASQPGVLEWGDGYYNGDIKTRKTILASEIKADQLGLRRSEQLRELYESLSVAESSSSGVAAGSQVTRRASAAALSPEDLADTKWYYLVCMSFVFNIGEGMPGRTFANSEPIWLCNAHTADSKVFSRSLLAKSASVVTVICFPFLGGVVEIGTTEHIIEDMNVIQCVKTSFLEAPDPYASLLPTRSDYHIDNVLDPQQILGDEIYAPMFGTETFPATSPSRTTSRFDPEHEQVAEDHDSFMAEGINGGASQVQSWQFMDEELSNCVHQSLNSSDCVSQTFVKAAAGRVSCNARKGRAQRLGHIQERQRNVKMLSFDPRNDDVHYQSVISTIFKTNHQLILGPQFRNCDKRSSFTRWKKLSSSSSGTASIVSPSQGMLKKILFEVPRVHQKEKLLLDSPGIGDETTNHAVLEKKRREKLNERFMILRSIIPSINKIDKVSILDDTIEYLQELERRVQELESCRESTDTETRGTMTVKRKKSHDAGERTSANCTNNETGNGKRVQVGETEPAETDYTGLTDNLRIGSFGNEVVIELRCAWREGVLLEIMDVISDLNLDSHSVQSSTGDGLLCLTVNCKHKGSKMTTTGMIKEALQKVAWIC

SEQ ID NO: 178 - DNA, 1917 bp, Thlaspi arvense
atgatggatggaatggttactgaacaaaacagaatatctgttccggagaatctgaaaaaacagctcgcagtttcagttcgaagaattcaatggagttacgcaatcttctggtctatttctgcttctcagcctggagtgttagaatggggagatggatactataatggagatatcaaaacgaggaagacgattctagcatcggagatcaaagctgatcagcttggtttacgaaggagcgagcaacttagggagctttacgagtctctttctgtcgctgaatcttcttcctccggcgtcgccgccggatctcaggtcactagacgagcttctgccgccgcactctcgccggaagatctcgccgacacagagtggtactacttggtttgtatgtctttcgtcttcaacatcggtgaaggaatgcctggacgaacgtttgcgaacagtgaaccgatatggttgtgcaacgctcacaccgcagatagtaaagtctttagccgctctcttctggcaaaaagtgcttcggttgtgacagtgatttgcttcccgtttcttggaggagtcgttgagatcggtactacagaacatatcatagaggacatgaatgtaatacaatgcgtgaagacatcattcctcgaagctccagatccatacgcttcactgttaccaacaagatccgattatcacatcgacaacgttctcgatccgcaacagatcctaggtgacgagatttacgcgcctatgtttggtactgagacttttccggcgacttctcctagcagaactaccagcaggttcgatcctgaacacgagcaagtagcagaagatcatgactcgttcatggccgaaggaatcaatggaggagcttctcaggttcaaagctggcagttcatggacgaagagcttagtaactgcgttcaccaatcgcttaattccagtgattgcgtctctcaaacgtttgttaaagcagcggctggacgagtttcttgcaacgcaagaaaaggaagggctcaaaggttagggcatattcaagagcggcagagaaatgtgaaaatgttgtcttttgatccaagaaacgatgacgttcattaccaaagtgtgatctccacaatttttaagaccaaccatcagttaattctcggaccgcagttccggaattgcgataagcggtcaagcttcacgaggtggaagaaattatcgtcatcatcatctggaaccgcgtcaatcgtatcaccgtcacaaggaatgttaaagaagattcttttcgaggttcctcgagtgcaccagaaagagaagttgttgttggattcaccagggatcggggatgaaaccacgaaccacgcggttttagagaagaaacggcgtgagaaattgaacgaacggttcatgatcttgagatcaatcattccatcaatcaataagatcgataaagtatcaattcttgacgatacgatagagtatcttcaagaactggaaagacgtgttcaagaactagaatcttgcagagaatcaaccgatacagaaacacgtgggacaatgacagtgaagaggaagaaatctcacgacgcaggggaaagaacttcagccaactgcacaaacaatgaaaccggaaacgggaagagagttcaggttggagaaaccgagccggcagagaccgattataccggtttaactaataatttaaggatcggttcgtttggtaatgaggtcgttattgagcttagatgtgcttggagagaaggagtattgcttgagataatggatgtcattagtgatctcaacttagattctcattcggtacaatcctcgacaggagatggtttactctgcttaaccgtcaactgcaagcacaagggttcaaaaatgacgacaacaggaatgatcaaagaggcacttcaaaaggttgcatggatctgttga

SEQ ID NO: 179 - protein, 638 aa, Thlaspi arvense
MMDGMVTEQNRISVPENLKKQLAVSVRRIQWSYAIFWSISASQPGVLEWGDGYYNGDIKTRKTILASEIKADQLGLRRSEQLRELYESLSVAESSSSGVAAGSQVTRRASAAALSPEDLADTEWYYLVCMSFVFNIGEGMPGRTFANSEPIWLCNAHTADSKVFSRSLLAKSASVVTVICFPFLGGVVEIGTTEHIIEDMNVIQCVKTSFLEAPDPYASLLPTRSDYHIDNVLDPQQILGDEIYAPMFGTETFPATSPSRTTSRFDPEHEQVAEDHDSFMAEGINGGASQVQSWQFMDEELSNCVHQSLNSSDCVSQTFVKAAAGRVSCNARKGRAQRLGHIQERQRNVKMLSFDPRNDDVHYQSVISTIFKTNHQLILGPQFRNCDKRSSFTRWKKLSSSSSGTASIVSPSQGMLKKILFEVPRVHQKEKLLLDSPGIGDETTNHAVLEKKRREKLNERFMILRSIIPSINKIDKVSILDDTIEYLQELERRVQELESCRESTDTETRGTMTVKRKKSHDAGERTSANCTNNETGNGKRVQVGETEPAETDYTGLTNNLRIGSFGNEVVIELRCAWREGVLLEIMDVISDLNLDSHSVQSSTGDGLLCLTVNCKHKGSKMTTTGMIKEALQKVAWIC

SEQ ID NO: 180 - DNA, 1041 bp, Thlaspi arvense
atgacaatcttggatcagaccgttgtaacaaccggatcgaagaaggcttgtgtcatcggtggcacaggaaacttagcttctactctcatcaagcatttgcttcaaagtggctacaaagttaacactacagttagagatccagagaatgagaagaaaatggctcacttaagggtacttcaagaacttggggacctcaagatcttcaaggcggaatttactgatgaagagagtttcgattcaccagtttcgggctgtgattacgttttccatgtcgcaacgcctatcaactttacatctgaagatcccgagaaagacatgatcaagccaaggatacaaggagtgaccaatgtgttgaaatcttgcttaaaatcgaaatcagtcaagcgtgtgatctacacttcttcagctgctgcggtttccatcaacaatctttctggacctggacttgtgatgaacgaagaaaactggactgaccttgattatctcacaaaggagaagccgtttaactggggctacccagtgtcaaagatactagcagaaaaggcagcttgtaaatttgcggaagagaacaagatcgatctagttaccgtgattccggcactcatatccggaaaatctctcctctcggatcctcctccgagcagctcatttctctctatgtctttaatcaccgggaatgaaatgtatctgaaaggtctcaaggaaatgcagaagcaatctggctccatctcgttcagccacgtgaaggatttggctcgtgcccatttgtttcttgcggagaaagaaactgcgtctggtcgttacatttgctgtacttacaacacaagtgttccggagattgcagattttctcaggcagagatatcctaagtacaatgtgctgtctgaattcgaagagtgcttatcaagtgcgaagctgacgctatcttcggaaaaactcatcaatgaaggctttcgattcgaatatgggattaatgagatctatgatgagatgatagagcacttcgagtccaaaggattaatcaaagctaaagaatcttga

SEQ ID NO: 181 - protein, 346 aa, Thlaspi arvense
MTILDQTVVTTGSKKACVIGGTGNLASTLIKHLLQSGYKVNTTVRDPENEKKMAHLRVLQELGDLKIFKAEFTDEESFDSPVSGCDYVFHVATPINFTSEDPEKDMIKPRIQGVTNVLKSCLKSKSVKRVIYTSSAAAVSINNLSGPGLVMNEENWTDLDYLTKEKPFNWGYPVSKILAEKAACKFAEENKIDLVTVIPALISGKSLLSDPPPSSSFLSMSLITGNEMYLKGLKEMQKQSGSISFSHVKDLARAHLFLAEKETASGRYICCTYNTSVPEIADFLRQRYPKYNVLSEFEECLSSAKLTLSSEKLINEGFRFEYGINEIYDEMIEHFESKGLIKAKES

SEQ ID NO: 182 - DNA, 1188 bp, Thlaspi arvense
atggtgatgggtacacaaccgtcgttggaagagatcagaaaggcacagagagcggatggccccgcaggcatcttggggataggcacggccaaccctgcgaaccatgtgatccaggcagagtatccggactactacttccgcatcaccaacagtgagcacatgactgacctcaaggagaagttcaagcgcatgtgcgacaagtcgatgatacggaaacggcacatgcacctgacggaggagttcctgaaggagaatccggacatgtgcgcctacatggctccttctcttgatgtgaggcaggacatcgtggtggtcgaggtccctaagctagggaaagaggcggcagtgaaggccatcaaggagtggggtcagcccaagtccaagatcacccacgtcgtcttctgcactacatccggagttgacatgcctggtgctgactaccagctcaccaagctcctcggtcttcgcccttccgtcaagcgtctcatgatgtaccagcaaggttgctacgccggcggcactgtcctccgactcgccaaggacctcgctgagaataaccgtggtgctcgtgtccttgtcgtctgctccgagatcacagccgtcaccttccgtggcccctctgacacacacctcgactccctcgttggtcaggctctcttcagtgacggtgctgccgcgctcattgttggtgcggaccctgatgcctccgtgggagagaagcctatcttcgagatggtgtctgctgcacagaccatcctcccagactcggacggagccatagatggacacttgagggaagttgggctcaccttccatctcctcaaggacgtccctgggctcatctcgaagaacatagagaagagtctagaagaagcgtttaaaccgctcgggataagtgactggaactctctcttttggatagctcaccctgaaggtcctgcgatcctggaccaggttgagttaaagctaggactcaaggaagagaagatgagggccacgcgtcacgtgctgagcgagtacggaaacatgtcgagcgcgtgcgttctcttcattatggacgagatgaggaggaagtccaaggaggatggtgtggccacgacaggagaagggttggagtggggtgtcttgtttggtttcggaccaggtctcaccgtagagacagtcgtcttgcacagcgtccctgtttga

SEQ ID NO: 183 - protein, 395 aa, Thlaspi arvense
MVMGTQPSLEEIRKAQRADGPAGILGIGTANPANHVIQAEYPDYYFRITNSEHMTDLKEKFKRMCDKSMIRKRHMHLTEEFLKENPDMCAYMAPSLDVRQDIVVVEVPKLGKEAAVKAIKEWGQPKSKITHVVFCTTSGVDMPGADYQLTKLLGLRPSVKRLMMYQQGCYAGGTVLRLAKDLAENNRGARVLVVCSEITAVTFRGPSDTHLDSLVGQALFSDGAAALIVGADPDASVGEKPIFEMVSAAQTILPDSDGAIDGHLREVGLTFHLLKDVPGLISKNIEKSLEEAFKPLGISDWNSLFWIAHPEGPAILDQVELKLGLKEEKMRATRHVLSEYGNMSSACVLFIMDEMRRKSKEDGVATTGEGLEWGVLFGFGPGLTVETVVLHSVPV